European Patent Application EP 4 745 238 A1, published May 20, 2026. Title: 靶向血管紧张素原的寡核苷酸及其用途. Applicant: 北京安龙生物医药有限公司. Application CN. The sequence listing filed with the application follows.

SEQUENCE LISTING (911 sequences)

SEQ ID NO: 1 - RNA, 21 nt, synthetic construct
  source 1..21: mol_type = other RNA
gtcatccacaatgagagtaca

SEQ ID NO: 2 - RNA, 21 nt, synthetic construct
  source 1..21: mol_type = other RNA
cttccacctcgtcatccacaa

SEQ ID NO: 3 - RNA, 21 nt, synthetic construct
  source 1..21: mol_type = other RNA
ccacctcgtcatccacaatga

SEQ ID NO: 4 - RNA, 21 nt, synthetic construct
  source 1..21: mol_type = other RNA
cctcgtcatccacaatgagaa

SEQ ID NO: 5 - RNA, 21 nt, synthetic construct
  source 1..21: mol_type = other RNA
cgtcatccacaatgagagtaa

SEQ ID NO: 6 - RNA, 21 nt, synthetic construct
  source 1..21: mol_type = other RNA
atccacaatgagagtacctga

SEQ ID NO: 7 - RNA, 21 nt, synthetic construct
  source 1..21: mol_type = other RNA
ccacaatgagagtacctgtga

SEQ ID NO: 8 - RNA, 21 nt, synthetic construct
  source 1..21: mol_type = other RNA
caatgagagtacctgtgagca

SEQ ID NO: 9 - RNA, 21 nt, synthetic construct
  source 1..21: mol_type = other RNA
gacaccgaagacaagttgaga

SEQ ID NO: 10 - RNA, 21 nt, synthetic construct
  source 1..21: mol_type = other RNA
gtcgggatgctggccaactta

SEQ ID NO: 11 - RNA, 21 nt, synthetic construct
  source 1..21: mol_type = other RNA
gggatgctggccaacttctta

SEQ ID NO: 12 - RNA, 21 nt, synthetic construct
  source 1..21: mol_type = other RNA
acttcttgggcttccgtatat

SEQ ID NO: 13 - RNA, 21 nt, synthetic construct
  source 1..21: mol_type = other RNA
atggcatgcacagtgagctat

SEQ ID NO: 14 - RNA, 21 nt, synthetic construct
  source 1..21: mol_type = other RNA
ggcatgcacagtgagctatga

SEQ ID NO: 15 - RNA, 21 nt, synthetic construct
  source 1..21: mol_type = other RNA
gctgacaggctacaggcaata

SEQ ID NO: 16 - RNA, 21 nt, synthetic construct
  source 1..21: mol_type = other RNA
gtgttccttggaaggacaaga

SEQ ID NO: 17 - RNA, 21 nt, synthetic construct
  source 1..21: mol_type = other RNA
gatgcgcacaaggtcctgtct

SEQ ID NO: 18 - RNA, 21 nt, synthetic construct
  source 1..21: mol_type = other RNA
ggctgtacagggcctgctagt

SEQ ID NO: 19 - RNA, 21 nt, synthetic construct
  source 1..21: mol_type = other RNA
ttgctgctgagaagattgaca

SEQ ID NO: 20 - RNA, 21 nt, synthetic construct
  source 1..21: mol_type = other RNA
gagaagattgacaggttcatg

SEQ ID NO: 21 - RNA, 21 nt, synthetic construct
  source 1..21: mol_type = other RNA
ggacagcaccctggctttcaa

SEQ ID NO: 22 - RNA, 21 nt, synthetic construct
  source 1..21: mol_type = other RNA
acagcaccctggctttcaaca

SEQ ID NO: 23 - RNA, 21 nt, synthetic construct
  source 1..21: mol_type = other RNA
aggagttctgggtggacaaca

SEQ ID NO: 24 - RNA, 21 nt, synthetic construct
  source 1..21: mol_type = other RNA
ggtggacaacagcacctcagt

SEQ ID NO: 25 - RNA, 21 nt, synthetic construct
  source 1..21: mol_type = other RNA
gtggacaacagcacctcagta

SEQ ID NO: 26 - RNA, 21 nt, synthetic construct
  source 1..21: mol_type = other RNA
gcctcactatgcctctgacct

SEQ ID NO: 27 - RNA, 21 nt, synthetic construct
  source 1..21: mol_type = other RNA
ggacaaggtggagggtctcaa

SEQ ID NO: 28 - RNA, 21 nt, synthetic construct
  source 1..21: mol_type = other RNA
gacaaggtggagggtctcact

SEQ ID NO: 29 - RNA, 21 nt, synthetic construct
  source 1..21: mol_type = other RNA
acaaggtggagggtctcactt

SEQ ID NO: 30 - RNA, 21 nt, synthetic construct
  source 1..21: mol_type = other RNA
ctcactttccagcaaaactca

SEQ ID NO: 31 - RNA, 21 nt, synthetic construct
  source 1..21: mol_type = other RNA
actccctcaactggatgaaga

SEQ ID NO: 32 - RNA, 21 nt, synthetic construct
  source 1..21: mol_type = other RNA
ccctcaactggatgaagaaaa

SEQ ID NO: 33 - RNA, 21 nt, synthetic construct
  source 1..21: mol_type = other RNA
cctcaactggatgaagaaact

SEQ ID NO: 34 - RNA, 21 nt, synthetic construct
  source 1..21: mol_type = other RNA
caactggatgaagaaactata

SEQ ID NO: 35 - RNA, 21 nt, synthetic construct
  source 1..21: mol_type = other RNA
aactggatgaagaaactatct

SEQ ID NO: 36 - RNA, 21 nt, synthetic construct
  source 1..21: mol_type = other RNA
ggtgctgcaaggatcttatga

SEQ ID NO: 37 - RNA, 21 nt, synthetic construct
  source 1..21: mol_type = other RNA
gctgcaaggatcttatgacct

SEQ ID NO: 38 - RNA, 21 nt, synthetic construct
  source 1..21: mol_type = other RNA
ggtgctgaacagcattttttt

SEQ ID NO: 39 - RNA, 21 nt, synthetic construct
  source 1..21: mol_type = other RNA
gtgctgaacagcatttttttt

SEQ ID NO: 40 - RNA, 21 nt, synthetic construct
  source 1..21: mol_type = other RNA
gctgaacagcattttttttga

SEQ ID NO: 41 - RNA, 21 nt, synthetic construct
  source 1..21: mol_type = other RNA
gaacagcattttttttgagct

SEQ ID NO: 42 - RNA, 21 nt, synthetic construct
  source 1..21: mol_type = other RNA
cagcattttttttgagcttga

SEQ ID NO: 43 - RNA, 21 nt, synthetic construct
  source 1..21: mol_type = other RNA
gagcttgaagcggatgagaga

SEQ ID NO: 44 - RNA, 21 nt, synthetic construct
  source 1..21: mol_type = other RNA
gcttgaagcggatgagagaga

SEQ ID NO: 45 - RNA, 21 nt, synthetic construct
  source 1..21: mol_type = other RNA
atgagagagagcccacagagt

SEQ ID NO: 46 - RNA, 21 nt, synthetic construct
  source 1..21: mol_type = other RNA
gagagagagcccacagagtct

SEQ ID NO: 47 - RNA, 21 nt, synthetic construct
  source 1..21: mol_type = other RNA
agagagagcccacagagtcta

SEQ ID NO: 48 - RNA, 21 nt, synthetic construct
  source 1..21: mol_type = other RNA
gagtctacccaacagcttaaa

SEQ ID NO: 49 - RNA, 21 nt, synthetic construct
  source 1..21: mol_type = other RNA
agtctacccaacagcttaaca

SEQ ID NO: 50 - RNA, 21 nt, synthetic construct
  source 1..21: mol_type = other RNA
cattcctgtttgctgtgtata

SEQ ID NO: 51 - RNA, 21 nt, synthetic construct
  source 1..21: mol_type = other RNA
cctgtttgctgtgtatgatca

SEQ ID NO: 52 - RNA, 21 nt, synthetic construct
  source 1..21: mol_type = other RNA
gtttgctgtgtatgatcaaaa

SEQ ID NO: 53 - RNA, 21 nt, synthetic construct
  source 1..21: mol_type = other RNA
gcaaaggccagcagcagataa

SEQ ID NO: 54 - RNA, 21 nt, synthetic construct
  source 1..21: mol_type = other RNA
cagcgatgtgtcacccccagt

SEQ ID NO: 55 - RNA, 21 nt, synthetic construct
  source 1..21: mol_type = other RNA
gcgatgtgtcacccccagtct

SEQ ID NO: 56 - RNA, 21 nt, synthetic construct
  source 1..21: mol_type = other RNA
gatgtgtcacccccagtctca

SEQ ID NO: 57 - RNA, 21 nt, synthetic construct
  source 1..21: mol_type = other RNA
gtgtcacccccagtctcccaa

SEQ ID NO: 58 - RNA, 21 nt, synthetic construct
  source 1..21: mol_type = other RNA
gtcacccccagtctcccacct

SEQ ID NO: 59 - RNA, 21 nt, synthetic construct
  source 1..21: mol_type = other RNA
cacccccagtctcccaccttt

SEQ ID NO: 60 - RNA, 21 nt, synthetic construct
  source 1..21: mol_type = other RNA
cccccagtctcccacctttta

SEQ ID NO: 61 - RNA, 21 nt, synthetic construct
  source 1..21: mol_type = other RNA
cccagtctcccaccttttctt

SEQ ID NO: 62 - RNA, 21 nt, synthetic construct
  source 1..21: mol_type = other RNA
cagtctcccaccttttcttct

SEQ ID NO: 63 - RNA, 21 nt, synthetic construct
  source 1..21: mol_type = other RNA
tctcccaccttttcttctaat

SEQ ID NO: 64 - RNA, 21 nt, synthetic construct
  source 1..21: mol_type = other RNA
caccttttcttcttaatgagt

SEQ ID NO: 65 - RNA, 21 nt, synthetic construct
  source 1..21: mol_type = other RNA
ccttttcttctaatgagtcga

SEQ ID NO: 66 - RNA, 21 nt, synthetic construct
  source 1..21: mol_type = other RNA
agccgtttctccttggtctaa

SEQ ID NO: 67 - RNA, 21 nt, synthetic construct
  source 1..21: mol_type = other RNA
gccgtttctccttggtctaaa

SEQ ID NO: 68 - RNA, 21 nt, synthetic construct
  source 1..21: mol_type = other RNA
ccagtttgctgggtttatttt

SEQ ID NO: 69 - RNA, 21 nt, synthetic construct
  source 1..21: mol_type = other RNA
cagtttgctgggtttatttta

SEQ ID NO: 70 - RNA, 21 nt, synthetic construct
  source 1..21: mol_type = other RNA
gtccacaatgagagtacctga

SEQ ID NO: 71 - RNA, 21 nt, synthetic construct
  source 1..21: mol_type = other RNA
ggcatgcacactgagctatga

SEQ ID NO: 72 - RNA, 21 nt, synthetic construct
  source 1..21: mol_type = other RNA
gagaagattgacaggttcata

SEQ ID NO: 73 - RNA, 21 nt, synthetic construct
  source 1..21: mol_type = other RNA
ggacagcaccgtggctttcaa

SEQ ID NO: 74 - RNA, 21 nt, synthetic construct
  source 1..21: mol_type = other RNA
gctgaacagcgttttttttga

SEQ ID NO: 75 - RNA, 21 nt, synthetic construct
  source 1..21: mol_type = other RNA
ccttttcttcgaatgagtcga

SEQ ID NO: 76 - RNA, 21 nt, synthetic construct
  source 1..21: mol_type = other RNA
agccgtttctgcttggtctaa

SEQ ID NO: 77 - RNA, 21 nt, synthetic construct
  source 1..21: mol_type = other RNA
gccgtttctgcttggtctaaa

SEQ ID NO: 78 - RNA, 21 nt, synthetic construct
  source 1..21: mol_type = other RNA
cgttgttctgggtactacaga

SEQ ID NO: 79 - RNA, 21 nt, synthetic construct
  source 1..21: mol_type = other RNA
gccacctcgtcatccacaata

SEQ ID NO: 80 - RNA, 21 nt, synthetic construct
  source 1..21: mol_type = other RNA
cacctcgtcatccacaatgaa

SEQ ID NO: 81 - RNA, 21 nt, synthetic construct
  source 1..21: mol_type = other RNA
atccacaatgcgagtacctga

SEQ ID NO: 82 - RNA, 21 nt, synthetic construct
  source 1..21: mol_type = other RNA
tccacaatgagagtacctgta

SEQ ID NO: 83 - RNA, 21 nt, synthetic construct
  source 1..21: mol_type = other RNA
gagcttgaaggggatgagaga

SEQ ID NO: 84 - RNA, 21 nt, synthetic construct
  source 1..21: mol_type = other RNA
gagagagagcgcacagagtct

SEQ ID NO: 85 - RNA, 21 nt, synthetic construct
  source 1..21: mol_type = other RNA
gttttttgagcttgaagcgga

SEQ ID NO: 86 - RNA, 21 nt, synthetic construct
  source 1..21: mol_type = other RNA
gttttgagcttgaagcggata

SEQ ID NO: 87 - RNA, 21 nt, synthetic construct
  source 1..21: mol_type = other RNA
gtttgagcttgaagcggatga

SEQ ID NO: 88 - RNA, 21 nt, synthetic construct
  source 1..21: mol_type = other RNA
ccagtctcccaccttttctta

SEQ ID NO: 89 - RNA, 21 nt, synthetic construct
  source 1..21: mol_type = other RNA
ccccagtctcccaccttttct

SEQ ID NO: 90 - RNA, 21 nt, synthetic construct
  source 1..21: mol_type = other RNA
gcgactttgagctggaaagca

SEQ ID NO: 91 - RNA, 21 nt, synthetic construct
  source 1..21: mol_type = other RNA
gcagccgtttctccttggtct

SEQ ID NO: 92 - RNA, 21 nt, synthetic construct
  source 1..21: mol_type = other RNA
ccgtttctccttggtctaagt

SEQ ID NO: 93 - RNA, 21 nt, synthetic construct
  source 1..21: mol_type = other RNA
gtccacaatgagagtacctgt

SEQ ID NO: 94 - RNA, 21 nt, synthetic construct
  source 1..21: mol_type = other RNA
atccacaatgagagtacctgt

SEQ ID NO: 95 - RNA, 21 nt, synthetic construct
  source 1..21: mol_type = other RNA
gcatccacaatgagagtacct

SEQ ID NO: 96 - RNA, 21 nt, synthetic construct
  source 1..21: mol_type = other RNA
cccagtctcccaccttttcta

SEQ ID NO: 97 - RNA, 21 nt, synthetic construct
  source 1..21: mol_type = other RNA
cagtctcccaccttttcttca

SEQ ID NO: 98 - RNA, 21 nt, synthetic construct
  source 1..21: mol_type = other RNA
ggtctcccaccttttcttcta

SEQ ID NO: 99 - RNA, 21 nt, synthetic construct
  source 1..21: mol_type = other RNA
gtctcccaccttttcttctaa

SEQ ID NO: 100 - RNA, 21 nt, synthetic construct
  source 1..21: mol_type = other RNA
cagccgtttctccttggtcta

SEQ ID NO: 101 - RNA, 21 nt, synthetic construct
  source 1..21: mol_type = other RNA
ggccgtttctccttggtctaa

SEQ ID NO: 102 - RNA, 21 nt, synthetic construct
  source 1..21: mol_type = other RNA
gccgtttctccttggtctaag

SEQ ID NO: 103 - RNA, 21 nt, synthetic construct
  source 1..21: mol_type = other RNA
cgtttctccttggtctaagtg

SEQ ID NO: 104 - RNA, 21 nt, synthetic construct
  source 1..21: mol_type = other RNA
cgtttctccttggtctaagta

SEQ ID NO: 105 - RNA, 21 nt, synthetic construct
  source 1..21: mol_type = other RNA
gtttctccttggtctaagtgt

SEQ ID NO: 106 - RNA, 21 nt, synthetic construct
  source 1..21: mol_type = other RNA
gtttctccttggtctaagtga

SEQ ID NO: 107 - RNA, 21 nt, synthetic construct
  source 1..21: mol_type = other RNA
cagtctcccagcttttcttct

SEQ ID NO: 108 - RNA, 21 nt, synthetic construct
  source 1..21: mol_type = other RNA
gccgtttctcgttggtctaaa

SEQ ID NO: 109 - RNA, 21 nt, synthetic construct
  source 1..21: mol_type = other RNA
ggccgtttctgcttggtctaa

SEQ ID NO: 110 - RNA, 21 nt, synthetic construct
  source 1..21: mol_type = other RNA
ggccgtttctacttggtctaa

SEQ ID NO: 111 - RNA, 21 nt, synthetic construct
  source 1..21: mol_type = other RNA
ccgtttctccttggtctaaga

SEQ ID NO: 112 - RNA, 21 nt, synthetic construct
  source 1..21: mol_type = other RNA
gcgtttctccttggtctaagt

SEQ ID NO: 113 - RNA, 21 nt, synthetic construct
  source 1..21: mol_type = other RNA
gcgtttctccttggtctaaga

SEQ ID NO: 114 - RNA, 21 nt, synthetic construct
  source 1..21: mol_type = other RNA
gcgtttctccgtggtctaagt

SEQ ID NO: 115 - RNA, 19 nt, synthetic construct
  source 1..19: mol_type = other RNA
tcccaccttttcttctaat

SEQ ID NO: 116 - RNA, 19 nt, synthetic construct
  source 1..19: mol_type = other RNA
gcccaccttttcttctaaa

SEQ ID NO: 117 - RNA, 19 nt, synthetic construct
  source 1..19: mol_type = other RNA
gcatccacaatgagagtaa

SEQ ID NO: 118 - RNA, 19 nt, synthetic construct
  source 1..19: mol_type = other RNA
gcgtcatccacaatgagaa

SEQ ID NO: 119 - RNA, 19 nt, synthetic construct
  source 1..19: mol_type = other RNA
cctcgtcatccacaatgaa

SEQ ID NO: 120 - RNA, 19 nt, synthetic construct
  source 1..19: mol_type = other RNA
cacctcgtcatccacaata

SEQ ID NO: 121 - RNA, 19 nt, synthetic construct
  source 1..19: mol_type = other RNA
gtccacaatgagagtacca

SEQ ID NO: 122 - RNA, 19 nt, synthetic construct
  source 1..19: mol_type = other RNA
gccacaatgagagtaccta

SEQ ID NO: 123 - RNA, 19 nt, synthetic construct
  source 1..19: mol_type = other RNA
cacaatgagagtacctgta

SEQ ID NO: 124 - RNA, 19 nt, synthetic construct
  source 1..19: mol_type = other RNA
gcaatgagagtacctgtga

SEQ ID NO: 125 - RNA, 19 nt, synthetic construct
  source 1..19: mol_type = other RNA
caatgagagtacctgtgaa

SEQ ID NO: 126 - RNA, 19 nt, synthetic construct
  source 1..19: mol_type = other RNA
gatgagagtacctgtgaga

SEQ ID NO: 127 - RNA, 19 nt, synthetic construct
  source 1..19: mol_type = other RNA
ggagagtacctgtgagcaa

SEQ ID NO: 128 - RNA, 19 nt, synthetic construct
  source 1..19: mol_type = other RNA
gagagtacctgtgagcaga

SEQ ID NO: 129 - RNA, 19 nt, synthetic construct
  source 1..19: mol_type = other RNA
ctcccaccttttcttctaa

SEQ ID NO: 130 - RNA, 19 nt, synthetic construct
  source 1..19: mol_type = other RNA
gctcccaccttttcttcta

SEQ ID NO: 131 - RNA, 19 nt, synthetic construct
  source 1..19: mol_type = other RNA
gtctcccaccttttcttca

SEQ ID NO: 132 - RNA, 19 nt, synthetic construct
  source 1..19: mol_type = other RNA
ggtctcccaccttttctta

SEQ ID NO: 133 - RNA, 19 nt, synthetic construct
  source 1..19: mol_type = other RNA
cccaccttttcttctaata

SEQ ID NO: 134 - RNA, 19 nt, synthetic construct
  source 1..19: mol_type = other RNA
ccaccttttcttctaatga

SEQ ID NO: 135 - RNA, 19 nt, synthetic construct
  source 1..19: mol_type = other RNA
caccttttcttctaatgaa

SEQ ID NO: 136 - RNA, 19 nt, synthetic construct
  source 1..19: mol_type = other RNA
gccttttcttctaatgaga

SEQ ID NO: 137 - RNA, 19 nt, synthetic construct
  source 1..19: mol_type = other RNA
ccttttcttctaatgagta

SEQ ID NO: 138 - RNA, 19 nt, synthetic construct
  source 1..19: mol_type = other RNA
cttttcttctaatgagtca

SEQ ID NO: 139 - RNA, 19 nt, synthetic construct
  source 1..19: mol_type = other RNA
agcacctgaatttctgttt

SEQ ID NO: 140 - RNA, 19 nt, synthetic construct
  source 1..19: mol_type = other RNA
gtctgtaataccttagttt

SEQ ID NO: 141 - RNA, 19 nt, synthetic construct
  source 1..19: mol_type = other RNA
caaatgcacctcccagttt

SEQ ID NO: 142 - RNA, 19 nt, synthetic construct
  source 1..19: mol_type = other RNA
tggacagcaccctggcttt

SEQ ID NO: 143 - RNA, 19 nt, synthetic construct
  source 1..19: mol_type = other RNA
cttctaatgagtcgacttt

SEQ ID NO: 144 - RNA, 19 nt, synthetic construct
  source 1..19: mol_type = other RNA
aggtggagggtctcacttt

SEQ ID NO: 145 - RNA, 19 nt, synthetic construct
  source 1..19: mol_type = other RNA
gaaccatagctggttattt

SEQ ID NO: 146 - RNA, 19 nt, synthetic construct
  source 1..19: mol_type = other RNA
ttgccttcggtttgtattt

SEQ ID NO: 147 - RNA, 19 nt, synthetic construct
  source 1..19: mol_type = other RNA
ggtttgtatttagtgtctt

SEQ ID NO: 148 - RNA, 19 nt, synthetic construct
  source 1..19: mol_type = other RNA
caagttgagaacaaaaatt

SEQ ID NO: 149 - RNA, 19 nt, synthetic construct
  source 1..19: mol_type = other RNA
gtttgtgaaacaaaaaagt

SEQ ID NO: 150 - RNA, 19 nt, synthetic construct
  source 1..19: mol_type = other RNA
tggacaaggtggagggtct

SEQ ID NO: 151 - RNA, 19 nt, synthetic construct
  source 1..19: mol_type = other RNA
ctcactttccagcaaaact

SEQ ID NO: 152 - RNA, 19 nt, synthetic construct
  source 1..19: mol_type = other RNA
acttcttgggcttccgtat

SEQ ID NO: 153 - RNA, 19 nt, synthetic construct
  source 1..19: mol_type = other RNA
gtcttgaatgtaagaacat

SEQ ID NO: 154 - RNA, 19 nt, synthetic construct
  source 1..19: mol_type = other RNA
ttcctgtttgctgtgtatg

SEQ ID NO: 155 - RNA, 19 nt, synthetic construct
  source 1..19: mol_type = other RNA
ggcaagaaccagtgtttag

SEQ ID NO: 156 - RNA, 19 nt, synthetic construct
  source 1..19: mol_type = other RNA
gattgacaggttcatgcag

SEQ ID NO: 157 - RNA, 19 nt, synthetic construct
  source 1..19: mol_type = other RNA
gtatatatggcatgcacag

SEQ ID NO: 158 - RNA, 19 nt, synthetic construct
  source 1..19: mol_type = other RNA
ccatagctggttatttctc

SEQ ID NO: 159 - RNA, 19 nt, synthetic construct
  source 1..19: mol_type = other RNA
atgtaagaacatgacctcc

SEQ ID NO: 160 - RNA, 19 nt, synthetic construct
  source 1..19: mol_type = other RNA
ccgtatatatggcatgcac

SEQ ID NO: 161 - RNA, 19 nt, synthetic construct
  source 1..19: mol_type = other RNA
gtgtcttgaatgtaagaac

SEQ ID NO: 162 - RNA, 19 nt, synthetic construct
  source 1..19: mol_type = other RNA
aggcaagaaccagtgttta

SEQ ID NO: 163 - RNA, 19 nt, synthetic construct
  source 1..19: mol_type = other RNA
cattcctgtttgctgtgta

SEQ ID NO: 164 - RNA, 19 nt, synthetic construct
  source 1..19: mol_type = other RNA
gggttttaaaattaaagta

SEQ ID NO: 165 - RNA, 19 nt, synthetic construct
  source 1..19: mol_type = other RNA
cttcttgggcttccgtata

SEQ ID NO: 166 - RNA, 19 nt, synthetic construct
  source 1..19: mol_type = other RNA
gttttaaaattaaagtata

SEQ ID NO: 167 - RNA, 19 nt, synthetic construct
  source 1..19: mol_type = other RNA
tatatggcatgcacagtga

SEQ ID NO: 168 - RNA, 19 nt, synthetic construct
  source 1..19: mol_type = other RNA
cttgaatgtaagaacatga

SEQ ID NO: 169 - RNA, 19 nt, synthetic construct
  source 1..19: mol_type = other RNA
gatcttatgacctgcagga

SEQ ID NO: 170 - RNA, 19 nt, synthetic construct
  source 1..19: mol_type = other RNA
ggtggacaacagcacctca

SEQ ID NO: 171 - RNA, 19 nt, synthetic construct
  source 1..19: mol_type = other RNA
agattgacaggttcatgca

SEQ ID NO: 172 - RNA, 19 nt, synthetic construct
  source 1..19: mol_type = other RNA
gttcatgcaggctgtgaca

SEQ ID NO: 173 - RNA, 19 nt, synthetic construct
  source 1..19: mol_type = other RNA
caggagttctgggtggaca

SEQ ID NO: 174 - RNA, 19 nt, synthetic construct
  source 1..19: mol_type = other RNA
cgtatatatggcatgcaca

SEQ ID NO: 175 - RNA, 19 nt, synthetic construct
  source 1..19: mol_type = other RNA
actccctcaactggatgaa

SEQ ID NO: 176 - RNA, 19 nt, synthetic construct
  source 1..19: mol_type = other RNA
gggtctcactttccagcaa

SEQ ID NO: 177 - RNA, 19 nt, synthetic construct
  source 1..19: mol_type = other RNA
aggagttctgggtggacaa

SEQ ID NO: 178 - RNA, 19 nt, synthetic construct
  source 1..19: mol_type = other RNA
gaccagcttgtttgtgaaa

SEQ ID NO: 179 - RNA, 19 nt, synthetic construct
  source 1..19: mol_type = other RNA
cctgtgagcagctggcaaa

SEQ ID NO: 180 - RNA, 19 nt, synthetic construct
  source 1..19: mol_type = other RNA
ggtctcactttccagcaaa

SEQ ID NO: 181 - RNA, 19 nt, synthetic construct
  source 1..19: mol_type = other RNA
caaaaattgggttttaaaa

SEQ ID NO: 182 - RNA, 19 nt, synthetic construct
  source 1..19: mol_type = other RNA
gcttgtttgtgaaacaaaa

SEQ ID NO: 183 - RNA, 19 nt, synthetic construct
  source 1..19: mol_type = other RNA
aagacgtttattactaaca

SEQ ID NO: 184 - RNA, 19 nt, synthetic construct
  source 1..19: mol_type = other RNA
cgaccagcttgtttgtgaa

SEQ ID NO: 185 - RNA, 19 nt, synthetic construct
  source 1..19: mol_type = other RNA
cttgtttgtgaaacaaaaa

SEQ ID NO: 186 - RNA, 19 nt, synthetic construct
  source 1..19: mol_type = other RNA
acaacttctcggtgactca

SEQ ID NO: 187 - RNA, 19 nt, synthetic construct
  source 1..19: mol_type = other RNA
tggtcgggatgctggccaa

SEQ ID NO: 188 - RNA, 19 nt, synthetic construct
  source 1..19: mol_type = other RNA
ctgaatttctgtttgaatg

SEQ ID NO: 189 - RNA, 19 nt, synthetic construct
  source 1..19: mol_type = other RNA
aggatcttatgacctgcag

SEQ ID NO: 190 - RNA, 19 nt, synthetic construct
  source 1..19: mol_type = other RNA
gagaagattgacaggttca

SEQ ID NO: 191 - RNA, 19 nt, synthetic construct
  source 1..19: mol_type = other RNA
gttccaaaaagaattccaa

SEQ ID NO: 192 - RNA, 19 nt, synthetic construct
  source 1..19: mol_type = other RNA
tgtaagaacatgacctccg

SEQ ID NO: 193 - RNA, 19 nt, synthetic construct
  source 1..19: mol_type = other RNA
ggctgtacagggcctgcta

SEQ ID NO: 194 - RNA, 19 nt, synthetic construct
  source 1..19: mol_type = other RNA
caactggatgaagaaacta

SEQ ID NO: 195 - RNA, 19 nt, synthetic construct
  source 1..19: mol_type = other RNA
ccctcaactggatgaagaa

SEQ ID NO: 196 - RNA, 19 nt, synthetic construct
  source 1..19: mol_type = other RNA
tacgtgaaagatgcaagca

SEQ ID NO: 197 - RNA, 19 nt, synthetic construct
  source 1..19: mol_type = other RNA
gcaaaggccagcagcagat

SEQ ID NO: 198 - RNA, 19 nt, synthetic construct
  source 1..19: mol_type = other RNA
gcaaggatcttatgacctg

SEQ ID NO: 199 - RNA, 19 nt, synthetic construct
  source 1..19: mol_type = other RNA
gctgacaggctacaggcaa

SEQ ID NO: 200 - RNA, 19 nt, synthetic construct
  source 1..19: mol_type = other RNA
cccttgtgttagtaataaa

SEQ ID NO: 201 - RNA, 19 nt, synthetic construct
  source 1..19: mol_type = other RNA
gcacctgaatttctgtttg

SEQ ID NO: 202 - RNA, 19 nt, synthetic construct
  source 1..19: mol_type = other RNA
gagcacagcatgaggccag

SEQ ID NO: 203 - RNA, 19 nt, synthetic construct
  source 1..19: mol_type = other RNA
ctcccttgtgttagtaata

SEQ ID NO: 204 - RNA, 19 nt, synthetic construct
  source 1..19: mol_type = other RNA
acaatacgtgaaagatgca

SEQ ID NO: 205 - RNA, 19 nt, synthetic construct
  source 1..19: mol_type = other RNA
gaacaatacgtgaaagatg

SEQ ID NO: 206 - RNA, 19 nt, synthetic construct
  source 1..19: mol_type = other RNA
tttctcccttgtgttagta

SEQ ID NO: 207 - RNA, 19 nt, synthetic construct
  source 1..19: mol_type = other RNA
ccaatgccgggaagcccaa

SEQ ID NO: 208 - RNA, 19 nt, synthetic construct
  source 1..19: mol_type = other RNA
tgcaagcacctgaatttct

SEQ ID NO: 209 - RNA, 19 nt, synthetic construct
  source 1..19: mol_type = other RNA
ggtgctgcaaggatcttat

SEQ ID NO: 210 - RNA, 19 nt, synthetic construct
  source 1..19: mol_type = other RNA
ccacacagctgacaggcta

SEQ ID NO: 211 - RNA, 19 nt, synthetic construct
  source 1..19: mol_type = other RNA
ttgaacaatacgtgaaaga

SEQ ID NO: 212 - RNA, 19 nt, synthetic construct
  source 1..19: mol_type = other RNA
gacaccgaagacaagttga

SEQ ID NO: 213 - RNA, 19 nt, synthetic construct
  source 1..19: mol_type = other RNA
gagccagtgtggacagcac

SEQ ID NO: 214 - RNA, 19 nt, synthetic construct
  source 1..19: mol_type = other RNA
tggaaggacaagaactgca

SEQ ID NO: 215 - RNA, 19 nt, synthetic construct
  source 1..19: mol_type = other RNA
caacttctcggtgactcaa

SEQ ID NO: 216 - RNA, 19 nt, synthetic construct
  source 1..19: mol_type = other RNA
aacgtcttgccacaataag

SEQ ID NO: 217 - RNA, 19 nt, synthetic construct
  source 1..19: mol_type = other RNA
ctgagaagattgacaggtt

SEQ ID NO: 218 - RNA, 19 nt, synthetic construct
  source 1..19: mol_type = other RNA
ccagtttgctgggtttatt

SEQ ID NO: 219 - RNA, 19 nt, synthetic construct
  source 1..19: mol_type = other RNA
acttctcggtgactcaagt

SEQ ID NO: 220 - RNA, 23 nt, synthetic construct
  source 1..23: mol_type = other RNA
tgtactctcattgtggatgacga

SEQ ID NO: 221 - RNA, 23 nt, synthetic construct
  source 1..23: mol_type = other RNA
ttgtggatgacgaggtggaaggg

SEQ ID NO: 222 - RNA, 23 nt, synthetic construct
  source 1..23: mol_type = other RNA
tcattgtggatgacgaggtggaa

SEQ ID NO: 223 - RNA, 23 nt, synthetic construct
  source 1..23: mol_type = other RNA
ttctcattgtggatgacgaggtg

SEQ ID NO: 224 - RNA, 23 nt, synthetic construct
  source 1..23: mol_type = other RNA
ttactctcattgtggatgacgag

SEQ ID NO: 225 - RNA, 23 nt, synthetic construct
  source 1..23: mol_type = other RNA
tcaggtactctcattgtggatga

SEQ ID NO: 226 - RNA, 23 nt, synthetic construct
  source 1..23: mol_type = other RNA
tcacaggtactctcattgtggat

SEQ ID NO: 227 - RNA, 23 nt, synthetic construct
  source 1..23: mol_type = other RNA
tgctcacaggtactctcattgtg

SEQ ID NO: 228 - RNA, 23 nt, synthetic construct
  source 1..23: mol_type = other RNA
tctcaacttgtcttcggtgtcaa

SEQ ID NO: 229 - RNA, 23 nt, synthetic construct
  source 1..23: mol_type = other RNA
taagttggccagcatcccgacca

SEQ ID NO: 230 - RNA, 23 nt, synthetic construct
  source 1..23: mol_type = other RNA
taagaagttggccagcatcccga

SEQ ID NO: 231 - RNA, 23 nt, synthetic construct
  source 1..23: mol_type = other RNA
atatacggaagcccaagaagttg

SEQ ID NO: 232 - RNA, 23 nt, synthetic construct
  source 1..23: mol_type = other RNA
atagctcactgtgcatgccatat

SEQ ID NO: 233 - RNA, 23 nt, synthetic construct
  source 1..23: mol_type = other RNA
tcatagctcactgtgcatgccat

SEQ ID NO: 234 - RNA, 23 nt, synthetic construct
  source 1..23: mol_type = other RNA
tattgcctgtagcctgtcagctg

SEQ ID NO: 235 - RNA, 23 nt, synthetic construct
  source 1..23: mol_type = other RNA
tcttgtccttccaaggaacaccc

SEQ ID NO: 236 - RNA, 23 nt, synthetic construct
  source 1..23: mol_type = other RNA
agacaggaccttgtgcgcatcca

SEQ ID NO: 237 - RNA, 23 nt, synthetic construct
  source 1..23: mol_type = other RNA
actagcaggccctgtacagcctg

SEQ ID NO: 238 - RNA, 23 nt, synthetic construct
  source 1..23: mol_type = other RNA
tgtcaatcttctcagcagcaaca

SEQ ID NO: 239 - RNA, 23 nt, synthetic construct
  source 1..23: mol_type = other RNA
catgaacctgtcaatcttctcag

SEQ ID NO: 240 - RNA, 23 nt, synthetic construct
  source 1..23: mol_type = other RNA
ttgaaagccagggtgctgtccac

SEQ ID NO: 241 - RNA, 23 nt, synthetic construct
  source 1..23: mol_type = other RNA
tgttgaaagccagggtgctgtcc

SEQ ID NO: 242 - RNA, 23 nt, synthetic construct
  source 1..23: mol_type = other RNA
tgttgtccacccagaactcctgg

SEQ ID NO: 243 - RNA, 23 nt, synthetic construct
  source 1..23: mol_type = other RNA
actgaggtgctgttgtccaccca

SEQ ID NO: 244 - RNA, 23 nt, synthetic construct
  source 1..23: mol_type = other RNA
tactgaggtgctgttgtccaccc

SEQ ID NO: 245 - RNA, 23 nt, synthetic construct
  source 1..23: mol_type = other RNA
aggtcagaggcatagtgaggctg

SEQ ID NO: 246 - RNA, 23 nt, synthetic construct
  source 1..23: mol_type = other RNA
ttgagaccctccaccttgtccag

SEQ ID NO: 247 - RNA, 23 nt, synthetic construct
  source 1..23: mol_type = other RNA
agtgagaccctccaccttgtcca

SEQ ID NO: 248 - RNA, 23 nt, synthetic construct
  source 1..23: mol_type = other RNA
aagtgagaccctccaccttgtcc

SEQ ID NO: 249 - RNA, 23 nt, synthetic construct
  source 1..23: mol_type = other RNA
tgagttttgctggaaagtgagac

SEQ ID NO: 250 - RNA, 23 nt, synthetic construct
  source 1..23: mol_type = other RNA
tcttcatccagttgagggagttt

SEQ ID NO: 251 - RNA, 23 nt, synthetic construct
  source 1..23: mol_type = other RNA
ttttcttcatccagttgagggag

SEQ ID NO: 252 - RNA, 23 nt, synthetic construct
  source 1..23: mol_type = other RNA
agtttcttcatccagttgaggga

SEQ ID NO: 253 - RNA, 23 nt, synthetic construct
  source 1..23: mol_type = other RNA
tatagtttcttcatccagttgag

SEQ ID NO: 254 - RNA, 23 nt, synthetic construct
  source 1..23: mol_type = other RNA
agatagtttcttcatccagttga

SEQ ID NO: 255 - RNA, 23 nt, synthetic construct
  source 1..23: mol_type = other RNA
tcataagatccttgcagcaccag

SEQ ID NO: 256 - RNA, 23 nt, synthetic construct
  source 1..23: mol_type = other RNA
aggtcataagatccttgcagcac

SEQ ID NO: 257 - RNA, 23 nt, synthetic construct
  source 1..23: mol_type = other RNA
aaaaaaatgctgttcagcacctc

SEQ ID NO: 258 - RNA, 23 nt, synthetic construct
  source 1..23: mol_type = other RNA
aaaaaaaatgctgttcagcacct

SEQ ID NO: 259 - RNA, 23 nt, synthetic construct
  source 1..23: mol_type = other RNA
tcaaaaaaaatgctgttcagcac

SEQ ID NO: 260 - RNA, 23 nt, synthetic construct
  source 1..23: mol_type = other RNA
agctcaaaaaaaatgctgttcag

SEQ ID NO: 261 - RNA, 23 nt, synthetic construct
  source 1..23: mol_type = other RNA
tcaagctcaaaaaaaatgctgtt

SEQ ID NO: 262 - RNA, 23 nt, synthetic construct
  source 1..23: mol_type = other RNA
tctctcatccgcttcaagctcaa

SEQ ID NO: 263 - RNA, 23 nt, synthetic construct
  source 1..23: mol_type = other RNA
tctctctcatccgcttcaagctc

SEQ ID NO: 264 - RNA, 23 nt, synthetic construct
  source 1..23: mol_type = other RNA
actctgtgggctctctctcatcc

SEQ ID NO: 265 - RNA, 23 nt, synthetic construct
  source 1..23: mol_type = other RNA
agactctgtgggctctctctcat

SEQ ID NO: 266 - RNA, 23 nt, synthetic construct
  source 1..23: mol_type = other RNA
tagactctgtgggctctctctca

SEQ ID NO: 267 - RNA, 23 nt, synthetic construct
  source 1..23: mol_type = other RNA
tttaagctgttgggtagactctg

SEQ ID NO: 268 - RNA, 23 nt, synthetic construct
  source 1..23: mol_type = other RNA
tgttaagctgttgggtagactct

SEQ ID NO: 269 - RNA, 23 nt, synthetic construct
  source 1..23: mol_type = other RNA
tatacacagcaaacaggaatggg

SEQ ID NO: 270 - RNA, 23 nt, synthetic construct
  source 1..23: mol_type = other RNA
tgatcatacacagcaaacaggaa

SEQ ID NO: 271 - RNA, 23 nt, synthetic construct
  source 1..23: mol_type = other RNA
ttttgatcatacacagcaaacag

SEQ ID NO: 272 - RNA, 23 nt, synthetic construct
  source 1..23: mol_type = other RNA
ttatctgctgctggcctttgcct

SEQ ID NO: 273 - RNA, 23 nt, synthetic construct
  source 1..23: mol_type = other RNA
actgggggtgacacatcgctgat

SEQ ID NO: 274 - RNA, 23 nt, synthetic construct
  source 1..23: mol_type = other RNA
agactgggggtgacacatcgctg

SEQ ID NO: 275 - RNA, 23 nt, synthetic construct
  source 1..23: mol_type = other RNA
tgagactgggggtgacacatcgc

SEQ ID NO: 276 - RNA, 23 nt, synthetic construct
  source 1..23: mol_type = other RNA
ttgggagactgggggtgacacat

SEQ ID NO: 277 - RNA, 23 nt, synthetic construct
  source 1..23: mol_type = other RNA
aggtgggagactgggggtgacac

SEQ ID NO: 278 - RNA, 23 nt, synthetic construct
  source 1..23: mol_type = other RNA
aaaggtgggagactgggggtgac

SEQ ID NO: 279 - RNA, 23 nt, synthetic construct
  source 1..23: mol_type = other RNA
taaaaggtgggagactgggggtg

SEQ ID NO: 280 - RNA, 23 nt, synthetic construct
  source 1..23: mol_type = other RNA
aagaaaaggtgggagactggggg

SEQ ID NO: 281 - RNA, 23 nt, synthetic construct
  source 1..23: mol_type = other RNA
agaagaaaaggtgggagactggg

SEQ ID NO: 282 - RNA, 23 nt, synthetic construct
  source 1..23: mol_type = other RNA
attagaagaaaaggtgggagact

SEQ ID NO: 283 - RNA, 23 nt, synthetic construct
  source 1..23: mol_type = other RNA
actcattaagaagaaaaggtggg

SEQ ID NO: 284 - RNA, 23 nt, synthetic construct
  source 1..23: mol_type = other RNA
tcgactcattagaagaaaaggtg

SEQ ID NO: 285 - RNA, 23 nt, synthetic construct
  source 1..23: mol_type = other RNA
ttagaccaaggagaaacggctgc

SEQ ID NO: 286 - RNA, 23 nt, synthetic construct
  source 1..23: mol_type = other RNA
tttagaccaaggagaaacggctg

SEQ ID NO: 287 - RNA, 23 nt, synthetic construct
  source 1..23: mol_type = other RNA
aaaataaacccagcaaactggga

SEQ ID NO: 288 - RNA, 23 nt, synthetic construct
  source 1..23: mol_type = other RNA
taaaataaacccagcaaactggg

SEQ ID NO: 289 - RNA, 23 nt, synthetic construct
  source 1..23: mol_type = other RNA
tcaggtactctcattgtggacga

SEQ ID NO: 290 - RNA, 23 nt, synthetic construct
  source 1..23: mol_type = other RNA
tatgaacctgtcaatcttctcag

SEQ ID NO: 291 - RNA, 23 nt, synthetic construct
  source 1..23: mol_type = other RNA
tctgtagtacccagaacaacggc

SEQ ID NO: 292 - RNA, 23 nt, synthetic construct
  source 1..23: mol_type = other RNA
tattgtggatgacgaggtggcag

SEQ ID NO: 293 - RNA, 23 nt, synthetic construct
  source 1..23: mol_type = other RNA
ttcattgtggatgacgaggtgga

SEQ ID NO: 294 - RNA, 23 nt, synthetic construct
  source 1..23: mol_type = other RNA
tacaggtactctcattgtggatg

SEQ ID NO: 295 - RNA, 23 nt, synthetic construct
  source 1..23: mol_type = other RNA
tccgcttcaagctcaaaaaacat

SEQ ID NO: 296 - RNA, 23 nt, synthetic construct
  source 1..23: mol_type = other RNA
tatccgcttcaagctcaaaacaa

SEQ ID NO: 297 - RNA, 23 nt, synthetic construct
  source 1..23: mol_type = other RNA
tcatccgcttcaagctcaaacaa

SEQ ID NO: 298 - RNA, 23 nt, synthetic construct
  source 1..23: mol_type = other RNA
taagaaaaggtgggagactgggg

SEQ ID NO: 299 - RNA, 23 nt, synthetic construct
  source 1..23: mol_type = other RNA
agaaaaggtgggagactggggag

SEQ ID NO: 300 - RNA, 23 nt, synthetic construct
  source 1..23: mol_type = other RNA
tgctttccagctcaaagtcgcct

SEQ ID NO: 301 - RNA, 23 nt, synthetic construct
  source 1..23: mol_type = other RNA
agaccaaggagaaacggctgctt

SEQ ID NO: 302 - RNA, 23 nt, synthetic construct
  source 1..23: mol_type = other RNA
acttagaccaaggagaaacggct

SEQ ID NO: 303 - RNA, 23 nt, synthetic construct
  source 1..23: mol_type = other RNA
acaggtactctcattgtggacga

SEQ ID NO: 304 - RNA, 23 nt, synthetic construct
  source 1..23: mol_type = other RNA
acaggtactctcattgtggatga

SEQ ID NO: 305 - RNA, 23 nt, synthetic construct
  source 1..23: mol_type = other RNA
aggtactctcattgtggatgccg

SEQ ID NO: 306 - RNA, 23 nt, synthetic construct
  source 1..23: mol_type = other RNA
tagaaaaggtgggagactggggg

SEQ ID NO: 307 - RNA, 23 nt, synthetic construct
  source 1..23: mol_type = other RNA
tgaagaaaaggtgggagactggg

SEQ ID NO: 308 - RNA, 23 nt, synthetic construct
  source 1..23: mol_type = other RNA
tagaagaaaaggtgggagaccgg

SEQ ID NO: 309 - RNA, 23 nt, synthetic construct
  source 1..23: mol_type = other RNA
ttagaagaaaaggtgggagactg

SEQ ID NO: 310 - RNA, 23 nt, synthetic construct
  source 1..23: mol_type = other RNA
tagaccaaggagaaacggctgct

SEQ ID NO: 311 - RNA, 23 nt, synthetic construct
  source 1..23: mol_type = other RNA
ttagaccaaggagaaacggccgc

SEQ ID NO: 312 - RNA, 23 nt, synthetic construct
  source 1..23: mol_type = other RNA
cttagaccaaggagaaacggctg

SEQ ID NO: 313 - RNA, 23 nt, synthetic construct
  source 1..23: mol_type = other RNA
cacttagaccaaggagaaacggc

SEQ ID NO: 314 - RNA, 23 nt, synthetic construct
  source 1..23: mol_type = other RNA
tacttagaccaaggagaaacggc

SEQ ID NO: 315 - RNA, 23 nt, synthetic construct
  source 1..23: mol_type = other RNA
acacttagaccaaggagaaacgg

SEQ ID NO: 316 - RNA, 23 nt, synthetic construct
  source 1..23: mol_type = other RNA
tcacttagaccaaggagaaacgg

SEQ ID NO: 317 - RNA, 23 nt, synthetic construct
  source 1..23: mol_type = other RNA
tcttagaccaaggagaaacggct

SEQ ID NO: 318 - RNA, 23 nt, synthetic construct
  source 1..23: mol_type = other RNA
acttagaccaaggagaaacgcct

SEQ ID NO: 319 - RNA, 23 nt, synthetic construct
  source 1..23: mol_type = other RNA
tcttagaccaaggagaaacgcct

SEQ ID NO: 320 - RNA, 21 nt, synthetic construct
  source 1..21: mol_type = other RNA
attagaagaaaaggtgggaga

SEQ ID NO: 321 - RNA, 21 nt, synthetic construct
  source 1..21: mol_type = other RNA
tttagaagaaaaggtgggcga

SEQ ID NO: 322 - RNA, 21 nt, synthetic construct
  source 1..21: mol_type = other RNA
ttactctcattgtggatgccg

SEQ ID NO: 323 - RNA, 21 nt, synthetic construct
  source 1..21: mol_type = other RNA
ttctcattgtggatgacgcgg

SEQ ID NO: 324 - RNA, 21 nt, synthetic construct
  source 1..21: mol_type = other RNA
ttcattgtggatgacgaggtg

SEQ ID NO: 325 - RNA, 21 nt, synthetic construct
  source 1..21: mol_type = other RNA
tattgtggatgacgaggtgga

SEQ ID NO: 326 - RNA, 21 nt, synthetic construct
  source 1..21: mol_type = other RNA
tggtactctcattgtggacga

SEQ ID NO: 327 - RNA, 21 nt, synthetic construct
  source 1..21: mol_type = other RNA
taggtactctcattgtggctg

SEQ ID NO: 328 - RNA, 21 nt, synthetic construct
  source 1..21: mol_type = other RNA
tacaggtactctcattgtgga

SEQ ID NO: 329 - RNA, 21 nt, synthetic construct
  source 1..21: mol_type = other RNA
tcacaggtactctcattgcgg

SEQ ID NO: 330 - RNA, 21 nt, synthetic construct
  source 1..21: mol_type = other RNA
ttcacaggtactctcattgtg

SEQ ID NO: 331 - RNA, 21 nt, synthetic construct
  source 1..21: mol_type = other RNA
tctcacaggtactctcatcgt

SEQ ID NO: 332 - RNA, 21 nt, synthetic construct
  source 1..21: mol_type = other RNA
ttgctcacaggtactctcctt

SEQ ID NO: 333 - RNA, 21 nt, synthetic construct
  source 1..21: mol_type = other RNA
tctgctcacaggtactctcat

SEQ ID NO: 334 - RNA, 21 nt, synthetic construct
  source 1..21: mol_type = other RNA
ttagaagaaaaggtgggagac

SEQ ID NO: 335 - RNA, 21 nt, synthetic construct
  source 1..21: mol_type = other RNA
tagaagaaaaggtgggagcct

SEQ ID NO: 336 - RNA, 21 nt, synthetic construct
  source 1..21: mol_type = other RNA
tgaagaaaaggtgggagactg

SEQ ID NO: 337 - RNA, 21 nt, synthetic construct
  source 1..21: mol_type = other RNA
taagaaaaggtgggagaccgg

SEQ ID NO: 338 - RNA, 21 nt, synthetic construct
  source 1..21: mol_type = other RNA
tattagaagaaaaggtgggag

SEQ ID NO: 339 - RNA, 21 nt, synthetic construct
  source 1..21: mol_type = other RNA
tcattagaagaaaaggtggga

SEQ ID NO: 340 - RNA, 21 nt, synthetic construct
  source 1..21: mol_type = other RNA
ttcattagaagaaaaggtggg

SEQ ID NO: 341 - RNA, 21 nt, synthetic construct
  source 1..21: mol_type = other RNA
tctcattagaagaaaaggcgg

SEQ ID NO: 342 - RNA, 21 nt, synthetic construct
  source 1..21: mol_type = other RNA
tactcattagaagaaaaggtg

SEQ ID NO: 343 - RNA, 21 nt, synthetic construct
  source 1..21: mol_type = other RNA
tgactcattagaagaaaaggt

SEQ ID NO: 344 - RNA, 21 nt, synthetic construct
  source 1..21: mol_type = other RNA
aaacagaaattcaggtgcttg

SEQ ID NO: 345 - RNA, 21 nt, synthetic construct
  source 1..21: mol_type = other RNA
aaactaaggtattacagacac

SEQ ID NO: 346 - RNA, 21 nt, synthetic construct
  source 1..21: mol_type = other RNA
aaactgggaggtgcatttgtg

SEQ ID NO: 347 - RNA, 21 nt, synthetic construct
  source 1..21: mol_type = other RNA
aaagccagggtgctgtccaca

SEQ ID NO: 348 - RNA, 21 nt, synthetic construct
  source 1..21: mol_type = other RNA
aaagtcgactcattagaagaa

SEQ ID NO: 349 - RNA, 21 nt, synthetic construct
  source 1..21: mol_type = other RNA
aaagtgagaccctccaccttg

SEQ ID NO: 350 - RNA, 21 nt, synthetic construct
  source 1..21: mol_type = other RNA
aaataaccagctatggttccg

SEQ ID NO: 351 - RNA, 21 nt, synthetic construct
  source 1..21: mol_type = other RNA
aaatacaaaccgaaggcaatg

SEQ ID NO: 352 - RNA, 21 nt, synthetic construct
  source 1..21: mol_type = other RNA
aagacactaaatacaaaccga

SEQ ID NO: 353 - RNA, 21 nt, synthetic construct
  source 1..21: mol_type = other RNA
aatttttgttctcaacttgaa

SEQ ID NO: 354 - RNA, 21 nt, synthetic construct
  source 1..21: mol_type = other RNA
acttttttgtttcacaaacaa

SEQ ID NO: 355 - RNA, 21 nt, synthetic construct
  source 1..21: mol_type = other RNA
agaccctccaccttgtccagg

SEQ ID NO: 356 - RNA, 21 nt, synthetic construct
  source 1..21: mol_type = other RNA
agttttgctggaaagtgagac

SEQ ID NO: 357 - RNA, 21 nt, synthetic construct
  source 1..21: mol_type = other RNA
atacggaagcccaagaagttg

SEQ ID NO: 358 - RNA, 21 nt, synthetic construct
  source 1..21: mol_type = other RNA
atgttcttacattcaagacac

SEQ ID NO: 359 - RNA, 21 nt, synthetic construct
  source 1..21: mol_type = other RNA
catacacagcaaacaggaatg

SEQ ID NO: 360 - RNA, 21 nt, synthetic construct
  source 1..21: mol_type = other RNA
ctaaacactggttcttgcctc

SEQ ID NO: 361 - RNA, 21 nt, synthetic construct
  source 1..21: mol_type = other RNA
ctgcatgaacctgtcaatctt

SEQ ID NO: 362 - RNA, 21 nt, synthetic construct
  source 1..21: mol_type = other RNA
ctgtgcatgccatatatacgg

SEQ ID NO: 363 - RNA, 21 nt, synthetic construct
  source 1..21: mol_type = other RNA
gagaaataaccagctatggtt

SEQ ID NO: 364 - RNA, 21 nt, synthetic construct
  source 1..21: mol_type = other RNA
ggaggtcatgttcttacattc

SEQ ID NO: 365 - RNA, 21 nt, synthetic construct
  source 1..21: mol_type = other RNA
gtgcatgccatatatacggaa

SEQ ID NO: 366 - RNA, 21 nt, synthetic construct
  source 1..21: mol_type = other RNA
gttcttacattcaagacacta

SEQ ID NO: 367 - RNA, 21 nt, synthetic construct
  source 1..21: mol_type = other RNA
taaacactggttcttgcctcc

SEQ ID NO: 368 - RNA, 21 nt, synthetic construct
  source 1..21: mol_type = other RNA
tacacagcaaacaggaatggg

SEQ ID NO: 369 - RNA, 21 nt, synthetic construct
  source 1..21: mol_type = other RNA
tactttaattttaaaacccaa

SEQ ID NO: 370 - RNA, 21 nt, synthetic construct
  source 1..21: mol_type = other RNA
tatacggaagcccaagaagtt

SEQ ID NO: 371 - RNA, 21 nt, synthetic construct
  source 1..21: mol_type = other RNA
tatactttaattttaaaaccc

SEQ ID NO: 372 - RNA, 21 nt, synthetic construct
  source 1..21: mol_type = other RNA
tcactgtgcatgccatatata

SEQ ID NO: 373 - RNA, 21 nt, synthetic construct
  source 1..21: mol_type = other RNA
tcatgttcttacattcaagac

SEQ ID NO: 374 - RNA, 21 nt, synthetic construct
  source 1..21: mol_type = other RNA
tcctgcaggtcataagatcct

SEQ ID NO: 375 - RNA, 21 nt, synthetic construct
  source 1..21: mol_type = other RNA
tgaggtgctgttgtccaccca

SEQ ID NO: 376 - RNA, 21 nt, synthetic construct
  source 1..21: mol_type = other RNA
tgcatgaacctgtcaatcttc

SEQ ID NO: 377 - RNA, 21 nt, synthetic construct
  source 1..21: mol_type = other RNA
tgtcacagcctgcatgaacct

SEQ ID NO: 378 - RNA, 21 nt, synthetic construct
  source 1..21: mol_type = other RNA
tgtccacccagaactcctggg

SEQ ID NO: 379 - RNA, 21 nt, synthetic construct
  source 1..21: mol_type = other RNA
tgtgcatgccatatatacgga

SEQ ID NO: 380 - RNA, 21 nt, synthetic construct
  source 1..21: mol_type = other RNA
ttcatccagttgagggagttt

SEQ ID NO: 381 - RNA, 21 nt, synthetic construct
  source 1..21: mol_type = other RNA
ttgctggaaagtgagaccctc

SEQ ID NO: 382 - RNA, 21 nt, synthetic construct
  source 1..21: mol_type = other RNA
ttgtccacccagaactcctgg

SEQ ID NO: 383 - RNA, 21 nt, synthetic construct
  source 1..21: mol_type = other RNA
tttcacaaacaagctggtcgg

SEQ ID NO: 384 - RNA, 21 nt, synthetic construct
  source 1..21: mol_type = other RNA
tttgccagctgctcacaggta

SEQ ID NO: 385 - RNA, 21 nt, synthetic construct
  source 1..21: mol_type = other RNA
tttgctggaaagtgagaccct

SEQ ID NO: 386 - RNA, 21 nt, synthetic construct
  source 1..21: mol_type = other RNA
ttttaaaacccaatttttgtt

SEQ ID NO: 387 - RNA, 21 nt, synthetic construct
  source 1..21: mol_type = other RNA
ttttgtttcacaaacaagctg

SEQ ID NO: 388 - RNA, 21 nt, synthetic construct
  source 1..21: mol_type = other RNA
tgttagtaataaacgtcttgc

SEQ ID NO: 389 - RNA, 21 nt, synthetic construct
  source 1..21: mol_type = other RNA
ttcacaaacaagctggtcggt

SEQ ID NO: 390 - RNA, 21 nt, synthetic construct
  source 1..21: mol_type = other RNA
tttttgtttcacaaacaagct

SEQ ID NO: 391 - RNA, 21 nt, synthetic construct
  source 1..21: mol_type = other RNA
tgagtcaccgagaagttgtcc

SEQ ID NO: 392 - RNA, 21 nt, synthetic construct
  source 1..21: mol_type = other RNA
ttggccagcatcccgaccatt

SEQ ID NO: 393 - RNA, 21 nt, synthetic construct
  source 1..21: mol_type = other RNA
cattcaaacagaaattcaggt

SEQ ID NO: 394 - RNA, 21 nt, synthetic construct
  source 1..21: mol_type = other RNA
ctgcaggtcataagatccttg

SEQ ID NO: 395 - RNA, 21 nt, synthetic construct
  source 1..21: mol_type = other RNA
tgaacctgtcaatcttctcag

SEQ ID NO: 396 - RNA, 21 nt, synthetic construct
  source 1..21: mol_type = other RNA
ttggaattctttttggaacag

SEQ ID NO: 397 - RNA, 21 nt, synthetic construct
  source 1..21: mol_type = other RNA
cggaggtcatgttcttacatt

SEQ ID NO: 398 - RNA, 21 nt, synthetic construct
  source 1..21: mol_type = other RNA
tagcaggccctgtacagcctg

SEQ ID NO: 399 - RNA, 21 nt, synthetic construct
  source 1..21: mol_type = other RNA
tagtttcttcatccagttgag

SEQ ID NO: 400 - RNA, 21 nt, synthetic construct
  source 1..21: mol_type = other RNA
ttcttcatccagttgagggag

SEQ ID NO: 401 - RNA, 21 nt, synthetic construct
  source 1..21: mol_type = other RNA
tgcttgcatctttcacgtatt

SEQ ID NO: 402 - RNA, 21 nt, synthetic construct
  source 1..21: mol_type = other RNA
atctgctgctggcctttgcct

SEQ ID NO: 403 - RNA, 21 nt, synthetic construct
  source 1..21: mol_type = other RNA
caggtcataagatccttgcag

SEQ ID NO: 404 - RNA, 21 nt, synthetic construct
  source 1..21: mol_type = other RNA
ttgcctgtagcctgtcagctg

SEQ ID NO: 405 - RNA, 21 nt, synthetic construct
  source 1..21: mol_type = other RNA
tttattactaacacaagggag

SEQ ID NO: 406 - RNA, 21 nt, synthetic construct
  source 1..21: mol_type = other RNA
caaacagaaattcaggtgctt

SEQ ID NO: 407 - RNA, 21 nt, synthetic construct
  source 1..21: mol_type = other RNA
ctggcctcatgctgtgctcag

SEQ ID NO: 408 - RNA, 21 nt, synthetic construct
  source 1..21: mol_type = other RNA
tattactaacacaagggagaa

SEQ ID NO: 409 - RNA, 21 nt, synthetic construct
  source 1..21: mol_type = other RNA
tgcatctttcacgtattgttc

SEQ ID NO: 410 - RNA, 21 nt, synthetic construct
  source 1..21: mol_type = other RNA
catctttcacgtattgttcaa

SEQ ID NO: 411 - RNA, 21 nt, synthetic construct
  source 1..21: mol_type = other RNA
tactaacacaagggagaaata

SEQ ID NO: 412 - RNA, 21 nt, synthetic construct
  source 1..21: mol_type = other RNA
ttgggcttcccggcattggcc

SEQ ID NO: 413 - RNA, 21 nt, synthetic construct
  source 1..21: mol_type = other RNA
agaaattcaggtgcttgcatc

SEQ ID NO: 414 - RNA, 21 nt, synthetic construct
  source 1..21: mol_type = other RNA
ataagatccttgcagcaccag

SEQ ID NO: 415 - RNA, 21 nt, synthetic construct
  source 1..21: mol_type = other RNA
tagcctgtcagctgtgtggtc

SEQ ID NO: 416 - RNA, 21 nt, synthetic construct
  source 1..21: mol_type = other RNA
tctttcacgtattgttcaaaa

SEQ ID NO: 417 - RNA, 21 nt, synthetic construct
  source 1..21: mol_type = other RNA
tcaacttgtcttcggtgtcaa

SEQ ID NO: 418 - RNA, 21 nt, synthetic construct
  source 1..21: mol_type = other RNA
gtgctgtccacactggctccc

SEQ ID NO: 419 - RNA, 21 nt, synthetic construct
  source 1..21: mol_type = other RNA
tgcagttcttgtccttccaag

SEQ ID NO: 420 - RNA, 21 nt, synthetic construct
  source 1..21: mol_type = other RNA
ttgagtcaccgagaagttgtc

SEQ ID NO: 421 - RNA, 21 nt, synthetic construct
  source 1..21: mol_type = other RNA
cttattgtggcaagacgttta

SEQ ID NO: 422 - RNA, 21 nt, synthetic construct
  source 1..21: mol_type = other RNA
aacctgtcaatcttctcagca

SEQ ID NO: 423 - RNA, 21 nt, synthetic construct
  source 1..21: mol_type = other RNA
aataaacccagcaaactggga

SEQ ID NO: 424 - RNA, 21 nt, synthetic construct
  source 1..21: mol_type = other RNA
acttgagtcaccgagaagttg

SEQ ID NO: 425 - RNA, 21 nt, synthetic construct
  modified_base 1..6: mod_base = OTHER; note = 2'-methoxy nucleoside; note (original language) = 2'-甲氧基核苷
  modified_base 8: mod_base = OTHER; note = 2'-methoxy nucleoside; note (original language) = 2'-甲氧基核苷
  modified_base 12..21: mod_base = OTHER; note = 2'-methoxy nucleoside; note (original language) = 2'-甲氧基核苷
  modified_base 7: mod_base = OTHER; note = 2'-fluoro nucleoside; note (original language) = 2'-氟核苷
  modified_base 9..11: mod_base = OTHER; note = 2'-fluoro nucleoside; note (original language) = 2'-氟核苷
  modified_base 1..3: mod_base = OTHER; note = phosphorothioate bond; note (original language) = 硫代磷酸酯键
  source 1..21: mol_type = other RNA
gtcatccacaatgagagtaca

SEQ ID NO: 426 - RNA, 21 nt, synthetic construct
  modified_base 1..6: mod_base = OTHER; note = 2'-methoxy nucleoside; note (original language) = 2'-甲氧基核苷
  modified_base 8: mod_base = OTHER; note = 2'-methoxy nucleoside; note (original language) = 2'-甲氧基核苷
  modified_base 12..21: mod_base = OTHER; note = 2'-methoxy nucleoside; note (original language) = 2'-甲氧基核苷
  modified_base 7: mod_base = OTHER; note = 2'-fluoro nucleoside; note (original language) = 2'-氟核苷
  modified_base 9..11: mod_base = OTHER; note = 2'-fluoro nucleoside; note (original language) = 2'-氟核苷
  modified_base 1..3: mod_base = OTHER; note = phosphorothioate bond; note (original language) = 硫代磷酸酯键
  source 1..21: mol_type = other RNA
ccacctcgtcatccacaatga

SEQ ID NO: 427 - RNA, 21 nt, synthetic construct
  modified_base 1..6: mod_base = OTHER; note = 2'-methoxy nucleoside; note (original language) = 2'-甲氧基核苷
  modified_base 8: mod_base = OTHER; note = 2'-methoxy nucleoside; note (original language) = 2'-甲氧基核苷
  modified_base 12..21: mod_base = OTHER; note = 2'-methoxy nucleoside; note (original language) = 2'-甲氧基核苷
  modified_base 7: mod_base = OTHER; note = 2'-fluoro nucleoside; note (original language) = 2'-氟核苷
  modified_base 9..11: mod_base = OTHER; note = 2'-fluoro nucleoside; note (original language) = 2'-氟核苷
  modified_base 1..3: mod_base = OTHER; note = phosphorothioate bond; note (original language) = 硫代磷酸酯键
  source 1..21: mol_type = other RNA
cctcgtcatccacaatgagaa

SEQ ID NO: 428 - RNA, 21 nt, synthetic construct
  modified_base 1..6: mod_base = OTHER; note = 2'-methoxy nucleoside; note (original language) = 2'-甲氧基核苷
  modified_base 8: mod_base = OTHER; note = 2'-methoxy nucleoside; note (original language) = 2'-甲氧基核苷
  modified_base 12..21: mod_base = OTHER; note = 2'-methoxy nucleoside; note (original language) = 2'-甲氧基核苷
  modified_base 7: mod_base = OTHER; note = 2'-fluoro nucleoside; note (original language) = 2'-氟核苷
  modified_base 9..11: mod_base = OTHER; note = 2'-fluoro nucleoside; note (original language) = 2'-氟核苷
  modified_base 1..3: mod_base = OTHER; note = phosphorothioate bond; note (original language) = 硫代磷酸酯键
  source 1..21: mol_type = other RNA
atccacaatgagagtacctga

SEQ ID NO: 429 - RNA, 21 nt, synthetic construct
  modified_base 1..6: mod_base = OTHER; note = 2'-methoxy nucleoside; note (original language) = 2'-甲氧基核苷
  modified_base 8: mod_base = OTHER; note = 2'-methoxy nucleoside; note (original language) = 2'-甲氧基核苷
  modified_base 12..21: mod_base = OTHER; note = 2'-methoxy nucleoside; note (original language) = 2'-甲氧基核苷
  modified_base 7: mod_base = OTHER; note = 2'-fluoro nucleoside; note (original language) = 2'-氟核苷
  modified_base 9..11: mod_base = OTHER; note = 2'-fluoro nucleoside; note (original language) = 2'-氟核苷
  modified_base 1..3: mod_base = OTHER; note = phosphorothioate bond; note (original language) = 硫代磷酸酯键
  source 1..21: mol_type = other RNA
ggcatgcacagtgagctatga

SEQ ID NO: 430 - RNA, 21 nt, synthetic construct
  modified_base 1..6: mod_base = OTHER; note = 2'-methoxy nucleoside; note (original language) = 2'-甲氧基核苷
  modified_base 8: mod_base = OTHER; note = 2'-methoxy nucleoside; note (original language) = 2'-甲氧基核苷
  modified_base 12..21: mod_base = OTHER; note = 2'-methoxy nucleoside; note (original language) = 2'-甲氧基核苷
  modified_base 7: mod_base = OTHER; note = 2'-fluoro nucleoside; note (original language) = 2'-氟核苷
  modified_base 9..11: mod_base = OTHER; note = 2'-fluoro nucleoside; note (original language) = 2'-氟核苷
  modified_base 1..3: mod_base = OTHER; note = phosphorothioate bond; note (original language) = 硫代磷酸酯键
  source 1..21: mol_type = other RNA
gagaagattgacaggttcatg

SEQ ID NO: 431 - RNA, 21 nt, synthetic construct
  modified_base 1..6: mod_base = OTHER; note = 2'-methoxy nucleoside; note (original language) = 2'-甲氧基核苷
  modified_base 8: mod_base = OTHER; note = 2'-methoxy nucleoside; note (original language) = 2'-甲氧基核苷
  modified_base 12..21: mod_base = OTHER; note = 2'-methoxy nucleoside; note (original language) = 2'-甲氧基核苷
  modified_base 7: mod_base = OTHER; note = 2'-fluoro nucleoside; note (original language) = 2'-氟核苷
  modified_base 9..11: mod_base = OTHER; note = 2'-fluoro nucleoside; note (original language) = 2'-氟核苷
  modified_base 1..3: mod_base = OTHER; note = phosphorothioate bond; note (original language) = 硫代磷酸酯键
  source 1..21: mol_type = other RNA
ggacagcaccctggctttcaa

SEQ ID NO: 432 - RNA, 21 nt, synthetic construct
  modified_base 1..6: mod_base = OTHER; note = 2'-methoxy nucleoside; note (original language) = 2'-甲氧基核苷
  modified_base 8: mod_base = OTHER; note = 2'-methoxy nucleoside; note (original language) = 2'-甲氧基核苷
  modified_base 12..21: mod_base = OTHER; note = 2'-methoxy nucleoside; note (original language) = 2'-甲氧基核苷
  modified_base 7: mod_base = OTHER; note = 2'-fluoro nucleoside; note (original language) = 2'-氟核苷
  modified_base 9..11: mod_base = OTHER; note = 2'-fluoro nucleoside; note (original language) = 2'-氟核苷
  modified_base 1..3: mod_base = OTHER; note = phosphorothioate bond; note (original language) = 硫代磷酸酯键
  source 1..21: mol_type = other RNA
gctgaacagcattttttttga

SEQ ID NO: 433 - RNA, 21 nt, synthetic construct
  modified_base 1..6: mod_base = OTHER; note = 2'-methoxy nucleoside; note (original language) = 2'-甲氧基核苷
  modified_base 8: mod_base = OTHER; note = 2'-methoxy nucleoside; note (original language) = 2'-甲氧基核苷
  modified_base 12..21: mod_base = OTHER; note = 2'-methoxy nucleoside; note (original language) = 2'-甲氧基核苷
  modified_base 7: mod_base = OTHER; note = 2'-fluoro nucleoside; note (original language) = 2'-氟核苷
  modified_base 9..11: mod_base = OTHER; note = 2'-fluoro nucleoside; note (original language) = 2'-氟核苷
  modified_base 1..3: mod_base = OTHER; note = phosphorothioate bond; note (original language) = 硫代磷酸酯键
  source 1..21: mol_type = other RNA
gagcttgaagcggatgagaga

SEQ ID NO: 434 - RNA, 21 nt, synthetic construct
  modified_base 1..6: mod_base = OTHER; note = 2'-methoxy nucleoside; note (original language) = 2'-甲氧基核苷
  modified_base 8: mod_base = OTHER; note = 2'-methoxy nucleoside; note (original language) = 2'-甲氧基核苷
  modified_base 12..21: mod_base = OTHER; note = 2'-methoxy nucleoside; note (original language) = 2'-甲氧基核苷
  modified_base 7: mod_base = OTHER; note = 2'-fluoro nucleoside; note (original language) = 2'-氟核苷
  modified_base 9..11: mod_base = OTHER; note = 2'-fluoro nucleoside; note (original language) = 2'-氟核苷
  modified_base 1..3: mod_base = OTHER; note = phosphorothioate bond; note (original language) = 硫代磷酸酯键
  source 1..21: mol_type = other RNA
gagagagagcccacagagtct

SEQ ID NO: 435 - RNA, 21 nt, synthetic construct
  modified_base 1..6: mod_base = OTHER; note = 2'-methoxy nucleoside; note (original language) = 2'-甲氧基核苷
  modified_base 8: mod_base = OTHER; note = 2'-methoxy nucleoside; note (original language) = 2'-甲氧基核苷
  modified_base 12..21: mod_base = OTHER; note = 2'-methoxy nucleoside; note (original language) = 2'-甲氧基核苷
  modified_base 7: mod_base = OTHER; note = 2'-fluoro nucleoside; note (original language) = 2'-氟核苷
  modified_base 9..11: mod_base = OTHER; note = 2'-fluoro nucleoside; note (original language) = 2'-氟核苷
  modified_base 1..3: mod_base = OTHER; note = phosphorothioate bond; note (original language) = 硫代磷酸酯键
  source 1..21: mol_type = other RNA
cccagtctcccaccttttctt

SEQ ID NO: 436 - RNA, 21 nt, synthetic construct
  modified_base 1..6: mod_base = OTHER; note = 2'-methoxy nucleoside; note (original language) = 2'-甲氧基核苷
  modified_base 8: mod_base = OTHER; note = 2'-methoxy nucleoside; note (original language) = 2'-甲氧基核苷
  modified_base 12..21: mod_base = OTHER; note = 2'-methoxy nucleoside; note (original language) = 2'-甲氧基核苷
  modified_base 7: mod_base = OTHER; note = 2'-fluoro nucleoside; note (original language) = 2'-氟核苷
  modified_base 9..11: mod_base = OTHER; note = 2'-fluoro nucleoside; note (original language) = 2'-氟核苷
  modified_base 1..3: mod_base = OTHER; note = phosphorothioate bond; note (original language) = 硫代磷酸酯键
  source 1..21: mol_type = other RNA
cagtctcccaccttttcttct

SEQ ID NO: 437 - RNA, 21 nt, synthetic construct
  modified_base 1..6: mod_base = OTHER; note = 2'-methoxy nucleoside; note (original language) = 2'-甲氧基核苷
  modified_base 8: mod_base = OTHER; note = 2'-methoxy nucleoside; note (original language) = 2'-甲氧基核苷
  modified_base 12..21: mod_base = OTHER; note = 2'-methoxy nucleoside; note (original language) = 2'-甲氧基核苷
  modified_base 7: mod_base = OTHER; note = 2'-fluoro nucleoside; note (original language) = 2'-氟核苷
  modified_base 9..11: mod_base = OTHER; note = 2'-fluoro nucleoside; note (original language) = 2'-氟核苷
  modified_base 1..3: mod_base = OTHER; note = phosphorothioate bond; note (original language) = 硫代磷酸酯键
  source 1..21: mol_type = other RNA
ccttttcttctaatgagtcga

SEQ ID NO: 438 - RNA, 21 nt, synthetic construct
  modified_base 1..6: mod_base = OTHER; note = 2'-methoxy nucleoside; note (original language) = 2'-甲氧基核苷
  modified_base 8: mod_base = OTHER; note = 2'-methoxy nucleoside; note (original language) = 2'-甲氧基核苷
  modified_base 12..21: mod_base = OTHER; note = 2'-methoxy nucleoside; note (original language) = 2'-甲氧基核苷
  modified_base 7: mod_base = OTHER; note = 2'-fluoro nucleoside; note (original language) = 2'-氟核苷
  modified_base 9..11: mod_base = OTHER; note = 2'-fluoro nucleoside; note (original language) = 2'-氟核苷
  modified_base 1..3: mod_base = OTHER; note = phosphorothioate bond; note (original language) = 硫代磷酸酯键
  source 1..21: mol_type = other RNA
agccgtttctccttggtctaa

SEQ ID NO: 439 - RNA, 21 nt, synthetic construct
  modified_base 1..6: mod_base = OTHER; note = 2'-methoxy nucleoside; note (original language) = 2'-甲氧基核苷
  modified_base 8: mod_base = OTHER; note = 2'-methoxy nucleoside; note (original language) = 2'-甲氧基核苷
  modified_base 12..21: mod_base = OTHER; note = 2'-methoxy nucleoside; note (original language) = 2'-甲氧基核苷
  modified_base 7: mod_base = OTHER; note = 2'-fluoro nucleoside; note (original language) = 2'-氟核苷
  modified_base 9..11: mod_base = OTHER; note = 2'-fluoro nucleoside; note (original language) = 2'-氟核苷
  modified_base 1..3: mod_base = OTHER; note = phosphorothioate bond; note (original language) = 硫代磷酸酯键
  source 1..21: mol_type = other RNA
gccgtttctccttggtctaaa

SEQ ID NO: 440 - RNA, 21 nt, synthetic construct
  modified_base 1..6: mod_base = OTHER; note = 2'-methoxy nucleoside; note (original language) = 2'-甲氧基核苷
  modified_base 8: mod_base = OTHER; note = 2'-methoxy nucleoside; note (original language) = 2'-甲氧基核苷
  modified_base 12..21: mod_base = OTHER; note = 2'-methoxy nucleoside; note (original language) = 2'-甲氧基核苷
  modified_base 7: mod_base = OTHER; note = 2'-fluoro nucleoside; note (original language) = 2'-氟核苷
  modified_base 9..11: mod_base = OTHER; note = 2'-fluoro nucleoside; note (original language) = 2'-氟核苷
  modified_base 1..3: mod_base = OTHER; note = phosphorothioate bond; note (original language) = 硫代磷酸酯键
  source 1..21: mol_type = other RNA
gtccacaatgagagtacctga

SEQ ID NO: 441 - RNA, 21 nt, synthetic construct
  modified_base 1..6: mod_base = OTHER; note = 2'-methoxy nucleoside; note (original language) = 2'-甲氧基核苷
  modified_base 8: mod_base = OTHER; note = 2'-methoxy nucleoside; note (original language) = 2'-甲氧基核苷
  modified_base 12..21: mod_base = OTHER; note = 2'-methoxy nucleoside; note (original language) = 2'-甲氧基核苷
  modified_base 7: mod_base = OTHER; note = 2'-fluoro nucleoside; note (original language) = 2'-氟核苷
  modified_base 9..11: mod_base = OTHER; note = 2'-fluoro nucleoside; note (original language) = 2'-氟核苷
  modified_base 1..3: mod_base = OTHER; note = phosphorothioate bond; note (original language) = 硫代磷酸酯键
  source 1..21: mol_type = other RNA
ggcatgcacactgagctatga

SEQ ID NO: 442 - RNA, 21 nt, synthetic construct
  modified_base 1..6: mod_base = OTHER; note = 2'-methoxy nucleoside; note (original language) = 2'-甲氧基核苷
  modified_base 8: mod_base = OTHER; note = 2'-methoxy nucleoside; note (original language) = 2'-甲氧基核苷
  modified_base 12..21: mod_base = OTHER; note = 2'-methoxy nucleoside; note (original language) = 2'-甲氧基核苷
  modified_base 7: mod_base = OTHER; note = 2'-fluoro nucleoside; note (original language) = 2'-氟核苷
  modified_base 9..11: mod_base = OTHER; note = 2'-fluoro nucleoside; note (original language) = 2'-氟核苷
  modified_base 1..3: mod_base = OTHER; note = phosphorothioate bond; note (original language) = 硫代磷酸酯键
  source 1..21: mol_type = other RNA
gagaagattgacaggttcata

SEQ ID NO: 443 - RNA, 21 nt, synthetic construct
  modified_base 1..6: mod_base = OTHER; note = 2'-methoxy nucleoside; note (original language) = 2'-甲氧基核苷
  modified_base 8: mod_base = OTHER; note = 2'-methoxy nucleoside; note (original language) = 2'-甲氧基核苷
  modified_base 12..21: mod_base = OTHER; note = 2'-methoxy nucleoside; note (original language) = 2'-甲氧基核苷
  modified_base 7: mod_base = OTHER; note = 2'-fluoro nucleoside; note (original language) = 2'-氟核苷
  modified_base 9..11: mod_base = OTHER; note = 2'-fluoro nucleoside; note (original language) = 2'-氟核苷
  modified_base 1..3: mod_base = OTHER; note = phosphorothioate bond; note (original language) = 硫代磷酸酯键
  source 1..21: mol_type = other RNA
ggacagcaccgtggctttcaa

SEQ ID NO: 444 - RNA, 21 nt, synthetic construct
  modified_base 1..6: mod_base = OTHER; note = 2'-methoxy nucleoside; note (original language) = 2'-甲氧基核苷
  modified_base 8: mod_base = OTHER; note = 2'-methoxy nucleoside; note (original language) = 2'-甲氧基核苷
  modified_base 12..21: mod_base = OTHER; note = 2'-methoxy nucleoside; note (original language) = 2'-甲氧基核苷
  modified_base 7: mod_base = OTHER; note = 2'-fluoro nucleoside; note (original language) = 2'-氟核苷
  modified_base 9..11: mod_base = OTHER; note = 2'-fluoro nucleoside; note (original language) = 2'-氟核苷
  modified_base 1..3: mod_base = OTHER; note = phosphorothioate bond; note (original language) = 硫代磷酸酯键
  source 1..21: mol_type = other RNA
gctgaacagcgttttttttga

SEQ ID NO: 445 - RNA, 21 nt, synthetic construct
  modified_base 1..6: mod_base = OTHER; note = 2'-methoxy nucleoside; note (original language) = 2'-甲氧基核苷
  modified_base 8: mod_base = OTHER; note = 2'-methoxy nucleoside; note (original language) = 2'-甲氧基核苷
  modified_base 12..21: mod_base = OTHER; note = 2'-methoxy nucleoside; note (original language) = 2'-甲氧基核苷
  modified_base 7: mod_base = OTHER; note = 2'-fluoro nucleoside; note (original language) = 2'-氟核苷
  modified_base 9..11: mod_base = OTHER; note = 2'-fluoro nucleoside; note (original language) = 2'-氟核苷
  modified_base 1..3: mod_base = OTHER; note = phosphorothioate bond; note (original language) = 硫代磷酸酯键
  source 1..21: mol_type = other RNA
ccttttcttcgaatgagtcga

SEQ ID NO: 446 - RNA, 21 nt, synthetic construct
  modified_base 1..6: mod_base = OTHER; note = 2'-methoxy nucleoside; note (original language) = 2'-甲氧基核苷
  modified_base 8: mod_base = OTHER; note = 2'-methoxy nucleoside; note (original language) = 2'-甲氧基核苷
  modified_base 12..21: mod_base = OTHER; note = 2'-methoxy nucleoside; note (original language) = 2'-甲氧基核苷
  modified_base 7: mod_base = OTHER; note = 2'-fluoro nucleoside; note (original language) = 2'-氟核苷
  modified_base 9..11: mod_base = OTHER; note = 2'-fluoro nucleoside; note (original language) = 2'-氟核苷
  modified_base 1..3: mod_base = OTHER; note = phosphorothioate bond; note (original language) = 硫代磷酸酯键
  source 1..21: mol_type = other RNA
agccgtttctgcttggtctaa

SEQ ID NO: 447 - RNA, 21 nt, synthetic construct
  modified_base 1..6: mod_base = OTHER; note = 2'-methoxy nucleoside; note (original language) = 2'-甲氧基核苷
  modified_base 8: mod_base = OTHER; note = 2'-methoxy nucleoside; note (original language) = 2'-甲氧基核苷
  modified_base 12..21: mod_base = OTHER; note = 2'-methoxy nucleoside; note (original language) = 2'-甲氧基核苷
  modified_base 7: mod_base = OTHER; note = 2'-fluoro nucleoside; note (original language) = 2'-氟核苷
  modified_base 9..11: mod_base = OTHER; note = 2'-fluoro nucleoside; note (original language) = 2'-氟核苷
  modified_base 1..3: mod_base = OTHER; note = phosphorothioate bond; note (original language) = 硫代磷酸酯键
  source 1..21: mol_type = other RNA
gccgtttctgcttggtctaaa

SEQ ID NO: 448 - RNA, 21 nt, synthetic construct
  modified_base 1..6: mod_base = OTHER; note = 2'-methoxy nucleoside; note (original language) = 2'-甲氧基核苷
  modified_base 8: mod_base = OTHER; note = 2'-methoxy nucleoside; note (original language) = 2'-甲氧基核苷
  modified_base 12..21: mod_base = OTHER; note = 2'-methoxy nucleoside; note (original language) = 2'-甲氧基核苷
  modified_base 7: mod_base = OTHER; note = 2'-fluoro nucleoside; note (original language) = 2'-氟核苷
  modified_base 9..11: mod_base = OTHER; note = 2'-fluoro nucleoside; note (original language) = 2'-氟核苷
  modified_base 1..3: mod_base = OTHER; note = phosphorothioate bond; note (original language) = 硫代磷酸酯键
  source 1..21: mol_type = other RNA
cgttgttctgggtactacaga

SEQ ID NO: 449 - RNA, 21 nt, synthetic construct
  modified_base 1..6: mod_base = OTHER; note = 2'-methoxy nucleoside; note (original language) = 2'-甲氧基核苷
  modified_base 8: mod_base = OTHER; note = 2'-methoxy nucleoside; note (original language) = 2'-甲氧基核苷
  modified_base 12..21: mod_base = OTHER; note = 2'-methoxy nucleoside; note (original language) = 2'-甲氧基核苷
  modified_base 7: mod_base = OTHER; note = 2'-fluoro nucleoside; note (original language) = 2'-氟核苷
  modified_base 9..11: mod_base = OTHER; note = 2'-fluoro nucleoside; note (original language) = 2'-氟核苷
  modified_base 1..3: mod_base = OTHER; note = phosphorothioate bond; note (original language) = 硫代磷酸酯键
  source 1..21: mol_type = other RNA
gccacctcgtcatccacaata

SEQ ID NO: 450 - RNA, 21 nt, synthetic construct
  modified_base 1..6: mod_base = OTHER; note = 2'-methoxy nucleoside; note (original language) = 2'-甲氧基核苷
  modified_base 8: mod_base = OTHER; note = 2'-methoxy nucleoside; note (original language) = 2'-甲氧基核苷
  modified_base 12..21: mod_base = OTHER; note = 2'-methoxy nucleoside; note (original language) = 2'-甲氧基核苷
  modified_base 7: mod_base = OTHER; note = 2'-fluoro nucleoside; note (original language) = 2'-氟核苷
  modified_base 9..11: mod_base = OTHER; note = 2'-fluoro nucleoside; note (original language) = 2'-氟核苷
  modified_base 1..3: mod_base = OTHER; note = phosphorothioate bond; note (original language) = 硫代磷酸酯键
  source 1..21: mol_type = other RNA
cacctcgtcatccacaatgaa

SEQ ID NO: 451 - RNA, 21 nt, synthetic construct
  modified_base 1..6: mod_base = OTHER; note = 2'-methoxy nucleoside; note (original language) = 2'-甲氧基核苷
  modified_base 8: mod_base = OTHER; note = 2'-methoxy nucleoside; note (original language) = 2'-甲氧基核苷
  modified_base 12..21: mod_base = OTHER; note = 2'-methoxy nucleoside; note (original language) = 2'-甲氧基核苷
  modified_base 7: mod_base = OTHER; note = 2'-fluoro nucleoside; note (original language) = 2'-氟核苷
  modified_base 9..11: mod_base = OTHER; note = 2'-fluoro nucleoside; note (original language) = 2'-氟核苷
  modified_base 1..3: mod_base = OTHER; note = phosphorothioate bond; note (original language) = 硫代磷酸酯键
  source 1..21: mol_type = other RNA
atccacaatgcgagtacctga

SEQ ID NO: 452 - RNA, 21 nt, synthetic construct
  modified_base 1..6: mod_base = OTHER; note = 2'-methoxy nucleoside; note (original language) = 2'-甲氧基核苷
  modified_base 8: mod_base = OTHER; note = 2'-methoxy nucleoside; note (original language) = 2'-甲氧基核苷
  modified_base 12..21: mod_base = OTHER; note = 2'-methoxy nucleoside; note (original language) = 2'-甲氧基核苷
  modified_base 7: mod_base = OTHER; note = 2'-fluoro nucleoside; note (original language) = 2'-氟核苷
  modified_base 9..11: mod_base = OTHER; note = 2'-fluoro nucleoside; note (original language) = 2'-氟核苷
  modified_base 1..3: mod_base = OTHER; note = phosphorothioate bond; note (original language) = 硫代磷酸酯键
  source 1..21: mol_type = other RNA
tccacaatgagagtacctgta

SEQ ID NO: 453 - RNA, 21 nt, synthetic construct
  modified_base 1..6: mod_base = OTHER; note = 2'-methoxy nucleoside; note (original language) = 2'-甲氧基核苷
  modified_base 8: mod_base = OTHER; note = 2'-methoxy nucleoside; note (original language) = 2'-甲氧基核苷
  modified_base 12..21: mod_base = OTHER; note = 2'-methoxy nucleoside; note (original language) = 2'-甲氧基核苷
  modified_base 7: mod_base = OTHER; note = 2'-fluoro nucleoside; note (original language) = 2'-氟核苷
  modified_base 9..11: mod_base = OTHER; note = 2'-fluoro nucleoside; note (original language) = 2'-氟核苷
  modified_base 1..3: mod_base = OTHER; note = phosphorothioate bond; note (original language) = 硫代磷酸酯键
  source 1..21: mol_type = other RNA
gagcttgaaggggatgagaga

SEQ ID NO: 454 - RNA, 21 nt, synthetic construct
  modified_base 1..6: mod_base = OTHER; note = 2'-methoxy nucleoside; note (original language) = 2'-甲氧基核苷
  modified_base 8: mod_base = OTHER; note = 2'-methoxy nucleoside; note (original language) = 2'-甲氧基核苷
  modified_base 12..21: mod_base = OTHER; note = 2'-methoxy nucleoside; note (original language) = 2'-甲氧基核苷
  modified_base 7: mod_base = OTHER; note = 2'-fluoro nucleoside; note (original language) = 2'-氟核苷
  modified_base 9..11: mod_base = OTHER; note = 2'-fluoro nucleoside; note (original language) = 2'-氟核苷
  modified_base 1..3: mod_base = OTHER; note = phosphorothioate bond; note (original language) = 硫代磷酸酯键
  source 1..21: mol_type = other RNA
gagagagagcgcacagagtct

SEQ ID NO: 455 - RNA, 21 nt, synthetic construct
  modified_base 1..6: mod_base = OTHER; note = 2'-methoxy nucleoside; note (original language) = 2'-甲氧基核苷
  modified_base 8: mod_base = OTHER; note = 2'-methoxy nucleoside; note (original language) = 2'-甲氧基核苷
  modified_base 12..21: mod_base = OTHER; note = 2'-methoxy nucleoside; note (original language) = 2'-甲氧基核苷
  modified_base 7: mod_base = OTHER; note = 2'-fluoro nucleoside; note (original language) = 2'-氟核苷
  modified_base 9..11: mod_base = OTHER; note = 2'-fluoro nucleoside; note (original language) = 2'-氟核苷
  modified_base 1..3: mod_base = OTHER; note = phosphorothioate bond; note (original language) = 硫代磷酸酯键
  source 1..21: mol_type = other RNA
gttttttgagcttgaagcgga

SEQ ID NO: 456 - RNA, 21 nt, synthetic construct
  modified_base 1..6: mod_base = OTHER; note = 2'-methoxy nucleoside; note (original language) = 2'-甲氧基核苷
  modified_base 8: mod_base = OTHER; note = 2'-methoxy nucleoside; note (original language) = 2'-甲氧基核苷
  modified_base 12..21: mod_base = OTHER; note = 2'-methoxy nucleoside; note (original language) = 2'-甲氧基核苷
  modified_base 7: mod_base = OTHER; note = 2'-fluoro nucleoside; note (original language) = 2'-氟核苷
  modified_base 9..11: mod_base = OTHER; note = 2'-fluoro nucleoside; note (original language) = 2'-氟核苷
  modified_base 1..3: mod_base = OTHER; note = phosphorothioate bond; note (original language) = 硫代磷酸酯键
  source 1..21: mol_type = other RNA
gttttgagcttgaagcggata

SEQ ID NO: 457 - RNA, 21 nt, synthetic construct
  modified_base 1..6: mod_base = OTHER; note = 2'-methoxy nucleoside; note (original language) = 2'-甲氧基核苷
  modified_base 8: mod_base = OTHER; note = 2'-methoxy nucleoside; note (original language) = 2'-甲氧基核苷
  modified_base 12..21: mod_base = OTHER; note = 2'-methoxy nucleoside; note (original language) = 2'-甲氧基核苷
  modified_base 7: mod_base = OTHER; note = 2'-fluoro nucleoside; note (original language) = 2'-氟核苷
  modified_base 9..11: mod_base = OTHER; note = 2'-fluoro nucleoside; note (original language) = 2'-氟核苷
  modified_base 1..3: mod_base = OTHER; note = phosphorothioate bond; note (original language) = 硫代磷酸酯键
  source 1..21: mol_type = other RNA
gtttgagcttgaagcggatga

SEQ ID NO: 458 - RNA, 21 nt, synthetic construct
  modified_base 1..6: mod_base = OTHER; note = 2'-methoxy nucleoside; note (original language) = 2'-甲氧基核苷
  modified_base 8: mod_base = OTHER; note = 2'-methoxy nucleoside; note (original language) = 2'-甲氧基核苷
  modified_base 12..21: mod_base = OTHER; note = 2'-methoxy nucleoside; note (original language) = 2'-甲氧基核苷
  modified_base 7: mod_base = OTHER; note = 2'-fluoro nucleoside; note (original language) = 2'-氟核苷
  modified_base 9..11: mod_base = OTHER; note = 2'-fluoro nucleoside; note (original language) = 2'-氟核苷
  modified_base 1..3: mod_base = OTHER; note = phosphorothioate bond; note (original language) = 硫代磷酸酯键
  source 1..21: mol_type = other RNA
ccagtctcccaccttttctta

SEQ ID NO: 459 - RNA, 21 nt, synthetic construct
  modified_base 1..6: mod_base = OTHER; note = 2'-methoxy nucleoside; note (original language) = 2'-甲氧基核苷
  modified_base 8: mod_base = OTHER; note = 2'-methoxy nucleoside; note (original language) = 2'-甲氧基核苷
  modified_base 12..21: mod_base = OTHER; note = 2'-methoxy nucleoside; note (original language) = 2'-甲氧基核苷
  modified_base 7: mod_base = OTHER; note = 2'-fluoro nucleoside; note (original language) = 2'-氟核苷
  modified_base 9..11: mod_base = OTHER; note = 2'-fluoro nucleoside; note (original language) = 2'-氟核苷
  modified_base 1..3: mod_base = OTHER; note = phosphorothioate bond; note (original language) = 硫代磷酸酯键
  source 1..21: mol_type = other RNA
ccccagtctcccaccttttct

SEQ ID NO: 460 - RNA, 21 nt, synthetic construct
  modified_base 1..6: mod_base = OTHER; note = 2'-methoxy nucleoside; note (original language) = 2'-甲氧基核苷
  modified_base 8: mod_base = OTHER; note = 2'-methoxy nucleoside; note (original language) = 2'-甲氧基核苷
  modified_base 12..21: mod_base = OTHER; note = 2'-methoxy nucleoside; note (original language) = 2'-甲氧基核苷
  modified_base 7: mod_base = OTHER; note = 2'-fluoro nucleoside; note (original language) = 2'-氟核苷
  modified_base 9..11: mod_base = OTHER; note = 2'-fluoro nucleoside; note (original language) = 2'-氟核苷
  modified_base 1..3: mod_base = OTHER; note = phosphorothioate bond; note (original language) = 硫代磷酸酯键
  source 1..21: mol_type = other RNA
gcgactttgagctggaaagca

SEQ ID NO: 461 - RNA, 21 nt, synthetic construct
  modified_base 1..6: mod_base = OTHER; note = 2'-methoxy nucleoside; note (original language) = 2'-甲氧基核苷
  modified_base 8: mod_base = OTHER; note = 2'-methoxy nucleoside; note (original language) = 2'-甲氧基核苷
  modified_base 12..21: mod_base = OTHER; note = 2'-methoxy nucleoside; note (original language) = 2'-甲氧基核苷
  modified_base 7: mod_base = OTHER; note = 2'-fluoro nucleoside; note (original language) = 2'-氟核苷
  modified_base 9..11: mod_base = OTHER; note = 2'-fluoro nucleoside; note (original language) = 2'-氟核苷
  modified_base 1..3: mod_base = OTHER; note = phosphorothioate bond; note (original language) = 硫代磷酸酯键
  source 1..21: mol_type = other RNA
gcagccgtttctccttggtct

SEQ ID NO: 462 - RNA, 21 nt, synthetic construct
  modified_base 1..6: mod_base = OTHER; note = 2'-methoxy nucleoside; note (original language) = 2'-甲氧基核苷
  modified_base 8: mod_base = OTHER; note = 2'-methoxy nucleoside; note (original language) = 2'-甲氧基核苷
  modified_base 12..21: mod_base = OTHER; note = 2'-methoxy nucleoside; note (original language) = 2'-甲氧基核苷
  modified_base 7: mod_base = OTHER; note = 2'-fluoro nucleoside; note (original language) = 2'-氟核苷
  modified_base 9..11: mod_base = OTHER; note = 2'-fluoro nucleoside; note (original language) = 2'-氟核苷
  modified_base 1..3: mod_base = OTHER; note = phosphorothioate bond; note (original language) = 硫代磷酸酯键
  source 1..21: mol_type = other RNA
ccgtttctccttggtctaagt

SEQ ID NO: 463 - RNA, 21 nt, synthetic construct
  modified_base 1..6: mod_base = OTHER; note = 2'-methoxy nucleoside; note (original language) = 2'-甲氧基核苷
  modified_base 8: mod_base = OTHER; note = 2'-methoxy nucleoside; note (original language) = 2'-甲氧基核苷
  modified_base 12..21: mod_base = OTHER; note = 2'-methoxy nucleoside; note (original language) = 2'-甲氧基核苷
  modified_base 7: mod_base = OTHER; note = 2'-fluoro nucleoside; note (original language) = 2'-氟核苷
  modified_base 9..11: mod_base = OTHER; note = 2'-fluoro nucleoside; note (original language) = 2'-氟核苷
  modified_base 1..3: mod_base = OTHER; note = phosphorothioate bond; note (original language) = 硫代磷酸酯键
  source 1..21: mol_type = other RNA
gtccacaatgagagtacctgt

SEQ ID NO: 464 - RNA, 21 nt, synthetic construct
  modified_base 1..6: mod_base = OTHER; note = 2'-methoxy nucleoside; note (original language) = 2'-甲氧基核苷
  modified_base 8: mod_base = OTHER; note = 2'-methoxy nucleoside; note (original language) = 2'-甲氧基核苷
  modified_base 12..21: mod_base = OTHER; note = 2'-methoxy nucleoside; note (original language) = 2'-甲氧基核苷
  modified_base 7: mod_base = OTHER; note = 2'-fluoro nucleoside; note (original language) = 2'-氟核苷
  modified_base 9..11: mod_base = OTHER; note = 2'-fluoro nucleoside; note (original language) = 2'-氟核苷
  modified_base 1..3: mod_base = OTHER; note = phosphorothioate bond; note (original language) = 硫代磷酸酯键
  source 1..21: mol_type = other RNA
atccacaatgagagtacctgt

SEQ ID NO: 465 - RNA, 21 nt, synthetic construct
  modified_base 1..6: mod_base = OTHER; note = 2'-methoxy nucleoside; note (original language) = 2'-甲氧基核苷
  modified_base 8: mod_base = OTHER; note = 2'-methoxy nucleoside; note (original language) = 2'-甲氧基核苷
  modified_base 12..21: mod_base = OTHER; note = 2'-methoxy nucleoside; note (original language) = 2'-甲氧基核苷
  modified_base 7: mod_base = OTHER; note = 2'-fluoro nucleoside; note (original language) = 2'-氟核苷
  modified_base 9..11: mod_base = OTHER; note = 2'-fluoro nucleoside; note (original language) = 2'-氟核苷
  modified_base 1..3: mod_base = OTHER; note = phosphorothioate bond; note (original language) = 硫代磷酸酯键
  source 1..21: mol_type = other RNA
gcatccacaatgagagtacct

SEQ ID NO: 466 - RNA, 21 nt, synthetic construct
  modified_base 1..6: mod_base = OTHER; note = 2'-methoxy nucleoside; note (original language) = 2'-甲氧基核苷
  modified_base 8: mod_base = OTHER; note = 2'-methoxy nucleoside; note (original language) = 2'-甲氧基核苷
  modified_base 12..21: mod_base = OTHER; note = 2'-methoxy nucleoside; note (original language) = 2'-甲氧基核苷
  modified_base 7: mod_base = OTHER; note = 2'-fluoro nucleoside; note (original language) = 2'-氟核苷
  modified_base 9..11: mod_base = OTHER; note = 2'-fluoro nucleoside; note (original language) = 2'-氟核苷
  modified_base 1..3: mod_base = OTHER; note = phosphorothioate bond; note (original language) = 硫代磷酸酯键
  source 1..21: mol_type = other RNA
cccagtctcccaccttttcta

SEQ ID NO: 467 - RNA, 21 nt, synthetic construct
  modified_base 1..6: mod_base = OTHER; note = 2'-methoxy nucleoside; note (original language) = 2'-甲氧基核苷
  modified_base 8: mod_base = OTHER; note = 2'-methoxy nucleoside; note (original language) = 2'-甲氧基核苷
  modified_base 12..21: mod_base = OTHER; note = 2'-methoxy nucleoside; note (original language) = 2'-甲氧基核苷
  modified_base 7: mod_base = OTHER; note = 2'-fluoro nucleoside; note (original language) = 2'-氟核苷
  modified_base 9..11: mod_base = OTHER; note = 2'-fluoro nucleoside; note (original language) = 2'-氟核苷
  modified_base 1..3: mod_base = OTHER; note = phosphorothioate bond; note (original language) = 硫代磷酸酯键
  source 1..21: mol_type = other RNA
cagtctcccaccttttcttca

SEQ ID NO: 468 - RNA, 21 nt, synthetic construct
  modified_base 1..6: mod_base = OTHER; note = 2'-methoxy nucleoside; note (original language) = 2'-甲氧基核苷
  modified_base 8: mod_base = OTHER; note = 2'-methoxy nucleoside; note (original language) = 2'-甲氧基核苷
  modified_base 12..21: mod_base = OTHER; note = 2'-methoxy nucleoside; note (original language) = 2'-甲氧基核苷
  modified_base 7: mod_base = OTHER; note = 2'-fluoro nucleoside; note (original language) = 2'-氟核苷
  modified_base 9..11: mod_base = OTHER; note = 2'-fluoro nucleoside; note (original language) = 2'-氟核苷
  modified_base 1..3: mod_base = OTHER; note = phosphorothioate bond; note (original language) = 硫代磷酸酯键
  source 1..21: mol_type = other RNA
ggtctcccaccttttcttcta

SEQ ID NO: 469 - RNA, 21 nt, synthetic construct
  modified_base 1..6: mod_base = OTHER; note = 2'-methoxy nucleoside; note (original language) = 2'-甲氧基核苷
  modified_base 8: mod_base = OTHER; note = 2'-methoxy nucleoside; note (original language) = 2'-甲氧基核苷
  modified_base 12..21: mod_base = OTHER; note = 2'-methoxy nucleoside; note (original language) = 2'-甲氧基核苷
  modified_base 7: mod_base = OTHER; note = 2'-fluoro nucleoside; note (original language) = 2'-氟核苷
  modified_base 9..11: mod_base = OTHER; note = 2'-fluoro nucleoside; note (original language) = 2'-氟核苷
  modified_base 1..3: mod_base = OTHER; note = phosphorothioate bond; note (original language) = 硫代磷酸酯键
  source 1..21: mol_type = other RNA
gtctcccaccttttcttctaa

SEQ ID NO: 470 - RNA, 21 nt, synthetic construct
  modified_base 1..6: mod_base = OTHER; note = 2'-methoxy nucleoside; note (original language) = 2'-甲氧基核苷
  modified_base 8: mod_base = OTHER; note = 2'-methoxy nucleoside; note (original language) = 2'-甲氧基核苷
  modified_base 12..21: mod_base = OTHER; note = 2'-methoxy nucleoside; note (original language) = 2'-甲氧基核苷
  modified_base 7: mod_base = OTHER; note = 2'-fluoro nucleoside; note (original language) = 2'-氟核苷
  modified_base 9..11: mod_base = OTHER; note = 2'-fluoro nucleoside; note (original language) = 2'-氟核苷
  modified_base 1..3: mod_base = OTHER; note = phosphorothioate bond; note (original language) = 硫代磷酸酯键
  source 1..21: mol_type = other RNA
cagccgtttctccttggtcta

SEQ ID NO: 471 - RNA, 21 nt, synthetic construct
  modified_base 1..6: mod_base = OTHER; note = 2'-methoxy nucleoside; note (original language) = 2'-甲氧基核苷
  modified_base 8: mod_base = OTHER; note = 2'-methoxy nucleoside; note (original language) = 2'-甲氧基核苷
  modified_base 12..21: mod_base = OTHER; note = 2'-methoxy nucleoside; note (original language) = 2'-甲氧基核苷
  modified_base 7: mod_base = OTHER; note = 2'-fluoro nucleoside; note (original language) = 2'-氟核苷
  modified_base 9..11: mod_base = OTHER; note = 2'-fluoro nucleoside; note (original language) = 2'-氟核苷
  modified_base 1..3: mod_base = OTHER; note = phosphorothioate bond; note (original language) = 硫代磷酸酯键
  source 1..21: mol_type = other RNA
ggccgtttctccttggtctaa

SEQ ID NO: 472 - RNA, 21 nt, synthetic construct
  modified_base 1..6: mod_base = OTHER; note = 2'-methoxy nucleoside; note (original language) = 2'-甲氧基核苷
  modified_base 8: mod_base = OTHER; note = 2'-methoxy nucleoside; note (original language) = 2'-甲氧基核苷
  modified_base 12..21: mod_base = OTHER; note = 2'-methoxy nucleoside; note (original language) = 2'-甲氧基核苷
  modified_base 7: mod_base = OTHER; note = 2'-fluoro nucleoside; note (original language) = 2'-氟核苷
  modified_base 9..11: mod_base = OTHER; note = 2'-fluoro nucleoside; note (original language) = 2'-氟核苷
  modified_base 1..3: mod_base = OTHER; note = phosphorothioate bond; note (original language) = 硫代磷酸酯键
  source 1..21: mol_type = other RNA
gccgtttctccttggtctaag

SEQ ID NO: 473 - RNA, 21 nt, synthetic construct
  modified_base 1..6: mod_base = OTHER; note = 2'-methoxy nucleoside; note (original language) = 2'-甲氧基核苷
  modified_base 8: mod_base = OTHER; note = 2'-methoxy nucleoside; note (original language) = 2'-甲氧基核苷
  modified_base 12..21: mod_base = OTHER; note = 2'-methoxy nucleoside; note (original language) = 2'-甲氧基核苷
  modified_base 7: mod_base = OTHER; note = 2'-fluoro nucleoside; note (original language) = 2'-氟核苷
  modified_base 9..11: mod_base = OTHER; note = 2'-fluoro nucleoside; note (original language) = 2'-氟核苷
  modified_base 1..3: mod_base = OTHER; note = phosphorothioate bond; note (original language) = 硫代磷酸酯键
  source 1..21: mol_type = other RNA
cgtttctccttggtctaagtg

SEQ ID NO: 474 - RNA, 21 nt, synthetic construct
  modified_base 1..6: mod_base = OTHER; note = 2'-methoxy nucleoside; note (original language) = 2'-甲氧基核苷
  modified_base 8: mod_base = OTHER; note = 2'-methoxy nucleoside; note (original language) = 2'-甲氧基核苷
  modified_base 12..21: mod_base = OTHER; note = 2'-methoxy nucleoside; note (original language) = 2'-甲氧基核苷
  modified_base 7: mod_base = OTHER; note = 2'-fluoro nucleoside; note (original language) = 2'-氟核苷
  modified_base 9..11: mod_base = OTHER; note = 2'-fluoro nucleoside; note (original language) = 2'-氟核苷
  modified_base 1..3: mod_base = OTHER; note = phosphorothioate bond; note (original language) = 硫代磷酸酯键
  source 1..21: mol_type = other RNA
cgtttctccttggtctaagta

SEQ ID NO: 475 - RNA, 21 nt, synthetic construct
  modified_base 1..6: mod_base = OTHER; note = 2'-methoxy nucleoside; note (original language) = 2'-甲氧基核苷
  modified_base 8: mod_base = OTHER; note = 2'-methoxy nucleoside; note (original language) = 2'-甲氧基核苷
  modified_base 12..21: mod_base = OTHER; note = 2'-methoxy nucleoside; note (original language) = 2'-甲氧基核苷
  modified_base 7: mod_base = OTHER; note = 2'-fluoro nucleoside; note (original language) = 2'-氟核苷
  modified_base 9..11: mod_base = OTHER; note = 2'-fluoro nucleoside; note (original language) = 2'-氟核苷
  modified_base 1..3: mod_base = OTHER; note = phosphorothioate bond; note (original language) = 硫代磷酸酯键
  source 1..21: mol_type = other RNA
gtttctccttggtctaagtgt

SEQ ID NO: 476 - RNA, 21 nt, synthetic construct
  modified_base 1..6: mod_base = OTHER; note = 2'-methoxy nucleoside; note (original language) = 2'-甲氧基核苷
  modified_base 8: mod_base = OTHER; note = 2'-methoxy nucleoside; note (original language) = 2'-甲氧基核苷
  modified_base 12..21: mod_base = OTHER; note = 2'-methoxy nucleoside; note (original language) = 2'-甲氧基核苷
  modified_base 7: mod_base = OTHER; note = 2'-fluoro nucleoside; note (original language) = 2'-氟核苷
  modified_base 9..11: mod_base = OTHER; note = 2'-fluoro nucleoside; note (original language) = 2'-氟核苷
  modified_base 1..3: mod_base = OTHER; note = phosphorothioate bond; note (original language) = 硫代磷酸酯键
  source 1..21: mol_type = other RNA
gtttctccttggtctaagtga

SEQ ID NO: 477 - RNA, 21 nt, synthetic construct
  modified_base 1..6: mod_base = OTHER; note = 2'-methoxy nucleoside; note (original language) = 2'-甲氧基核苷
  modified_base 8: mod_base = OTHER; note = 2'-methoxy nucleoside; note (original language) = 2'-甲氧基核苷
  modified_base 12..21: mod_base = OTHER; note = 2'-methoxy nucleoside; note (original language) = 2'-甲氧基核苷
  modified_base 7: mod_base = OTHER; note = 2'-fluoro nucleoside; note (original language) = 2'-氟核苷
  modified_base 9..11: mod_base = OTHER; note = 2'-fluoro nucleoside; note (original language) = 2'-氟核苷
  modified_base 1..3: mod_base = OTHER; note = phosphorothioate bond; note (original language) = 硫代磷酸酯键
  source 1..21: mol_type = other RNA
cagtctcccagcttttcttct

SEQ ID NO: 478 - RNA, 21 nt, synthetic construct
  modified_base 1..6: mod_base = OTHER; note = 2'-methoxy nucleoside; note (original language) = 2'-甲氧基核苷
  modified_base 8: mod_base = OTHER; note = 2'-methoxy nucleoside; note (original language) = 2'-甲氧基核苷
  modified_base 12..21: mod_base = OTHER; note = 2'-methoxy nucleoside; note (original language) = 2'-甲氧基核苷
  modified_base 7: mod_base = OTHER; note = 2'-fluoro nucleoside; note (original language) = 2'-氟核苷
  modified_base 9..11: mod_base = OTHER; note = 2'-fluoro nucleoside; note (original language) = 2'-氟核苷
  modified_base 1..3: mod_base = OTHER; note = phosphorothioate bond; note (original language) = 硫代磷酸酯键
  source 1..21: mol_type = other RNA
gccgtttctcgttggtctaaa

SEQ ID NO: 479 - RNA, 21 nt, synthetic construct
  modified_base 1..6: mod_base = OTHER; note = 2'-methoxy nucleoside; note (original language) = 2'-甲氧基核苷
  modified_base 8: mod_base = OTHER; note = 2'-methoxy nucleoside; note (original language) = 2'-甲氧基核苷
  modified_base 12..21: mod_base = OTHER; note = 2'-methoxy nucleoside; note (original language) = 2'-甲氧基核苷
  modified_base 7: mod_base = OTHER; note = 2'-fluoro nucleoside; note (original language) = 2'-氟核苷
  modified_base 9..11: mod_base = OTHER; note = 2'-fluoro nucleoside; note (original language) = 2'-氟核苷
  modified_base 1..3: mod_base = OTHER; note = phosphorothioate bond; note (original language) = 硫代磷酸酯键
  source 1..21: mol_type = other RNA
ggccgtttctgcttggtctaa

SEQ ID NO: 480 - RNA, 21 nt, synthetic construct
  modified_base 1..6: mod_base = OTHER; note = 2'-methoxy nucleoside; note (original language) = 2'-甲氧基核苷
  modified_base 8: mod_base = OTHER; note = 2'-methoxy nucleoside; note (original language) = 2'-甲氧基核苷
  modified_base 12..21: mod_base = OTHER; note = 2'-methoxy nucleoside; note (original language) = 2'-甲氧基核苷
  modified_base 7: mod_base = OTHER; note = 2'-fluoro nucleoside; note (original language) = 2'-氟核苷
  modified_base 9..11: mod_base = OTHER; note = 2'-fluoro nucleoside; note (original language) = 2'-氟核苷
  modified_base 1..3: mod_base = OTHER; note = phosphorothioate bond; note (original language) = 硫代磷酸酯键
  source 1..21: mol_type = other RNA
ggccgtttctacttggtctaa

SEQ ID NO: 481 - RNA, 21 nt, synthetic construct
  modified_base 1..6: mod_base = OTHER; note = 2'-methoxy nucleoside; note (original language) = 2'-甲氧基核苷
  modified_base 8: mod_base = OTHER; note = 2'-methoxy nucleoside; note (original language) = 2'-甲氧基核苷
  modified_base 12..21: mod_base = OTHER; note = 2'-methoxy nucleoside; note (original language) = 2'-甲氧基核苷
  modified_base 7: mod_base = OTHER; note = 2'-fluoro nucleoside; note (original language) = 2'-氟核苷
  modified_base 9..11: mod_base = OTHER; note = 2'-fluoro nucleoside; note (original language) = 2'-氟核苷
  modified_base 1..3: mod_base = OTHER; note = phosphorothioate bond; note (original language) = 硫代磷酸酯键
  source 1..21: mol_type = other RNA
ccgtttctccttggtctaaga

SEQ ID NO: 482 - RNA, 21 nt, synthetic construct
  modified_base 1..6: mod_base = OTHER; note = 2'-methoxy nucleoside; note (original language) = 2'-甲氧基核苷
  modified_base 8: mod_base = OTHER; note = 2'-methoxy nucleoside; note (original language) = 2'-甲氧基核苷
  modified_base 12..21: mod_base = OTHER; note = 2'-methoxy nucleoside; note (original language) = 2'-甲氧基核苷
  modified_base 7: mod_base = OTHER; note = 2'-fluoro nucleoside; note (original language) = 2'-氟核苷
  modified_base 9..11: mod_base = OTHER; note = 2'-fluoro nucleoside; note (original language) = 2'-氟核苷
  modified_base 1..3: mod_base = OTHER; note = phosphorothioate bond; note (original language) = 硫代磷酸酯键
  source 1..21: mol_type = other RNA
gcgtttctccttggtctaagt

SEQ ID NO: 483 - RNA, 21 nt, synthetic construct
  modified_base 1..6: mod_base = OTHER; note = 2'-methoxy nucleoside; note (original language) = 2'-甲氧基核苷
  modified_base 8: mod_base = OTHER; note = 2'-methoxy nucleoside; note (original language) = 2'-甲氧基核苷
  modified_base 12..21: mod_base = OTHER; note = 2'-methoxy nucleoside; note (original language) = 2'-甲氧基核苷
  modified_base 7: mod_base = OTHER; note = 2'-fluoro nucleoside; note (original language) = 2'-氟核苷
  modified_base 9..11: mod_base = OTHER; note = 2'-fluoro nucleoside; note (original language) = 2'-氟核苷
  modified_base 1..3: mod_base = OTHER; note = phosphorothioate bond; note (original language) = 硫代磷酸酯键
  source 1..21: mol_type = other RNA
gcgtttctccttggtctaaga

SEQ ID NO: 484 - RNA, 21 nt, synthetic construct
  modified_base 1..6: mod_base = OTHER; note = 2'-methoxy nucleoside; note (original language) = 2'-甲氧基核苷
  modified_base 8: mod_base = OTHER; note = 2'-methoxy nucleoside; note (original language) = 2'-甲氧基核苷
  modified_base 12..21: mod_base = OTHER; note = 2'-methoxy nucleoside; note (original language) = 2'-甲氧基核苷
  modified_base 7: mod_base = OTHER; note = 2'-fluoro nucleoside; note (original language) = 2'-氟核苷
  modified_base 9..11: mod_base = OTHER; note = 2'-fluoro nucleoside; note (original language) = 2'-氟核苷
  modified_base 1..3: mod_base = OTHER; note = phosphorothioate bond; note (original language) = 硫代磷酸酯键
  source 1..21: mol_type = other RNA
gcgtttctccgtggtctaagt

SEQ ID NO: 485 - RNA, 19 nt, synthetic construct
  modified_base 1..4: mod_base = OTHER; note = 2'-methoxy nucleoside; note (original language) = 2'-甲氧基核苷
  modified_base 6: mod_base = OTHER; note = 2'-methoxy nucleoside; note (original language) = 2'-甲氧基核苷
  modified_base 10..19: mod_base = OTHER; note = 2'-methoxy nucleoside; note (original language) = 2'-甲氧基核苷
  modified_base 5: mod_base = OTHER; note = 2'-fluoro nucleoside; note (original language) = 2'-氟核苷
  modified_base 7..9: mod_base = OTHER; note = 2'-fluoro nucleoside; note (original language) = 2'-氟核苷
  modified_base 1..3: mod_base = OTHER; note = phosphorothioate bond; note (original language) = 硫代磷酸酯键
  source 1..19: mol_type = other RNA
tcccaccttttcttctaat

SEQ ID NO: 486 - RNA, 19 nt, synthetic construct
  modified_base 1..4: mod_base = OTHER; note = 2'-methoxy nucleoside; note (original language) = 2'-甲氧基核苷
  modified_base 6: mod_base = OTHER; note = 2'-methoxy nucleoside; note (original language) = 2'-甲氧基核苷
  modified_base 10..19: mod_base = OTHER; note = 2'-methoxy nucleoside; note (original language) = 2'-甲氧基核苷
  modified_base 5: mod_base = OTHER; note = 2'-fluoro nucleoside; note (original language) = 2'-氟核苷
  modified_base 7..9: mod_base = OTHER; note = 2'-fluoro nucleoside; note (original language) = 2'-氟核苷
  modified_base 1..3: mod_base = OTHER; note = phosphorothioate bond; note (original language) = 硫代磷酸酯键
  source 1..19: mol_type = other RNA
gcccaccttttcttctaaa

SEQ ID NO: 487 - RNA, 19 nt, synthetic construct
  modified_base 1..4: mod_base = OTHER; note = 2'-methoxy nucleoside; note (original language) = 2'-甲氧基核苷
  modified_base 6: mod_base = OTHER; note = 2'-methoxy nucleoside; note (original language) = 2'-甲氧基核苷
  modified_base 10..19: mod_base = OTHER; note = 2'-methoxy nucleoside; note (original language) = 2'-甲氧基核苷
  modified_base 5: mod_base = OTHER; note = 2'-fluoro nucleoside; note (original language) = 2'-氟核苷
  modified_base 7..9: mod_base = OTHER; note = 2'-fluoro nucleoside; note (original language) = 2'-氟核苷
  modified_base 1..3: mod_base = OTHER; note = phosphorothioate bond; note (original language) = 硫代磷酸酯键
  source 1..19: mol_type = other RNA
gcatccacaatgagagtaa

SEQ ID NO: 488 - RNA, 19 nt, synthetic construct
  modified_base 1..4: mod_base = OTHER; note = 2'-methoxy nucleoside; note (original language) = 2'-甲氧基核苷
  modified_base 6: mod_base = OTHER; note = 2'-methoxy nucleoside; note (original language) = 2'-甲氧基核苷
  modified_base 10..19: mod_base = OTHER; note = 2'-methoxy nucleoside; note (original language) = 2'-甲氧基核苷
  modified_base 5: mod_base = OTHER; note = 2'-fluoro nucleoside; note (original language) = 2'-氟核苷
  modified_base 7..9: mod_base = OTHER; note = 2'-fluoro nucleoside; note (original language) = 2'-氟核苷
  modified_base 1..3: mod_base = OTHER; note = phosphorothioate bond; note (original language) = 硫代磷酸酯键
  source 1..19: mol_type = other RNA
gcgtcatccacaatgagaa

SEQ ID NO: 489 - RNA, 19 nt, synthetic construct
  modified_base 1..4: mod_base = OTHER; note = 2'-methoxy nucleoside; note (original language) = 2'-甲氧基核苷
  modified_base 6: mod_base = OTHER; note = 2'-methoxy nucleoside; note (original language) = 2'-甲氧基核苷
  modified_base 10..19: mod_base = OTHER; note = 2'-methoxy nucleoside; note (original language) = 2'-甲氧基核苷
  modified_base 5: mod_base = OTHER; note = 2'-fluoro nucleoside; note (original language) = 2'-氟核苷
  modified_base 7..9: mod_base = OTHER; note = 2'-fluoro nucleoside; note (original language) = 2'-氟核苷
  modified_base 1..3: mod_base = OTHER; note = phosphorothioate bond; note (original language) = 硫代磷酸酯键
  source 1..19: mol_type = other RNA
cctcgtcatccacaatgaa

SEQ ID NO: 490 - RNA, 19 nt, synthetic construct
  modified_base 1..4: mod_base = OTHER; note = 2'-methoxy nucleoside; note (original language) = 2'-甲氧基核苷
  modified_base 6: mod_base = OTHER; note = 2'-methoxy nucleoside; note (original language) = 2'-甲氧基核苷
  modified_base 10..19: mod_base = OTHER; note = 2'-methoxy nucleoside; note (original language) = 2'-甲氧基核苷
  modified_base 5: mod_base = OTHER; note = 2'-fluoro nucleoside; note (original language) = 2'-氟核苷
  modified_base 7..9: mod_base = OTHER; note = 2'-fluoro nucleoside; note (original language) = 2'-氟核苷
  modified_base 1..3: mod_base = OTHER; note = phosphorothioate bond; note (original language) = 硫代磷酸酯键
  source 1..19: mol_type = other RNA
cacctcgtcatccacaata

SEQ ID NO: 491 - RNA, 19 nt, synthetic construct
  modified_base 1..4: mod_base = OTHER; note = 2'-methoxy nucleoside; note (original language) = 2'-甲氧基核苷
  modified_base 6: mod_base = OTHER; note = 2'-methoxy nucleoside; note (original language) = 2'-甲氧基核苷
  modified_base 10..19: mod_base = OTHER; note = 2'-methoxy nucleoside; note (original language) = 2'-甲氧基核苷
  modified_base 5: mod_base = OTHER; note = 2'-fluoro nucleoside; note (original language) = 2'-氟核苷
  modified_base 7..9: mod_base = OTHER; note = 2'-fluoro nucleoside; note (original language) = 2'-氟核苷
  modified_base 1..3: mod_base = OTHER; note = phosphorothioate bond; note (original language) = 硫代磷酸酯键
  source 1..19: mol_type = other RNA
gtccacaatgagagtacca

SEQ ID NO: 492 - RNA, 19 nt, synthetic construct
  modified_base 1..4: mod_base = OTHER; note = 2'-methoxy nucleoside; note (original language) = 2'-甲氧基核苷
  modified_base 6: mod_base = OTHER; note = 2'-methoxy nucleoside; note (original language) = 2'-甲氧基核苷
  modified_base 10..19: mod_base = OTHER; note = 2'-methoxy nucleoside; note (original language) = 2'-甲氧基核苷
  modified_base 5: mod_base = OTHER; note = 2'-fluoro nucleoside; note (original language) = 2'-氟核苷
  modified_base 7..9: mod_base = OTHER; note = 2'-fluoro nucleoside; note (original language) = 2'-氟核苷
  modified_base 1..3: mod_base = OTHER; note = phosphorothioate bond; note (original language) = 硫代磷酸酯键
  source 1..19: mol_type = other RNA
gccacaatgagagtaccta

SEQ ID NO: 493 - RNA, 19 nt, synthetic construct
  modified_base 1..4: mod_base = OTHER; note = 2'-methoxy nucleoside; note (original language) = 2'-甲氧基核苷
  modified_base 6: mod_base = OTHER; note = 2'-methoxy nucleoside; note (original language) = 2'-甲氧基核苷
  modified_base 10..19: mod_base = OTHER; note = 2'-methoxy nucleoside; note (original language) = 2'-甲氧基核苷
  modified_base 5: mod_base = OTHER; note = 2'-fluoro nucleoside; note (original language) = 2'-氟核苷
  modified_base 7..9: mod_base = OTHER; note = 2'-fluoro nucleoside; note (original language) = 2'-氟核苷
  modified_base 1..3: mod_base = OTHER; note = phosphorothioate bond; note (original language) = 硫代磷酸酯键
  source 1..19: mol_type = other RNA
cacaatgagagtacctgta

SEQ ID NO: 494 - RNA, 19 nt, synthetic construct
  modified_base 1..4: mod_base = OTHER; note = 2'-methoxy nucleoside; note (original language) = 2'-甲氧基核苷
  modified_base 6: mod_base = OTHER; note = 2'-methoxy nucleoside; note (original language) = 2'-甲氧基核苷
  modified_base 10..19: mod_base = OTHER; note = 2'-methoxy nucleoside; note (original language) = 2'-甲氧基核苷
  modified_base 5: mod_base = OTHER; note = 2'-fluoro nucleoside; note (original language) = 2'-氟核苷
  modified_base 7..9: mod_base = OTHER; note = 2'-fluoro nucleoside; note (original language) = 2'-氟核苷
  modified_base 1..3: mod_base = OTHER; note = phosphorothioate bond; note (original language) = 硫代磷酸酯键
  source 1..19: mol_type = other RNA
gcaatgagagtacctgtga

SEQ ID NO: 495 - RNA, 19 nt, synthetic construct
  modified_base 1..4: mod_base = OTHER; note = 2'-methoxy nucleoside; note (original language) = 2'-甲氧基核苷
  modified_base 6: mod_base = OTHER; note = 2'-methoxy nucleoside; note (original language) = 2'-甲氧基核苷
  modified_base 10..19: mod_base = OTHER; note = 2'-methoxy nucleoside; note (original language) = 2'-甲氧基核苷
  modified_base 5: mod_base = OTHER; note = 2'-fluoro nucleoside; note (original language) = 2'-氟核苷
  modified_base 7..9: mod_base = OTHER; note = 2'-fluoro nucleoside; note (original language) = 2'-氟核苷
  modified_base 1..3: mod_base = OTHER; note = phosphorothioate bond; note (original language) = 硫代磷酸酯键
  source 1..19: mol_type = other RNA
caatgagagtacctgtgaa

SEQ ID NO: 496 - RNA, 19 nt, synthetic construct
  modified_base 1..4: mod_base = OTHER; note = 2'-methoxy nucleoside; note (original language) = 2'-甲氧基核苷
  modified_base 6: mod_base = OTHER; note = 2'-methoxy nucleoside; note (original language) = 2'-甲氧基核苷
  modified_base 10..19: mod_base = OTHER; note = 2'-methoxy nucleoside; note (original language) = 2'-甲氧基核苷
  modified_base 5: mod_base = OTHER; note = 2'-fluoro nucleoside; note (original language) = 2'-氟核苷
  modified_base 7..9: mod_base = OTHER; note = 2'-fluoro nucleoside; note (original language) = 2'-氟核苷
  modified_base 1..3: mod_base = OTHER; note = phosphorothioate bond; note (original language) = 硫代磷酸酯键
  source 1..19: mol_type = other RNA
gatgagagtacctgtgaga

SEQ ID NO: 497 - RNA, 19 nt, synthetic construct
  modified_base 1..4: mod_base = OTHER; note = 2'-methoxy nucleoside; note (original language) = 2'-甲氧基核苷
  modified_base 6: mod_base = OTHER; note = 2'-methoxy nucleoside; note (original language) = 2'-甲氧基核苷
  modified_base 10..19: mod_base = OTHER; note = 2'-methoxy nucleoside; note (original language) = 2'-甲氧基核苷
  modified_base 5: mod_base = OTHER; note = 2'-fluoro nucleoside; note (original language) = 2'-氟核苷
  modified_base 7..9: mod_base = OTHER; note = 2'-fluoro nucleoside; note (original language) = 2'-氟核苷
  modified_base 1..3: mod_base = OTHER; note = phosphorothioate bond; note (original language) = 硫代磷酸酯键
  source 1..19: mol_type = other RNA
ggagagtacctgtgagcaa

SEQ ID NO: 498 - RNA, 19 nt, synthetic construct
  modified_base 1..4: mod_base = OTHER; note = 2'-methoxy nucleoside; note (original language) = 2'-甲氧基核苷
  modified_base 6: mod_base = OTHER; note = 2'-methoxy nucleoside; note (original language) = 2'-甲氧基核苷
  modified_base 10..19: mod_base = OTHER; note = 2'-methoxy nucleoside; note (original language) = 2'-甲氧基核苷
  modified_base 5: mod_base = OTHER; note = 2'-fluoro nucleoside; note (original language) = 2'-氟核苷
  modified_base 7..9: mod_base = OTHER; note = 2'-fluoro nucleoside; note (original language) = 2'-氟核苷
  modified_base 1..3: mod_base = OTHER; note = phosphorothioate bond; note (original language) = 硫代磷酸酯键
  source 1..19: mol_type = other RNA
gagagtacctgtgagcaga

SEQ ID NO: 499 - RNA, 19 nt, synthetic construct
  modified_base 1..4: mod_base = OTHER; note = 2'-methoxy nucleoside; note (original language) = 2'-甲氧基核苷
  modified_base 6: mod_base = OTHER; note = 2'-methoxy nucleoside; note (original language) = 2'-甲氧基核苷
  modified_base 10..19: mod_base = OTHER; note = 2'-methoxy nucleoside; note (original language) = 2'-甲氧基核苷
  modified_base 5: mod_base = OTHER; note = 2'-fluoro nucleoside; note (original language) = 2'-氟核苷
  modified_base 7..9: mod_base = OTHER; note = 2'-fluoro nucleoside; note (original language) = 2'-氟核苷
  modified_base 1..3: mod_base = OTHER; note = phosphorothioate bond; note (original language) = 硫代磷酸酯键
  source 1..19: mol_type = other RNA
ctcccaccttttcttctaa

SEQ ID NO: 500 - RNA, 19 nt, synthetic construct
  modified_base 1..4: mod_base = OTHER; note = 2'-methoxy nucleoside; note (original language) = 2'-甲氧基核苷
  modified_base 6: mod_base = OTHER; note = 2'-methoxy nucleoside; note (original language) = 2'-甲氧基核苷
  modified_base 10..19: mod_base = OTHER; note = 2'-methoxy nucleoside; note (original language) = 2'-甲氧基核苷
  modified_base 5: mod_base = OTHER; note = 2'-fluoro nucleoside; note (original language) = 2'-氟核苷
  modified_base 7..9: mod_base = OTHER; note = 2'-fluoro nucleoside; note (original language) = 2'-氟核苷
  modified_base 1..3: mod_base = OTHER; note = phosphorothioate bond; note (original language) = 硫代磷酸酯键
  source 1..19: mol_type = other RNA
gctcccaccttttcttcta

SEQ ID NO: 501 - RNA, 19 nt, synthetic construct
  modified_base 1..4: mod_base = OTHER; note = 2'-methoxy nucleoside; note (original language) = 2'-甲氧基核苷
  modified_base 6: mod_base = OTHER; note = 2'-methoxy nucleoside; note (original language) = 2'-甲氧基核苷
  modified_base 10..19: mod_base = OTHER; note = 2'-methoxy nucleoside; note (original language) = 2'-甲氧基核苷
  modified_base 5: mod_base = OTHER; note = 2'-fluoro nucleoside; note (original language) = 2'-氟核苷
  modified_base 7..9: mod_base = OTHER; note = 2'-fluoro nucleoside; note (original language) = 2'-氟核苷
  modified_base 1..3: mod_base = OTHER; note = phosphorothioate bond; note (original language) = 硫代磷酸酯键
  source 1..19: mol_type = other RNA
gtctcccaccttttcttca

SEQ ID NO: 502 - RNA, 19 nt, synthetic construct
  modified_base 1..4: mod_base = OTHER; note = 2'-methoxy nucleoside; note (original language) = 2'-甲氧基核苷
  modified_base 6: mod_base = OTHER; note = 2'-methoxy nucleoside; note (original language) = 2'-甲氧基核苷
  modified_base 10..19: mod_base = OTHER; note = 2'-methoxy nucleoside; note (original language) = 2'-甲氧基核苷
  modified_base 5: mod_base = OTHER; note = 2'-fluoro nucleoside; note (original language) = 2'-氟核苷
  modified_base 7..9: mod_base = OTHER; note = 2'-fluoro nucleoside; note (original language) = 2'-氟核苷
  modified_base 1..3: mod_base = OTHER; note = phosphorothioate bond; note (original language) = 硫代磷酸酯键
  source 1..19: mol_type = other RNA
ggtctcccaccttttctta

SEQ ID NO: 503 - RNA, 19 nt, synthetic construct
  modified_base 1..4: mod_base = OTHER; note = 2'-methoxy nucleoside; note (original language) = 2'-甲氧基核苷
  modified_base 6: mod_base = OTHER; note = 2'-methoxy nucleoside; note (original language) = 2'-甲氧基核苷
  modified_base 10..19: mod_base = OTHER; note = 2'-methoxy nucleoside; note (original language) = 2'-甲氧基核苷
  modified_base 5: mod_base = OTHER; note = 2'-fluoro nucleoside; note (original language) = 2'-氟核苷
  modified_base 7..9: mod_base = OTHER; note = 2'-fluoro nucleoside; note (original language) = 2'-氟核苷
  modified_base 1..3: mod_base = OTHER; note = phosphorothioate bond; note (original language) = 硫代磷酸酯键
  source 1..19: mol_type = other RNA
cccaccttttcttctaata

SEQ ID NO: 504 - RNA, 19 nt, synthetic construct
  modified_base 1..4: mod_base = OTHER; note = 2'-methoxy nucleoside; note (original language) = 2'-甲氧基核苷
  modified_base 6: mod_base = OTHER; note = 2'-methoxy nucleoside; note (original language) = 2'-甲氧基核苷
  modified_base 10..19: mod_base = OTHER; note = 2'-methoxy nucleoside; note (original language) = 2'-甲氧基核苷
  modified_base 5: mod_base = OTHER; note = 2'-fluoro nucleoside; note (original language) = 2'-氟核苷
  modified_base 7..9: mod_base = OTHER; note = 2'-fluoro nucleoside; note (original language) = 2'-氟核苷
  modified_base 1..3: mod_base = OTHER; note = phosphorothioate bond; note (original language) = 硫代磷酸酯键
  source 1..19: mol_type = other RNA
ccaccttttcttctaatga

SEQ ID NO: 505 - RNA, 19 nt, synthetic construct
  modified_base 1..4: mod_base = OTHER; note = 2'-methoxy nucleoside; note (original language) = 2'-甲氧基核苷
  modified_base 6: mod_base = OTHER; note = 2'-methoxy nucleoside; note (original language) = 2'-甲氧基核苷
  modified_base 10..19: mod_base = OTHER; note = 2'-methoxy nucleoside; note (original language) = 2'-甲氧基核苷
  modified_base 5: mod_base = OTHER; note = 2'-fluoro nucleoside; note (original language) = 2'-氟核苷
  modified_base 7..9: mod_base = OTHER; note = 2'-fluoro nucleoside; note (original language) = 2'-氟核苷
  modified_base 1..3: mod_base = OTHER; note = phosphorothioate bond; note (original language) = 硫代磷酸酯键
  source 1..19: mol_type = other RNA
caccttttcttctaatgaa

SEQ ID NO: 506 - RNA, 19 nt, synthetic construct
  modified_base 1..4: mod_base = OTHER; note = 2'-methoxy nucleoside; note (original language) = 2'-甲氧基核苷
  modified_base 6: mod_base = OTHER; note = 2'-methoxy nucleoside; note (original language) = 2'-甲氧基核苷
  modified_base 10..19: mod_base = OTHER; note = 2'-methoxy nucleoside; note (original language) = 2'-甲氧基核苷
  modified_base 5: mod_base = OTHER; note = 2'-fluoro nucleoside; note (original language) = 2'-氟核苷
  modified_base 7..9: mod_base = OTHER; note = 2'-fluoro nucleoside; note (original language) = 2'-氟核苷
  modified_base 1..3: mod_base = OTHER; note = phosphorothioate bond; note (original language) = 硫代磷酸酯键
  source 1..19: mol_type = other RNA
gccttttcttctaatgaga

SEQ ID NO: 507 - RNA, 19 nt, synthetic construct
  modified_base 1..4: mod_base = OTHER; note = 2'-methoxy nucleoside; note (original language) = 2'-甲氧基核苷
  modified_base 6: mod_base = OTHER; note = 2'-methoxy nucleoside; note (original language) = 2'-甲氧基核苷
  modified_base 10..19: mod_base = OTHER; note = 2'-methoxy nucleoside; note (original language) = 2'-甲氧基核苷
  modified_base 5: mod_base = OTHER; note = 2'-fluoro nucleoside; note (original language) = 2'-氟核苷
  modified_base 7..9: mod_base = OTHER; note = 2'-fluoro nucleoside; note (original language) = 2'-氟核苷
  modified_base 1..3: mod_base = OTHER; note = phosphorothioate bond; note (original language) = 硫代磷酸酯键
  source 1..19: mol_type = other RNA
ccttttcttctaatgagta

SEQ ID NO: 508 - RNA, 19 nt, synthetic construct
  modified_base 1..4: mod_base = OTHER; note = 2'-methoxy nucleoside; note (original language) = 2'-甲氧基核苷
  modified_base 6: mod_base = OTHER; note = 2'-methoxy nucleoside; note (original language) = 2'-甲氧基核苷
  modified_base 10..19: mod_base = OTHER; note = 2'-methoxy nucleoside; note (original language) = 2'-甲氧基核苷
  modified_base 5: mod_base = OTHER; note = 2'-fluoro nucleoside; note (original language) = 2'-氟核苷
  modified_base 7..9: mod_base = OTHER; note = 2'-fluoro nucleoside; note (original language) = 2'-氟核苷
  modified_base 1..3: mod_base = OTHER; note = phosphorothioate bond; note (original language) = 硫代磷酸酯键
  source 1..19: mol_type = other RNA
cttttcttctaatgagtca

SEQ ID NO: 509 - RNA, 19 nt, synthetic construct
  modified_base 1..6: mod_base = OTHER; note = 2'-methoxy nucleoside; note (original language) = 2'-甲氧基核苷
  modified_base 10..19: mod_base = OTHER; note = 2'-methoxy nucleoside; note (original language) = 2'-甲氧基核苷
  modified_base 7..9: mod_base = OTHER; note = 2'-fluoro nucleoside; note (original language) = 2'-氟核苷
  modified_base 1..3: mod_base = OTHER; note = phosphorothioate bond; note (original language) = 硫代磷酸酯键
  source 1..19: mol_type = other RNA
agcacctgaatttctgttt

SEQ ID NO: 510 - RNA, 19 nt, synthetic construct
  modified_base 1..6: mod_base = OTHER; note = 2'-methoxy nucleoside; note (original language) = 2'-甲氧基核苷
  modified_base 10..19: mod_base = OTHER; note = 2'-methoxy nucleoside; note (original language) = 2'-甲氧基核苷
  modified_base 7..9: mod_base = OTHER; note = 2'-fluoro nucleoside; note (original language) = 2'-氟核苷
  modified_base 1..3: mod_base = OTHER; note = phosphorothioate bond; note (original language) = 硫代磷酸酯键
  source 1..19: mol_type = other RNA
gtctgtaataccttagttt

SEQ ID NO: 511 - RNA, 19 nt, synthetic construct
  modified_base 1..6: mod_base = OTHER; note = 2'-methoxy nucleoside; note (original language) = 2'-甲氧基核苷
  modified_base 10..19: mod_base = OTHER; note = 2'-methoxy nucleoside; note (original language) = 2'-甲氧基核苷
  modified_base 7..9: mod_base = OTHER; note = 2'-fluoro nucleoside; note (original language) = 2'-氟核苷
  modified_base 1..3: mod_base = OTHER; note = phosphorothioate bond; note (original language) = 硫代磷酸酯键
  source 1..19: mol_type = other RNA
caaatgcacctcccagttt

SEQ ID NO: 512 - RNA, 19 nt, synthetic construct
  modified_base 1..6: mod_base = OTHER; note = 2'-methoxy nucleoside; note (original language) = 2'-甲氧基核苷
  modified_base 10..19: mod_base = OTHER; note = 2'-methoxy nucleoside; note (original language) = 2'-甲氧基核苷
  modified_base 7..9: mod_base = OTHER; note = 2'-fluoro nucleoside; note (original language) = 2'-氟核苷
  modified_base 1..3: mod_base = OTHER; note = phosphorothioate bond; note (original language) = 硫代磷酸酯键
  source 1..19: mol_type = other RNA
tggacagcaccctggcttt

SEQ ID NO: 513 - RNA, 19 nt, synthetic construct
  modified_base 1..6: mod_base = OTHER; note = 2'-methoxy nucleoside; note (original language) = 2'-甲氧基核苷
  modified_base 10..19: mod_base = OTHER; note = 2'-methoxy nucleoside; note (original language) = 2'-甲氧基核苷
  modified_base 7..9: mod_base = OTHER; note = 2'-fluoro nucleoside; note (original language) = 2'-氟核苷
  modified_base 1..3: mod_base = OTHER; note = phosphorothioate bond; note (original language) = 硫代磷酸酯键
  source 1..19: mol_type = other RNA
cttctaatgagtcgacttt

SEQ ID NO: 514 - RNA, 19 nt, synthetic construct
  modified_base 1..6: mod_base = OTHER; note = 2'-methoxy nucleoside; note (original language) = 2'-甲氧基核苷
  modified_base 10..19: mod_base = OTHER; note = 2'-methoxy nucleoside; note (original language) = 2'-甲氧基核苷
  modified_base 7..9: mod_base = OTHER; note = 2'-fluoro nucleoside; note (original language) = 2'-氟核苷
  modified_base 1..3: mod_base = OTHER; note = phosphorothioate bond; note (original language) = 硫代磷酸酯键
  source 1..19: mol_type = other RNA
aggtggagggtctcacttt

SEQ ID NO: 515 - RNA, 19 nt, synthetic construct
  modified_base 1..6: mod_base = OTHER; note = 2'-methoxy nucleoside; note (original language) = 2'-甲氧基核苷
  modified_base 10..19: mod_base = OTHER; note = 2'-methoxy nucleoside; note (original language) = 2'-甲氧基核苷
  modified_base 7..9: mod_base = OTHER; note = 2'-fluoro nucleoside; note (original language) = 2'-氟核苷
  modified_base 1..3: mod_base = OTHER; note = phosphorothioate bond; note (original language) = 硫代磷酸酯键
  source 1..19: mol_type = other RNA
gaaccatagctggttattt

SEQ ID NO: 516 - RNA, 19 nt, synthetic construct
  modified_base 1..6: mod_base = OTHER; note = 2'-methoxy nucleoside; note (original language) = 2'-甲氧基核苷
  modified_base 10..19: mod_base = OTHER; note = 2'-methoxy nucleoside; note (original language) = 2'-甲氧基核苷
  modified_base 7..9: mod_base = OTHER; note = 2'-fluoro nucleoside; note (original language) = 2'-氟核苷
  modified_base 1..3: mod_base = OTHER; note = phosphorothioate bond; note (original language) = 硫代磷酸酯键
  source 1..19: mol_type = other RNA
ttgccttcggtttgtattt

SEQ ID NO: 517 - RNA, 19 nt, synthetic construct
  modified_base 1..6: mod_base = OTHER; note = 2'-methoxy nucleoside; note (original language) = 2'-甲氧基核苷
  modified_base 10..19: mod_base = OTHER; note = 2'-methoxy nucleoside; note (original language) = 2'-甲氧基核苷
  modified_base 7..9: mod_base = OTHER; note = 2'-fluoro nucleoside; note (original language) = 2'-氟核苷
  modified_base 1..3: mod_base = OTHER; note = phosphorothioate bond; note (original language) = 硫代磷酸酯键
  source 1..19: mol_type = other RNA
ggtttgtatttagtgtctt

SEQ ID NO: 518 - RNA, 19 nt, synthetic construct
  modified_base 1..6: mod_base = OTHER; note = 2'-methoxy nucleoside; note (original language) = 2'-甲氧基核苷
  modified_base 10..19: mod_base = OTHER; note = 2'-methoxy nucleoside; note (original language) = 2'-甲氧基核苷
  modified_base 7..9: mod_base = OTHER; note = 2'-fluoro nucleoside; note (original language) = 2'-氟核苷
  modified_base 1..3: mod_base = OTHER; note = phosphorothioate bond; note (original language) = 硫代磷酸酯键
  source 1..19: mol_type = other RNA
caagttgagaacaaaaatt

SEQ ID NO: 519 - RNA, 19 nt, synthetic construct
  modified_base 1..6: mod_base = OTHER; note = 2'-methoxy nucleoside; note (original language) = 2'-甲氧基核苷
  modified_base 10..19: mod_base = OTHER; note = 2'-methoxy nucleoside; note (original language) = 2'-甲氧基核苷
  modified_base 7..9: mod_base = OTHER; note = 2'-fluoro nucleoside; note (original language) = 2'-氟核苷
  modified_base 1..3: mod_base = OTHER; note = phosphorothioate bond; note (original language) = 硫代磷酸酯键
  source 1..19: mol_type = other RNA
gtttgtgaaacaaaaaagt

SEQ ID NO: 520 - RNA, 19 nt, synthetic construct
  modified_base 1..6: mod_base = OTHER; note = 2'-methoxy nucleoside; note (original language) = 2'-甲氧基核苷
  modified_base 10..19: mod_base = OTHER; note = 2'-methoxy nucleoside; note (original language) = 2'-甲氧基核苷
  modified_base 7..9: mod_base = OTHER; note = 2'-fluoro nucleoside; note (original language) = 2'-氟核苷
  modified_base 1..3: mod_base = OTHER; note = phosphorothioate bond; note (original language) = 硫代磷酸酯键
  source 1..19: mol_type = other RNA
tggacaaggtggagggtct

SEQ ID NO: 521 - RNA, 19 nt, synthetic construct
  modified_base 1..6: mod_base = OTHER; note = 2'-methoxy nucleoside; note (original language) = 2'-甲氧基核苷
  modified_base 10..19: mod_base = OTHER; note = 2'-methoxy nucleoside; note (original language) = 2'-甲氧基核苷
  modified_base 7..9: mod_base = OTHER; note = 2'-fluoro nucleoside; note (original language) = 2'-氟核苷
  modified_base 1..3: mod_base = OTHER; note = phosphorothioate bond; note (original language) = 硫代磷酸酯键
  source 1..19: mol_type = other RNA
ctcactttccagcaaaact

SEQ ID NO: 522 - RNA, 19 nt, synthetic construct
  modified_base 1..6: mod_base = OTHER; note = 2'-methoxy nucleoside; note (original language) = 2'-甲氧基核苷
  modified_base 10..19: mod_base = OTHER; note = 2'-methoxy nucleoside; note (original language) = 2'-甲氧基核苷
  modified_base 7..9: mod_base = OTHER; note = 2'-fluoro nucleoside; note (original language) = 2'-氟核苷
  modified_base 1..3: mod_base = OTHER; note = phosphorothioate bond; note (original language) = 硫代磷酸酯键
  source 1..19: mol_type = other RNA
acttcttgggcttccgtat

SEQ ID NO: 523 - RNA, 19 nt, synthetic construct
  modified_base 1..6: mod_base = OTHER; note = 2'-methoxy nucleoside; note (original language) = 2'-甲氧基核苷
  modified_base 10..19: mod_base = OTHER; note = 2'-methoxy nucleoside; note (original language) = 2'-甲氧基核苷
  modified_base 7..9: mod_base = OTHER; note = 2'-fluoro nucleoside; note (original language) = 2'-氟核苷
  modified_base 1..3: mod_base = OTHER; note = phosphorothioate bond; note (original language) = 硫代磷酸酯键
  source 1..19: mol_type = other RNA
gtcttgaatgtaagaacat

SEQ ID NO: 524 - RNA, 19 nt, synthetic construct
  modified_base 1..6: mod_base = OTHER; note = 2'-methoxy nucleoside; note (original language) = 2'-甲氧基核苷
  modified_base 10..19: mod_base = OTHER; note = 2'-methoxy nucleoside; note (original language) = 2'-甲氧基核苷
  modified_base 7..9: mod_base = OTHER; note = 2'-fluoro nucleoside; note (original language) = 2'-氟核苷
  modified_base 1..3: mod_base = OTHER; note = phosphorothioate bond; note (original language) = 硫代磷酸酯键
  source 1..19: mol_type = other RNA
ttcctgtttgctgtgtatg

SEQ ID NO: 525 - RNA, 19 nt, synthetic construct
  modified_base 1..6: mod_base = OTHER; note = 2'-methoxy nucleoside; note (original language) = 2'-甲氧基核苷
  modified_base 10..19: mod_base = OTHER; note = 2'-methoxy nucleoside; note (original language) = 2'-甲氧基核苷
  modified_base 7..9: mod_base = OTHER; note = 2'-fluoro nucleoside; note (original language) = 2'-氟核苷
  modified_base 1..3: mod_base = OTHER; note = phosphorothioate bond; note (original language) = 硫代磷酸酯键
  source 1..19: mol_type = other RNA
ggcaagaaccagtgtttag

SEQ ID NO: 526 - RNA, 19 nt, synthetic construct
  modified_base 1..6: mod_base = OTHER; note = 2'-methoxy nucleoside; note (original language) = 2'-甲氧基核苷
  modified_base 10..19: mod_base = OTHER; note = 2'-methoxy nucleoside; note (original language) = 2'-甲氧基核苷
  modified_base 7..9: mod_base = OTHER; note = 2'-fluoro nucleoside; note (original language) = 2'-氟核苷
  modified_base 1..3: mod_base = OTHER; note = phosphorothioate bond; note (original language) = 硫代磷酸酯键
  source 1..19: mol_type = other RNA
gattgacaggttcatgcag

SEQ ID NO: 527 - RNA, 19 nt, synthetic construct
  modified_base 1..6: mod_base = OTHER; note = 2'-methoxy nucleoside; note (original language) = 2'-甲氧基核苷
  modified_base 10..19: mod_base = OTHER; note = 2'-methoxy nucleoside; note (original language) = 2'-甲氧基核苷
  modified_base 7..9: mod_base = OTHER; note = 2'-fluoro nucleoside; note (original language) = 2'-氟核苷
  modified_base 1..3: mod_base = OTHER; note = phosphorothioate bond; note (original language) = 硫代磷酸酯键
  source 1..19: mol_type = other RNA
gtatatatggcatgcacag

SEQ ID NO: 528 - RNA, 19 nt, synthetic construct
  modified_base 1..6: mod_base = OTHER; note = 2'-methoxy nucleoside; note (original language) = 2'-甲氧基核苷
  modified_base 10..19: mod_base = OTHER; note = 2'-methoxy nucleoside; note (original language) = 2'-甲氧基核苷
  modified_base 7..9: mod_base = OTHER; note = 2'-fluoro nucleoside; note (original language) = 2'-氟核苷
  modified_base 1..3: mod_base = OTHER; note = phosphorothioate bond; note (original language) = 硫代磷酸酯键
  source 1..19: mol_type = other RNA
ccatagctggttatttctc

SEQ ID NO: 529 - RNA, 19 nt, synthetic construct
  modified_base 1..6: mod_base = OTHER; note = 2'-methoxy nucleoside; note (original language) = 2'-甲氧基核苷
  modified_base 10..19: mod_base = OTHER; note = 2'-methoxy nucleoside; note (original language) = 2'-甲氧基核苷
  modified_base 7..9: mod_base = OTHER; note = 2'-fluoro nucleoside; note (original language) = 2'-氟核苷
  modified_base 1..3: mod_base = OTHER; note = phosphorothioate bond; note (original language) = 硫代磷酸酯键
  source 1..19: mol_type = other RNA
atgtaagaacatgacctcc

SEQ ID NO: 530 - RNA, 19 nt, synthetic construct
  modified_base 1..6: mod_base = OTHER; note = 2'-methoxy nucleoside; note (original language) = 2'-甲氧基核苷
  modified_base 10..19: mod_base = OTHER; note = 2'-methoxy nucleoside; note (original language) = 2'-甲氧基核苷
  modified_base 7..9: mod_base = OTHER; note = 2'-fluoro nucleoside; note (original language) = 2'-氟核苷
  modified_base 1..3: mod_base = OTHER; note = phosphorothioate bond; note (original language) = 硫代磷酸酯键
  source 1..19: mol_type = other RNA
ccgtatatatggcatgcac

SEQ ID NO: 531 - RNA, 19 nt, synthetic construct
  modified_base 1..6: mod_base = OTHER; note = 2'-methoxy nucleoside; note (original language) = 2'-甲氧基核苷
  modified_base 10..19: mod_base = OTHER; note = 2'-methoxy nucleoside; note (original language) = 2'-甲氧基核苷
  modified_base 7..9: mod_base = OTHER; note = 2'-fluoro nucleoside; note (original language) = 2'-氟核苷
  modified_base 1..3: mod_base = OTHER; note = phosphorothioate bond; note (original language) = 硫代磷酸酯键
  source 1..19: mol_type = other RNA
gtgtcttgaatgtaagaac

SEQ ID NO: 532 - RNA, 19 nt, synthetic construct
  modified_base 1..6: mod_base = OTHER; note = 2'-methoxy nucleoside; note (original language) = 2'-甲氧基核苷
  modified_base 10..19: mod_base = OTHER; note = 2'-methoxy nucleoside; note (original language) = 2'-甲氧基核苷
  modified_base 7..9: mod_base = OTHER; note = 2'-fluoro nucleoside; note (original language) = 2'-氟核苷
  modified_base 1..3: mod_base = OTHER; note = phosphorothioate bond; note (original language) = 硫代磷酸酯键
  source 1..19: mol_type = other RNA
aggcaagaaccagtgttta

SEQ ID NO: 533 - RNA, 19 nt, synthetic construct
  modified_base 1..6: mod_base = OTHER; note = 2'-methoxy nucleoside; note (original language) = 2'-甲氧基核苷
  modified_base 10..19: mod_base = OTHER; note = 2'-methoxy nucleoside; note (original language) = 2'-甲氧基核苷
  modified_base 7..9: mod_base = OTHER; note = 2'-fluoro nucleoside; note (original language) = 2'-氟核苷
  modified_base 1..3: mod_base = OTHER; note = phosphorothioate bond; note (original language) = 硫代磷酸酯键
  source 1..19: mol_type = other RNA
cattcctgtttgctgtgta

SEQ ID NO: 534 - RNA, 19 nt, synthetic construct
  modified_base 1..6: mod_base = OTHER; note = 2'-methoxy nucleoside; note (original language) = 2'-甲氧基核苷
  modified_base 10..19: mod_base = OTHER; note = 2'-methoxy nucleoside; note (original language) = 2'-甲氧基核苷
  modified_base 7..9: mod_base = OTHER; note = 2'-fluoro nucleoside; note (original language) = 2'-氟核苷
  modified_base 1..3: mod_base = OTHER; note = phosphorothioate bond; note (original language) = 硫代磷酸酯键
  source 1..19: mol_type = other RNA
gggttttaaaattaaagta

SEQ ID NO: 535 - RNA, 19 nt, synthetic construct
  modified_base 1..6: mod_base = OTHER; note = 2'-methoxy nucleoside; note (original language) = 2'-甲氧基核苷
  modified_base 10..19: mod_base = OTHER; note = 2'-methoxy nucleoside; note (original language) = 2'-甲氧基核苷
  modified_base 7..9: mod_base = OTHER; note = 2'-fluoro nucleoside; note (original language) = 2'-氟核苷
  modified_base 1..3: mod_base = OTHER; note = phosphorothioate bond; note (original language) = 硫代磷酸酯键
  source 1..19: mol_type = other RNA
cttcttgggcttccgtata

SEQ ID NO: 536 - RNA, 19 nt, synthetic construct
  modified_base 1..6: mod_base = OTHER; note = 2'-methoxy nucleoside; note (original language) = 2'-甲氧基核苷
  modified_base 10..19: mod_base = OTHER; note = 2'-methoxy nucleoside; note (original language) = 2'-甲氧基核苷
  modified_base 7..9: mod_base = OTHER; note = 2'-fluoro nucleoside; note (original language) = 2'-氟核苷
  modified_base 1..3: mod_base = OTHER; note = phosphorothioate bond; note (original language) = 硫代磷酸酯键
  source 1..19: mol_type = other RNA
gttttaaaattaaagtata

SEQ ID NO: 537 - RNA, 19 nt, synthetic construct
  modified_base 1..6: mod_base = OTHER; note = 2'-methoxy nucleoside; note (original language) = 2'-甲氧基核苷
  modified_base 10..19: mod_base = OTHER; note = 2'-methoxy nucleoside; note (original language) = 2'-甲氧基核苷
  modified_base 7..9: mod_base = OTHER; note = 2'-fluoro nucleoside; note (original language) = 2'-氟核苷
  modified_base 1..3: mod_base = OTHER; note = phosphorothioate bond; note (original language) = 硫代磷酸酯键
  source 1..19: mol_type = other RNA
tatatggcatgcacagtga

SEQ ID NO: 538 - RNA, 19 nt, synthetic construct
  modified_base 1..6: mod_base = OTHER; note = 2'-methoxy nucleoside; note (original language) = 2'-甲氧基核苷
  modified_base 10..19: mod_base = OTHER; note = 2'-methoxy nucleoside; note (original language) = 2'-甲氧基核苷
  modified_base 7..9: mod_base = OTHER; note = 2'-fluoro nucleoside; note (original language) = 2'-氟核苷
  modified_base 1..3: mod_base = OTHER; note = phosphorothioate bond; note (original language) = 硫代磷酸酯键
  source 1..19: mol_type = other RNA
cttgaatgtaagaacatga

SEQ ID NO: 539 - RNA, 19 nt, synthetic construct
  modified_base 1..6: mod_base = OTHER; note = 2'-methoxy nucleoside; note (original language) = 2'-甲氧基核苷
  modified_base 10..19: mod_base = OTHER; note = 2'-methoxy nucleoside; note (original language) = 2'-甲氧基核苷
  modified_base 7..9: mod_base = OTHER; note = 2'-fluoro nucleoside; note (original language) = 2'-氟核苷
  modified_base 1..3: mod_base = OTHER; note = phosphorothioate bond; note (original language) = 硫代磷酸酯键
  source 1..19: mol_type = other RNA
gatcttatgacctgcagga

SEQ ID NO: 540 - RNA, 19 nt, synthetic construct
  modified_base 1..6: mod_base = OTHER; note = 2'-methoxy nucleoside; note (original language) = 2'-甲氧基核苷
  modified_base 10..19: mod_base = OTHER; note = 2'-methoxy nucleoside; note (original language) = 2'-甲氧基核苷
  modified_base 7..9: mod_base = OTHER; note = 2'-fluoro nucleoside; note (original language) = 2'-氟核苷
  modified_base 1..3: mod_base = OTHER; note = phosphorothioate bond; note (original language) = 硫代磷酸酯键
  source 1..19: mol_type = other RNA
ggtggacaacagcacctca

SEQ ID NO: 541 - RNA, 19 nt, synthetic construct
  modified_base 1..6: mod_base = OTHER; note = 2'-methoxy nucleoside; note (original language) = 2'-甲氧基核苷
  modified_base 10..19: mod_base = OTHER; note = 2'-methoxy nucleoside; note (original language) = 2'-甲氧基核苷
  modified_base 7..9: mod_base = OTHER; note = 2'-fluoro nucleoside; note (original language) = 2'-氟核苷
  modified_base 1..3: mod_base = OTHER; note = phosphorothioate bond; note (original language) = 硫代磷酸酯键
  source 1..19: mol_type = other RNA
agattgacaggttcatgca

SEQ ID NO: 542 - RNA, 19 nt, synthetic construct
  modified_base 1..6: mod_base = OTHER; note = 2'-methoxy nucleoside; note (original language) = 2'-甲氧基核苷
  modified_base 10..19: mod_base = OTHER; note = 2'-methoxy nucleoside; note (original language) = 2'-甲氧基核苷
  modified_base 7..9: mod_base = OTHER; note = 2'-fluoro nucleoside; note (original language) = 2'-氟核苷
  modified_base 1..3: mod_base = OTHER; note = phosphorothioate bond; note (original language) = 硫代磷酸酯键
  source 1..19: mol_type = other RNA
gttcatgcaggctgtgaca

SEQ ID NO: 543 - RNA, 19 nt, synthetic construct
  modified_base 1..6: mod_base = OTHER; note = 2'-methoxy nucleoside; note (original language) = 2'-甲氧基核苷
  modified_base 10..19: mod_base = OTHER; note = 2'-methoxy nucleoside; note (original language) = 2'-甲氧基核苷
  modified_base 7..9: mod_base = OTHER; note = 2'-fluoro nucleoside; note (original language) = 2'-氟核苷
  modified_base 1..3: mod_base = OTHER; note = phosphorothioate bond; note (original language) = 硫代磷酸酯键
  source 1..19: mol_type = other RNA
caggagttctgggtggaca

SEQ ID NO: 544 - RNA, 19 nt, synthetic construct
  modified_base 1..6: mod_base = OTHER; note = 2'-methoxy nucleoside; note (original language) = 2'-甲氧基核苷
  modified_base 10..19: mod_base = OTHER; note = 2'-methoxy nucleoside; note (original language) = 2'-甲氧基核苷
  modified_base 7..9: mod_base = OTHER; note = 2'-fluoro nucleoside; note (original language) = 2'-氟核苷
  modified_base 1..3: mod_base = OTHER; note = phosphorothioate bond; note (original language) = 硫代磷酸酯键
  source 1..19: mol_type = other RNA
cgtatatatggcatgcaca

SEQ ID NO: 545 - RNA, 19 nt, synthetic construct
  modified_base 1..6: mod_base = OTHER; note = 2'-methoxy nucleoside; note (original language) = 2'-甲氧基核苷
  modified_base 10..19: mod_base = OTHER; note = 2'-methoxy nucleoside; note (original language) = 2'-甲氧基核苷
  modified_base 7..9: mod_base = OTHER; note = 2'-fluoro nucleoside; note (original language) = 2'-氟核苷
  modified_base 1..3: mod_base = OTHER; note = phosphorothioate bond; note (original language) = 硫代磷酸酯键
  source 1..19: mol_type = other RNA
actccctcaactggatgaa

SEQ ID NO: 546 - RNA, 19 nt, synthetic construct
  modified_base 1..6: mod_base = OTHER; note = 2'-methoxy nucleoside; note (original language) = 2'-甲氧基核苷
  modified_base 10..19: mod_base = OTHER; note = 2'-methoxy nucleoside; note (original language) = 2'-甲氧基核苷
  modified_base 7..9: mod_base = OTHER; note = 2'-fluoro nucleoside; note (original language) = 2'-氟核苷
  modified_base 1..3: mod_base = OTHER; note = phosphorothioate bond; note (original language) = 硫代磷酸酯键
  source 1..19: mol_type = other RNA
gggtctcactttccagcaa

SEQ ID NO: 547 - RNA, 19 nt, synthetic construct
  modified_base 1..6: mod_base = OTHER; note = 2'-methoxy nucleoside; note (original language) = 2'-甲氧基核苷
  modified_base 10..19: mod_base = OTHER; note = 2'-methoxy nucleoside; note (original language) = 2'-甲氧基核苷
  modified_base 7..9: mod_base = OTHER; note = 2'-fluoro nucleoside; note (original language) = 2'-氟核苷
  modified_base 1..3: mod_base = OTHER; note = phosphorothioate bond; note (original language) = 硫代磷酸酯键
  source 1..19: mol_type = other RNA
aggagttctgggtggacaa

SEQ ID NO: 548 - RNA, 19 nt, synthetic construct
  modified_base 1..6: mod_base = OTHER; note = 2'-methoxy nucleoside; note (original language) = 2'-甲氧基核苷
  modified_base 10..19: mod_base = OTHER; note = 2'-methoxy nucleoside; note (original language) = 2'-甲氧基核苷
  modified_base 7..9: mod_base = OTHER; note = 2'-fluoro nucleoside; note (original language) = 2'-氟核苷
  modified_base 1..3: mod_base = OTHER; note = phosphorothioate bond; note (original language) = 硫代磷酸酯键
  source 1..19: mol_type = other RNA
gaccagcttgtttgtgaaa

SEQ ID NO: 549 - RNA, 19 nt, synthetic construct
  modified_base 1..6: mod_base = OTHER; note = 2'-methoxy nucleoside; note (original language) = 2'-甲氧基核苷
  modified_base 10..19: mod_base = OTHER; note = 2'-methoxy nucleoside; note (original language) = 2'-甲氧基核苷
  modified_base 7..9: mod_base = OTHER; note = 2'-fluoro nucleoside; note (original language) = 2'-氟核苷
  modified_base 1..3: mod_base = OTHER; note = phosphorothioate bond; note (original language) = 硫代磷酸酯键
  source 1..19: mol_type = other RNA
cctgtgagcagctggcaaa

SEQ ID NO: 550 - RNA, 19 nt, synthetic construct
  modified_base 1..6: mod_base = OTHER; note = 2'-methoxy nucleoside; note (original language) = 2'-甲氧基核苷
  modified_base 10..19: mod_base = OTHER; note = 2'-methoxy nucleoside; note (original language) = 2'-甲氧基核苷
  modified_base 7..9: mod_base = OTHER; note = 2'-fluoro nucleoside; note (original language) = 2'-氟核苷
  modified_base 1..3: mod_base = OTHER; note = phosphorothioate bond; note (original language) = 硫代磷酸酯键
  source 1..19: mol_type = other RNA
ggtctcactttccagcaaa

SEQ ID NO: 551 - RNA, 19 nt, synthetic construct
  modified_base 1..6: mod_base = OTHER; note = 2'-methoxy nucleoside; note (original language) = 2'-甲氧基核苷
  modified_base 10..19: mod_base = OTHER; note = 2'-methoxy nucleoside; note (original language) = 2'-甲氧基核苷
  modified_base 7..9: mod_base = OTHER; note = 2'-fluoro nucleoside; note (original language) = 2'-氟核苷
  modified_base 1..3: mod_base = OTHER; note = phosphorothioate bond; note (original language) = 硫代磷酸酯键
  source 1..19: mol_type = other RNA
caaaaattgggttttaaaa

SEQ ID NO: 552 - RNA, 19 nt, synthetic construct
  modified_base 1..6: mod_base = OTHER; note = 2'-methoxy nucleoside; note (original language) = 2'-甲氧基核苷
  modified_base 10..19: mod_base = OTHER; note = 2'-methoxy nucleoside; note (original language) = 2'-甲氧基核苷
  modified_base 7..9: mod_base = OTHER; note = 2'-fluoro nucleoside; note (original language) = 2'-氟核苷
  modified_base 1..3: mod_base = OTHER; note = phosphorothioate bond; note (original language) = 硫代磷酸酯键
  source 1..19: mol_type = other RNA
gcttgtttgtgaaacaaaa

SEQ ID NO: 553 - RNA, 19 nt, synthetic construct
  modified_base 1..6: mod_base = OTHER; note = 2'-methoxy nucleoside; note (original language) = 2'-甲氧基核苷
  modified_base 10..19: mod_base = OTHER; note = 2'-methoxy nucleoside; note (original language) = 2'-甲氧基核苷
  modified_base 7..9: mod_base = OTHER; note = 2'-fluoro nucleoside; note (original language) = 2'-氟核苷
  modified_base 1..3: mod_base = OTHER; note = phosphorothioate bond; note (original language) = 硫代磷酸酯键
  source 1..19: mol_type = other RNA
aagacgtttattactaaca

SEQ ID NO: 554 - RNA, 19 nt, synthetic construct
  modified_base 1..6: mod_base = OTHER; note = 2'-methoxy nucleoside; note (original language) = 2'-甲氧基核苷
  modified_base 10..19: mod_base = OTHER; note = 2'-methoxy nucleoside; note (original language) = 2'-甲氧基核苷
  modified_base 7..9: mod_base = OTHER; note = 2'-fluoro nucleoside; note (original language) = 2'-氟核苷
  modified_base 1..3: mod_base = OTHER; note = phosphorothioate bond; note (original language) = 硫代磷酸酯键
  source 1..19: mol_type = other RNA
cgaccagcttgtttgtgaa

SEQ ID NO: 555 - RNA, 19 nt, synthetic construct
  modified_base 1..6: mod_base = OTHER; note = 2'-methoxy nucleoside; note (original language) = 2'-甲氧基核苷
  modified_base 10..19: mod_base = OTHER; note = 2'-methoxy nucleoside; note (original language) = 2'-甲氧基核苷
  modified_base 7..9: mod_base = OTHER; note = 2'-fluoro nucleoside; note (original language) = 2'-氟核苷
  modified_base 1..3: mod_base = OTHER; note = phosphorothioate bond; note (original language) = 硫代磷酸酯键
  source 1..19: mol_type = other RNA
cttgtttgtgaaacaaaaa

SEQ ID NO: 556 - RNA, 19 nt, synthetic construct
  modified_base 1..6: mod_base = OTHER; note = 2'-methoxy nucleoside; note (original language) = 2'-甲氧基核苷
  modified_base 10..19: mod_base = OTHER; note = 2'-methoxy nucleoside; note (original language) = 2'-甲氧基核苷
  modified_base 7..9: mod_base = OTHER; note = 2'-fluoro nucleoside; note (original language) = 2'-氟核苷
  modified_base 1..3: mod_base = OTHER; note = phosphorothioate bond; note (original language) = 硫代磷酸酯键
  source 1..19: mol_type = other RNA
acaacttctcggtgactca

SEQ ID NO: 557 - RNA, 19 nt, synthetic construct
  modified_base 1..6: mod_base = OTHER; note = 2'-methoxy nucleoside; note (original language) = 2'-甲氧基核苷
  modified_base 10..19: mod_base = OTHER; note = 2'-methoxy nucleoside; note (original language) = 2'-甲氧基核苷
  modified_base 7..9: mod_base = OTHER; note = 2'-fluoro nucleoside; note (original language) = 2'-氟核苷
  modified_base 1..3: mod_base = OTHER; note = phosphorothioate bond; note (original language) = 硫代磷酸酯键
  source 1..19: mol_type = other RNA
tggtcgggatgctggccaa

SEQ ID NO: 558 - RNA, 19 nt, synthetic construct
  modified_base 1..6: mod_base = OTHER; note = 2'-methoxy nucleoside; note (original language) = 2'-甲氧基核苷
  modified_base 10..19: mod_base = OTHER; note = 2'-methoxy nucleoside; note (original language) = 2'-甲氧基核苷
  modified_base 7..9: mod_base = OTHER; note = 2'-fluoro nucleoside; note (original language) = 2'-氟核苷
  modified_base 1..3: mod_base = OTHER; note = phosphorothioate bond; note (original language) = 硫代磷酸酯键
  source 1..19: mol_type = other RNA
ctgaatttctgtttgaatg

SEQ ID NO: 559 - RNA, 19 nt, synthetic construct
  modified_base 1..6: mod_base = OTHER; note = 2'-methoxy nucleoside; note (original language) = 2'-甲氧基核苷
  modified_base 10..19: mod_base = OTHER; note = 2'-methoxy nucleoside; note (original language) = 2'-甲氧基核苷
  modified_base 7..9: mod_base = OTHER; note = 2'-fluoro nucleoside; note (original language) = 2'-氟核苷
  modified_base 1..3: mod_base = OTHER; note = phosphorothioate bond; note (original language) = 硫代磷酸酯键
  source 1..19: mol_type = other RNA
aggatcttatgacctgcag

SEQ ID NO: 560 - RNA, 19 nt, synthetic construct
  modified_base 1..6: mod_base = OTHER; note = 2'-methoxy nucleoside; note (original language) = 2'-甲氧基核苷
  modified_base 10..19: mod_base = OTHER; note = 2'-methoxy nucleoside; note (original language) = 2'-甲氧基核苷
  modified_base 7..9: mod_base = OTHER; note = 2'-fluoro nucleoside; note (original language) = 2'-氟核苷
  modified_base 1..3: mod_base = OTHER; note = phosphorothioate bond; note (original language) = 硫代磷酸酯键
  source 1..19: mol_type = other RNA
gagaagattgacaggttca

SEQ ID NO: 561 - RNA, 19 nt, synthetic construct
  modified_base 1..6: mod_base = OTHER; note = 2'-methoxy nucleoside; note (original language) = 2'-甲氧基核苷
  modified_base 10..19: mod_base = OTHER; note = 2'-methoxy nucleoside; note (original language) = 2'-甲氧基核苷
  modified_base 7..9: mod_base = OTHER; note = 2'-fluoro nucleoside; note (original language) = 2'-氟核苷
  modified_base 1..3: mod_base = OTHER; note = phosphorothioate bond; note (original language) = 硫代磷酸酯键
  source 1..19: mol_type = other RNA
gttccaaaaagaattccaa

SEQ ID NO: 562 - RNA, 19 nt, synthetic construct
  modified_base 1..6: mod_base = OTHER; note = 2'-methoxy nucleoside; note (original language) = 2'-甲氧基核苷
  modified_base 10..19: mod_base = OTHER; note = 2'-methoxy nucleoside; note (original language) = 2'-甲氧基核苷
  modified_base 7..9: mod_base = OTHER; note = 2'-fluoro nucleoside; note (original language) = 2'-氟核苷
  modified_base 1..3: mod_base = OTHER; note = phosphorothioate bond; note (original language) = 硫代磷酸酯键
  source 1..19: mol_type = other RNA
tgtaagaacatgacctccg

SEQ ID NO: 563 - RNA, 19 nt, synthetic construct
  modified_base 1..6: mod_base = OTHER; note = 2'-methoxy nucleoside; note (original language) = 2'-甲氧基核苷
  modified_base 10..19: mod_base = OTHER; note = 2'-methoxy nucleoside; note (original language) = 2'-甲氧基核苷
  modified_base 7..9: mod_base = OTHER; note = 2'-fluoro nucleoside; note (original language) = 2'-氟核苷
  modified_base 1..3: mod_base = OTHER; note = phosphorothioate bond; note (original language) = 硫代磷酸酯键
  source 1..19: mol_type = other RNA
ggctgtacagggcctgcta

SEQ ID NO: 564 - RNA, 19 nt, synthetic construct
  modified_base 1..6: mod_base = OTHER; note = 2'-methoxy nucleoside; note (original language) = 2'-甲氧基核苷
  modified_base 10..19: mod_base = OTHER; note = 2'-methoxy nucleoside; note (original language) = 2'-甲氧基核苷
  modified_base 7..9: mod_base = OTHER; note = 2'-fluoro nucleoside; note (original language) = 2'-氟核苷
  modified_base 1..3: mod_base = OTHER; note = phosphorothioate bond; note (original language) = 硫代磷酸酯键
  source 1..19: mol_type = other RNA
caactggatgaagaaacta

SEQ ID NO: 565 - RNA, 19 nt, synthetic construct
  modified_base 1..6: mod_base = OTHER; note = 2'-methoxy nucleoside; note (original language) = 2'-甲氧基核苷
  modified_base 10..19: mod_base = OTHER; note = 2'-methoxy nucleoside; note (original language) = 2'-甲氧基核苷
  modified_base 7..9: mod_base = OTHER; note = 2'-fluoro nucleoside; note (original language) = 2'-氟核苷
  modified_base 1..3: mod_base = OTHER; note = phosphorothioate bond; note (original language) = 硫代磷酸酯键
  source 1..19: mol_type = other RNA
ccctcaactggatgaagaa

SEQ ID NO: 566 - RNA, 19 nt, synthetic construct
  modified_base 1..6: mod_base = OTHER; note = 2'-methoxy nucleoside; note (original language) = 2'-甲氧基核苷
  modified_base 10..19: mod_base = OTHER; note = 2'-methoxy nucleoside; note (original language) = 2'-甲氧基核苷
  modified_base 7..9: mod_base = OTHER; note = 2'-fluoro nucleoside; note (original language) = 2'-氟核苷
  modified_base 1..3: mod_base = OTHER; note = phosphorothioate bond; note (original language) = 硫代磷酸酯键
  source 1..19: mol_type = other RNA
tacgtgaaagatgcaagca

SEQ ID NO: 567 - RNA, 19 nt, synthetic construct
  modified_base 1..6: mod_base = OTHER; note = 2'-methoxy nucleoside; note (original language) = 2'-甲氧基核苷
  modified_base 10..19: mod_base = OTHER; note = 2'-methoxy nucleoside; note (original language) = 2'-甲氧基核苷
  modified_base 7..9: mod_base = OTHER; note = 2'-fluoro nucleoside; note (original language) = 2'-氟核苷
  modified_base 1..3: mod_base = OTHER; note = phosphorothioate bond; note (original language) = 硫代磷酸酯键
  source 1..19: mol_type = other RNA
gcaaaggccagcagcagat

SEQ ID NO: 568 - RNA, 19 nt, synthetic construct
  modified_base 1..6: mod_base = OTHER; note = 2'-methoxy nucleoside; note (original language) = 2'-甲氧基核苷
  modified_base 10..19: mod_base = OTHER; note = 2'-methoxy nucleoside; note (original language) = 2'-甲氧基核苷
  modified_base 7..9: mod_base = OTHER; note = 2'-fluoro nucleoside; note (original language) = 2'-氟核苷
  modified_base 1..3: mod_base = OTHER; note = phosphorothioate bond; note (original language) = 硫代磷酸酯键
  source 1..19: mol_type = other RNA
gcaaggatcttatgacctg

SEQ ID NO: 569 - RNA, 19 nt, synthetic construct
  modified_base 1..6: mod_base = OTHER; note = 2'-methoxy nucleoside; note (original language) = 2'-甲氧基核苷
  modified_base 10..19: mod_base = OTHER; note = 2'-methoxy nucleoside; note (original language) = 2'-甲氧基核苷
  modified_base 7..9: mod_base = OTHER; note = 2'-fluoro nucleoside; note (original language) = 2'-氟核苷
  modified_base 1..3: mod_base = OTHER; note = phosphorothioate bond; note (original language) = 硫代磷酸酯键
  source 1..19: mol_type = other RNA
gctgacaggctacaggcaa

SEQ ID NO: 570 - RNA, 19 nt, synthetic construct
  modified_base 1..6: mod_base = OTHER; note = 2'-methoxy nucleoside; note (original language) = 2'-甲氧基核苷
  modified_base 10..19: mod_base = OTHER; note = 2'-methoxy nucleoside; note (original language) = 2'-甲氧基核苷
  modified_base 7..9: mod_base = OTHER; note = 2'-fluoro nucleoside; note (original language) = 2'-氟核苷
  modified_base 1..3: mod_base = OTHER; note = phosphorothioate bond; note (original language) = 硫代磷酸酯键
  source 1..19: mol_type = other RNA
cccttgtgttagtaataaa

SEQ ID NO: 571 - RNA, 19 nt, synthetic construct
  modified_base 1..6: mod_base = OTHER; note = 2'-methoxy nucleoside; note (original language) = 2'-甲氧基核苷
  modified_base 10..19: mod_base = OTHER; note = 2'-methoxy nucleoside; note (original language) = 2'-甲氧基核苷
  modified_base 7..9: mod_base = OTHER; note = 2'-fluoro nucleoside; note (original language) = 2'-氟核苷
  modified_base 1..3: mod_base = OTHER; note = phosphorothioate bond; note (original language) = 硫代磷酸酯键
  source 1..19: mol_type = other RNA
gcacctgaatttctgtttg

SEQ ID NO: 572 - RNA, 19 nt, synthetic construct
  modified_base 1..6: mod_base = OTHER; note = 2'-methoxy nucleoside; note (original language) = 2'-甲氧基核苷
  modified_base 10..19: mod_base = OTHER; note = 2'-methoxy nucleoside; note (original language) = 2'-甲氧基核苷
  modified_base 7..9: mod_base = OTHER; note = 2'-fluoro nucleoside; note (original language) = 2'-氟核苷
  modified_base 1..3: mod_base = OTHER; note = phosphorothioate bond; note (original language) = 硫代磷酸酯键
  source 1..19: mol_type = other RNA
gagcacagcatgaggccag

SEQ ID NO: 573 - RNA, 19 nt, synthetic construct
  modified_base 1..6: mod_base = OTHER; note = 2'-methoxy nucleoside; note (original language) = 2'-甲氧基核苷
  modified_base 10..19: mod_base = OTHER; note = 2'-methoxy nucleoside; note (original language) = 2'-甲氧基核苷
  modified_base 7..9: mod_base = OTHER; note = 2'-fluoro nucleoside; note (original language) = 2'-氟核苷
  modified_base 1..3: mod_base = OTHER; note = phosphorothioate bond; note (original language) = 硫代磷酸酯键
  source 1..19: mol_type = other RNA
ctcccttgtgttagtaata

SEQ ID NO: 574 - RNA, 19 nt, synthetic construct
  modified_base 1..6: mod_base = OTHER; note = 2'-methoxy nucleoside; note (original language) = 2'-甲氧基核苷
  modified_base 10..19: mod_base = OTHER; note = 2'-methoxy nucleoside; note (original language) = 2'-甲氧基核苷
  modified_base 7..9: mod_base = OTHER; note = 2'-fluoro nucleoside; note (original language) = 2'-氟核苷
  modified_base 1..3: mod_base = OTHER; note = phosphorothioate bond; note (original language) = 硫代磷酸酯键
  source 1..19: mol_type = other RNA
acaatacgtgaaagatgca

SEQ ID NO: 575 - RNA, 19 nt, synthetic construct
  modified_base 1..6: mod_base = OTHER; note = 2'-methoxy nucleoside; note (original language) = 2'-甲氧基核苷
  modified_base 10..19: mod_base = OTHER; note = 2'-methoxy nucleoside; note (original language) = 2'-甲氧基核苷
  modified_base 7..9: mod_base = OTHER; note = 2'-fluoro nucleoside; note (original language) = 2'-氟核苷
  modified_base 1..3: mod_base = OTHER; note = phosphorothioate bond; note (original language) = 硫代磷酸酯键
  source 1..19: mol_type = other RNA
gaacaatacgtgaaagatg

SEQ ID NO: 576 - RNA, 19 nt, synthetic construct
  modified_base 1..6: mod_base = OTHER; note = 2'-methoxy nucleoside; note (original language) = 2'-甲氧基核苷
  modified_base 10..19: mod_base = OTHER; note = 2'-methoxy nucleoside; note (original language) = 2'-甲氧基核苷
  modified_base 7..9: mod_base = OTHER; note = 2'-fluoro nucleoside; note (original language) = 2'-氟核苷
  modified_base 1..3: mod_base = OTHER; note = phosphorothioate bond; note (original language) = 硫代磷酸酯键
  source 1..19: mol_type = other RNA
tttctcccttgtgttagta

SEQ ID NO: 577 - RNA, 19 nt, synthetic construct
  modified_base 1..6: mod_base = OTHER; note = 2'-methoxy nucleoside; note (original language) = 2'-甲氧基核苷
  modified_base 10..19: mod_base = OTHER; note = 2'-methoxy nucleoside; note (original language) = 2'-甲氧基核苷
  modified_base 7..9: mod_base = OTHER; note = 2'-fluoro nucleoside; note (original language) = 2'-氟核苷
  modified_base 1..3: mod_base = OTHER; note = phosphorothioate bond; note (original language) = 硫代磷酸酯键
  source 1..19: mol_type = other RNA
ccaatgccgggaagcccaa

SEQ ID NO: 578 - RNA, 19 nt, synthetic construct
  modified_base 1..6: mod_base = OTHER; note = 2'-methoxy nucleoside; note (original language) = 2'-甲氧基核苷
  modified_base 10..19: mod_base = OTHER; note = 2'-methoxy nucleoside; note (original language) = 2'-甲氧基核苷
  modified_base 7..9: mod_base = OTHER; note = 2'-fluoro nucleoside; note (original language) = 2'-氟核苷
  modified_base 1..3: mod_base = OTHER; note = phosphorothioate bond; note (original language) = 硫代磷酸酯键
  source 1..19: mol_type = other RNA
tgcaagcacctgaatttct

SEQ ID NO: 579 - RNA, 19 nt, synthetic construct
  modified_base 1..6: mod_base = OTHER; note = 2'-methoxy nucleoside; note (original language) = 2'-甲氧基核苷
  modified_base 10..19: mod_base = OTHER; note = 2'-methoxy nucleoside; note (original language) = 2'-甲氧基核苷
  modified_base 7..9: mod_base = OTHER; note = 2'-fluoro nucleoside; note (original language) = 2'-氟核苷
  modified_base 1..3: mod_base = OTHER; note = phosphorothioate bond; note (original language) = 硫代磷酸酯键
  source 1..19: mol_type = other RNA
ggtgctgcaaggatcttat

SEQ ID NO: 580 - RNA, 19 nt, synthetic construct
  modified_base 1..6: mod_base = OTHER; note = 2'-methoxy nucleoside; note (original language) = 2'-甲氧基核苷
  modified_base 10..19: mod_base = OTHER; note = 2'-methoxy nucleoside; note (original language) = 2'-甲氧基核苷
  modified_base 7..9: mod_base = OTHER; note = 2'-fluoro nucleoside; note (original language) = 2'-氟核苷
  modified_base 1..3: mod_base = OTHER; note = phosphorothioate bond; note (original language) = 硫代磷酸酯键
  source 1..19: mol_type = other RNA
ccacacagctgacaggcta

SEQ ID NO: 581 - RNA, 19 nt, synthetic construct
  modified_base 1..6: mod_base = OTHER; note = 2'-methoxy nucleoside; note (original language) = 2'-甲氧基核苷
  modified_base 10..19: mod_base = OTHER; note = 2'-methoxy nucleoside; note (original language) = 2'-甲氧基核苷
  modified_base 7..9: mod_base = OTHER; note = 2'-fluoro nucleoside; note (original language) = 2'-氟核苷
  modified_base 1..3: mod_base = OTHER; note = phosphorothioate bond; note (original language) = 硫代磷酸酯键
  source 1..19: mol_type = other RNA
ttgaacaatacgtgaaaga

SEQ ID NO: 582 - RNA, 19 nt, synthetic construct
  modified_base 1..6: mod_base = OTHER; note = 2'-methoxy nucleoside; note (original language) = 2'-甲氧基核苷
  modified_base 10..19: mod_base = OTHER; note = 2'-methoxy nucleoside; note (original language) = 2'-甲氧基核苷
  modified_base 7..9: mod_base = OTHER; note = 2'-fluoro nucleoside; note (original language) = 2'-氟核苷
  modified_base 1..3: mod_base = OTHER; note = phosphorothioate bond; note (original language) = 硫代磷酸酯键
  source 1..19: mol_type = other RNA
gacaccgaagacaagttga

SEQ ID NO: 583 - RNA, 19 nt, synthetic construct
  modified_base 1..6: mod_base = OTHER; note = 2'-methoxy nucleoside; note (original language) = 2'-甲氧基核苷
  modified_base 10..19: mod_base = OTHER; note = 2'-methoxy nucleoside; note (original language) = 2'-甲氧基核苷
  modified_base 7..9: mod_base = OTHER; note = 2'-fluoro nucleoside; note (original language) = 2'-氟核苷
  modified_base 1..3: mod_base = OTHER; note = phosphorothioate bond; note (original language) = 硫代磷酸酯键
  source 1..19: mol_type = other RNA
gagccagtgtggacagcac

SEQ ID NO: 584 - RNA, 19 nt, synthetic construct
  modified_base 1..6: mod_base = OTHER; note = 2'-methoxy nucleoside; note (original language) = 2'-甲氧基核苷
  modified_base 10..19: mod_base = OTHER; note = 2'-methoxy nucleoside; note (original language) = 2'-甲氧基核苷
  modified_base 7..9: mod_base = OTHER; note = 2'-fluoro nucleoside; note (original language) = 2'-氟核苷
  modified_base 1..3: mod_base = OTHER; note = phosphorothioate bond; note (original language) = 硫代磷酸酯键
  source 1..19: mol_type = other RNA
tggaaggacaagaactgca

SEQ ID NO: 585 - RNA, 19 nt, synthetic construct
  modified_base 1..6: mod_base = OTHER; note = 2'-methoxy nucleoside; note (original language) = 2'-甲氧基核苷
  modified_base 10..19: mod_base = OTHER; note = 2'-methoxy nucleoside; note (original language) = 2'-甲氧基核苷
  modified_base 7..9: mod_base = OTHER; note = 2'-fluoro nucleoside; note (original language) = 2'-氟核苷
  modified_base 1..3: mod_base = OTHER; note = phosphorothioate bond; note (original language) = 硫代磷酸酯键
  source 1..19: mol_type = other RNA
caacttctcggtgactcaa

SEQ ID NO: 586 - RNA, 19 nt, synthetic construct
  modified_base 1..6: mod_base = OTHER; note = 2'-methoxy nucleoside; note (original language) = 2'-甲氧基核苷
  modified_base 10..19: mod_base = OTHER; note = 2'-methoxy nucleoside; note (original language) = 2'-甲氧基核苷
  modified_base 7..9: mod_base = OTHER; note = 2'-fluoro nucleoside; note (original language) = 2'-氟核苷
  modified_base 1..3: mod_base = OTHER; note = phosphorothioate bond; note (original language) = 硫代磷酸酯键
  source 1..19: mol_type = other RNA
aacgtcttgccacaataag

SEQ ID NO: 587 - RNA, 19 nt, synthetic construct
  modified_base 1..6: mod_base = OTHER; note = 2'-methoxy nucleoside; note (original language) = 2'-甲氧基核苷
  modified_base 10..19: mod_base = OTHER; note = 2'-methoxy nucleoside; note (original language) = 2'-甲氧基核苷
  modified_base 7..9: mod_base = OTHER; note = 2'-fluoro nucleoside; note (original language) = 2'-氟核苷
  modified_base 1..3: mod_base = OTHER; note = phosphorothioate bond; note (original language) = 硫代磷酸酯键
  source 1..19: mol_type = other RNA
ctgagaagattgacaggtt

SEQ ID NO: 588 - RNA, 19 nt, synthetic construct
  modified_base 1..6: mod_base = OTHER; note = 2'-methoxy nucleoside; note (original language) = 2'-甲氧基核苷
  modified_base 10..19: mod_base = OTHER; note = 2'-methoxy nucleoside; note (original language) = 2'-甲氧基核苷
  modified_base 7..9: mod_base = OTHER; note = 2'-fluoro nucleoside; note (original language) = 2'-氟核苷
  modified_base 1..3: mod_base = OTHER; note = phosphorothioate bond; note (original language) = 硫代磷酸酯键
  source 1..19: mol_type = other RNA
ccagtttgctgggtttatt

SEQ ID NO: 589 - RNA, 19 nt, synthetic construct
  modified_base 1..6: mod_base = OTHER; note = 2'-methoxy nucleoside; note (original language) = 2'-甲氧基核苷
  modified_base 10..19: mod_base = OTHER; note = 2'-methoxy nucleoside; note (original language) = 2'-甲氧基核苷
  modified_base 7..9: mod_base = OTHER; note = 2'-fluoro nucleoside; note (original language) = 2'-氟核苷
  modified_base 1..3: mod_base = OTHER; note = phosphorothioate bond; note (original language) = 硫代磷酸酯键
  source 1..19: mol_type = other RNA
acttctcggtgactcaagt

SEQ ID NO: 590 - RNA, 21 nt, synthetic construct
  modified_base 1..8: mod_base = OTHER; note = 2'-methoxy nucleoside; note (original language) = 2'-甲氧基核苷
  modified_base 12..21: mod_base = OTHER; note = 2'-methoxy nucleoside; note (original language) = 2'-甲氧基核苷
  modified_base 9..11: mod_base = OTHER; note = 2'-fluoro nucleoside; note (original language) = 2'-氟核苷
  modified_base 1..3: mod_base = OTHER; note = phosphorothioate bond; note (original language) = 硫代磷酸酯键
  source 1..21: mol_type = other RNA
ccgtttctccttggtctaaga

SEQ ID NO: 591 - RNA, 21 nt, synthetic construct
  modified_base 1..8: mod_base = OTHER; note = 2'-methoxy nucleoside; note (original language) = 2'-甲氧基核苷
  modified_base 12..21: mod_base = OTHER; note = 2'-methoxy nucleoside; note (original language) = 2'-甲氧基核苷
  modified_base 9..11: mod_base = OTHER; note = 2'-fluoro nucleoside; note (original language) = 2'-氟核苷
  modified_base 1..3: mod_base = OTHER; note = phosphorothioate bond; note (original language) = 硫代磷酸酯键
  source 1..21: mol_type = other RNA
gccgtttctcgttggtctaaa

SEQ ID NO: 592 - RNA, 21 nt, synthetic construct
  modified_base 1..8: mod_base = OTHER; note = 2'-methoxy nucleoside; note (original language) = 2'-甲氧基核苷
  modified_base 12..21: mod_base = OTHER; note = 2'-methoxy nucleoside; note (original language) = 2'-甲氧基核苷
  modified_base 9..11: mod_base = OTHER; note = 2'-fluoro nucleoside; note (original language) = 2'-氟核苷
  modified_base 1..3: mod_base = OTHER; note = phosphorothioate bond; note (original language) = 硫代磷酸酯键
  source 1..21: mol_type = other RNA
gcgtttctccttggtctaaga

SEQ ID NO: 593 - RNA, 21 nt, synthetic construct
  modified_base 1..8: mod_base = OTHER; note = 2'-methoxy nucleoside; note (original language) = 2'-甲氧基核苷
  modified_base 12..21: mod_base = OTHER; note = 2'-methoxy nucleoside; note (original language) = 2'-甲氧基核苷
  modified_base 9..11: mod_base = OTHER; note = 2'-fluoro nucleoside; note (original language) = 2'-氟核苷
  modified_base 1..3: mod_base = OTHER; note = phosphorothioate bond; note (original language) = 硫代磷酸酯键
  source 1..21: mol_type = other RNA
cagtctcccagcttttcttct

SEQ ID NO: 594 - RNA, 21 nt, synthetic construct
  modified_base 1..8: mod_base = OTHER; note = 2'-methoxy nucleoside; note (original language) = 2'-甲氧基核苷
  modified_base 12..21: mod_base = OTHER; note = 2'-methoxy nucleoside; note (original language) = 2'-甲氧基核苷
  modified_base 9..11: mod_base = OTHER; note = 2'-fluoro nucleoside; note (original language) = 2'-氟核苷
  modified_base 1..3: mod_base = OTHER; note = phosphorothioate bond; note (original language) = 硫代磷酸酯键
  source 1..21: mol_type = other RNA
gcgtttctccttggtctaagt

SEQ ID NO: 595 - RNA, 19 nt, synthetic construct
  modified_base 1..6: mod_base = OTHER; note = 2'-methoxy nucleoside; note (original language) = 2'-甲氧基核苷
  modified_base 10..19: mod_base = OTHER; note = 2'-methoxy nucleoside; note (original language) = 2'-甲氧基核苷
  modified_base 7..9: mod_base = OTHER; note = 2'-fluoro nucleoside; note (original language) = 2'-氟核苷
  modified_base 1..3: mod_base = OTHER; note = phosphorothioate bond; note (original language) = 硫代磷酸酯键
  source 1..19: mol_type = other RNA
ctcccaccttttcttctaa

SEQ ID NO: 596 - RNA, 19 nt, synthetic construct
  modified_base 1..6: mod_base = OTHER; note = 2'-methoxy nucleoside; note (original language) = 2'-甲氧基核苷
  modified_base 10..19: mod_base = OTHER; note = 2'-methoxy nucleoside; note (original language) = 2'-甲氧基核苷
  modified_base 7..9: mod_base = OTHER; note = 2'-fluoro nucleoside; note (original language) = 2'-氟核苷
  modified_base 1..3: mod_base = OTHER; note = phosphorothioate bond; note (original language) = 硫代磷酸酯键
  source 1..19: mol_type = other RNA
cccaccttttcttctaata

SEQ ID NO: 597 - RNA, 19 nt, synthetic construct
  modified_base 1..6: mod_base = OTHER; note = 2'-methoxy nucleoside; note (original language) = 2'-甲氧基核苷
  modified_base 10..19: mod_base = OTHER; note = 2'-methoxy nucleoside; note (original language) = 2'-甲氧基核苷
  modified_base 7..9: mod_base = OTHER; note = 2'-fluoro nucleoside; note (original language) = 2'-氟核苷
  modified_base 1..3: mod_base = OTHER; note = phosphorothioate bond; note (original language) = 硫代磷酸酯键
  source 1..19: mol_type = other RNA
caccttttcttctaatgaa

SEQ ID NO: 598 - RNA, 19 nt, synthetic construct
  modified_base 1..6: mod_base = OTHER; note = 2'-methoxy nucleoside; note (original language) = 2'-甲氧基核苷
  modified_base 10..19: mod_base = OTHER; note = 2'-methoxy nucleoside; note (original language) = 2'-甲氧基核苷
  modified_base 7..9: mod_base = OTHER; note = 2'-fluoro nucleoside; note (original language) = 2'-氟核苷
  modified_base 1..3: mod_base = OTHER; note = phosphorothioate bond; note (original language) = 硫代磷酸酯键
  source 1..19: mol_type = other RNA
ccttttcttctaatgagta

SEQ ID NO: 599 - RNA, 23 nt, synthetic construct
  modified_base 1: mod_base = OTHER; note = 2'-methoxy nucleoside; note (original language) = 2'-甲氧基核苷
  modified_base 3..5: mod_base = OTHER; note = 2'-methoxy nucleoside; note (original language) = 2'-甲氧基核苷
  modified_base 7..13: mod_base = OTHER; note = 2'-methoxy nucleoside; note (original language) = 2'-甲氧基核苷
  modified_base 15: mod_base = OTHER; note = 2'-methoxy nucleoside; note (original language) = 2'-甲氧基核苷
  modified_base 17..23: mod_base = OTHER; note = 2'-methoxy nucleoside; note (original language) = 2'-甲氧基核苷
  modified_base 2: mod_base = OTHER; note = 2'-fluoro nucleoside; note (original language) = 2'-氟核苷
  modified_base 6: mod_base = OTHER; note = 2'-fluoro nucleoside; note (original language) = 2'-氟核苷
  modified_base 14: mod_base = OTHER; note = 2'-fluoro nucleoside; note (original language) = 2'-氟核苷
  modified_base 16: mod_base = OTHER; note = 2'-fluoro nucleoside; note (original language) = 2'-氟核苷
  modified_base 1..3: mod_base = OTHER; note = phosphorothioate bond; note (original language) = 硫代磷酸酯键
  modified_base 21..23: mod_base = OTHER; note = phosphorothioate bond; note (original language) = 硫代磷酸酯键
  source 1..23: mol_type = other RNA
tgtactctcattgtggatgacga

SEQ ID NO: 600 - RNA, 23 nt, synthetic construct
  modified_base 1: mod_base = OTHER; note = 2'-methoxy nucleoside; note (original language) = 2'-甲氧基核苷
  modified_base 3..5: mod_base = OTHER; note = 2'-methoxy nucleoside; note (original language) = 2'-甲氧基核苷
  modified_base 7..8: mod_base = OTHER; note = 2'-methoxy nucleoside; note (original language) = 2'-甲氧基核苷
  modified_base 10..13: mod_base = OTHER; note = 2'-methoxy nucleoside; note (original language) = 2'-甲氧基核苷
  modified_base 15: mod_base = OTHER; note = 2'-methoxy nucleoside; note (original language) = 2'-甲氧基核苷
  modified_base 17..23: mod_base = OTHER; note = 2'-methoxy nucleoside; note (original language) = 2'-甲氧基核苷
  modified_base 2: mod_base = OTHER; note = 2'-fluoro nucleoside; note (original language) = 2'-氟核苷
  modified_base 6: mod_base = OTHER; note = 2'-fluoro nucleoside; note (original language) = 2'-氟核苷
  modified_base 9: mod_base = OTHER; note = 2'-fluoro nucleoside; note (original language) = 2'-氟核苷
  modified_base 14: mod_base = OTHER; note = 2'-fluoro nucleoside; note (original language) = 2'-氟核苷
  modified_base 16: mod_base = OTHER; note = 2'-fluoro nucleoside; note (original language) = 2'-氟核苷
  modified_base 1..3: mod_base = OTHER; note = phosphorothioate bond; note (original language) = 硫代磷酸酯键
  modified_base 21..23: mod_base = OTHER; note = phosphorothioate bond; note (original language) = 硫代磷酸酯键
  source 1..23: mol_type = other RNA
tcattgtggatgacgaggtggaa

SEQ ID NO: 601 - RNA, 23 nt, synthetic construct
  modified_base 1: mod_base = OTHER; note = 2'-methoxy nucleoside; note (original language) = 2'-甲氧基核苷
  modified_base 3..5: mod_base = OTHER; note = 2'-methoxy nucleoside; note (original language) = 2'-甲氧基核苷
  modified_base 7..8: mod_base = OTHER; note = 2'-methoxy nucleoside; note (original language) = 2'-甲氧基核苷
  modified_base 10..13: mod_base = OTHER; note = 2'-methoxy nucleoside; note (original language) = 2'-甲氧基核苷
  modified_base 15: mod_base = OTHER; note = 2'-methoxy nucleoside; note (original language) = 2'-甲氧基核苷
  modified_base 17..23: mod_base = OTHER; note = 2'-methoxy nucleoside; note (original language) = 2'-甲氧基核苷
  modified_base 2: mod_base = OTHER; note = 2'-fluoro nucleoside; note (original language) = 2'-氟核苷
  modified_base 6: mod_base = OTHER; note = 2'-fluoro nucleoside; note (original language) = 2'-氟核苷
  modified_base 9: mod_base = OTHER; note = 2'-fluoro nucleoside; note (original language) = 2'-氟核苷
  modified_base 14: mod_base = OTHER; note = 2'-fluoro nucleoside; note (original language) = 2'-氟核苷
  modified_base 16: mod_base = OTHER; note = 2'-fluoro nucleoside; note (original language) = 2'-氟核苷
  modified_base 1..3: mod_base = OTHER; note = phosphorothioate bond; note (original language) = 硫代磷酸酯键
  modified_base 21..23: mod_base = OTHER; note = phosphorothioate bond; note (original language) = 硫代磷酸酯键
  source 1..23: mol_type = other RNA
ttctcattgtggatgacgaggtg

SEQ ID NO: 602 - RNA, 23 nt, synthetic construct
  modified_base 1: mod_base = OTHER; note = 2'-methoxy nucleoside; note (original language) = 2'-甲氧基核苷
  modified_base 3..5: mod_base = OTHER; note = 2'-methoxy nucleoside; note (original language) = 2'-甲氧基核苷
  modified_base 7..8: mod_base = OTHER; note = 2'-methoxy nucleoside; note (original language) = 2'-甲氧基核苷
  modified_base 10..13: mod_base = OTHER; note = 2'-methoxy nucleoside; note (original language) = 2'-甲氧基核苷
  modified_base 15: mod_base = OTHER; note = 2'-methoxy nucleoside; note (original language) = 2'-甲氧基核苷
  modified_base 17..23: mod_base = OTHER; note = 2'-methoxy nucleoside; note (original language) = 2'-甲氧基核苷
  modified_base 2: mod_base = OTHER; note = 2'-fluoro nucleoside; note (original language) = 2'-氟核苷
  modified_base 6: mod_base = OTHER; note = 2'-fluoro nucleoside; note (original language) = 2'-氟核苷
  modified_base 9: mod_base = OTHER; note = 2'-fluoro nucleoside; note (original language) = 2'-氟核苷
  modified_base 14: mod_base = OTHER; note = 2'-fluoro nucleoside; note (original language) = 2'-氟核苷
  modified_base 16: mod_base = OTHER; note = 2'-fluoro nucleoside; note (original language) = 2'-氟核苷
  modified_base 1..3: mod_base = OTHER; note = phosphorothioate bond; note (original language) = 硫代磷酸酯键
  modified_base 21..23: mod_base = OTHER; note = phosphorothioate bond; note (original language) = 硫代磷酸酯键
  source 1..23: mol_type = other RNA
tcaggtactctcattgtggatga

SEQ ID NO: 603 - RNA, 23 nt, synthetic construct
  modified_base 1: mod_base = OTHER; note = 2'-methoxy nucleoside; note (original language) = 2'-甲氧基核苷
  modified_base 3..5: mod_base = OTHER; note = 2'-methoxy nucleoside; note (original language) = 2'-甲氧基核苷
  modified_base 7..8: mod_base = OTHER; note = 2'-methoxy nucleoside; note (original language) = 2'-甲氧基核苷
  modified_base 10..13: mod_base = OTHER; note = 2'-methoxy nucleoside; note (original language) = 2'-甲氧基核苷
  modified_base 15: mod_base = OTHER; note = 2'-methoxy nucleoside; note (original language) = 2'-甲氧基核苷
  modified_base 17..23: mod_base = OTHER; note = 2'-methoxy nucleoside; note (original language) = 2'-甲氧基核苷
  modified_base 2: mod_base = OTHER; note = 2'-fluoro nucleoside; note (original language) = 2'-氟核苷
  modified_base 6: mod_base = OTHER; note = 2'-fluoro nucleoside; note (original language) = 2'-氟核苷
  modified_base 9: mod_base = OTHER; note = 2'-fluoro nucleoside; note (original language) = 2'-氟核苷
  modified_base 14: mod_base = OTHER; note = 2'-fluoro nucleoside; note (original language) = 2'-氟核苷
  modified_base 16: mod_base = OTHER; note = 2'-fluoro nucleoside; note (original language) = 2'-氟核苷
  modified_base 1..3: mod_base = OTHER; note = phosphorothioate bond; note (original language) = 硫代磷酸酯键
  modified_base 21..23: mod_base = OTHER; note = phosphorothioate bond; note (original language) = 硫代磷酸酯键
  source 1..23: mol_type = other RNA
tcatagctcactgtgcatgccat

SEQ ID NO: 604 - RNA, 23 nt, synthetic construct
  modified_base 1: mod_base = OTHER; note = 2'-methoxy nucleoside; note (original language) = 2'-甲氧基核苷
  modified_base 3..5: mod_base = OTHER; note = 2'-methoxy nucleoside; note (original language) = 2'-甲氧基核苷
  modified_base 7..8: mod_base = OTHER; note = 2'-methoxy nucleoside; note (original language) = 2'-甲氧基核苷
  modified_base 10..13: mod_base = OTHER; note = 2'-methoxy nucleoside; note (original language) = 2'-甲氧基核苷
  modified_base 15: mod_base = OTHER; note = 2'-methoxy nucleoside; note (original language) = 2'-甲氧基核苷
  modified_base 17..23: mod_base = OTHER; note = 2'-methoxy nucleoside; note (original language) = 2'-甲氧基核苷
  modified_base 2: mod_base = OTHER; note = 2'-fluoro nucleoside; note (original language) = 2'-氟核苷
  modified_base 6: mod_base = OTHER; note = 2'-fluoro nucleoside; note (original language) = 2'-氟核苷
  modified_base 9: mod_base = OTHER; note = 2'-fluoro nucleoside; note (original language) = 2'-氟核苷
  modified_base 14: mod_base = OTHER; note = 2'-fluoro nucleoside; note (original language) = 2'-氟核苷
  modified_base 16: mod_base = OTHER; note = 2'-fluoro nucleoside; note (original language) = 2'-氟核苷
  modified_base 1..3: mod_base = OTHER; note = phosphorothioate bond; note (original language) = 硫代磷酸酯键
  modified_base 21..23: mod_base = OTHER; note = phosphorothioate bond; note (original language) = 硫代磷酸酯键
  source 1..23: mol_type = other RNA
catgaacctgtcaatcttctcag

SEQ ID NO: 605 - RNA, 23 nt, synthetic construct
  modified_base 1: mod_base = OTHER; note = 2'-methoxy nucleoside; note (original language) = 2'-甲氧基核苷
  modified_base 3..5: mod_base = OTHER; note = 2'-methoxy nucleoside; note (original language) = 2'-甲氧基核苷
  modified_base 7..8: mod_base = OTHER; note = 2'-methoxy nucleoside; note (original language) = 2'-甲氧基核苷
  modified_base 10..13: mod_base = OTHER; note = 2'-methoxy nucleoside; note (original language) = 2'-甲氧基核苷
  modified_base 15: mod_base = OTHER; note = 2'-methoxy nucleoside; note (original language) = 2'-甲氧基核苷
  modified_base 17..23: mod_base = OTHER; note = 2'-methoxy nucleoside; note (original language) = 2'-甲氧基核苷
  modified_base 2: mod_base = OTHER; note = 2'-fluoro nucleoside; note (original language) = 2'-氟核苷
  modified_base 6: mod_base = OTHER; note = 2'-fluoro nucleoside; note (original language) = 2'-氟核苷
  modified_base 9: mod_base = OTHER; note = 2'-fluoro nucleoside; note (original language) = 2'-氟核苷
  modified_base 14: mod_base = OTHER; note = 2'-fluoro nucleoside; note (original language) = 2'-氟核苷
  modified_base 16: mod_base = OTHER; note = 2'-fluoro nucleoside; note (original language) = 2'-氟核苷
  modified_base 1..3: mod_base = OTHER; note = phosphorothioate bond; note (original language) = 硫代磷酸酯键
  modified_base 21..23: mod_base = OTHER; note = phosphorothioate bond; note (original language) = 硫代磷酸酯键
  source 1..23: mol_type = other RNA
ttgaaagccagggtgctgtccac

SEQ ID NO: 606 - RNA, 23 nt, synthetic construct
  modified_base 1: mod_base = OTHER; note = 2'-methoxy nucleoside; note (original language) = 2'-甲氧基核苷
  modified_base 3..5: mod_base = OTHER; note = 2'-methoxy nucleoside; note (original language) = 2'-甲氧基核苷
  modified_base 7..8: mod_base = OTHER; note = 2'-methoxy nucleoside; note (original language) = 2'-甲氧基核苷
  modified_base 10..13: mod_base = OTHER; note = 2'-methoxy nucleoside; note (original language) = 2'-甲氧基核苷
  modified_base 15: mod_base = OTHER; note = 2'-methoxy nucleoside; note (original language) = 2'-甲氧基核苷
  modified_base 17..23: mod_base = OTHER; note = 2'-methoxy nucleoside; note (original language) = 2'-甲氧基核苷
  modified_base 2: mod_base = OTHER; note = 2'-fluoro nucleoside; note (original language) = 2'-氟核苷
  modified_base 6: mod_base = OTHER; note = 2'-fluoro nucleoside; note (original language) = 2'-氟核苷
  modified_base 9: mod_base = OTHER; note = 2'-fluoro nucleoside; note (original language) = 2'-氟核苷
  modified_base 14: mod_base = OTHER; note = 2'-fluoro nucleoside; note (original language) = 2'-氟核苷
  modified_base 16: mod_base = OTHER; note = 2'-fluoro nucleoside; note (original language) = 2'-氟核苷
  modified_base 1..3: mod_base = OTHER; note = phosphorothioate bond; note (original language) = 硫代磷酸酯键
  modified_base 21..23: mod_base = OTHER; note = phosphorothioate bond; note (original language) = 硫代磷酸酯键
  source 1..23: mol_type = other RNA
tcaaaaaaaatgctgttcagcac

SEQ ID NO: 607 - RNA, 23 nt, synthetic construct
  modified_base 1: mod_base = OTHER; note = 2'-methoxy nucleoside; note (original language) = 2'-甲氧基核苷
  modified_base 3..5: mod_base = OTHER; note = 2'-methoxy nucleoside; note (original language) = 2'-甲氧基核苷
  modified_base 7..8: mod_base = OTHER; note = 2'-methoxy nucleoside; note (original language) = 2'-甲氧基核苷
  modified_base 10..13: mod_base = OTHER; note = 2'-methoxy nucleoside; note (original language) = 2'-甲氧基核苷
  modified_base 15: mod_base = OTHER; note = 2'-methoxy nucleoside; note (original language) = 2'-甲氧基核苷
  modified_base 17..23: mod_base = OTHER; note = 2'-methoxy nucleoside; note (original language) = 2'-甲氧基核苷
  modified_base 2: mod_base = OTHER; note = 2'-fluoro nucleoside; note (original language) = 2'-氟核苷
  modified_base 6: mod_base = OTHER; note = 2'-fluoro nucleoside; note (original language) = 2'-氟核苷
  modified_base 9: mod_base = OTHER; note = 2'-fluoro nucleoside; note (original language) = 2'-氟核苷
  modified_base 14: mod_base = OTHER; note = 2'-fluoro nucleoside; note (original language) = 2'-氟核苷
  modified_base 16: mod_base = OTHER; note = 2'-fluoro nucleoside; note (original language) = 2'-氟核苷
  modified_base 1..3: mod_base = OTHER; note = phosphorothioate bond; note (original language) = 硫代磷酸酯键
  modified_base 21..23: mod_base = OTHER; note = phosphorothioate bond; note (original language) = 硫代磷酸酯键
  source 1..23: mol_type = other RNA
tctctcatccgcttcaagctcaa

SEQ ID NO: 608 - RNA, 23 nt, synthetic construct
  modified_base 1: mod_base = OTHER; note = 2'-methoxy nucleoside; note (original language) = 2'-甲氧基核苷
  modified_base 3..5: mod_base = OTHER; note = 2'-methoxy nucleoside; note (original language) = 2'-甲氧基核苷
  modified_base 7..8: mod_base = OTHER; note = 2'-methoxy nucleoside; note (original language) = 2'-甲氧基核苷
  modified_base 10..13: mod_base = OTHER; note = 2'-methoxy nucleoside; note (original language) = 2'-甲氧基核苷
  modified_base 15: mod_base = OTHER; note = 2'-methoxy nucleoside; note (original language) = 2'-甲氧基核苷
  modified_base 17..23: mod_base = OTHER; note = 2'-methoxy nucleoside; note (original language) = 2'-甲氧基核苷
  modified_base 2: mod_base = OTHER; note = 2'-fluoro nucleoside; note (original language) = 2'-氟核苷
  modified_base 6: mod_base = OTHER; note = 2'-fluoro nucleoside; note (original language) = 2'-氟核苷
  modified_base 9: mod_base = OTHER; note = 2'-fluoro nucleoside; note (original language) = 2'-氟核苷
  modified_base 14: mod_base = OTHER; note = 2'-fluoro nucleoside; note (original language) = 2'-氟核苷
  modified_base 16: mod_base = OTHER; note = 2'-fluoro nucleoside; note (original language) = 2'-氟核苷
  modified_base 1..3: mod_base = OTHER; note = phosphorothioate bond; note (original language) = 硫代磷酸酯键
  modified_base 21..23: mod_base = OTHER; note = phosphorothioate bond; note (original language) = 硫代磷酸酯键
  source 1..23: mol_type = other RNA
agactctgtgggctctctctcat

SEQ ID NO: 609 - RNA, 23 nt, synthetic construct
  modified_base 1: mod_base = OTHER; note = 2'-methoxy nucleoside; note (original language) = 2'-甲氧基核苷
  modified_base 3..5: mod_base = OTHER; note = 2'-methoxy nucleoside; note (original language) = 2'-甲氧基核苷
  modified_base 7..8: mod_base = OTHER; note = 2'-methoxy nucleoside; note (original language) = 2'-甲氧基核苷
  modified_base 10..13: mod_base = OTHER; note = 2'-methoxy nucleoside; note (original language) = 2'-甲氧基核苷
  modified_base 15: mod_base = OTHER; note = 2'-methoxy nucleoside; note (original language) = 2'-甲氧基核苷
  modified_base 17..23: mod_base = OTHER; note = 2'-methoxy nucleoside; note (original language) = 2'-甲氧基核苷
  modified_base 2: mod_base = OTHER; note = 2'-fluoro nucleoside; note (original language) = 2'-氟核苷
  modified_base 6: mod_base = OTHER; note = 2'-fluoro nucleoside; note (original language) = 2'-氟核苷
  modified_base 9: mod_base = OTHER; note = 2'-fluoro nucleoside; note (original language) = 2'-氟核苷
  modified_base 14: mod_base = OTHER; note = 2'-fluoro nucleoside; note (original language) = 2'-氟核苷
  modified_base 16: mod_base = OTHER; note = 2'-fluoro nucleoside; note (original language) = 2'-氟核苷
  modified_base 1..3: mod_base = OTHER; note = phosphorothioate bond; note (original language) = 硫代磷酸酯键
  modified_base 21..23: mod_base = OTHER; note = phosphorothioate bond; note (original language) = 硫代磷酸酯键
  source 1..23: mol_type = other RNA
aagaaaaggtgggagactggggg

SEQ ID NO: 610 - RNA, 23 nt, synthetic construct
  modified_base 1: mod_base = OTHER; note = 2'-methoxy nucleoside; note (original language) = 2'-甲氧基核苷
  modified_base 3..5: mod_base = OTHER; note = 2'-methoxy nucleoside; note (original language) = 2'-甲氧基核苷
  modified_base 7..8: mod_base = OTHER; note = 2'-methoxy nucleoside; note (original language) = 2'-甲氧基核苷
  modified_base 10..13: mod_base = OTHER; note = 2'-methoxy nucleoside; note (original language) = 2'-甲氧基核苷
  modified_base 15: mod_base = OTHER; note = 2'-methoxy nucleoside; note (original language) = 2'-甲氧基核苷
  modified_base 17..23: mod_base = OTHER; note = 2'-methoxy nucleoside; note (original language) = 2'-甲氧基核苷
  modified_base 2: mod_base = OTHER; note = 2'-fluoro nucleoside; note (original language) = 2'-氟核苷
  modified_base 6: mod_base = OTHER; note = 2'-fluoro nucleoside; note (original language) = 2'-氟核苷
  modified_base 9: mod_base = OTHER; note = 2'-fluoro nucleoside; note (original language) = 2'-氟核苷
  modified_base 14: mod_base = OTHER; note = 2'-fluoro nucleoside; note (original language) = 2'-氟核苷
  modified_base 16: mod_base = OTHER; note = 2'-fluoro nucleoside; note (original language) = 2'-氟核苷
  modified_base 1..3: mod_base = OTHER; note = phosphorothioate bond; note (original language) = 硫代磷酸酯键
  modified_base 21..23: mod_base = OTHER; note = phosphorothioate bond; note (original language) = 硫代磷酸酯键
  source 1..23: mol_type = other RNA
agaagaaaaggtgggagactggg

SEQ ID NO: 611 - RNA, 23 nt, synthetic construct
  modified_base 1: mod_base = OTHER; note = 2'-methoxy nucleoside; note (original language) = 2'-甲氧基核苷
  modified_base 3..5: mod_base = OTHER; note = 2'-methoxy nucleoside; note (original language) = 2'-甲氧基核苷
  modified_base 7..8: mod_base = OTHER; note = 2'-methoxy nucleoside; note (original language) = 2'-甲氧基核苷
  modified_base 10..13: mod_base = OTHER; note = 2'-methoxy nucleoside; note (original language) = 2'-甲氧基核苷
  modified_base 15: mod_base = OTHER; note = 2'-methoxy nucleoside; note (original language) = 2'-甲氧基核苷
  modified_base 17..23: mod_base = OTHER; note = 2'-methoxy nucleoside; note (original language) = 2'-甲氧基核苷
  modified_base 2: mod_base = OTHER; note = 2'-fluoro nucleoside; note (original language) = 2'-氟核苷
  modified_base 6: mod_base = OTHER; note = 2'-fluoro nucleoside; note (original language) = 2'-氟核苷
  modified_base 9: mod_base = OTHER; note = 2'-fluoro nucleoside; note (original language) = 2'-氟核苷
  modified_base 14: mod_base = OTHER; note = 2'-fluoro nucleoside; note (original language) = 2'-氟核苷
  modified_base 16: mod_base = OTHER; note = 2'-fluoro nucleoside; note (original language) = 2'-氟核苷
  modified_base 1..3: mod_base = OTHER; note = phosphorothioate bond; note (original language) = 硫代磷酸酯键
  modified_base 21..23: mod_base = OTHER; note = phosphorothioate bond; note (original language) = 硫代磷酸酯键
  source 1..23: mol_type = other RNA
tcgactcattagaagaaaaggtg

SEQ ID NO: 612 - RNA, 23 nt, synthetic construct
  modified_base 1: mod_base = OTHER; note = 2'-methoxy nucleoside; note (original language) = 2'-甲氧基核苷
  modified_base 3..5: mod_base = OTHER; note = 2'-methoxy nucleoside; note (original language) = 2'-甲氧基核苷
  modified_base 7..8: mod_base = OTHER; note = 2'-methoxy nucleoside; note (original language) = 2'-甲氧基核苷
  modified_base 10..13: mod_base = OTHER; note = 2'-methoxy nucleoside; note (original language) = 2'-甲氧基核苷
  modified_base 15: mod_base = OTHER; note = 2'-methoxy nucleoside; note (original language) = 2'-甲氧基核苷
  modified_base 17..23: mod_base = OTHER; note = 2'-methoxy nucleoside; note (original language) = 2'-甲氧基核苷
  modified_base 2: mod_base = OTHER; note = 2'-fluoro nucleoside; note (original language) = 2'-氟核苷
  modified_base 6: mod_base = OTHER; note = 2'-fluoro nucleoside; note (original language) = 2'-氟核苷
  modified_base 9: mod_base = OTHER; note = 2'-fluoro nucleoside; note (original language) = 2'-氟核苷
  modified_base 14: mod_base = OTHER; note = 2'-fluoro nucleoside; note (original language) = 2'-氟核苷
  modified_base 16: mod_base = OTHER; note = 2'-fluoro nucleoside; note (original language) = 2'-氟核苷
  modified_base 1..3: mod_base = OTHER; note = phosphorothioate bond; note (original language) = 硫代磷酸酯键
  modified_base 21..23: mod_base = OTHER; note = phosphorothioate bond; note (original language) = 硫代磷酸酯键
  source 1..23: mol_type = other RNA
ttagaccaaggagaaacggctgc

SEQ ID NO: 613 - RNA, 23 nt, synthetic construct
  modified_base 1: mod_base = OTHER; note = 2'-methoxy nucleoside; note (original language) = 2'-甲氧基核苷
  modified_base 3..5: mod_base = OTHER; note = 2'-methoxy nucleoside; note (original language) = 2'-甲氧基核苷
  modified_base 7..8: mod_base = OTHER; note = 2'-methoxy nucleoside; note (original language) = 2'-甲氧基核苷
  modified_base 10..13: mod_base = OTHER; note = 2'-methoxy nucleoside; note (original language) = 2'-甲氧基核苷
  modified_base 15: mod_base = OTHER; note = 2'-methoxy nucleoside; note (original language) = 2'-甲氧基核苷
  modified_base 17..23: mod_base = OTHER; note = 2'-methoxy nucleoside; note (original language) = 2'-甲氧基核苷
  modified_base 2: mod_base = OTHER; note = 2'-fluoro nucleoside; note (original language) = 2'-氟核苷
  modified_base 6: mod_base = OTHER; note = 2'-fluoro nucleoside; note (original language) = 2'-氟核苷
  modified_base 9: mod_base = OTHER; note = 2'-fluoro nucleoside; note (original language) = 2'-氟核苷
  modified_base 14: mod_base = OTHER; note = 2'-fluoro nucleoside; note (original language) = 2'-氟核苷
  modified_base 16: mod_base = OTHER; note = 2'-fluoro nucleoside; note (original language) = 2'-氟核苷
  modified_base 1..3: mod_base = OTHER; note = phosphorothioate bond; note (original language) = 硫代磷酸酯键
  modified_base 21..23: mod_base = OTHER; note = phosphorothioate bond; note (original language) = 硫代磷酸酯键
  source 1..23: mol_type = other RNA
tttagaccaaggagaaacggctg

SEQ ID NO: 614 - RNA, 23 nt, synthetic construct
  modified_base 1: mod_base = OTHER; note = 2'-methoxy nucleoside; note (original language) = 2'-甲氧基核苷
  modified_base 3..5: mod_base = OTHER; note = 2'-methoxy nucleoside; note (original language) = 2'-甲氧基核苷
  modified_base 7..8: mod_base = OTHER; note = 2'-methoxy nucleoside; note (original language) = 2'-甲氧基核苷
  modified_base 10..13: mod_base = OTHER; note = 2'-methoxy nucleoside; note (original language) = 2'-甲氧基核苷
  modified_base 15: mod_base = OTHER; note = 2'-methoxy nucleoside; note (original language) = 2'-甲氧基核苷
  modified_base 17..23: mod_base = OTHER; note = 2'-methoxy nucleoside; note (original language) = 2'-甲氧基核苷
  modified_base 2: mod_base = OTHER; note = 2'-fluoro nucleoside; note (original language) = 2'-氟核苷
  modified_base 6: mod_base = OTHER; note = 2'-fluoro nucleoside; note (original language) = 2'-氟核苷
  modified_base 9: mod_base = OTHER; note = 2'-fluoro nucleoside; note (original language) = 2'-氟核苷
  modified_base 14: mod_base = OTHER; note = 2'-fluoro nucleoside; note (original language) = 2'-氟核苷
  modified_base 16: mod_base = OTHER; note = 2'-fluoro nucleoside; note (original language) = 2'-氟核苷
  modified_base 1..3: mod_base = OTHER; note = phosphorothioate bond; note (original language) = 硫代磷酸酯键
  modified_base 21..23: mod_base = OTHER; note = phosphorothioate bond; note (original language) = 硫代磷酸酯键
  source 1..23: mol_type = other RNA
tcaggtactctcattgtggacga

SEQ ID NO: 615 - RNA, 23 nt, synthetic construct
  modified_base 1: mod_base = OTHER; note = 2'-methoxy nucleoside; note (original language) = 2'-甲氧基核苷
  modified_base 3..5: mod_base = OTHER; note = 2'-methoxy nucleoside; note (original language) = 2'-甲氧基核苷
  modified_base 7..8: mod_base = OTHER; note = 2'-methoxy nucleoside; note (original language) = 2'-甲氧基核苷
  modified_base 10..13: mod_base = OTHER; note = 2'-methoxy nucleoside; note (original language) = 2'-甲氧基核苷
  modified_base 15: mod_base = OTHER; note = 2'-methoxy nucleoside; note (original language) = 2'-甲氧基核苷
  modified_base 17..23: mod_base = OTHER; note = 2'-methoxy nucleoside; note (original language) = 2'-甲氧基核苷
  modified_base 2: mod_base = OTHER; note = 2'-fluoro nucleoside; note (original language) = 2'-氟核苷
  modified_base 6: mod_base = OTHER; note = 2'-fluoro nucleoside; note (original language) = 2'-氟核苷
  modified_base 9: mod_base = OTHER; note = 2'-fluoro nucleoside; note (original language) = 2'-氟核苷
  modified_base 14: mod_base = OTHER; note = 2'-fluoro nucleoside; note (original language) = 2'-氟核苷
  modified_base 16: mod_base = OTHER; note = 2'-fluoro nucleoside; note (original language) = 2'-氟核苷
  modified_base 1..3: mod_base = OTHER; note = phosphorothioate bond; note (original language) = 硫代磷酸酯键
  modified_base 21..23: mod_base = OTHER; note = phosphorothioate bond; note (original language) = 硫代磷酸酯键
  source 1..23: mol_type = other RNA
tatgaacctgtcaatcttctcag

SEQ ID NO: 616 - RNA, 23 nt, synthetic construct
  modified_base 1: mod_base = OTHER; note = 2'-methoxy nucleoside; note (original language) = 2'-甲氧基核苷
  modified_base 3..5: mod_base = OTHER; note = 2'-methoxy nucleoside; note (original language) = 2'-甲氧基核苷
  modified_base 7..8: mod_base = OTHER; note = 2'-methoxy nucleoside; note (original language) = 2'-甲氧基核苷
  modified_base 10..13: mod_base = OTHER; note = 2'-methoxy nucleoside; note (original language) = 2'-甲氧基核苷
  modified_base 15: mod_base = OTHER; note = 2'-methoxy nucleoside; note (original language) = 2'-甲氧基核苷
  modified_base 17..23: mod_base = OTHER; note = 2'-methoxy nucleoside; note (original language) = 2'-甲氧基核苷
  modified_base 2: mod_base = OTHER; note = 2'-fluoro nucleoside; note (original language) = 2'-氟核苷
  modified_base 6: mod_base = OTHER; note = 2'-fluoro nucleoside; note (original language) = 2'-氟核苷
  modified_base 9: mod_base = OTHER; note = 2'-fluoro nucleoside; note (original language) = 2'-氟核苷
  modified_base 14: mod_base = OTHER; note = 2'-fluoro nucleoside; note (original language) = 2'-氟核苷
  modified_base 16: mod_base = OTHER; note = 2'-fluoro nucleoside; note (original language) = 2'-氟核苷
  modified_base 1..3: mod_base = OTHER; note = phosphorothioate bond; note (original language) = 硫代磷酸酯键
  modified_base 21..23: mod_base = OTHER; note = phosphorothioate bond; note (original language) = 硫代磷酸酯键
  source 1..23: mol_type = other RNA
tctgtagtacccagaacaacggc

SEQ ID NO: 617 - RNA, 23 nt, synthetic construct
  modified_base 1: mod_base = OTHER; note = 2'-methoxy nucleoside; note (original language) = 2'-甲氧基核苷
  modified_base 3..5: mod_base = OTHER; note = 2'-methoxy nucleoside; note (original language) = 2'-甲氧基核苷
  modified_base 7..8: mod_base = OTHER; note = 2'-methoxy nucleoside; note (original language) = 2'-甲氧基核苷
  modified_base 10..13: mod_base = OTHER; note = 2'-methoxy nucleoside; note (original language) = 2'-甲氧基核苷
  modified_base 15: mod_base = OTHER; note = 2'-methoxy nucleoside; note (original language) = 2'-甲氧基核苷
  modified_base 17..23: mod_base = OTHER; note = 2'-methoxy nucleoside; note (original language) = 2'-甲氧基核苷
  modified_base 2: mod_base = OTHER; note = 2'-fluoro nucleoside; note (original language) = 2'-氟核苷
  modified_base 6: mod_base = OTHER; note = 2'-fluoro nucleoside; note (original language) = 2'-氟核苷
  modified_base 9: mod_base = OTHER; note = 2'-fluoro nucleoside; note (original language) = 2'-氟核苷
  modified_base 14: mod_base = OTHER; note = 2'-fluoro nucleoside; note (original language) = 2'-氟核苷
  modified_base 16: mod_base = OTHER; note = 2'-fluoro nucleoside; note (original language) = 2'-氟核苷
  modified_base 1..3: mod_base = OTHER; note = phosphorothioate bond; note (original language) = 硫代磷酸酯键
  modified_base 21..23: mod_base = OTHER; note = phosphorothioate bond; note (original language) = 硫代磷酸酯键
  source 1..23: mol_type = other RNA
tattgtggatgacgaggtggcag

SEQ ID NO: 618 - RNA, 23 nt, synthetic construct
  modified_base 1: mod_base = OTHER; note = 2'-methoxy nucleoside; note (original language) = 2'-甲氧基核苷
  modified_base 3..5: mod_base = OTHER; note = 2'-methoxy nucleoside; note (original language) = 2'-甲氧基核苷
  modified_base 7..8: mod_base = OTHER; note = 2'-methoxy nucleoside; note (original language) = 2'-甲氧基核苷
  modified_base 10..13: mod_base = OTHER; note = 2'-methoxy nucleoside; note (original language) = 2'-甲氧基核苷
  modified_base 15: mod_base = OTHER; note = 2'-methoxy nucleoside; note (original language) = 2'-甲氧基核苷
  modified_base 17..23: mod_base = OTHER; note = 2'-methoxy nucleoside; note (original language) = 2'-甲氧基核苷
  modified_base 2: mod_base = OTHER; note = 2'-fluoro nucleoside; note (original language) = 2'-氟核苷
  modified_base 6: mod_base = OTHER; note = 2'-fluoro nucleoside; note (original language) = 2'-氟核苷
  modified_base 9: mod_base = OTHER; note = 2'-fluoro nucleoside; note (original language) = 2'-氟核苷
  modified_base 14: mod_base = OTHER; note = 2'-fluoro nucleoside; note (original language) = 2'-氟核苷
  modified_base 16: mod_base = OTHER; note = 2'-fluoro nucleoside; note (original language) = 2'-氟核苷
  modified_base 1..3: mod_base = OTHER; note = phosphorothioate bond; note (original language) = 硫代磷酸酯键
  modified_base 21..23: mod_base = OTHER; note = phosphorothioate bond; note (original language) = 硫代磷酸酯键
  source 1..23: mol_type = other RNA
ttcattgtggatgacgaggtgga

SEQ ID NO: 619 - RNA, 23 nt, synthetic construct
  modified_base 1: mod_base = OTHER; note = 2'-methoxy nucleoside; note (original language) = 2'-甲氧基核苷
  modified_base 3..5: mod_base = OTHER; note = 2'-methoxy nucleoside; note (original language) = 2'-甲氧基核苷
  modified_base 7..8: mod_base = OTHER; note = 2'-methoxy nucleoside; note (original language) = 2'-甲氧基核苷
  modified_base 10..13: mod_base = OTHER; note = 2'-methoxy nucleoside; note (original language) = 2'-甲氧基核苷
  modified_base 15: mod_base = OTHER; note = 2'-methoxy nucleoside; note (original language) = 2'-甲氧基核苷
  modified_base 17..23: mod_base = OTHER; note = 2'-methoxy nucleoside; note (original language) = 2'-甲氧基核苷
  modified_base 2: mod_base = OTHER; note = 2'-fluoro nucleoside; note (original language) = 2'-氟核苷
  modified_base 6: mod_base = OTHER; note = 2'-fluoro nucleoside; note (original language) = 2'-氟核苷
  modified_base 9: mod_base = OTHER; note = 2'-fluoro nucleoside; note (original language) = 2'-氟核苷
  modified_base 14: mod_base = OTHER; note = 2'-fluoro nucleoside; note (original language) = 2'-氟核苷
  modified_base 16: mod_base = OTHER; note = 2'-fluoro nucleoside; note (original language) = 2'-氟核苷
  modified_base 1..3: mod_base = OTHER; note = phosphorothioate bond; note (original language) = 硫代磷酸酯键
  modified_base 21..23: mod_base = OTHER; note = phosphorothioate bond; note (original language) = 硫代磷酸酯键
  source 1..23: mol_type = other RNA
tacaggtactctcattgtggatg

SEQ ID NO: 620 - RNA, 23 nt, synthetic construct
  modified_base 1: mod_base = OTHER; note = 2'-methoxy nucleoside; note (original language) = 2'-甲氧基核苷
  modified_base 3..5: mod_base = OTHER; note = 2'-methoxy nucleoside; note (original language) = 2'-甲氧基核苷
  modified_base 7..8: mod_base = OTHER; note = 2'-methoxy nucleoside; note (original language) = 2'-甲氧基核苷
  modified_base 10..13: mod_base = OTHER; note = 2'-methoxy nucleoside; note (original language) = 2'-甲氧基核苷
  modified_base 15: mod_base = OTHER; note = 2'-methoxy nucleoside; note (original language) = 2'-甲氧基核苷
  modified_base 17..23: mod_base = OTHER; note = 2'-methoxy nucleoside; note (original language) = 2'-甲氧基核苷
  modified_base 2: mod_base = OTHER; note = 2'-fluoro nucleoside; note (original language) = 2'-氟核苷
  modified_base 6: mod_base = OTHER; note = 2'-fluoro nucleoside; note (original language) = 2'-氟核苷
  modified_base 9: mod_base = OTHER; note = 2'-fluoro nucleoside; note (original language) = 2'-氟核苷
  modified_base 14: mod_base = OTHER; note = 2'-fluoro nucleoside; note (original language) = 2'-氟核苷
  modified_base 16: mod_base = OTHER; note = 2'-fluoro nucleoside; note (original language) = 2'-氟核苷
  modified_base 1..3: mod_base = OTHER; note = phosphorothioate bond; note (original language) = 硫代磷酸酯键
  modified_base 21..23: mod_base = OTHER; note = phosphorothioate bond; note (original language) = 硫代磷酸酯键
  source 1..23: mol_type = other RNA
tccgcttcaagctcaaaaaacat

SEQ ID NO: 621 - RNA, 23 nt, synthetic construct
  modified_base 1: mod_base = OTHER; note = 2'-methoxy nucleoside; note (original language) = 2'-甲氧基核苷
  modified_base 3..5: mod_base = OTHER; note = 2'-methoxy nucleoside; note (original language) = 2'-甲氧基核苷
  modified_base 7..8: mod_base = OTHER; note = 2'-methoxy nucleoside; note (original language) = 2'-甲氧基核苷
  modified_base 10..13: mod_base = OTHER; note = 2'-methoxy nucleoside; note (original language) = 2'-甲氧基核苷
  modified_base 15: mod_base = OTHER; note = 2'-methoxy nucleoside; note (original language) = 2'-甲氧基核苷
  modified_base 17..23: mod_base = OTHER; note = 2'-methoxy nucleoside; note (original language) = 2'-甲氧基核苷
  modified_base 2: mod_base = OTHER; note = 2'-fluoro nucleoside; note (original language) = 2'-氟核苷
  modified_base 6: mod_base = OTHER; note = 2'-fluoro nucleoside; note (original language) = 2'-氟核苷
  modified_base 9: mod_base = OTHER; note = 2'-fluoro nucleoside; note (original language) = 2'-氟核苷
  modified_base 14: mod_base = OTHER; note = 2'-fluoro nucleoside; note (original language) = 2'-氟核苷
  modified_base 16: mod_base = OTHER; note = 2'-fluoro nucleoside; note (original language) = 2'-氟核苷
  modified_base 1..3: mod_base = OTHER; note = phosphorothioate bond; note (original language) = 硫代磷酸酯键
  modified_base 21..23: mod_base = OTHER; note = phosphorothioate bond; note (original language) = 硫代磷酸酯键
  source 1..23: mol_type = other RNA
tatccgcttcaagctcaaaacaa

SEQ ID NO: 622 - RNA, 23 nt, synthetic construct
  modified_base 1: mod_base = OTHER; note = 2'-methoxy nucleoside; note (original language) = 2'-甲氧基核苷
  modified_base 3..5: mod_base = OTHER; note = 2'-methoxy nucleoside; note (original language) = 2'-甲氧基核苷
  modified_base 7..8: mod_base = OTHER; note = 2'-methoxy nucleoside; note (original language) = 2'-甲氧基核苷
  modified_base 10..13: mod_base = OTHER; note = 2'-methoxy nucleoside; note (original language) = 2'-甲氧基核苷
  modified_base 15: mod_base = OTHER; note = 2'-methoxy nucleoside; note (original language) = 2'-甲氧基核苷
  modified_base 17..23: mod_base = OTHER; note = 2'-methoxy nucleoside; note (original language) = 2'-甲氧基核苷
  modified_base 2: mod_base = OTHER; note = 2'-fluoro nucleoside; note (original language) = 2'-氟核苷
  modified_base 6: mod_base = OTHER; note = 2'-fluoro nucleoside; note (original language) = 2'-氟核苷
  modified_base 9: mod_base = OTHER; note = 2'-fluoro nucleoside; note (original language) = 2'-氟核苷
  modified_base 14: mod_base = OTHER; note = 2'-fluoro nucleoside; note (original language) = 2'-氟核苷
  modified_base 16: mod_base = OTHER; note = 2'-fluoro nucleoside; note (original language) = 2'-氟核苷
  modified_base 1..3: mod_base = OTHER; note = phosphorothioate bond; note (original language) = 硫代磷酸酯键
  modified_base 21..23: mod_base = OTHER; note = phosphorothioate bond; note (original language) = 硫代磷酸酯键
  source 1..23: mol_type = other RNA
tcatccgcttcaagctcaaacaa

SEQ ID NO: 623 - RNA, 23 nt, synthetic construct
  modified_base 1: mod_base = OTHER; note = 2'-methoxy nucleoside; note (original language) = 2'-甲氧基核苷
  modified_base 3..5: mod_base = OTHER; note = 2'-methoxy nucleoside; note (original language) = 2'-甲氧基核苷
  modified_base 7..8: mod_base = OTHER; note = 2'-methoxy nucleoside; note (original language) = 2'-甲氧基核苷
  modified_base 10..13: mod_base = OTHER; note = 2'-methoxy nucleoside; note (original language) = 2'-甲氧基核苷
  modified_base 15: mod_base = OTHER; note = 2'-methoxy nucleoside; note (original language) = 2'-甲氧基核苷
  modified_base 17..23: mod_base = OTHER; note = 2'-methoxy nucleoside; note (original language) = 2'-甲氧基核苷
  modified_base 2: mod_base = OTHER; note = 2'-fluoro nucleoside; note (original language) = 2'-氟核苷
  modified_base 6: mod_base = OTHER; note = 2'-fluoro nucleoside; note (original language) = 2'-氟核苷
  modified_base 9: mod_base = OTHER; note = 2'-fluoro nucleoside; note (original language) = 2'-氟核苷
  modified_base 14: mod_base = OTHER; note = 2'-fluoro nucleoside; note (original language) = 2'-氟核苷
  modified_base 16: mod_base = OTHER; note = 2'-fluoro nucleoside; note (original language) = 2'-氟核苷
  modified_base 1..3: mod_base = OTHER; note = phosphorothioate bond; note (original language) = 硫代磷酸酯键
  modified_base 21..23: mod_base = OTHER; note = phosphorothioate bond; note (original language) = 硫代磷酸酯键
  source 1..23: mol_type = other RNA
taagaaaaggtgggagactgggg

SEQ ID NO: 624 - RNA, 23 nt, synthetic construct
  modified_base 1: mod_base = OTHER; note = 2'-methoxy nucleoside; note (original language) = 2'-甲氧基核苷
  modified_base 3..5: mod_base = OTHER; note = 2'-methoxy nucleoside; note (original language) = 2'-甲氧基核苷
  modified_base 7..8: mod_base = OTHER; note = 2'-methoxy nucleoside; note (original language) = 2'-甲氧基核苷
  modified_base 10..13: mod_base = OTHER; note = 2'-methoxy nucleoside; note (original language) = 2'-甲氧基核苷
  modified_base 15: mod_base = OTHER; note = 2'-methoxy nucleoside; note (original language) = 2'-甲氧基核苷
  modified_base 17..23: mod_base = OTHER; note = 2'-methoxy nucleoside; note (original language) = 2'-甲氧基核苷
  modified_base 2: mod_base = OTHER; note = 2'-fluoro nucleoside; note (original language) = 2'-氟核苷
  modified_base 6: mod_base = OTHER; note = 2'-fluoro nucleoside; note (original language) = 2'-氟核苷
  modified_base 9: mod_base = OTHER; note = 2'-fluoro nucleoside; note (original language) = 2'-氟核苷
  modified_base 14: mod_base = OTHER; note = 2'-fluoro nucleoside; note (original language) = 2'-氟核苷
  modified_base 16: mod_base = OTHER; note = 2'-fluoro nucleoside; note (original language) = 2'-氟核苷
  modified_base 1..3: mod_base = OTHER; note = phosphorothioate bond; note (original language) = 硫代磷酸酯键
  modified_base 21..23: mod_base = OTHER; note = phosphorothioate bond; note (original language) = 硫代磷酸酯键
  source 1..23: mol_type = other RNA
agaaaaggtgggagactggggag

SEQ ID NO: 625 - RNA, 23 nt, synthetic construct
  modified_base 1: mod_base = OTHER; note = 2'-methoxy nucleoside; note (original language) = 2'-甲氧基核苷
  modified_base 3..5: mod_base = OTHER; note = 2'-methoxy nucleoside; note (original language) = 2'-甲氧基核苷
  modified_base 7..8: mod_base = OTHER; note = 2'-methoxy nucleoside; note (original language) = 2'-甲氧基核苷
  modified_base 10..13: mod_base = OTHER; note = 2'-methoxy nucleoside; note (original language) = 2'-甲氧基核苷
  modified_base 15: mod_base = OTHER; note = 2'-methoxy nucleoside; note (original language) = 2'-甲氧基核苷
  modified_base 17..23: mod_base = OTHER; note = 2'-methoxy nucleoside; note (original language) = 2'-甲氧基核苷
  modified_base 2: mod_base = OTHER; note = 2'-fluoro nucleoside; note (original language) = 2'-氟核苷
  modified_base 6: mod_base = OTHER; note = 2'-fluoro nucleoside; note (original language) = 2'-氟核苷
  modified_base 9: mod_base = OTHER; note = 2'-fluoro nucleoside; note (original language) = 2'-氟核苷
  modified_base 14: mod_base = OTHER; note = 2'-fluoro nucleoside; note (original language) = 2'-氟核苷
  modified_base 16: mod_base = OTHER; note = 2'-fluoro nucleoside; note (original language) = 2'-氟核苷
  modified_base 1..3: mod_base = OTHER; note = phosphorothioate bond; note (original language) = 硫代磷酸酯键
  modified_base 21..23: mod_base = OTHER; note = phosphorothioate bond; note (original language) = 硫代磷酸酯键
  source 1..23: mol_type = other RNA
tgctttccagctcaaagtcgcct

SEQ ID NO: 626 - RNA, 23 nt, synthetic construct
  modified_base 1: mod_base = OTHER; note = 2'-methoxy nucleoside; note (original language) = 2'-甲氧基核苷
  modified_base 3..5: mod_base = OTHER; note = 2'-methoxy nucleoside; note (original language) = 2'-甲氧基核苷
  modified_base 7..8: mod_base = OTHER; note = 2'-methoxy nucleoside; note (original language) = 2'-甲氧基核苷
  modified_base 10..13: mod_base = OTHER; note = 2'-methoxy nucleoside; note (original language) = 2'-甲氧基核苷
  modified_base 15: mod_base = OTHER; note = 2'-methoxy nucleoside; note (original language) = 2'-甲氧基核苷
  modified_base 17..23: mod_base = OTHER; note = 2'-methoxy nucleoside; note (original language) = 2'-甲氧基核苷
  modified_base 2: mod_base = OTHER; note = 2'-fluoro nucleoside; note (original language) = 2'-氟核苷
  modified_base 6: mod_base = OTHER; note = 2'-fluoro nucleoside; note (original language) = 2'-氟核苷
  modified_base 9: mod_base = OTHER; note = 2'-fluoro nucleoside; note (original language) = 2'-氟核苷
  modified_base 14: mod_base = OTHER; note = 2'-fluoro nucleoside; note (original language) = 2'-氟核苷
  modified_base 16: mod_base = OTHER; note = 2'-fluoro nucleoside; note (original language) = 2'-氟核苷
  modified_base 1..3: mod_base = OTHER; note = phosphorothioate bond; note (original language) = 硫代磷酸酯键
  modified_base 21..23: mod_base = OTHER; note = phosphorothioate bond; note (original language) = 硫代磷酸酯键
  source 1..23: mol_type = other RNA
agaccaaggagaaacggctgctt

SEQ ID NO: 627 - RNA, 23 nt, synthetic construct
  modified_base 1: mod_base = OTHER; note = 2'-methoxy nucleoside; note (original language) = 2'-甲氧基核苷
  modified_base 3..5: mod_base = OTHER; note = 2'-methoxy nucleoside; note (original language) = 2'-甲氧基核苷
  modified_base 7..8: mod_base = OTHER; note = 2'-methoxy nucleoside; note (original language) = 2'-甲氧基核苷
  modified_base 10..13: mod_base = OTHER; note = 2'-methoxy nucleoside; note (original language) = 2'-甲氧基核苷
  modified_base 15: mod_base = OTHER; note = 2'-methoxy nucleoside; note (original language) = 2'-甲氧基核苷
  modified_base 17..23: mod_base = OTHER; note = 2'-methoxy nucleoside; note (original language) = 2'-甲氧基核苷
  modified_base 2: mod_base = OTHER; note = 2'-fluoro nucleoside; note (original language) = 2'-氟核苷
  modified_base 6: mod_base = OTHER; note = 2'-fluoro nucleoside; note (original language) = 2'-氟核苷
  modified_base 9: mod_base = OTHER; note = 2'-fluoro nucleoside; note (original language) = 2'-氟核苷
  modified_base 14: mod_base = OTHER; note = 2'-fluoro nucleoside; note (original language) = 2'-氟核苷
  modified_base 16: mod_base = OTHER; note = 2'-fluoro nucleoside; note (original language) = 2'-氟核苷
  modified_base 1..3: mod_base = OTHER; note = phosphorothioate bond; note (original language) = 硫代磷酸酯键
  modified_base 21..23: mod_base = OTHER; note = phosphorothioate bond; note (original language) = 硫代磷酸酯键
  source 1..23: mol_type = other RNA
acttagaccaaggagaaacggct

SEQ ID NO: 628 - RNA, 23 nt, synthetic construct
  modified_base 1: mod_base = OTHER; note = 2'-methoxy nucleoside; note (original language) = 2'-甲氧基核苷
  modified_base 3..5: mod_base = OTHER; note = 2'-methoxy nucleoside; note (original language) = 2'-甲氧基核苷
  modified_base 7..8: mod_base = OTHER; note = 2'-methoxy nucleoside; note (original language) = 2'-甲氧基核苷
  modified_base 10..13: mod_base = OTHER; note = 2'-methoxy nucleoside; note (original language) = 2'-甲氧基核苷
  modified_base 15: mod_base = OTHER; note = 2'-methoxy nucleoside; note (original language) = 2'-甲氧基核苷
  modified_base 17..23: mod_base = OTHER; note = 2'-methoxy nucleoside; note (original language) = 2'-甲氧基核苷
  modified_base 2: mod_base = OTHER; note = 2'-fluoro nucleoside; note (original language) = 2'-氟核苷
  modified_base 6: mod_base = OTHER; note = 2'-fluoro nucleoside; note (original language) = 2'-氟核苷
  modified_base 9: mod_base = OTHER; note = 2'-fluoro nucleoside; note (original language) = 2'-氟核苷
  modified_base 14: mod_base = OTHER; note = 2'-fluoro nucleoside; note (original language) = 2'-氟核苷
  modified_base 16: mod_base = OTHER; note = 2'-fluoro nucleoside; note (original language) = 2'-氟核苷
  modified_base 1..3: mod_base = OTHER; note = phosphorothioate bond; note (original language) = 硫代磷酸酯键
  modified_base 21..23: mod_base = OTHER; note = phosphorothioate bond; note (original language) = 硫代磷酸酯键
  source 1..23: mol_type = other RNA
acaggtactctcattgtggacga

SEQ ID NO: 629 - RNA, 23 nt, synthetic construct
  modified_base 1: mod_base = OTHER; note = 2'-methoxy nucleoside; note (original language) = 2'-甲氧基核苷
  modified_base 3..5: mod_base = OTHER; note = 2'-methoxy nucleoside; note (original language) = 2'-甲氧基核苷
  modified_base 7..8: mod_base = OTHER; note = 2'-methoxy nucleoside; note (original language) = 2'-甲氧基核苷
  modified_base 10..13: mod_base = OTHER; note = 2'-methoxy nucleoside; note (original language) = 2'-甲氧基核苷
  modified_base 15: mod_base = OTHER; note = 2'-methoxy nucleoside; note (original language) = 2'-甲氧基核苷
  modified_base 17..23: mod_base = OTHER; note = 2'-methoxy nucleoside; note (original language) = 2'-甲氧基核苷
  modified_base 2: mod_base = OTHER; note = 2'-fluoro nucleoside; note (original language) = 2'-氟核苷
  modified_base 6: mod_base = OTHER; note = 2'-fluoro nucleoside; note (original language) = 2'-氟核苷
  modified_base 9: mod_base = OTHER; note = 2'-fluoro nucleoside; note (original language) = 2'-氟核苷
  modified_base 14: mod_base = OTHER; note = 2'-fluoro nucleoside; note (original language) = 2'-氟核苷
  modified_base 16: mod_base = OTHER; note = 2'-fluoro nucleoside; note (original language) = 2'-氟核苷
  modified_base 1..3: mod_base = OTHER; note = phosphorothioate bond; note (original language) = 硫代磷酸酯键
  modified_base 21..23: mod_base = OTHER; note = phosphorothioate bond; note (original language) = 硫代磷酸酯键
  source 1..23: mol_type = other RNA
acaggtactctcattgtggatga

SEQ ID NO: 630 - RNA, 23 nt, synthetic construct
  modified_base 1: mod_base = OTHER; note = 2'-methoxy nucleoside; note (original language) = 2'-甲氧基核苷
  modified_base 3..5: mod_base = OTHER; note = 2'-methoxy nucleoside; note (original language) = 2'-甲氧基核苷
  modified_base 7..8: mod_base = OTHER; note = 2'-methoxy nucleoside; note (original language) = 2'-甲氧基核苷
  modified_base 10..13: mod_base = OTHER; note = 2'-methoxy nucleoside; note (original language) = 2'-甲氧基核苷
  modified_base 15: mod_base = OTHER; note = 2'-methoxy nucleoside; note (original language) = 2'-甲氧基核苷
  modified_base 17..23: mod_base = OTHER; note = 2'-methoxy nucleoside; note (original language) = 2'-甲氧基核苷
  modified_base 2: mod_base = OTHER; note = 2'-fluoro nucleoside; note (original language) = 2'-氟核苷
  modified_base 6: mod_base = OTHER; note = 2'-fluoro nucleoside; note (original language) = 2'-氟核苷
  modified_base 9: mod_base = OTHER; note = 2'-fluoro nucleoside; note (original language) = 2'-氟核苷
  modified_base 14: mod_base = OTHER; note = 2'-fluoro nucleoside; note (original language) = 2'-氟核苷
  modified_base 16: mod_base = OTHER; note = 2'-fluoro nucleoside; note (original language) = 2'-氟核苷
  modified_base 1..3: mod_base = OTHER; note = phosphorothioate bond; note (original language) = 硫代磷酸酯键
  modified_base 21..23: mod_base = OTHER; note = phosphorothioate bond; note (original language) = 硫代磷酸酯键
  source 1..23: mol_type = other RNA
aggtactctcattgtggatgccg

SEQ ID NO: 631 - RNA, 23 nt, synthetic construct
  modified_base 1: mod_base = OTHER; note = 2'-methoxy nucleoside; note (original language) = 2'-甲氧基核苷
  modified_base 3..5: mod_base = OTHER; note = 2'-methoxy nucleoside; note (original language) = 2'-甲氧基核苷
  modified_base 7..8: mod_base = OTHER; note = 2'-methoxy nucleoside; note (original language) = 2'-甲氧基核苷
  modified_base 10..13: mod_base = OTHER; note = 2'-methoxy nucleoside; note (original language) = 2'-甲氧基核苷
  modified_base 15: mod_base = OTHER; note = 2'-methoxy nucleoside; note (original language) = 2'-甲氧基核苷
  modified_base 17..23: mod_base = OTHER; note = 2'-methoxy nucleoside; note (original language) = 2'-甲氧基核苷
  modified_base 2: mod_base = OTHER; note = 2'-fluoro nucleoside; note (original language) = 2'-氟核苷
  modified_base 6: mod_base = OTHER; note = 2'-fluoro nucleoside; note (original language) = 2'-氟核苷
  modified_base 9: mod_base = OTHER; note = 2'-fluoro nucleoside; note (original language) = 2'-氟核苷
  modified_base 14: mod_base = OTHER; note = 2'-fluoro nucleoside; note (original language) = 2'-氟核苷
  modified_base 16: mod_base = OTHER; note = 2'-fluoro nucleoside; note (original language) = 2'-氟核苷
  modified_base 1..3: mod_base = OTHER; note = phosphorothioate bond; note (original language) = 硫代磷酸酯键
  modified_base 21..23: mod_base = OTHER; note = phosphorothioate bond; note (original language) = 硫代磷酸酯键
  source 1..23: mol_type = other RNA
tagaaaaggtgggagactggggg

SEQ ID NO: 632 - RNA, 23 nt, synthetic construct
  modified_base 1: mod_base = OTHER; note = 2'-methoxy nucleoside; note (original language) = 2'-甲氧基核苷
  modified_base 3..5: mod_base = OTHER; note = 2'-methoxy nucleoside; note (original language) = 2'-甲氧基核苷
  modified_base 7..8: mod_base = OTHER; note = 2'-methoxy nucleoside; note (original language) = 2'-甲氧基核苷
  modified_base 10..13: mod_base = OTHER; note = 2'-methoxy nucleoside; note (original language) = 2'-甲氧基核苷
  modified_base 15: mod_base = OTHER; note = 2'-methoxy nucleoside; note (original language) = 2'-甲氧基核苷
  modified_base 17..23: mod_base = OTHER; note = 2'-methoxy nucleoside; note (original language) = 2'-甲氧基核苷
  modified_base 2: mod_base = OTHER; note = 2'-fluoro nucleoside; note (original language) = 2'-氟核苷
  modified_base 6: mod_base = OTHER; note = 2'-fluoro nucleoside; note (original language) = 2'-氟核苷
  modified_base 9: mod_base = OTHER; note = 2'-fluoro nucleoside; note (original language) = 2'-氟核苷
  modified_base 14: mod_base = OTHER; note = 2'-fluoro nucleoside; note (original language) = 2'-氟核苷
  modified_base 16: mod_base = OTHER; note = 2'-fluoro nucleoside; note (original language) = 2'-氟核苷
  modified_base 1..3: mod_base = OTHER; note = phosphorothioate bond; note (original language) = 硫代磷酸酯键
  modified_base 21..23: mod_base = OTHER; note = phosphorothioate bond; note (original language) = 硫代磷酸酯键
  source 1..23: mol_type = other RNA
tgaagaaaaggtgggagactggg

SEQ ID NO: 633 - RNA, 23 nt, synthetic construct
  modified_base 1: mod_base = OTHER; note = 2'-methoxy nucleoside; note (original language) = 2'-甲氧基核苷
  modified_base 3..5: mod_base = OTHER; note = 2'-methoxy nucleoside; note (original language) = 2'-甲氧基核苷
  modified_base 7..8: mod_base = OTHER; note = 2'-methoxy nucleoside; note (original language) = 2'-甲氧基核苷
  modified_base 10..13: mod_base = OTHER; note = 2'-methoxy nucleoside; note (original language) = 2'-甲氧基核苷
  modified_base 15: mod_base = OTHER; note = 2'-methoxy nucleoside; note (original language) = 2'-甲氧基核苷
  modified_base 17..23: mod_base = OTHER; note = 2'-methoxy nucleoside; note (original language) = 2'-甲氧基核苷
  modified_base 2: mod_base = OTHER; note = 2'-fluoro nucleoside; note (original language) = 2'-氟核苷
  modified_base 6: mod_base = OTHER; note = 2'-fluoro nucleoside; note (original language) = 2'-氟核苷
  modified_base 9: mod_base = OTHER; note = 2'-fluoro nucleoside; note (original language) = 2'-氟核苷
  modified_base 14: mod_base = OTHER; note = 2'-fluoro nucleoside; note (original language) = 2'-氟核苷
  modified_base 16: mod_base = OTHER; note = 2'-fluoro nucleoside; note (original language) = 2'-氟核苷
  modified_base 1..3: mod_base = OTHER; note = phosphorothioate bond; note (original language) = 硫代磷酸酯键
  modified_base 21..23: mod_base = OTHER; note = phosphorothioate bond; note (original language) = 硫代磷酸酯键
  source 1..23: mol_type = other RNA
tagaagaaaaggtgggagaccgg

SEQ ID NO: 634 - RNA, 23 nt, synthetic construct
  modified_base 1: mod_base = OTHER; note = 2'-methoxy nucleoside; note (original language) = 2'-甲氧基核苷
  modified_base 3..5: mod_base = OTHER; note = 2'-methoxy nucleoside; note (original language) = 2'-甲氧基核苷
  modified_base 7..8: mod_base = OTHER; note = 2'-methoxy nucleoside; note (original language) = 2'-甲氧基核苷
  modified_base 10..13: mod_base = OTHER; note = 2'-methoxy nucleoside; note (original language) = 2'-甲氧基核苷
  modified_base 15: mod_base = OTHER; note = 2'-methoxy nucleoside; note (original language) = 2'-甲氧基核苷
  modified_base 17..23: mod_base = OTHER; note = 2'-methoxy nucleoside; note (original language) = 2'-甲氧基核苷
  modified_base 2: mod_base = OTHER; note = 2'-fluoro nucleoside; note (original language) = 2'-氟核苷
  modified_base 6: mod_base = OTHER; note = 2'-fluoro nucleoside; note (original language) = 2'-氟核苷
  modified_base 9: mod_base = OTHER; note = 2'-fluoro nucleoside; note (original language) = 2'-氟核苷
  modified_base 14: mod_base = OTHER; note = 2'-fluoro nucleoside; note (original language) = 2'-氟核苷
  modified_base 16: mod_base = OTHER; note = 2'-fluoro nucleoside; note (original language) = 2'-氟核苷
  modified_base 1..3: mod_base = OTHER; note = phosphorothioate bond; note (original language) = 硫代磷酸酯键
  modified_base 21..23: mod_base = OTHER; note = phosphorothioate bond; note (original language) = 硫代磷酸酯键
  source 1..23: mol_type = other RNA
ttagaagaaaaggtgggagactg

SEQ ID NO: 635 - RNA, 23 nt, synthetic construct
  modified_base 1: mod_base = OTHER; note = 2'-methoxy nucleoside; note (original language) = 2'-甲氧基核苷
  modified_base 3..5: mod_base = OTHER; note = 2'-methoxy nucleoside; note (original language) = 2'-甲氧基核苷
  modified_base 7..8: mod_base = OTHER; note = 2'-methoxy nucleoside; note (original language) = 2'-甲氧基核苷
  modified_base 10..13: mod_base = OTHER; note = 2'-methoxy nucleoside; note (original language) = 2'-甲氧基核苷
  modified_base 15: mod_base = OTHER; note = 2'-methoxy nucleoside; note (original language) = 2'-甲氧基核苷
  modified_base 17..23: mod_base = OTHER; note = 2'-methoxy nucleoside; note (original language) = 2'-甲氧基核苷
  modified_base 2: mod_base = OTHER; note = 2'-fluoro nucleoside; note (original language) = 2'-氟核苷
  modified_base 6: mod_base = OTHER; note = 2'-fluoro nucleoside; note (original language) = 2'-氟核苷
  modified_base 9: mod_base = OTHER; note = 2'-fluoro nucleoside; note (original language) = 2'-氟核苷
  modified_base 14: mod_base = OTHER; note = 2'-fluoro nucleoside; note (original language) = 2'-氟核苷
  modified_base 16: mod_base = OTHER; note = 2'-fluoro nucleoside; note (original language) = 2'-氟核苷
  modified_base 1..3: mod_base = OTHER; note = phosphorothioate bond; note (original language) = 硫代磷酸酯键
  modified_base 21..23: mod_base = OTHER; note = phosphorothioate bond; note (original language) = 硫代磷酸酯键
  source 1..23: mol_type = other RNA
tagaccaaggagaaacggctgct

SEQ ID NO: 636 - RNA, 23 nt, synthetic construct
  modified_base 1: mod_base = OTHER; note = 2'-methoxy nucleoside; note (original language) = 2'-甲氧基核苷
  modified_base 3..5: mod_base = OTHER; note = 2'-methoxy nucleoside; note (original language) = 2'-甲氧基核苷
  modified_base 7..8: mod_base = OTHER; note = 2'-methoxy nucleoside; note (original language) = 2'-甲氧基核苷
  modified_base 10..13: mod_base = OTHER; note = 2'-methoxy nucleoside; note (original language) = 2'-甲氧基核苷
  modified_base 15: mod_base = OTHER; note = 2'-methoxy nucleoside; note (original language) = 2'-甲氧基核苷
  modified_base 17..23: mod_base = OTHER; note = 2'-methoxy nucleoside; note (original language) = 2'-甲氧基核苷
  modified_base 2: mod_base = OTHER; note = 2'-fluoro nucleoside; note (original language) = 2'-氟核苷
  modified_base 6: mod_base = OTHER; note = 2'-fluoro nucleoside; note (original language) = 2'-氟核苷
  modified_base 9: mod_base = OTHER; note = 2'-fluoro nucleoside; note (original language) = 2'-氟核苷
  modified_base 14: mod_base = OTHER; note = 2'-fluoro nucleoside; note (original language) = 2'-氟核苷
  modified_base 16: mod_base = OTHER; note = 2'-fluoro nucleoside; note (original language) = 2'-氟核苷
  modified_base 1..3: mod_base = OTHER; note = phosphorothioate bond; note (original language) = 硫代磷酸酯键
  modified_base 21..23: mod_base = OTHER; note = phosphorothioate bond; note (original language) = 硫代磷酸酯键
  source 1..23: mol_type = other RNA
ttagaccaaggagaaacggccgc

SEQ ID NO: 637 - RNA, 23 nt, synthetic construct
  modified_base 1: mod_base = OTHER; note = 2'-methoxy nucleoside; note (original language) = 2'-甲氧基核苷
  modified_base 3..5: mod_base = OTHER; note = 2'-methoxy nucleoside; note (original language) = 2'-甲氧基核苷
  modified_base 7..8: mod_base = OTHER; note = 2'-methoxy nucleoside; note (original language) = 2'-甲氧基核苷
  modified_base 10..13: mod_base = OTHER; note = 2'-methoxy nucleoside; note (original language) = 2'-甲氧基核苷
  modified_base 15: mod_base = OTHER; note = 2'-methoxy nucleoside; note (original language) = 2'-甲氧基核苷
  modified_base 17..23: mod_base = OTHER; note = 2'-methoxy nucleoside; note (original language) = 2'-甲氧基核苷
  modified_base 2: mod_base = OTHER; note = 2'-fluoro nucleoside; note (original language) = 2'-氟核苷
  modified_base 6: mod_base = OTHER; note = 2'-fluoro nucleoside; note (original language) = 2'-氟核苷
  modified_base 9: mod_base = OTHER; note = 2'-fluoro nucleoside; note (original language) = 2'-氟核苷
  modified_base 14: mod_base = OTHER; note = 2'-fluoro nucleoside; note (original language) = 2'-氟核苷
  modified_base 16: mod_base = OTHER; note = 2'-fluoro nucleoside; note (original language) = 2'-氟核苷
  modified_base 1..3: mod_base = OTHER; note = phosphorothioate bond; note (original language) = 硫代磷酸酯键
  modified_base 21..23: mod_base = OTHER; note = phosphorothioate bond; note (original language) = 硫代磷酸酯键
  source 1..23: mol_type = other RNA
cttagaccaaggagaaacggctg

SEQ ID NO: 638 - RNA, 23 nt, synthetic construct
  modified_base 1: mod_base = OTHER; note = 2'-methoxy nucleoside; note (original language) = 2'-甲氧基核苷
  modified_base 3..5: mod_base = OTHER; note = 2'-methoxy nucleoside; note (original language) = 2'-甲氧基核苷
  modified_base 7..8: mod_base = OTHER; note = 2'-methoxy nucleoside; note (original language) = 2'-甲氧基核苷
  modified_base 10..13: mod_base = OTHER; note = 2'-methoxy nucleoside; note (original language) = 2'-甲氧基核苷
  modified_base 15: mod_base = OTHER; note = 2'-methoxy nucleoside; note (original language) = 2'-甲氧基核苷
  modified_base 17..23: mod_base = OTHER; note = 2'-methoxy nucleoside; note (original language) = 2'-甲氧基核苷
  modified_base 2: mod_base = OTHER; note = 2'-fluoro nucleoside; note (original language) = 2'-氟核苷
  modified_base 6: mod_base = OTHER; note = 2'-fluoro nucleoside; note (original language) = 2'-氟核苷
  modified_base 9: mod_base = OTHER; note = 2'-fluoro nucleoside; note (original language) = 2'-氟核苷
  modified_base 14: mod_base = OTHER; note = 2'-fluoro nucleoside; note (original language) = 2'-氟核苷
  modified_base 16: mod_base = OTHER; note = 2'-fluoro nucleoside; note (original language) = 2'-氟核苷
  modified_base 1..3: mod_base = OTHER; note = phosphorothioate bond; note (original language) = 硫代磷酸酯键
  modified_base 21..23: mod_base = OTHER; note = phosphorothioate bond; note (original language) = 硫代磷酸酯键
  source 1..23: mol_type = other RNA
cacttagaccaaggagaaacggc

SEQ ID NO: 639 - RNA, 23 nt, synthetic construct
  modified_base 1: mod_base = OTHER; note = 2'-methoxy nucleoside; note (original language) = 2'-甲氧基核苷
  modified_base 3..5: mod_base = OTHER; note = 2'-methoxy nucleoside; note (original language) = 2'-甲氧基核苷
  modified_base 7..8: mod_base = OTHER; note = 2'-methoxy nucleoside; note (original language) = 2'-甲氧基核苷
  modified_base 10..13: mod_base = OTHER; note = 2'-methoxy nucleoside; note (original language) = 2'-甲氧基核苷
  modified_base 15: mod_base = OTHER; note = 2'-methoxy nucleoside; note (original language) = 2'-甲氧基核苷
  modified_base 17..23: mod_base = OTHER; note = 2'-methoxy nucleoside; note (original language) = 2'-甲氧基核苷
  modified_base 2: mod_base = OTHER; note = 2'-fluoro nucleoside; note (original language) = 2'-氟核苷
  modified_base 6: mod_base = OTHER; note = 2'-fluoro nucleoside; note (original language) = 2'-氟核苷
  modified_base 9: mod_base = OTHER; note = 2'-fluoro nucleoside; note (original language) = 2'-氟核苷
  modified_base 14: mod_base = OTHER; note = 2'-fluoro nucleoside; note (original language) = 2'-氟核苷
  modified_base 16: mod_base = OTHER; note = 2'-fluoro nucleoside; note (original language) = 2'-氟核苷
  modified_base 1..3: mod_base = OTHER; note = phosphorothioate bond; note (original language) = 硫代磷酸酯键
  modified_base 21..23: mod_base = OTHER; note = phosphorothioate bond; note (original language) = 硫代磷酸酯键
  source 1..23: mol_type = other RNA
tacttagaccaaggagaaacggc

SEQ ID NO: 640 - RNA, 23 nt, synthetic construct
  modified_base 1: mod_base = OTHER; note = 2'-methoxy nucleoside; note (original language) = 2'-甲氧基核苷
  modified_base 3..5: mod_base = OTHER; note = 2'-methoxy nucleoside; note (original language) = 2'-甲氧基核苷
  modified_base 7..8: mod_base = OTHER; note = 2'-methoxy nucleoside; note (original language) = 2'-甲氧基核苷
  modified_base 10..13: mod_base = OTHER; note = 2'-methoxy nucleoside; note (original language) = 2'-甲氧基核苷
  modified_base 15: mod_base = OTHER; note = 2'-methoxy nucleoside; note (original language) = 2'-甲氧基核苷
  modified_base 17..23: mod_base = OTHER; note = 2'-methoxy nucleoside; note (original language) = 2'-甲氧基核苷
  modified_base 2: mod_base = OTHER; note = 2'-fluoro nucleoside; note (original language) = 2'-氟核苷
  modified_base 6: mod_base = OTHER; note = 2'-fluoro nucleoside; note (original language) = 2'-氟核苷
  modified_base 9: mod_base = OTHER; note = 2'-fluoro nucleoside; note (original language) = 2'-氟核苷
  modified_base 14: mod_base = OTHER; note = 2'-fluoro nucleoside; note (original language) = 2'-氟核苷
  modified_base 16: mod_base = OTHER; note = 2'-fluoro nucleoside; note (original language) = 2'-氟核苷
  modified_base 1..3: mod_base = OTHER; note = phosphorothioate bond; note (original language) = 硫代磷酸酯键
  modified_base 21..23: mod_base = OTHER; note = phosphorothioate bond; note (original language) = 硫代磷酸酯键
  source 1..23: mol_type = other RNA
acacttagaccaaggagaaacgg

SEQ ID NO: 641 - RNA, 23 nt, synthetic construct
  modified_base 1: mod_base = OTHER; note = 2'-methoxy nucleoside; note (original language) = 2'-甲氧基核苷
  modified_base 3..5: mod_base = OTHER; note = 2'-methoxy nucleoside; note (original language) = 2'-甲氧基核苷
  modified_base 7..8: mod_base = OTHER; note = 2'-methoxy nucleoside; note (original language) = 2'-甲氧基核苷
  modified_base 10..13: mod_base = OTHER; note = 2'-methoxy nucleoside; note (original language) = 2'-甲氧基核苷
  modified_base 15: mod_base = OTHER; note = 2'-methoxy nucleoside; note (original language) = 2'-甲氧基核苷
  modified_base 17..23: mod_base = OTHER; note = 2'-methoxy nucleoside; note (original language) = 2'-甲氧基核苷
  modified_base 2: mod_base = OTHER; note = 2'-fluoro nucleoside; note (original language) = 2'-氟核苷
  modified_base 6: mod_base = OTHER; note = 2'-fluoro nucleoside; note (original language) = 2'-氟核苷
  modified_base 9: mod_base = OTHER; note = 2'-fluoro nucleoside; note (original language) = 2'-氟核苷
  modified_base 14: mod_base = OTHER; note = 2'-fluoro nucleoside; note (original language) = 2'-氟核苷
  modified_base 16: mod_base = OTHER; note = 2'-fluoro nucleoside; note (original language) = 2'-氟核苷
  modified_base 1..3: mod_base = OTHER; note = phosphorothioate bond; note (original language) = 硫代磷酸酯键
  modified_base 21..23: mod_base = OTHER; note = phosphorothioate bond; note (original language) = 硫代磷酸酯键
  source 1..23: mol_type = other RNA
tcacttagaccaaggagaaacgg

SEQ ID NO: 642 - RNA, 23 nt, synthetic construct
  modified_base 1: mod_base = OTHER; note = 2'-methoxy nucleoside; note (original language) = 2'-甲氧基核苷
  modified_base 3..5: mod_base = OTHER; note = 2'-methoxy nucleoside; note (original language) = 2'-甲氧基核苷
  modified_base 7..8: mod_base = OTHER; note = 2'-methoxy nucleoside; note (original language) = 2'-甲氧基核苷
  modified_base 10..13: mod_base = OTHER; note = 2'-methoxy nucleoside; note (original language) = 2'-甲氧基核苷
  modified_base 15: mod_base = OTHER; note = 2'-methoxy nucleoside; note (original language) = 2'-甲氧基核苷
  modified_base 17..23: mod_base = OTHER; note = 2'-methoxy nucleoside; note (original language) = 2'-甲氧基核苷
  modified_base 2: mod_base = OTHER; note = 2'-fluoro nucleoside; note (original language) = 2'-氟核苷
  modified_base 6: mod_base = OTHER; note = 2'-fluoro nucleoside; note (original language) = 2'-氟核苷
  modified_base 9: mod_base = OTHER; note = 2'-fluoro nucleoside; note (original language) = 2'-氟核苷
  modified_base 14: mod_base = OTHER; note = 2'-fluoro nucleoside; note (original language) = 2'-氟核苷
  modified_base 16: mod_base = OTHER; note = 2'-fluoro nucleoside; note (original language) = 2'-氟核苷
  modified_base 1..3: mod_base = OTHER; note = phosphorothioate bond; note (original language) = 硫代磷酸酯键
  modified_base 21..23: mod_base = OTHER; note = phosphorothioate bond; note (original language) = 硫代磷酸酯键
  source 1..23: mol_type = other RNA
tgtactctcattgtggatgacga

SEQ ID NO: 643 - RNA, 23 nt, synthetic construct
  modified_base 1: mod_base = OTHER; note = 2'-methoxy nucleoside; note (original language) = 2'-甲氧基核苷
  modified_base 3..5: mod_base = OTHER; note = 2'-methoxy nucleoside; note (original language) = 2'-甲氧基核苷
  modified_base 7..13: mod_base = OTHER; note = 2'-methoxy nucleoside; note (original language) = 2'-甲氧基核苷
  modified_base 15: mod_base = OTHER; note = 2'-methoxy nucleoside; note (original language) = 2'-甲氧基核苷
  modified_base 17..23: mod_base = OTHER; note = 2'-methoxy nucleoside; note (original language) = 2'-甲氧基核苷
  modified_base 2: mod_base = OTHER; note = 2'-fluoro nucleoside; note (original language) = 2'-氟核苷
  modified_base 6: mod_base = OTHER; note = 2'-fluoro nucleoside; note (original language) = 2'-氟核苷
  modified_base 14: mod_base = OTHER; note = 2'-fluoro nucleoside; note (original language) = 2'-氟核苷
  modified_base 16: mod_base = OTHER; note = 2'-fluoro nucleoside; note (original language) = 2'-氟核苷
  modified_base 1..3: mod_base = OTHER; note = phosphorothioate bond; note (original language) = 硫代磷酸酯键
  modified_base 21..23: mod_base = OTHER; note = phosphorothioate bond; note (original language) = 硫代磷酸酯键
  source 1..23: mol_type = other RNA
agaagaaaaggtgggagactggg

SEQ ID NO: 644 - RNA, 23 nt, synthetic construct
  modified_base 1: mod_base = OTHER; note = 2'-methoxy nucleoside; note (original language) = 2'-甲氧基核苷
  modified_base 3..5: mod_base = OTHER; note = 2'-methoxy nucleoside; note (original language) = 2'-甲氧基核苷
  modified_base 7..13: mod_base = OTHER; note = 2'-methoxy nucleoside; note (original language) = 2'-甲氧基核苷
  modified_base 15: mod_base = OTHER; note = 2'-methoxy nucleoside; note (original language) = 2'-甲氧基核苷
  modified_base 17..23: mod_base = OTHER; note = 2'-methoxy nucleoside; note (original language) = 2'-甲氧基核苷
  modified_base 2: mod_base = OTHER; note = 2'-fluoro nucleoside; note (original language) = 2'-氟核苷
  modified_base 6: mod_base = OTHER; note = 2'-fluoro nucleoside; note (original language) = 2'-氟核苷
  modified_base 14: mod_base = OTHER; note = 2'-fluoro nucleoside; note (original language) = 2'-氟核苷
  modified_base 16: mod_base = OTHER; note = 2'-fluoro nucleoside; note (original language) = 2'-氟核苷
  modified_base 1..3: mod_base = OTHER; note = phosphorothioate bond; note (original language) = 硫代磷酸酯键
  modified_base 21..23: mod_base = OTHER; note = phosphorothioate bond; note (original language) = 硫代磷酸酯键
  source 1..23: mol_type = other RNA
ttagaccaaggagaaacggccgc

SEQ ID NO: 645 - RNA, 23 nt, synthetic construct
  modified_base 1: mod_base = OTHER; note = 2'-methoxy nucleoside; note (original language) = 2'-甲氧基核苷
  modified_base 3..5: mod_base = OTHER; note = 2'-methoxy nucleoside; note (original language) = 2'-甲氧基核苷
  modified_base 7..13: mod_base = OTHER; note = 2'-methoxy nucleoside; note (original language) = 2'-甲氧基核苷
  modified_base 15: mod_base = OTHER; note = 2'-methoxy nucleoside; note (original language) = 2'-甲氧基核苷
  modified_base 17..23: mod_base = OTHER; note = 2'-methoxy nucleoside; note (original language) = 2'-甲氧基核苷
  modified_base 2: mod_base = OTHER; note = 2'-fluoro nucleoside; note (original language) = 2'-氟核苷
  modified_base 6: mod_base = OTHER; note = 2'-fluoro nucleoside; note (original language) = 2'-氟核苷
  modified_base 14: mod_base = OTHER; note = 2'-fluoro nucleoside; note (original language) = 2'-氟核苷
  modified_base 16: mod_base = OTHER; note = 2'-fluoro nucleoside; note (original language) = 2'-氟核苷
  modified_base 1..3: mod_base = OTHER; note = phosphorothioate bond; note (original language) = 硫代磷酸酯键
  modified_base 21..23: mod_base = OTHER; note = phosphorothioate bond; note (original language) = 硫代磷酸酯键
  source 1..23: mol_type = other RNA
tttagaccaaggagaaacggctg

SEQ ID NO: 646 - RNA, 23 nt, synthetic construct
  modified_base 1: mod_base = OTHER; note = 2'-methoxy nucleoside; note (original language) = 2'-甲氧基核苷
  modified_base 3..5: mod_base = OTHER; note = 2'-methoxy nucleoside; note (original language) = 2'-甲氧基核苷
  modified_base 7..13: mod_base = OTHER; note = 2'-methoxy nucleoside; note (original language) = 2'-甲氧基核苷
  modified_base 15: mod_base = OTHER; note = 2'-methoxy nucleoside; note (original language) = 2'-甲氧基核苷
  modified_base 17..23: mod_base = OTHER; note = 2'-methoxy nucleoside; note (original language) = 2'-甲氧基核苷
  modified_base 2: mod_base = OTHER; note = 2'-fluoro nucleoside; note (original language) = 2'-氟核苷
  modified_base 6: mod_base = OTHER; note = 2'-fluoro nucleoside; note (original language) = 2'-氟核苷
  modified_base 14: mod_base = OTHER; note = 2'-fluoro nucleoside; note (original language) = 2'-氟核苷
  modified_base 16: mod_base = OTHER; note = 2'-fluoro nucleoside; note (original language) = 2'-氟核苷
  modified_base 1..3: mod_base = OTHER; note = phosphorothioate bond; note (original language) = 硫代磷酸酯键
  modified_base 21..23: mod_base = OTHER; note = phosphorothioate bond; note (original language) = 硫代磷酸酯键
  source 1..23: mol_type = other RNA
tcttagaccaaggagaaacggct

SEQ ID NO: 647 - RNA, 23 nt, synthetic construct
  modified_base 1: mod_base = OTHER; note = 2'-methoxy nucleoside; note (original language) = 2'-甲氧基核苷
  modified_base 3..5: mod_base = OTHER; note = 2'-methoxy nucleoside; note (original language) = 2'-甲氧基核苷
  modified_base 7..13: mod_base = OTHER; note = 2'-methoxy nucleoside; note (original language) = 2'-甲氧基核苷
  modified_base 15: mod_base = OTHER; note = 2'-methoxy nucleoside; note (original language) = 2'-甲氧基核苷
  modified_base 17..23: mod_base = OTHER; note = 2'-methoxy nucleoside; note (original language) = 2'-甲氧基核苷
  modified_base 2: mod_base = OTHER; note = 2'-fluoro nucleoside; note (original language) = 2'-氟核苷
  modified_base 6: mod_base = OTHER; note = 2'-fluoro nucleoside; note (original language) = 2'-氟核苷
  modified_base 14: mod_base = OTHER; note = 2'-fluoro nucleoside; note (original language) = 2'-氟核苷
  modified_base 16: mod_base = OTHER; note = 2'-fluoro nucleoside; note (original language) = 2'-氟核苷
  modified_base 1..3: mod_base = OTHER; note = phosphorothioate bond; note (original language) = 硫代磷酸酯键
  modified_base 21..23: mod_base = OTHER; note = phosphorothioate bond; note (original language) = 硫代磷酸酯键
  source 1..23: mol_type = other RNA
acttagaccaaggagaaacgcct

SEQ ID NO: 648 - RNA, 23 nt, synthetic construct
  modified_base 1: mod_base = OTHER; note = 2'-methoxy nucleoside; note (original language) = 2'-甲氧基核苷
  modified_base 3..5: mod_base = OTHER; note = 2'-methoxy nucleoside; note (original language) = 2'-甲氧基核苷
  modified_base 7..13: mod_base = OTHER; note = 2'-methoxy nucleoside; note (original language) = 2'-甲氧基核苷
  modified_base 15: mod_base = OTHER; note = 2'-methoxy nucleoside; note (original language) = 2'-甲氧基核苷
  modified_base 17..23: mod_base = OTHER; note = 2'-methoxy nucleoside; note (original language) = 2'-甲氧基核苷
  modified_base 2: mod_base = OTHER; note = 2'-fluoro nucleoside; note (original language) = 2'-氟核苷
  modified_base 6: mod_base = OTHER; note = 2'-fluoro nucleoside; note (original language) = 2'-氟核苷
  modified_base 14: mod_base = OTHER; note = 2'-fluoro nucleoside; note (original language) = 2'-氟核苷
  modified_base 16: mod_base = OTHER; note = 2'-fluoro nucleoside; note (original language) = 2'-氟核苷
  modified_base 1..3: mod_base = OTHER; note = phosphorothioate bond; note (original language) = 硫代磷酸酯键
  modified_base 21..23: mod_base = OTHER; note = phosphorothioate bond; note (original language) = 硫代磷酸酯键
  source 1..23: mol_type = other RNA
tcttagaccaaggagaaacgcct

SEQ ID NO: 649 - RNA, 23 nt, synthetic construct
  modified_base 1: mod_base = OTHER; note = 2'-methoxy nucleoside; note (original language) = 2'-甲氧基核苷
  modified_base 3..5: mod_base = OTHER; note = 2'-methoxy nucleoside; note (original language) = 2'-甲氧基核苷
  modified_base 7..13: mod_base = OTHER; note = 2'-methoxy nucleoside; note (original language) = 2'-甲氧基核苷
  modified_base 15: mod_base = OTHER; note = 2'-methoxy nucleoside; note (original language) = 2'-甲氧基核苷
  modified_base 17..23: mod_base = OTHER; note = 2'-methoxy nucleoside; note (original language) = 2'-甲氧基核苷
  modified_base 2: mod_base = OTHER; note = 2'-fluoro nucleoside; note (original language) = 2'-氟核苷
  modified_base 6: mod_base = OTHER; note = 2'-fluoro nucleoside; note (original language) = 2'-氟核苷
  modified_base 14: mod_base = OTHER; note = 2'-fluoro nucleoside; note (original language) = 2'-氟核苷
  modified_base 16: mod_base = OTHER; note = 2'-fluoro nucleoside; note (original language) = 2'-氟核苷
  modified_base 2..3: mod_base = OTHER; note = phosphorothioate bond; note (original language) = 硫代磷酸酯键
  modified_base 21..23: mod_base = OTHER; note = phosphorothioate bond; note (original language) = 硫代磷酸酯键
  modified_base 1: mod_base = OTHER; note = 2'-methoxy-5'-vinyl phosphonate nucleoside; note (original language) = 2'-甲氧基-5'-乙烯基膦酸核苷
  source 1..23: mol_type = other RNA
tcttagaccaaggagaaacggct

SEQ ID NO: 650 - RNA, 21 nt, synthetic construct
  modified_base 1: mod_base = OTHER; note = 2'-methoxy nucleoside; note (original language) = 2'-甲氧基核苷
  modified_base 3..5: mod_base = OTHER; note = 2'-methoxy nucleoside; note (original language) = 2'-甲氧基核苷
  modified_base 7..13: mod_base = OTHER; note = 2'-methoxy nucleoside; note (original language) = 2'-甲氧基核苷
  modified_base 15: mod_base = OTHER; note = 2'-methoxy nucleoside; note (original language) = 2'-甲氧基核苷
  modified_base 17..21: mod_base = OTHER; note = 2'-methoxy nucleoside; note (original language) = 2'-甲氧基核苷
  modified_base 2: mod_base = OTHER; note = 2'-fluoro nucleoside; note (original language) = 2'-氟核苷
  modified_base 6: mod_base = OTHER; note = 2'-fluoro nucleoside; note (original language) = 2'-氟核苷
  modified_base 14: mod_base = OTHER; note = 2'-fluoro nucleoside; note (original language) = 2'-氟核苷
  modified_base 16: mod_base = OTHER; note = 2'-fluoro nucleoside; note (original language) = 2'-氟核苷
  modified_base 1..3: mod_base = OTHER; note = phosphorothioate bond; note (original language) = 硫代磷酸酯键
  modified_base 19..21: mod_base = OTHER; note = phosphorothioate bond; note (original language) = 硫代磷酸酯键
  source 1..21: mol_type = other RNA
attagaagaaaaggtgggaga

SEQ ID NO: 651 - RNA, 21 nt, synthetic construct
  modified_base 1: mod_base = OTHER; note = 2'-methoxy nucleoside; note (original language) = 2'-甲氧基核苷
  modified_base 3..5: mod_base = OTHER; note = 2'-methoxy nucleoside; note (original language) = 2'-甲氧基核苷
  modified_base 7..13: mod_base = OTHER; note = 2'-methoxy nucleoside; note (original language) = 2'-甲氧基核苷
  modified_base 15: mod_base = OTHER; note = 2'-methoxy nucleoside; note (original language) = 2'-甲氧基核苷
  modified_base 17..21: mod_base = OTHER; note = 2'-methoxy nucleoside; note (original language) = 2'-甲氧基核苷
  modified_base 2: mod_base = OTHER; note = 2'-fluoro nucleoside; note (original language) = 2'-氟核苷
  modified_base 6: mod_base = OTHER; note = 2'-fluoro nucleoside; note (original language) = 2'-氟核苷
  modified_base 14: mod_base = OTHER; note = 2'-fluoro nucleoside; note (original language) = 2'-氟核苷
  modified_base 16: mod_base = OTHER; note = 2'-fluoro nucleoside; note (original language) = 2'-氟核苷
  modified_base 1..3: mod_base = OTHER; note = phosphorothioate bond; note (original language) = 硫代磷酸酯键
  modified_base 19..21: mod_base = OTHER; note = phosphorothioate bond; note (original language) = 硫代磷酸酯键
  source 1..21: mol_type = other RNA
tttagaagaaaaggtgggcga

SEQ ID NO: 652 - RNA, 21 nt, synthetic construct
  modified_base 1: mod_base = OTHER; note = 2'-methoxy nucleoside; note (original language) = 2'-甲氧基核苷
  modified_base 3..5: mod_base = OTHER; note = 2'-methoxy nucleoside; note (original language) = 2'-甲氧基核苷
  modified_base 7..13: mod_base = OTHER; note = 2'-methoxy nucleoside; note (original language) = 2'-甲氧基核苷
  modified_base 15: mod_base = OTHER; note = 2'-methoxy nucleoside; note (original language) = 2'-甲氧基核苷
  modified_base 17..21: mod_base = OTHER; note = 2'-methoxy nucleoside; note (original language) = 2'-甲氧基核苷
  modified_base 2: mod_base = OTHER; note = 2'-fluoro nucleoside; note (original language) = 2'-氟核苷
  modified_base 6: mod_base = OTHER; note = 2'-fluoro nucleoside; note (original language) = 2'-氟核苷
  modified_base 14: mod_base = OTHER; note = 2'-fluoro nucleoside; note (original language) = 2'-氟核苷
  modified_base 16: mod_base = OTHER; note = 2'-fluoro nucleoside; note (original language) = 2'-氟核苷
  modified_base 1..3: mod_base = OTHER; note = phosphorothioate bond; note (original language) = 硫代磷酸酯键
  modified_base 19..21: mod_base = OTHER; note = phosphorothioate bond; note (original language) = 硫代磷酸酯键
  source 1..21: mol_type = other RNA
ttactctcattgtggatgccg

SEQ ID NO: 653 - RNA, 21 nt, synthetic construct
  modified_base 1: mod_base = OTHER; note = 2'-methoxy nucleoside; note (original language) = 2'-甲氧基核苷
  modified_base 3..5: mod_base = OTHER; note = 2'-methoxy nucleoside; note (original language) = 2'-甲氧基核苷
  modified_base 7..13: mod_base = OTHER; note = 2'-methoxy nucleoside; note (original language) = 2'-甲氧基核苷
  modified_base 15: mod_base = OTHER; note = 2'-methoxy nucleoside; note (original language) = 2'-甲氧基核苷
  modified_base 17..21: mod_base = OTHER; note = 2'-methoxy nucleoside; note (original language) = 2'-甲氧基核苷
  modified_base 2: mod_base = OTHER; note = 2'-fluoro nucleoside; note (original language) = 2'-氟核苷
  modified_base 6: mod_base = OTHER; note = 2'-fluoro nucleoside; note (original language) = 2'-氟核苷
  modified_base 14: mod_base = OTHER; note = 2'-fluoro nucleoside; note (original language) = 2'-氟核苷
  modified_base 16: mod_base = OTHER; note = 2'-fluoro nucleoside; note (original language) = 2'-氟核苷
  modified_base 1..3: mod_base = OTHER; note = phosphorothioate bond; note (original language) = 硫代磷酸酯键
  modified_base 19..21: mod_base = OTHER; note = phosphorothioate bond; note (original language) = 硫代磷酸酯键
  source 1..21: mol_type = other RNA
ttctcattgtggatgacgcgg

SEQ ID NO: 654 - RNA, 21 nt, synthetic construct
  modified_base 1: mod_base = OTHER; note = 2'-methoxy nucleoside; note (original language) = 2'-甲氧基核苷
  modified_base 3..5: mod_base = OTHER; note = 2'-methoxy nucleoside; note (original language) = 2'-甲氧基核苷
  modified_base 7..13: mod_base = OTHER; note = 2'-methoxy nucleoside; note (original language) = 2'-甲氧基核苷
  modified_base 15: mod_base = OTHER; note = 2'-methoxy nucleoside; note (original language) = 2'-甲氧基核苷
  modified_base 17..21: mod_base = OTHER; note = 2'-methoxy nucleoside; note (original language) = 2'-甲氧基核苷
  modified_base 2: mod_base = OTHER; note = 2'-fluoro nucleoside; note (original language) = 2'-氟核苷
  modified_base 6: mod_base = OTHER; note = 2'-fluoro nucleoside; note (original language) = 2'-氟核苷
  modified_base 14: mod_base = OTHER; note = 2'-fluoro nucleoside; note (original language) = 2'-氟核苷
  modified_base 16: mod_base = OTHER; note = 2'-fluoro nucleoside; note (original language) = 2'-氟核苷
  modified_base 1..3: mod_base = OTHER; note = phosphorothioate bond; note (original language) = 硫代磷酸酯键
  modified_base 19..21: mod_base = OTHER; note = phosphorothioate bond; note (original language) = 硫代磷酸酯键
  source 1..21: mol_type = other RNA
ttcattgtggatgacgaggtg

SEQ ID NO: 655 - RNA, 21 nt, synthetic construct
  modified_base 1: mod_base = OTHER; note = 2'-methoxy nucleoside; note (original language) = 2'-甲氧基核苷
  modified_base 3..5: mod_base = OTHER; note = 2'-methoxy nucleoside; note (original language) = 2'-甲氧基核苷
  modified_base 7..13: mod_base = OTHER; note = 2'-methoxy nucleoside; note (original language) = 2'-甲氧基核苷
  modified_base 15: mod_base = OTHER; note = 2'-methoxy nucleoside; note (original language) = 2'-甲氧基核苷
  modified_base 17..21: mod_base = OTHER; note = 2'-methoxy nucleoside; note (original language) = 2'-甲氧基核苷
  modified_base 2: mod_base = OTHER; note = 2'-fluoro nucleoside; note (original language) = 2'-氟核苷
  modified_base 6: mod_base = OTHER; note = 2'-fluoro nucleoside; note (original language) = 2'-氟核苷
  modified_base 14: mod_base = OTHER; note = 2'-fluoro nucleoside; note (original language) = 2'-氟核苷
  modified_base 16: mod_base = OTHER; note = 2'-fluoro nucleoside; note (original language) = 2'-氟核苷
  modified_base 1..3: mod_base = OTHER; note = phosphorothioate bond; note (original language) = 硫代磷酸酯键
  modified_base 19..21: mod_base = OTHER; note = phosphorothioate bond; note (original language) = 硫代磷酸酯键
  source 1..21: mol_type = other RNA
tattgtggatgacgaggtgga

SEQ ID NO: 656 - RNA, 21 nt, synthetic construct
  modified_base 1: mod_base = OTHER; note = 2'-methoxy nucleoside; note (original language) = 2'-甲氧基核苷
  modified_base 3..5: mod_base = OTHER; note = 2'-methoxy nucleoside; note (original language) = 2'-甲氧基核苷
  modified_base 7..13: mod_base = OTHER; note = 2'-methoxy nucleoside; note (original language) = 2'-甲氧基核苷
  modified_base 15: mod_base = OTHER; note = 2'-methoxy nucleoside; note (original language) = 2'-甲氧基核苷
  modified_base 17..21: mod_base = OTHER; note = 2'-methoxy nucleoside; note (original language) = 2'-甲氧基核苷
  modified_base 2: mod_base = OTHER; note = 2'-fluoro nucleoside; note (original language) = 2'-氟核苷
  modified_base 6: mod_base = OTHER; note = 2'-fluoro nucleoside; note (original language) = 2'-氟核苷
  modified_base 14: mod_base = OTHER; note = 2'-fluoro nucleoside; note (original language) = 2'-氟核苷
  modified_base 16: mod_base = OTHER; note = 2'-fluoro nucleoside; note (original language) = 2'-氟核苷
  modified_base 1..3: mod_base = OTHER; note = phosphorothioate bond; note (original language) = 硫代磷酸酯键
  modified_base 19..21: mod_base = OTHER; note = phosphorothioate bond; note (original language) = 硫代磷酸酯键
  source 1..21: mol_type = other RNA
tggtactctcattgtggacga

SEQ ID NO: 657 - RNA, 21 nt, synthetic construct
  modified_base 1: mod_base = OTHER; note = 2'-methoxy nucleoside; note (original language) = 2'-甲氧基核苷
  modified_base 3..5: mod_base = OTHER; note = 2'-methoxy nucleoside; note (original language) = 2'-甲氧基核苷
  modified_base 7..13: mod_base = OTHER; note = 2'-methoxy nucleoside; note (original language) = 2'-甲氧基核苷
  modified_base 15: mod_base = OTHER; note = 2'-methoxy nucleoside; note (original language) = 2'-甲氧基核苷
  modified_base 17..21: mod_base = OTHER; note = 2'-methoxy nucleoside; note (original language) = 2'-甲氧基核苷
  modified_base 2: mod_base = OTHER; note = 2'-fluoro nucleoside; note (original language) = 2'-氟核苷
  modified_base 6: mod_base = OTHER; note = 2'-fluoro nucleoside; note (original language) = 2'-氟核苷
  modified_base 14: mod_base = OTHER; note = 2'-fluoro nucleoside; note (original language) = 2'-氟核苷
  modified_base 16: mod_base = OTHER; note = 2'-fluoro nucleoside; note (original language) = 2'-氟核苷
  modified_base 1..3: mod_base = OTHER; note = phosphorothioate bond; note (original language) = 硫代磷酸酯键
  modified_base 19..21: mod_base = OTHER; note = phosphorothioate bond; note (original language) = 硫代磷酸酯键
  source 1..21: mol_type = other RNA
taggtactctcattgtggctg

SEQ ID NO: 658 - RNA, 21 nt, synthetic construct
  modified_base 1: mod_base = OTHER; note = 2'-methoxy nucleoside; note (original language) = 2'-甲氧基核苷
  modified_base 3..5: mod_base = OTHER; note = 2'-methoxy nucleoside; note (original language) = 2'-甲氧基核苷
  modified_base 7..13: mod_base = OTHER; note = 2'-methoxy nucleoside; note (original language) = 2'-甲氧基核苷
  modified_base 15: mod_base = OTHER; note = 2'-methoxy nucleoside; note (original language) = 2'-甲氧基核苷
  modified_base 17..21: mod_base = OTHER; note = 2'-methoxy nucleoside; note (original language) = 2'-甲氧基核苷
  modified_base 2: mod_base = OTHER; note = 2'-fluoro nucleoside; note (original language) = 2'-氟核苷
  modified_base 6: mod_base = OTHER; note = 2'-fluoro nucleoside; note (original language) = 2'-氟核苷
  modified_base 14: mod_base = OTHER; note = 2'-fluoro nucleoside; note (original language) = 2'-氟核苷
  modified_base 16: mod_base = OTHER; note = 2'-fluoro nucleoside; note (original language) = 2'-氟核苷
  modified_base 1..3: mod_base = OTHER; note = phosphorothioate bond; note (original language) = 硫代磷酸酯键
  modified_base 19..21: mod_base = OTHER; note = phosphorothioate bond; note (original language) = 硫代磷酸酯键
  source 1..21: mol_type = other RNA
tacaggtactctcattgtgga

SEQ ID NO: 659 - RNA, 21 nt, synthetic construct
  modified_base 1: mod_base = OTHER; note = 2'-methoxy nucleoside; note (original language) = 2'-甲氧基核苷
  modified_base 3..5: mod_base = OTHER; note = 2'-methoxy nucleoside; note (original language) = 2'-甲氧基核苷
  modified_base 7..13: mod_base = OTHER; note = 2'-methoxy nucleoside; note (original language) = 2'-甲氧基核苷
  modified_base 15: mod_base = OTHER; note = 2'-methoxy nucleoside; note (original language) = 2'-甲氧基核苷
  modified_base 17..21: mod_base = OTHER; note = 2'-methoxy nucleoside; note (original language) = 2'-甲氧基核苷
  modified_base 2: mod_base = OTHER; note = 2'-fluoro nucleoside; note (original language) = 2'-氟核苷
  modified_base 6: mod_base = OTHER; note = 2'-fluoro nucleoside; note (original language) = 2'-氟核苷
  modified_base 14: mod_base = OTHER; note = 2'-fluoro nucleoside; note (original language) = 2'-氟核苷
  modified_base 16: mod_base = OTHER; note = 2'-fluoro nucleoside; note (original language) = 2'-氟核苷
  modified_base 1..3: mod_base = OTHER; note = phosphorothioate bond; note (original language) = 硫代磷酸酯键
  modified_base 19..21: mod_base = OTHER; note = phosphorothioate bond; note (original language) = 硫代磷酸酯键
  source 1..21: mol_type = other RNA
tcacaggtactctcattgcgg

SEQ ID NO: 660 - RNA, 21 nt, synthetic construct
  modified_base 1: mod_base = OTHER; note = 2'-methoxy nucleoside; note (original language) = 2'-甲氧基核苷
  modified_base 3..5: mod_base = OTHER; note = 2'-methoxy nucleoside; note (original language) = 2'-甲氧基核苷
  modified_base 7..13: mod_base = OTHER; note = 2'-methoxy nucleoside; note (original language) = 2'-甲氧基核苷
  modified_base 15: mod_base = OTHER; note = 2'-methoxy nucleoside; note (original language) = 2'-甲氧基核苷
  modified_base 17..21: mod_base = OTHER; note = 2'-methoxy nucleoside; note (original language) = 2'-甲氧基核苷
  modified_base 2: mod_base = OTHER; note = 2'-fluoro nucleoside; note (original language) = 2'-氟核苷
  modified_base 6: mod_base = OTHER; note = 2'-fluoro nucleoside; note (original language) = 2'-氟核苷
  modified_base 14: mod_base = OTHER; note = 2'-fluoro nucleoside; note (original language) = 2'-氟核苷
  modified_base 16: mod_base = OTHER; note = 2'-fluoro nucleoside; note (original language) = 2'-氟核苷
  modified_base 1..3: mod_base = OTHER; note = phosphorothioate bond; note (original language) = 硫代磷酸酯键
  modified_base 19..21: mod_base = OTHER; note = phosphorothioate bond; note (original language) = 硫代磷酸酯键
  source 1..21: mol_type = other RNA
ttcacaggtactctcattgtg

SEQ ID NO: 661 - RNA, 21 nt, synthetic construct
  modified_base 1: mod_base = OTHER; note = 2'-methoxy nucleoside; note (original language) = 2'-甲氧基核苷
  modified_base 3..5: mod_base = OTHER; note = 2'-methoxy nucleoside; note (original language) = 2'-甲氧基核苷
  modified_base 7..13: mod_base = OTHER; note = 2'-methoxy nucleoside; note (original language) = 2'-甲氧基核苷
  modified_base 15: mod_base = OTHER; note = 2'-methoxy nucleoside; note (original language) = 2'-甲氧基核苷
  modified_base 17..21: mod_base = OTHER; note = 2'-methoxy nucleoside; note (original language) = 2'-甲氧基核苷
  modified_base 2: mod_base = OTHER; note = 2'-fluoro nucleoside; note (original language) = 2'-氟核苷
  modified_base 6: mod_base = OTHER; note = 2'-fluoro nucleoside; note (original language) = 2'-氟核苷
  modified_base 14: mod_base = OTHER; note = 2'-fluoro nucleoside; note (original language) = 2'-氟核苷
  modified_base 16: mod_base = OTHER; note = 2'-fluoro nucleoside; note (original language) = 2'-氟核苷
  modified_base 1..3: mod_base = OTHER; note = phosphorothioate bond; note (original language) = 硫代磷酸酯键
  modified_base 19..21: mod_base = OTHER; note = phosphorothioate bond; note (original language) = 硫代磷酸酯键
  source 1..21: mol_type = other RNA
tctcacaggtactctcatcgt

SEQ ID NO: 662 - RNA, 21 nt, synthetic construct
  modified_base 1: mod_base = OTHER; note = 2'-methoxy nucleoside; note (original language) = 2'-甲氧基核苷
  modified_base 3..5: mod_base = OTHER; note = 2'-methoxy nucleoside; note (original language) = 2'-甲氧基核苷
  modified_base 7..13: mod_base = OTHER; note = 2'-methoxy nucleoside; note (original language) = 2'-甲氧基核苷
  modified_base 15: mod_base = OTHER; note = 2'-methoxy nucleoside; note (original language) = 2'-甲氧基核苷
  modified_base 17..21: mod_base = OTHER; note = 2'-methoxy nucleoside; note (original language) = 2'-甲氧基核苷
  modified_base 2: mod_base = OTHER; note = 2'-fluoro nucleoside; note (original language) = 2'-氟核苷
  modified_base 6: mod_base = OTHER; note = 2'-fluoro nucleoside; note (original language) = 2'-氟核苷
  modified_base 14: mod_base = OTHER; note = 2'-fluoro nucleoside; note (original language) = 2'-氟核苷
  modified_base 16: mod_base = OTHER; note = 2'-fluoro nucleoside; note (original language) = 2'-氟核苷
  modified_base 1..3: mod_base = OTHER; note = phosphorothioate bond; note (original language) = 硫代磷酸酯键
  modified_base 19..21: mod_base = OTHER; note = phosphorothioate bond; note (original language) = 硫代磷酸酯键
  source 1..21: mol_type = other RNA
ttgctcacaggtactctcctt

SEQ ID NO: 663 - RNA, 21 nt, synthetic construct
  modified_base 1: mod_base = OTHER; note = 2'-methoxy nucleoside; note (original language) = 2'-甲氧基核苷
  modified_base 3..5: mod_base = OTHER; note = 2'-methoxy nucleoside; note (original language) = 2'-甲氧基核苷
  modified_base 7..13: mod_base = OTHER; note = 2'-methoxy nucleoside; note (original language) = 2'-甲氧基核苷
  modified_base 15: mod_base = OTHER; note = 2'-methoxy nucleoside; note (original language) = 2'-甲氧基核苷
  modified_base 17..21: mod_base = OTHER; note = 2'-methoxy nucleoside; note (original language) = 2'-甲氧基核苷
  modified_base 2: mod_base = OTHER; note = 2'-fluoro nucleoside; note (original language) = 2'-氟核苷
  modified_base 6: mod_base = OTHER; note = 2'-fluoro nucleoside; note (original language) = 2'-氟核苷
  modified_base 14: mod_base = OTHER; note = 2'-fluoro nucleoside; note (original language) = 2'-氟核苷
  modified_base 16: mod_base = OTHER; note = 2'-fluoro nucleoside; note (original language) = 2'-氟核苷
  modified_base 1..3: mod_base = OTHER; note = phosphorothioate bond; note (original language) = 硫代磷酸酯键
  modified_base 19..21: mod_base = OTHER; note = phosphorothioate bond; note (original language) = 硫代磷酸酯键
  source 1..21: mol_type = other RNA
tctgctcacaggtactctcat

SEQ ID NO: 664 - RNA, 21 nt, synthetic construct
  modified_base 1: mod_base = OTHER; note = 2'-methoxy nucleoside; note (original language) = 2'-甲氧基核苷
  modified_base 3..5: mod_base = OTHER; note = 2'-methoxy nucleoside; note (original language) = 2'-甲氧基核苷
  modified_base 7..13: mod_base = OTHER; note = 2'-methoxy nucleoside; note (original language) = 2'-甲氧基核苷
  modified_base 15: mod_base = OTHER; note = 2'-methoxy nucleoside; note (original language) = 2'-甲氧基核苷
  modified_base 17..21: mod_base = OTHER; note = 2'-methoxy nucleoside; note (original language) = 2'-甲氧基核苷
  modified_base 2: mod_base = OTHER; note = 2'-fluoro nucleoside; note (original language) = 2'-氟核苷
  modified_base 6: mod_base = OTHER; note = 2'-fluoro nucleoside; note (original language) = 2'-氟核苷
  modified_base 14: mod_base = OTHER; note = 2'-fluoro nucleoside; note (original language) = 2'-氟核苷
  modified_base 16: mod_base = OTHER; note = 2'-fluoro nucleoside; note (original language) = 2'-氟核苷
  modified_base 1..3: mod_base = OTHER; note = phosphorothioate bond; note (original language) = 硫代磷酸酯键
  modified_base 19..21: mod_base = OTHER; note = phosphorothioate bond; note (original language) = 硫代磷酸酯键
  source 1..21: mol_type = other RNA
ttagaagaaaaggtgggagac

SEQ ID NO: 665 - RNA, 21 nt, synthetic construct
  modified_base 1: mod_base = OTHER; note = 2'-methoxy nucleoside; note (original language) = 2'-甲氧基核苷
  modified_base 3..5: mod_base = OTHER; note = 2'-methoxy nucleoside; note (original language) = 2'-甲氧基核苷
  modified_base 7..13: mod_base = OTHER; note = 2'-methoxy nucleoside; note (original language) = 2'-甲氧基核苷
  modified_base 15: mod_base = OTHER; note = 2'-methoxy nucleoside; note (original language) = 2'-甲氧基核苷
  modified_base 17..21: mod_base = OTHER; note = 2'-methoxy nucleoside; note (original language) = 2'-甲氧基核苷
  modified_base 2: mod_base = OTHER; note = 2'-fluoro nucleoside; note (original language) = 2'-氟核苷
  modified_base 6: mod_base = OTHER; note = 2'-fluoro nucleoside; note (original language) = 2'-氟核苷
  modified_base 14: mod_base = OTHER; note = 2'-fluoro nucleoside; note (original language) = 2'-氟核苷
  modified_base 16: mod_base = OTHER; note = 2'-fluoro nucleoside; note (original language) = 2'-氟核苷
  modified_base 1..3: mod_base = OTHER; note = phosphorothioate bond; note (original language) = 硫代磷酸酯键
  modified_base 19..21: mod_base = OTHER; note = phosphorothioate bond; note (original language) = 硫代磷酸酯键
  source 1..21: mol_type = other RNA
tagaagaaaaggtgggagcct

SEQ ID NO: 666 - RNA, 21 nt, synthetic construct
  modified_base 1: mod_base = OTHER; note = 2'-methoxy nucleoside; note (original language) = 2'-甲氧基核苷
  modified_base 3..5: mod_base = OTHER; note = 2'-methoxy nucleoside; note (original language) = 2'-甲氧基核苷
  modified_base 7..13: mod_base = OTHER; note = 2'-methoxy nucleoside; note (original language) = 2'-甲氧基核苷
  modified_base 15: mod_base = OTHER; note = 2'-methoxy nucleoside; note (original language) = 2'-甲氧基核苷
  modified_base 17..21: mod_base = OTHER; note = 2'-methoxy nucleoside; note (original language) = 2'-甲氧基核苷
  modified_base 2: mod_base = OTHER; note = 2'-fluoro nucleoside; note (original language) = 2'-氟核苷
  modified_base 6: mod_base = OTHER; note = 2'-fluoro nucleoside; note (original language) = 2'-氟核苷
  modified_base 14: mod_base = OTHER; note = 2'-fluoro nucleoside; note (original language) = 2'-氟核苷
  modified_base 16: mod_base = OTHER; note = 2'-fluoro nucleoside; note (original language) = 2'-氟核苷
  modified_base 1..3: mod_base = OTHER; note = phosphorothioate bond; note (original language) = 硫代磷酸酯键
  modified_base 19..21: mod_base = OTHER; note = phosphorothioate bond; note (original language) = 硫代磷酸酯键
  source 1..21: mol_type = other RNA
tgaagaaaaggtgggagactg

SEQ ID NO: 667 - RNA, 21 nt, synthetic construct
  modified_base 1: mod_base = OTHER; note = 2'-methoxy nucleoside; note (original language) = 2'-甲氧基核苷
  modified_base 3..5: mod_base = OTHER; note = 2'-methoxy nucleoside; note (original language) = 2'-甲氧基核苷
  modified_base 7..13: mod_base = OTHER; note = 2'-methoxy nucleoside; note (original language) = 2'-甲氧基核苷
  modified_base 15: mod_base = OTHER; note = 2'-methoxy nucleoside; note (original language) = 2'-甲氧基核苷
  modified_base 17..21: mod_base = OTHER; note = 2'-methoxy nucleoside; note (original language) = 2'-甲氧基核苷
  modified_base 2: mod_base = OTHER; note = 2'-fluoro nucleoside; note (original language) = 2'-氟核苷
  modified_base 6: mod_base = OTHER; note = 2'-fluoro nucleoside; note (original language) = 2'-氟核苷
  modified_base 14: mod_base = OTHER; note = 2'-fluoro nucleoside; note (original language) = 2'-氟核苷
  modified_base 16: mod_base = OTHER; note = 2'-fluoro nucleoside; note (original language) = 2'-氟核苷
  modified_base 1..3: mod_base = OTHER; note = phosphorothioate bond; note (original language) = 硫代磷酸酯键
  modified_base 19..21: mod_base = OTHER; note = phosphorothioate bond; note (original language) = 硫代磷酸酯键
  source 1..21: mol_type = other RNA
taagaaaaggtgggagaccgg

SEQ ID NO: 668 - RNA, 21 nt, synthetic construct
  modified_base 1: mod_base = OTHER; note = 2'-methoxy nucleoside; note (original language) = 2'-甲氧基核苷
  modified_base 3..5: mod_base = OTHER; note = 2'-methoxy nucleoside; note (original language) = 2'-甲氧基核苷
  modified_base 7..13: mod_base = OTHER; note = 2'-methoxy nucleoside; note (original language) = 2'-甲氧基核苷
  modified_base 15: mod_base = OTHER; note = 2'-methoxy nucleoside; note (original language) = 2'-甲氧基核苷
  modified_base 17..21: mod_base = OTHER; note = 2'-methoxy nucleoside; note (original language) = 2'-甲氧基核苷
  modified_base 2: mod_base = OTHER; note = 2'-fluoro nucleoside; note (original language) = 2'-氟核苷
  modified_base 6: mod_base = OTHER; note = 2'-fluoro nucleoside; note (original language) = 2'-氟核苷
  modified_base 14: mod_base = OTHER; note = 2'-fluoro nucleoside; note (original language) = 2'-氟核苷
  modified_base 16: mod_base = OTHER; note = 2'-fluoro nucleoside; note (original language) = 2'-氟核苷
  modified_base 1..3: mod_base = OTHER; note = phosphorothioate bond; note (original language) = 硫代磷酸酯键
  modified_base 19..21: mod_base = OTHER; note = phosphorothioate bond; note (original language) = 硫代磷酸酯键
  source 1..21: mol_type = other RNA
tattagaagaaaaggtgggag

SEQ ID NO: 669 - RNA, 21 nt, synthetic construct
  modified_base 1: mod_base = OTHER; note = 2'-methoxy nucleoside; note (original language) = 2'-甲氧基核苷
  modified_base 3..5: mod_base = OTHER; note = 2'-methoxy nucleoside; note (original language) = 2'-甲氧基核苷
  modified_base 7..13: mod_base = OTHER; note = 2'-methoxy nucleoside; note (original language) = 2'-甲氧基核苷
  modified_base 15: mod_base = OTHER; note = 2'-methoxy nucleoside; note (original language) = 2'-甲氧基核苷
  modified_base 17..21: mod_base = OTHER; note = 2'-methoxy nucleoside; note (original language) = 2'-甲氧基核苷
  modified_base 2: mod_base = OTHER; note = 2'-fluoro nucleoside; note (original language) = 2'-氟核苷
  modified_base 6: mod_base = OTHER; note = 2'-fluoro nucleoside; note (original language) = 2'-氟核苷
  modified_base 14: mod_base = OTHER; note = 2'-fluoro nucleoside; note (original language) = 2'-氟核苷
  modified_base 16: mod_base = OTHER; note = 2'-fluoro nucleoside; note (original language) = 2'-氟核苷
  modified_base 1..3: mod_base = OTHER; note = phosphorothioate bond; note (original language) = 硫代磷酸酯键
  modified_base 19..21: mod_base = OTHER; note = phosphorothioate bond; note (original language) = 硫代磷酸酯键
  source 1..21: mol_type = other RNA
tcattagaagaaaaggtggga

SEQ ID NO: 670 - RNA, 21 nt, synthetic construct
  modified_base 1: mod_base = OTHER; note = 2'-methoxy nucleoside; note (original language) = 2'-甲氧基核苷
  modified_base 3..5: mod_base = OTHER; note = 2'-methoxy nucleoside; note (original language) = 2'-甲氧基核苷
  modified_base 7..13: mod_base = OTHER; note = 2'-methoxy nucleoside; note (original language) = 2'-甲氧基核苷
  modified_base 15: mod_base = OTHER; note = 2'-methoxy nucleoside; note (original language) = 2'-甲氧基核苷
  modified_base 17..21: mod_base = OTHER; note = 2'-methoxy nucleoside; note (original language) = 2'-甲氧基核苷
  modified_base 2: mod_base = OTHER; note = 2'-fluoro nucleoside; note (original language) = 2'-氟核苷
  modified_base 6: mod_base = OTHER; note = 2'-fluoro nucleoside; note (original language) = 2'-氟核苷
  modified_base 14: mod_base = OTHER; note = 2'-fluoro nucleoside; note (original language) = 2'-氟核苷
  modified_base 16: mod_base = OTHER; note = 2'-fluoro nucleoside; note (original language) = 2'-氟核苷
  modified_base 1..3: mod_base = OTHER; note = phosphorothioate bond; note (original language) = 硫代磷酸酯键
  modified_base 19..21: mod_base = OTHER; note = phosphorothioate bond; note (original language) = 硫代磷酸酯键
  source 1..21: mol_type = other RNA
ttcattagaagaaaaggtggg

SEQ ID NO: 671 - RNA, 21 nt, synthetic construct
  modified_base 1: mod_base = OTHER; note = 2'-methoxy nucleoside; note (original language) = 2'-甲氧基核苷
  modified_base 3..5: mod_base = OTHER; note = 2'-methoxy nucleoside; note (original language) = 2'-甲氧基核苷
  modified_base 7..13: mod_base = OTHER; note = 2'-methoxy nucleoside; note (original language) = 2'-甲氧基核苷
  modified_base 15: mod_base = OTHER; note = 2'-methoxy nucleoside; note (original language) = 2'-甲氧基核苷
  modified_base 17..21: mod_base = OTHER; note = 2'-methoxy nucleoside; note (original language) = 2'-甲氧基核苷
  modified_base 2: mod_base = OTHER; note = 2'-fluoro nucleoside; note (original language) = 2'-氟核苷
  modified_base 6: mod_base = OTHER; note = 2'-fluoro nucleoside; note (original language) = 2'-氟核苷
  modified_base 14: mod_base = OTHER; note = 2'-fluoro nucleoside; note (original language) = 2'-氟核苷
  modified_base 16: mod_base = OTHER; note = 2'-fluoro nucleoside; note (original language) = 2'-氟核苷
  modified_base 1..3: mod_base = OTHER; note = phosphorothioate bond; note (original language) = 硫代磷酸酯键
  modified_base 19..21: mod_base = OTHER; note = phosphorothioate bond; note (original language) = 硫代磷酸酯键
  source 1..21: mol_type = other RNA
tctcattagaagaaaaggcgg

SEQ ID NO: 672 - RNA, 21 nt, synthetic construct
  modified_base 1: mod_base = OTHER; note = 2'-methoxy nucleoside; note (original language) = 2'-甲氧基核苷
  modified_base 3..5: mod_base = OTHER; note = 2'-methoxy nucleoside; note (original language) = 2'-甲氧基核苷
  modified_base 7..13: mod_base = OTHER; note = 2'-methoxy nucleoside; note (original language) = 2'-甲氧基核苷
  modified_base 15: mod_base = OTHER; note = 2'-methoxy nucleoside; note (original language) = 2'-甲氧基核苷
  modified_base 17..21: mod_base = OTHER; note = 2'-methoxy nucleoside; note (original language) = 2'-甲氧基核苷
  modified_base 2: mod_base = OTHER; note = 2'-fluoro nucleoside; note (original language) = 2'-氟核苷
  modified_base 6: mod_base = OTHER; note = 2'-fluoro nucleoside; note (original language) = 2'-氟核苷
  modified_base 14: mod_base = OTHER; note = 2'-fluoro nucleoside; note (original language) = 2'-氟核苷
  modified_base 16: mod_base = OTHER; note = 2'-fluoro nucleoside; note (original language) = 2'-氟核苷
  modified_base 1..3: mod_base = OTHER; note = phosphorothioate bond; note (original language) = 硫代磷酸酯键
  modified_base 19..21: mod_base = OTHER; note = phosphorothioate bond; note (original language) = 硫代磷酸酯键
  source 1..21: mol_type = other RNA
tactcattagaagaaaaggtg

SEQ ID NO: 673 - RNA, 23 nt, synthetic construct
  modified_base 3..5: mod_base = OTHER; note = 2'-methoxy nucleoside; note (original language) = 2'-甲氧基核苷
  modified_base 7..13: mod_base = OTHER; note = 2'-methoxy nucleoside; note (original language) = 2'-甲氧基核苷
  modified_base 15: mod_base = OTHER; note = 2'-methoxy nucleoside; note (original language) = 2'-甲氧基核苷
  modified_base 17..23: mod_base = OTHER; note = 2'-methoxy nucleoside; note (original language) = 2'-甲氧基核苷
  modified_base 2: mod_base = OTHER; note = 2'-fluoro nucleoside; note (original language) = 2'-氟核苷
  modified_base 6: mod_base = OTHER; note = 2'-fluoro nucleoside; note (original language) = 2'-氟核苷
  modified_base 14: mod_base = OTHER; note = 2'-fluoro nucleoside; note (original language) = 2'-氟核苷
  modified_base 16: mod_base = OTHER; note = 2'-fluoro nucleoside; note (original language) = 2'-氟核苷
  modified_base 1..3: mod_base = OTHER; note = phosphorothioate bond; note (original language) = 硫代磷酸酯键
  modified_base 21..23: mod_base = OTHER; note = phosphorothioate bond; note (original language) = 硫代磷酸酯键
  modified_base 1: mod_base = OTHER; note = 2'-acetamido-5'-vinyl phosphonate nucleoside; note (original language) = 2'-乙酰氨基-5'-乙烯基膦酸核苷
  source 1..23: mol_type = other RNA
ttagaccaaggagaaacggccgc

SEQ ID NO: 674 - RNA, 23 nt, synthetic construct
  modified_base 3..5: mod_base = OTHER; note = 2'-methoxy nucleoside; note (original language) = 2'-甲氧基核苷
  modified_base 7..13: mod_base = OTHER; note = 2'-methoxy nucleoside; note (original language) = 2'-甲氧基核苷
  modified_base 15: mod_base = OTHER; note = 2'-methoxy nucleoside; note (original language) = 2'-甲氧基核苷
  modified_base 17..23: mod_base = OTHER; note = 2'-methoxy nucleoside; note (original language) = 2'-甲氧基核苷
  modified_base 2: mod_base = OTHER; note = 2'-fluoro nucleoside; note (original language) = 2'-氟核苷
  modified_base 6: mod_base = OTHER; note = 2'-fluoro nucleoside; note (original language) = 2'-氟核苷
  modified_base 14: mod_base = OTHER; note = 2'-fluoro nucleoside; note (original language) = 2'-氟核苷
  modified_base 16: mod_base = OTHER; note = 2'-fluoro nucleoside; note (original language) = 2'-氟核苷
  modified_base 1..3: mod_base = OTHER; note = phosphorothioate bond; note (original language) = 硫代磷酸酯键
  modified_base 21..23: mod_base = OTHER; note = phosphorothioate bond; note (original language) = 硫代磷酸酯键
  modified_base 1: mod_base = OTHER; note = 2'-acetamido-5'-vinyl phosphonate nucleoside; note (original language) = 2'-乙酰氨基-5'-乙烯基膦酸核苷
  source 1..23: mol_type = other RNA
tttagaccaaggagaaacggctg

SEQ ID NO: 675 - RNA, 23 nt, synthetic construct
  modified_base 3..5: mod_base = OTHER; note = 2'-methoxy nucleoside; note (original language) = 2'-甲氧基核苷
  modified_base 7..13: mod_base = OTHER; note = 2'-methoxy nucleoside; note (original language) = 2'-甲氧基核苷
  modified_base 15: mod_base = OTHER; note = 2'-methoxy nucleoside; note (original language) = 2'-甲氧基核苷
  modified_base 17..23: mod_base = OTHER; note = 2'-methoxy nucleoside; note (original language) = 2'-甲氧基核苷
  modified_base 2: mod_base = OTHER; note = 2'-fluoro nucleoside; note (original language) = 2'-氟核苷
  modified_base 6: mod_base = OTHER; note = 2'-fluoro nucleoside; note (original language) = 2'-氟核苷
  modified_base 14: mod_base = OTHER; note = 2'-fluoro nucleoside; note (original language) = 2'-氟核苷
  modified_base 16: mod_base = OTHER; note = 2'-fluoro nucleoside; note (original language) = 2'-氟核苷
  modified_base 1..3: mod_base = OTHER; note = phosphorothioate bond; note (original language) = 硫代磷酸酯键
  modified_base 21..23: mod_base = OTHER; note = phosphorothioate bond; note (original language) = 硫代磷酸酯键
  modified_base 1: mod_base = OTHER; note = 2'-acetamido-5'-vinyl phosphonate nucleoside; note (original language) = 2'-乙酰氨基-5'-乙烯基膦酸核苷
  source 1..23: mol_type = other RNA
tcttagaccaaggagaaacgcct

SEQ ID NO: 676 - RNA, 23 nt, synthetic construct
  modified_base 3..5: mod_base = OTHER; note = 2'-methoxy nucleoside; note (original language) = 2'-甲氧基核苷
  modified_base 7..13: mod_base = OTHER; note = 2'-methoxy nucleoside; note (original language) = 2'-甲氧基核苷
  modified_base 15: mod_base = OTHER; note = 2'-methoxy nucleoside; note (original language) = 2'-甲氧基核苷
  modified_base 17..23: mod_base = OTHER; note = 2'-methoxy nucleoside; note (original language) = 2'-甲氧基核苷
  modified_base 2: mod_base = OTHER; note = 2'-fluoro nucleoside; note (original language) = 2'-氟核苷
  modified_base 6: mod_base = OTHER; note = 2'-fluoro nucleoside; note (original language) = 2'-氟核苷
  modified_base 14: mod_base = OTHER; note = 2'-fluoro nucleoside; note (original language) = 2'-氟核苷
  modified_base 16: mod_base = OTHER; note = 2'-fluoro nucleoside; note (original language) = 2'-氟核苷
  modified_base 1..3: mod_base = OTHER; note = phosphorothioate bond; note (original language) = 硫代磷酸酯键
  modified_base 21..23: mod_base = OTHER; note = phosphorothioate bond; note (original language) = 硫代磷酸酯键
  modified_base 1: mod_base = OTHER; note = 2'-acetamido-5'-vinyl phosphonate nucleoside; note (original language) = 2'-乙酰氨基-5'-乙烯基膦酸核苷
  source 1..23: mol_type = other RNA
tcttagaccaaggagaaacggct

SEQ ID NO: 677 - RNA, 23 nt, synthetic construct
  modified_base 1: mod_base = OTHER; note = 2'-methoxy nucleoside; note (original language) = 2'-甲氧基核苷
  modified_base 3..5: mod_base = OTHER; note = 2'-methoxy nucleoside; note (original language) = 2'-甲氧基核苷
  modified_base 7..13: mod_base = OTHER; note = 2'-methoxy nucleoside; note (original language) = 2'-甲氧基核苷
  modified_base 15: mod_base = OTHER; note = 2'-methoxy nucleoside; note (original language) = 2'-甲氧基核苷
  modified_base 17..23: mod_base = OTHER; note = 2'-methoxy nucleoside; note (original language) = 2'-甲氧基核苷
  modified_base 2: mod_base = OTHER; note = 2'-fluoro nucleoside; note (original language) = 2'-氟核苷
  modified_base 14: mod_base = OTHER; note = 2'-fluoro nucleoside; note (original language) = 2'-氟核苷
  modified_base 16: mod_base = OTHER; note = 2'-fluoro nucleoside; note (original language) = 2'-氟核苷
  modified_base 1..3: mod_base = OTHER; note = phosphorothioate bond; note (original language) = 硫代磷酸酯键
  modified_base 21..23: mod_base = OTHER; note = phosphorothioate bond; note (original language) = 硫代磷酸酯键
  modified_base 6: mod_base = OTHER; note = 2,3-dihydroxypropyl nucleoside; note (original language) = 2,3-二羟丙基核苷
  modified_base 6: mod_base = OTHER; note = thymine; note (original language) = 胸腺嘧啶
  source 1..23: mol_type = other RNA
tgtactctcattgtggatgacga

SEQ ID NO: 678 - RNA, 23 nt, synthetic construct
  modified_base 1: mod_base = OTHER; note = 2'-methoxy nucleoside; note (original language) = 2'-甲氧基核苷
  modified_base 3..5: mod_base = OTHER; note = 2'-methoxy nucleoside; note (original language) = 2'-甲氧基核苷
  modified_base 7..13: mod_base = OTHER; note = 2'-methoxy nucleoside; note (original language) = 2'-甲氧基核苷
  modified_base 15: mod_base = OTHER; note = 2'-methoxy nucleoside; note (original language) = 2'-甲氧基核苷
  modified_base 17..23: mod_base = OTHER; note = 2'-methoxy nucleoside; note (original language) = 2'-甲氧基核苷
  modified_base 2: mod_base = OTHER; note = 2'-fluoro nucleoside; note (original language) = 2'-氟核苷
  modified_base 6: mod_base = OTHER; note = 2'-fluoro nucleoside; note (original language) = 2'-氟核苷
  modified_base 14: mod_base = OTHER; note = 2'-fluoro nucleoside; note (original language) = 2'-氟核苷
  modified_base 16: mod_base = OTHER; note = 2'-fluoro nucleoside; note (original language) = 2'-氟核苷
  modified_base 1..3: mod_base = OTHER; note = phosphorothioate bond; note (original language) = 硫代磷酸酯键
  modified_base 21..23: mod_base = OTHER; note = phosphorothioate bond; note (original language) = 硫代磷酸酯键
  modified_base 1: mod_base = OTHER; note = 2'-methoxy-5'-vinyl phosphonate nucleoside; note (original language) = 2'-甲氧基-5'-乙烯基膦酸核苷
  source 1..23: mol_type = other RNA
ttagaccaaggagaaacggccgc

SEQ ID NO: 679 - RNA, 23 nt, synthetic construct
  modified_base 1: mod_base = OTHER; note = 2'-methoxy nucleoside; note (original language) = 2'-甲氧基核苷
  modified_base 3..5: mod_base = OTHER; note = 2'-methoxy nucleoside; note (original language) = 2'-甲氧基核苷
  modified_base 7..13: mod_base = OTHER; note = 2'-methoxy nucleoside; note (original language) = 2'-甲氧基核苷
  modified_base 15: mod_base = OTHER; note = 2'-methoxy nucleoside; note (original language) = 2'-甲氧基核苷
  modified_base 17..23: mod_base = OTHER; note = 2'-methoxy nucleoside; note (original language) = 2'-甲氧基核苷
  modified_base 2: mod_base = OTHER; note = 2'-fluoro nucleoside; note (original language) = 2'-氟核苷
  modified_base 6: mod_base = OTHER; note = 2'-fluoro nucleoside; note (original language) = 2'-氟核苷
  modified_base 14: mod_base = OTHER; note = 2'-fluoro nucleoside; note (original language) = 2'-氟核苷
  modified_base 16: mod_base = OTHER; note = 2'-fluoro nucleoside; note (original language) = 2'-氟核苷
  modified_base 1..3: mod_base = OTHER; note = phosphorothioate bond; note (original language) = 硫代磷酸酯键
  modified_base 21..23: mod_base = OTHER; note = phosphorothioate bond; note (original language) = 硫代磷酸酯键
  modified_base 1: mod_base = OTHER; note = 2'-methoxy-5'-vinyl phosphonate nucleoside; note (original language) = 2'-甲氧基-5'-乙烯基膦酸核苷
  source 1..23: mol_type = other RNA
tttagaccaaggagaaacggctg

SEQ ID NO: 680 - RNA, 23 nt, synthetic construct
  modified_base 1: mod_base = OTHER; note = 2'-methoxy nucleoside; note (original language) = 2'-甲氧基核苷
  modified_base 3..5: mod_base = OTHER; note = 2'-methoxy nucleoside; note (original language) = 2'-甲氧基核苷
  modified_base 7..13: mod_base = OTHER; note = 2'-methoxy nucleoside; note (original language) = 2'-甲氧基核苷
  modified_base 15: mod_base = OTHER; note = 2'-methoxy nucleoside; note (original language) = 2'-甲氧基核苷
  modified_base 17..23: mod_base = OTHER; note = 2'-methoxy nucleoside; note (original language) = 2'-甲氧基核苷
  modified_base 2: mod_base = OTHER; note = 2'-fluoro nucleoside; note (original language) = 2'-氟核苷
  modified_base 6: mod_base = OTHER; note = 2'-fluoro nucleoside; note (original language) = 2'-氟核苷
  modified_base 14: mod_base = OTHER; note = 2'-fluoro nucleoside; note (original language) = 2'-氟核苷
  modified_base 16: mod_base = OTHER; note = 2'-fluoro nucleoside; note (original language) = 2'-氟核苷
  modified_base 1..3: mod_base = OTHER; note = phosphorothioate bond; note (original language) = 硫代磷酸酯键
  modified_base 21..23: mod_base = OTHER; note = phosphorothioate bond; note (original language) = 硫代磷酸酯键
  modified_base 1: mod_base = OTHER; note = 2'-methoxy-5'-vinyl phosphonate nucleoside; note (original language) = 2'-甲氧基-5'-乙烯基膦酸核苷
  source 1..23: mol_type = other RNA
tcttagaccaaggagaaacgcct

SEQ ID NO: 681 - RNA, 23 nt, synthetic construct
  modified_base 1: mod_base = OTHER; note = 2'-methoxy nucleoside; note (original language) = 2'-甲氧基核苷
  modified_base 3..5: mod_base = OTHER; note = 2'-methoxy nucleoside; note (original language) = 2'-甲氧基核苷
  modified_base 7..13: mod_base = OTHER; note = 2'-methoxy nucleoside; note (original language) = 2'-甲氧基核苷
  modified_base 15: mod_base = OTHER; note = 2'-methoxy nucleoside; note (original language) = 2'-甲氧基核苷
  modified_base 17..23: mod_base = OTHER; note = 2'-methoxy nucleoside; note (original language) = 2'-甲氧基核苷
  modified_base 2: mod_base = OTHER; note = 2'-fluoro nucleoside; note (original language) = 2'-氟核苷
  modified_base 6: mod_base = OTHER; note = 2'-fluoro nucleoside; note (original language) = 2'-氟核苷
  modified_base 14: mod_base = OTHER; note = 2'-fluoro nucleoside; note (original language) = 2'-氟核苷
  modified_base 16: mod_base = OTHER; note = 2'-fluoro nucleoside; note (original language) = 2'-氟核苷
  modified_base 1..3: mod_base = OTHER; note = phosphorothioate bond; note (original language) = 硫代磷酸酯键
  modified_base 21..23: mod_base = OTHER; note = phosphorothioate bond; note (original language) = 硫代磷酸酯键
  modified_base 1: mod_base = OTHER; note = 2'-methoxy-5'-vinyl phosphonate nucleoside; note (original language) = 2'-甲氧基-5'-乙烯基膦酸核苷
  source 1..23: mol_type = other RNA
tcttagaccaaggagaaacggct

SEQ ID NO: 682 - RNA, 21 nt, synthetic construct
  modified_base 1: mod_base = OTHER; note = 2'-methoxy nucleoside; note (original language) = 2'-甲氧基核苷
  modified_base 3..5: mod_base = OTHER; note = 2'-methoxy nucleoside; note (original language) = 2'-甲氧基核苷
  modified_base 7..13: mod_base = OTHER; note = 2'-methoxy nucleoside; note (original language) = 2'-甲氧基核苷
  modified_base 15: mod_base = OTHER; note = 2'-methoxy nucleoside; note (original language) = 2'-甲氧基核苷
  modified_base 17..21: mod_base = OTHER; note = 2'-methoxy nucleoside; note (original language) = 2'-甲氧基核苷
  modified_base 2: mod_base = OTHER; note = 2'-fluoro nucleoside; note (original language) = 2'-氟核苷
  modified_base 6: mod_base = OTHER; note = 2'-fluoro nucleoside; note (original language) = 2'-氟核苷
  modified_base 14: mod_base = OTHER; note = 2'-fluoro nucleoside; note (original language) = 2'-氟核苷
  modified_base 16: mod_base = OTHER; note = 2'-fluoro nucleoside; note (original language) = 2'-氟核苷
  modified_base 1..3: mod_base = OTHER; note = phosphorothioate bond; note (original language) = 硫代磷酸酯键
  modified_base 19..21: mod_base = OTHER; note = phosphorothioate bond; note (original language) = 硫代磷酸酯键
  source 1..21: mol_type = other RNA
aaacagaaattcaggtgcttg

SEQ ID NO: 683 - RNA, 21 nt, synthetic construct
  modified_base 1: mod_base = OTHER; note = 2'-methoxy nucleoside; note (original language) = 2'-甲氧基核苷
  modified_base 3..5: mod_base = OTHER; note = 2'-methoxy nucleoside; note (original language) = 2'-甲氧基核苷
  modified_base 7..13: mod_base = OTHER; note = 2'-methoxy nucleoside; note (original language) = 2'-甲氧基核苷
  modified_base 15: mod_base = OTHER; note = 2'-methoxy nucleoside; note (original language) = 2'-甲氧基核苷
  modified_base 17..21: mod_base = OTHER; note = 2'-methoxy nucleoside; note (original language) = 2'-甲氧基核苷
  modified_base 2: mod_base = OTHER; note = 2'-fluoro nucleoside; note (original language) = 2'-氟核苷
  modified_base 6: mod_base = OTHER; note = 2'-fluoro nucleoside; note (original language) = 2'-氟核苷
  modified_base 14: mod_base = OTHER; note = 2'-fluoro nucleoside; note (original language) = 2'-氟核苷
  modified_base 16: mod_base = OTHER; note = 2'-fluoro nucleoside; note (original language) = 2'-氟核苷
  modified_base 1..3: mod_base = OTHER; note = phosphorothioate bond; note (original language) = 硫代磷酸酯键
  modified_base 19..21: mod_base = OTHER; note = phosphorothioate bond; note (original language) = 硫代磷酸酯键
  source 1..21: mol_type = other RNA
aaactaaggtattacagacac

SEQ ID NO: 684 - RNA, 21 nt, synthetic construct
  modified_base 1: mod_base = OTHER; note = 2'-methoxy nucleoside; note (original language) = 2'-甲氧基核苷
  modified_base 3..5: mod_base = OTHER; note = 2'-methoxy nucleoside; note (original language) = 2'-甲氧基核苷
  modified_base 7..13: mod_base = OTHER; note = 2'-methoxy nucleoside; note (original language) = 2'-甲氧基核苷
  modified_base 15: mod_base = OTHER; note = 2'-methoxy nucleoside; note (original language) = 2'-甲氧基核苷
  modified_base 17..21: mod_base = OTHER; note = 2'-methoxy nucleoside; note (original language) = 2'-甲氧基核苷
  modified_base 2: mod_base = OTHER; note = 2'-fluoro nucleoside; note (original language) = 2'-氟核苷
  modified_base 6: mod_base = OTHER; note = 2'-fluoro nucleoside; note (original language) = 2'-氟核苷
  modified_base 14: mod_base = OTHER; note = 2'-fluoro nucleoside; note (original language) = 2'-氟核苷
  modified_base 16: mod_base = OTHER; note = 2'-fluoro nucleoside; note (original language) = 2'-氟核苷
  modified_base 1..3: mod_base = OTHER; note = phosphorothioate bond; note (original language) = 硫代磷酸酯键
  modified_base 19..21: mod_base = OTHER; note = phosphorothioate bond; note (original language) = 硫代磷酸酯键
  source 1..21: mol_type = other RNA
aaactgggaggtgcatttgtg

SEQ ID NO: 685 - RNA, 21 nt, synthetic construct
  modified_base 1: mod_base = OTHER; note = 2'-methoxy nucleoside; note (original language) = 2'-甲氧基核苷
  modified_base 3..5: mod_base = OTHER; note = 2'-methoxy nucleoside; note (original language) = 2'-甲氧基核苷
  modified_base 7..13: mod_base = OTHER; note = 2'-methoxy nucleoside; note (original language) = 2'-甲氧基核苷
  modified_base 15: mod_base = OTHER; note = 2'-methoxy nucleoside; note (original language) = 2'-甲氧基核苷
  modified_base 17..21: mod_base = OTHER; note = 2'-methoxy nucleoside; note (original language) = 2'-甲氧基核苷
  modified_base 2: mod_base = OTHER; note = 2'-fluoro nucleoside; note (original language) = 2'-氟核苷
  modified_base 6: mod_base = OTHER; note = 2'-fluoro nucleoside; note (original language) = 2'-氟核苷
  modified_base 14: mod_base = OTHER; note = 2'-fluoro nucleoside; note (original language) = 2'-氟核苷
  modified_base 16: mod_base = OTHER; note = 2'-fluoro nucleoside; note (original language) = 2'-氟核苷
  modified_base 1..3: mod_base = OTHER; note = phosphorothioate bond; note (original language) = 硫代磷酸酯键
  modified_base 19..21: mod_base = OTHER; note = phosphorothioate bond; note (original language) = 硫代磷酸酯键
  source 1..21: mol_type = other RNA
aaagccagggtgctgtccaca

SEQ ID NO: 686 - RNA, 21 nt, synthetic construct
  modified_base 1: mod_base = OTHER; note = 2'-methoxy nucleoside; note (original language) = 2'-甲氧基核苷
  modified_base 3..5: mod_base = OTHER; note = 2'-methoxy nucleoside; note (original language) = 2'-甲氧基核苷
  modified_base 7..13: mod_base = OTHER; note = 2'-methoxy nucleoside; note (original language) = 2'-甲氧基核苷
  modified_base 15: mod_base = OTHER; note = 2'-methoxy nucleoside; note (original language) = 2'-甲氧基核苷
  modified_base 17..21: mod_base = OTHER; note = 2'-methoxy nucleoside; note (original language) = 2'-甲氧基核苷
  modified_base 2: mod_base = OTHER; note = 2'-fluoro nucleoside; note (original language) = 2'-氟核苷
  modified_base 6: mod_base = OTHER; note = 2'-fluoro nucleoside; note (original language) = 2'-氟核苷
  modified_base 14: mod_base = OTHER; note = 2'-fluoro nucleoside; note (original language) = 2'-氟核苷
  modified_base 16: mod_base = OTHER; note = 2'-fluoro nucleoside; note (original language) = 2'-氟核苷
  modified_base 1..3: mod_base = OTHER; note = phosphorothioate bond; note (original language) = 硫代磷酸酯键
  modified_base 19..21: mod_base = OTHER; note = phosphorothioate bond; note (original language) = 硫代磷酸酯键
  source 1..21: mol_type = other RNA
aaagtcgactcattagaagaa

SEQ ID NO: 687 - RNA, 21 nt, synthetic construct
  modified_base 1: mod_base = OTHER; note = 2'-methoxy nucleoside; note (original language) = 2'-甲氧基核苷
  modified_base 3..5: mod_base = OTHER; note = 2'-methoxy nucleoside; note (original language) = 2'-甲氧基核苷
  modified_base 7..13: mod_base = OTHER; note = 2'-methoxy nucleoside; note (original language) = 2'-甲氧基核苷
  modified_base 15: mod_base = OTHER; note = 2'-methoxy nucleoside; note (original language) = 2'-甲氧基核苷
  modified_base 17..21: mod_base = OTHER; note = 2'-methoxy nucleoside; note (original language) = 2'-甲氧基核苷
  modified_base 2: mod_base = OTHER; note = 2'-fluoro nucleoside; note (original language) = 2'-氟核苷
  modified_base 6: mod_base = OTHER; note = 2'-fluoro nucleoside; note (original language) = 2'-氟核苷
  modified_base 14: mod_base = OTHER; note = 2'-fluoro nucleoside; note (original language) = 2'-氟核苷
  modified_base 16: mod_base = OTHER; note = 2'-fluoro nucleoside; note (original language) = 2'-氟核苷
  modified_base 1..3: mod_base = OTHER; note = phosphorothioate bond; note (original language) = 硫代磷酸酯键
  modified_base 19..21: mod_base = OTHER; note = phosphorothioate bond; note (original language) = 硫代磷酸酯键
  source 1..21: mol_type = other RNA
aaagtgagaccctccaccttg

SEQ ID NO: 688 - RNA, 21 nt, synthetic construct
  modified_base 1: mod_base = OTHER; note = 2'-methoxy nucleoside; note (original language) = 2'-甲氧基核苷
  modified_base 3..5: mod_base = OTHER; note = 2'-methoxy nucleoside; note (original language) = 2'-甲氧基核苷
  modified_base 7..13: mod_base = OTHER; note = 2'-methoxy nucleoside; note (original language) = 2'-甲氧基核苷
  modified_base 15: mod_base = OTHER; note = 2'-methoxy nucleoside; note (original language) = 2'-甲氧基核苷
  modified_base 17..21: mod_base = OTHER; note = 2'-methoxy nucleoside; note (original language) = 2'-甲氧基核苷
  modified_base 2: mod_base = OTHER; note = 2'-fluoro nucleoside; note (original language) = 2'-氟核苷
  modified_base 6: mod_base = OTHER; note = 2'-fluoro nucleoside; note (original language) = 2'-氟核苷
  modified_base 14: mod_base = OTHER; note = 2'-fluoro nucleoside; note (original language) = 2'-氟核苷
  modified_base 16: mod_base = OTHER; note = 2'-fluoro nucleoside; note (original language) = 2'-氟核苷
  modified_base 1..3: mod_base = OTHER; note = phosphorothioate bond; note (original language) = 硫代磷酸酯键
  modified_base 19..21: mod_base = OTHER; note = phosphorothioate bond; note (original language) = 硫代磷酸酯键
  source 1..21: mol_type = other RNA
aaataaccagctatggttccg

SEQ ID NO: 689 - RNA, 21 nt, synthetic construct
  modified_base 1: mod_base = OTHER; note = 2'-methoxy nucleoside; note (original language) = 2'-甲氧基核苷
  modified_base 3..5: mod_base = OTHER; note = 2'-methoxy nucleoside; note (original language) = 2'-甲氧基核苷
  modified_base 7..13: mod_base = OTHER; note = 2'-methoxy nucleoside; note (original language) = 2'-甲氧基核苷
  modified_base 15: mod_base = OTHER; note = 2'-methoxy nucleoside; note (original language) = 2'-甲氧基核苷
  modified_base 17..21: mod_base = OTHER; note = 2'-methoxy nucleoside; note (original language) = 2'-甲氧基核苷
  modified_base 2: mod_base = OTHER; note = 2'-fluoro nucleoside; note (original language) = 2'-氟核苷
  modified_base 6: mod_base = OTHER; note = 2'-fluoro nucleoside; note (original language) = 2'-氟核苷
  modified_base 14: mod_base = OTHER; note = 2'-fluoro nucleoside; note (original language) = 2'-氟核苷
  modified_base 16: mod_base = OTHER; note = 2'-fluoro nucleoside; note (original language) = 2'-氟核苷
  modified_base 1..3: mod_base = OTHER; note = phosphorothioate bond; note (original language) = 硫代磷酸酯键
  modified_base 19..21: mod_base = OTHER; note = phosphorothioate bond; note (original language) = 硫代磷酸酯键
  source 1..21: mol_type = other RNA
aaatacaaaccgaaggcaatg

SEQ ID NO: 690 - RNA, 21 nt, synthetic construct
  modified_base 1: mod_base = OTHER; note = 2'-methoxy nucleoside; note (original language) = 2'-甲氧基核苷
  modified_base 3..5: mod_base = OTHER; note = 2'-methoxy nucleoside; note (original language) = 2'-甲氧基核苷
  modified_base 7..13: mod_base = OTHER; note = 2'-methoxy nucleoside; note (original language) = 2'-甲氧基核苷
  modified_base 15: mod_base = OTHER; note = 2'-methoxy nucleoside; note (original language) = 2'-甲氧基核苷
  modified_base 17..21: mod_base = OTHER; note = 2'-methoxy nucleoside; note (original language) = 2'-甲氧基核苷
  modified_base 2: mod_base = OTHER; note = 2'-fluoro nucleoside; note (original language) = 2'-氟核苷
  modified_base 6: mod_base = OTHER; note = 2'-fluoro nucleoside; note (original language) = 2'-氟核苷
  modified_base 14: mod_base = OTHER; note = 2'-fluoro nucleoside; note (original language) = 2'-氟核苷
  modified_base 16: mod_base = OTHER; note = 2'-fluoro nucleoside; note (original language) = 2'-氟核苷
  modified_base 1..3: mod_base = OTHER; note = phosphorothioate bond; note (original language) = 硫代磷酸酯键
  modified_base 19..21: mod_base = OTHER; note = phosphorothioate bond; note (original language) = 硫代磷酸酯键
  source 1..21: mol_type = other RNA
aagacactaaatacaaaccga

SEQ ID NO: 691 - RNA, 21 nt, synthetic construct
  modified_base 1: mod_base = OTHER; note = 2'-methoxy nucleoside; note (original language) = 2'-甲氧基核苷
  modified_base 3..5: mod_base = OTHER; note = 2'-methoxy nucleoside; note (original language) = 2'-甲氧基核苷
  modified_base 7..13: mod_base = OTHER; note = 2'-methoxy nucleoside; note (original language) = 2'-甲氧基核苷
  modified_base 15: mod_base = OTHER; note = 2'-methoxy nucleoside; note (original language) = 2'-甲氧基核苷
  modified_base 17..21: mod_base = OTHER; note = 2'-methoxy nucleoside; note (original language) = 2'-甲氧基核苷
  modified_base 2: mod_base = OTHER; note = 2'-fluoro nucleoside; note (original language) = 2'-氟核苷
  modified_base 6: mod_base = OTHER; note = 2'-fluoro nucleoside; note (original language) = 2'-氟核苷
  modified_base 14: mod_base = OTHER; note = 2'-fluoro nucleoside; note (original language) = 2'-氟核苷
  modified_base 16: mod_base = OTHER; note = 2'-fluoro nucleoside; note (original language) = 2'-氟核苷
  modified_base 1..3: mod_base = OTHER; note = phosphorothioate bond; note (original language) = 硫代磷酸酯键
  modified_base 19..21: mod_base = OTHER; note = phosphorothioate bond; note (original language) = 硫代磷酸酯键
  source 1..21: mol_type = other RNA
aatttttgttctcaacttgaa

SEQ ID NO: 692 - RNA, 21 nt, synthetic construct
  modified_base 1: mod_base = OTHER; note = 2'-methoxy nucleoside; note (original language) = 2'-甲氧基核苷
  modified_base 3..5: mod_base = OTHER; note = 2'-methoxy nucleoside; note (original language) = 2'-甲氧基核苷
  modified_base 7..13: mod_base = OTHER; note = 2'-methoxy nucleoside; note (original language) = 2'-甲氧基核苷
  modified_base 15: mod_base = OTHER; note = 2'-methoxy nucleoside; note (original language) = 2'-甲氧基核苷
  modified_base 17..21: mod_base = OTHER; note = 2'-methoxy nucleoside; note (original language) = 2'-甲氧基核苷
  modified_base 2: mod_base = OTHER; note = 2'-fluoro nucleoside; note (original language) = 2'-氟核苷
  modified_base 6: mod_base = OTHER; note = 2'-fluoro nucleoside; note (original language) = 2'-氟核苷
  modified_base 14: mod_base = OTHER; note = 2'-fluoro nucleoside; note (original language) = 2'-氟核苷
  modified_base 16: mod_base = OTHER; note = 2'-fluoro nucleoside; note (original language) = 2'-氟核苷
  modified_base 1..3: mod_base = OTHER; note = phosphorothioate bond; note (original language) = 硫代磷酸酯键
  modified_base 19..21: mod_base = OTHER; note = phosphorothioate bond; note (original language) = 硫代磷酸酯键
  source 1..21: mol_type = other RNA
acttttttgtttcacaaacaa

SEQ ID NO: 693 - RNA, 21 nt, synthetic construct
  modified_base 1: mod_base = OTHER; note = 2'-methoxy nucleoside; note (original language) = 2'-甲氧基核苷
  modified_base 3..5: mod_base = OTHER; note = 2'-methoxy nucleoside; note (original language) = 2'-甲氧基核苷
  modified_base 7..13: mod_base = OTHER; note = 2'-methoxy nucleoside; note (original language) = 2'-甲氧基核苷
  modified_base 15: mod_base = OTHER; note = 2'-methoxy nucleoside; note (original language) = 2'-甲氧基核苷
  modified_base 17..21: mod_base = OTHER; note = 2'-methoxy nucleoside; note (original language) = 2'-甲氧基核苷
  modified_base 2: mod_base = OTHER; note = 2'-fluoro nucleoside; note (original language) = 2'-氟核苷
  modified_base 6: mod_base = OTHER; note = 2'-fluoro nucleoside; note (original language) = 2'-氟核苷
  modified_base 14: mod_base = OTHER; note = 2'-fluoro nucleoside; note (original language) = 2'-氟核苷
  modified_base 16: mod_base = OTHER; note = 2'-fluoro nucleoside; note (original language) = 2'-氟核苷
  modified_base 1..3: mod_base = OTHER; note = phosphorothioate bond; note (original language) = 硫代磷酸酯键
  modified_base 19..21: mod_base = OTHER; note = phosphorothioate bond; note (original language) = 硫代磷酸酯键
  source 1..21: mol_type = other RNA
agaccctccaccttgtccagg

SEQ ID NO: 694 - RNA, 21 nt, synthetic construct
  modified_base 1: mod_base = OTHER; note = 2'-methoxy nucleoside; note (original language) = 2'-甲氧基核苷
  modified_base 3..5: mod_base = OTHER; note = 2'-methoxy nucleoside; note (original language) = 2'-甲氧基核苷
  modified_base 7..13: mod_base = OTHER; note = 2'-methoxy nucleoside; note (original language) = 2'-甲氧基核苷
  modified_base 15: mod_base = OTHER; note = 2'-methoxy nucleoside; note (original language) = 2'-甲氧基核苷
  modified_base 17..21: mod_base = OTHER; note = 2'-methoxy nucleoside; note (original language) = 2'-甲氧基核苷
  modified_base 2: mod_base = OTHER; note = 2'-fluoro nucleoside; note (original language) = 2'-氟核苷
  modified_base 6: mod_base = OTHER; note = 2'-fluoro nucleoside; note (original language) = 2'-氟核苷
  modified_base 14: mod_base = OTHER; note = 2'-fluoro nucleoside; note (original language) = 2'-氟核苷
  modified_base 16: mod_base = OTHER; note = 2'-fluoro nucleoside; note (original language) = 2'-氟核苷
  modified_base 1..3: mod_base = OTHER; note = phosphorothioate bond; note (original language) = 硫代磷酸酯键
  modified_base 19..21: mod_base = OTHER; note = phosphorothioate bond; note (original language) = 硫代磷酸酯键
  source 1..21: mol_type = other RNA
agttttgctggaaagtgagac

SEQ ID NO: 695 - RNA, 21 nt, synthetic construct
  modified_base 1: mod_base = OTHER; note = 2'-methoxy nucleoside; note (original language) = 2'-甲氧基核苷
  modified_base 3..5: mod_base = OTHER; note = 2'-methoxy nucleoside; note (original language) = 2'-甲氧基核苷
  modified_base 7..13: mod_base = OTHER; note = 2'-methoxy nucleoside; note (original language) = 2'-甲氧基核苷
  modified_base 15: mod_base = OTHER; note = 2'-methoxy nucleoside; note (original language) = 2'-甲氧基核苷
  modified_base 17..21: mod_base = OTHER; note = 2'-methoxy nucleoside; note (original language) = 2'-甲氧基核苷
  modified_base 2: mod_base = OTHER; note = 2'-fluoro nucleoside; note (original language) = 2'-氟核苷
  modified_base 6: mod_base = OTHER; note = 2'-fluoro nucleoside; note (original language) = 2'-氟核苷
  modified_base 14: mod_base = OTHER; note = 2'-fluoro nucleoside; note (original language) = 2'-氟核苷
  modified_base 16: mod_base = OTHER; note = 2'-fluoro nucleoside; note (original language) = 2'-氟核苷
  modified_base 1..3: mod_base = OTHER; note = phosphorothioate bond; note (original language) = 硫代磷酸酯键
  modified_base 19..21: mod_base = OTHER; note = phosphorothioate bond; note (original language) = 硫代磷酸酯键
  source 1..21: mol_type = other RNA
atacggaagcccaagaagttg

SEQ ID NO: 696 - RNA, 21 nt, synthetic construct
  modified_base 1: mod_base = OTHER; note = 2'-methoxy nucleoside; note (original language) = 2'-甲氧基核苷
  modified_base 3..5: mod_base = OTHER; note = 2'-methoxy nucleoside; note (original language) = 2'-甲氧基核苷
  modified_base 7..13: mod_base = OTHER; note = 2'-methoxy nucleoside; note (original language) = 2'-甲氧基核苷
  modified_base 15: mod_base = OTHER; note = 2'-methoxy nucleoside; note (original language) = 2'-甲氧基核苷
  modified_base 17..21: mod_base = OTHER; note = 2'-methoxy nucleoside; note (original language) = 2'-甲氧基核苷
  modified_base 2: mod_base = OTHER; note = 2'-fluoro nucleoside; note (original language) = 2'-氟核苷
  modified_base 6: mod_base = OTHER; note = 2'-fluoro nucleoside; note (original language) = 2'-氟核苷
  modified_base 14: mod_base = OTHER; note = 2'-fluoro nucleoside; note (original language) = 2'-氟核苷
  modified_base 16: mod_base = OTHER; note = 2'-fluoro nucleoside; note (original language) = 2'-氟核苷
  modified_base 1..3: mod_base = OTHER; note = phosphorothioate bond; note (original language) = 硫代磷酸酯键
  modified_base 19..21: mod_base = OTHER; note = phosphorothioate bond; note (original language) = 硫代磷酸酯键
  source 1..21: mol_type = other RNA
atgttcttacattcaagacac

SEQ ID NO: 697 - RNA, 21 nt, synthetic construct
  modified_base 1: mod_base = OTHER; note = 2'-methoxy nucleoside; note (original language) = 2'-甲氧基核苷
  modified_base 3..5: mod_base = OTHER; note = 2'-methoxy nucleoside; note (original language) = 2'-甲氧基核苷
  modified_base 7..13: mod_base = OTHER; note = 2'-methoxy nucleoside; note (original language) = 2'-甲氧基核苷
  modified_base 15: mod_base = OTHER; note = 2'-methoxy nucleoside; note (original language) = 2'-甲氧基核苷
  modified_base 17..21: mod_base = OTHER; note = 2'-methoxy nucleoside; note (original language) = 2'-甲氧基核苷
  modified_base 2: mod_base = OTHER; note = 2'-fluoro nucleoside; note (original language) = 2'-氟核苷
  modified_base 6: mod_base = OTHER; note = 2'-fluoro nucleoside; note (original language) = 2'-氟核苷
  modified_base 14: mod_base = OTHER; note = 2'-fluoro nucleoside; note (original language) = 2'-氟核苷
  modified_base 16: mod_base = OTHER; note = 2'-fluoro nucleoside; note (original language) = 2'-氟核苷
  modified_base 1..3: mod_base = OTHER; note = phosphorothioate bond; note (original language) = 硫代磷酸酯键
  modified_base 19..21: mod_base = OTHER; note = phosphorothioate bond; note (original language) = 硫代磷酸酯键
  source 1..21: mol_type = other RNA
catacacagcaaacaggaatg

SEQ ID NO: 698 - RNA, 21 nt, synthetic construct
  modified_base 1: mod_base = OTHER; note = 2'-methoxy nucleoside; note (original language) = 2'-甲氧基核苷
  modified_base 3..5: mod_base = OTHER; note = 2'-methoxy nucleoside; note (original language) = 2'-甲氧基核苷
  modified_base 7..13: mod_base = OTHER; note = 2'-methoxy nucleoside; note (original language) = 2'-甲氧基核苷
  modified_base 15: mod_base = OTHER; note = 2'-methoxy nucleoside; note (original language) = 2'-甲氧基核苷
  modified_base 17..21: mod_base = OTHER; note = 2'-methoxy nucleoside; note (original language) = 2'-甲氧基核苷
  modified_base 2: mod_base = OTHER; note = 2'-fluoro nucleoside; note (original language) = 2'-氟核苷
  modified_base 6: mod_base = OTHER; note = 2'-fluoro nucleoside; note (original language) = 2'-氟核苷
  modified_base 14: mod_base = OTHER; note = 2'-fluoro nucleoside; note (original language) = 2'-氟核苷
  modified_base 16: mod_base = OTHER; note = 2'-fluoro nucleoside; note (original language) = 2'-氟核苷
  modified_base 1..3: mod_base = OTHER; note = phosphorothioate bond; note (original language) = 硫代磷酸酯键
  modified_base 19..21: mod_base = OTHER; note = phosphorothioate bond; note (original language) = 硫代磷酸酯键
  source 1..21: mol_type = other RNA
ctaaacactggttcttgcctc

SEQ ID NO: 699 - RNA, 21 nt, synthetic construct
  modified_base 1: mod_base = OTHER; note = 2'-methoxy nucleoside; note (original language) = 2'-甲氧基核苷
  modified_base 3..5: mod_base = OTHER; note = 2'-methoxy nucleoside; note (original language) = 2'-甲氧基核苷
  modified_base 7..13: mod_base = OTHER; note = 2'-methoxy nucleoside; note (original language) = 2'-甲氧基核苷
  modified_base 15: mod_base = OTHER; note = 2'-methoxy nucleoside; note (original language) = 2'-甲氧基核苷
  modified_base 17..21: mod_base = OTHER; note = 2'-methoxy nucleoside; note (original language) = 2'-甲氧基核苷
  modified_base 2: mod_base = OTHER; note = 2'-fluoro nucleoside; note (original language) = 2'-氟核苷
  modified_base 6: mod_base = OTHER; note = 2'-fluoro nucleoside; note (original language) = 2'-氟核苷
  modified_base 14: mod_base = OTHER; note = 2'-fluoro nucleoside; note (original language) = 2'-氟核苷
  modified_base 16: mod_base = OTHER; note = 2'-fluoro nucleoside; note (original language) = 2'-氟核苷
  modified_base 1..3: mod_base = OTHER; note = phosphorothioate bond; note (original language) = 硫代磷酸酯键
  modified_base 19..21: mod_base = OTHER; note = phosphorothioate bond; note (original language) = 硫代磷酸酯键
  source 1..21: mol_type = other RNA
ctgcatgaacctgtcaatctt

SEQ ID NO: 700 - RNA, 21 nt, synthetic construct
  modified_base 1: mod_base = OTHER; note = 2'-methoxy nucleoside; note (original language) = 2'-甲氧基核苷
  modified_base 3..5: mod_base = OTHER; note = 2'-methoxy nucleoside; note (original language) = 2'-甲氧基核苷
  modified_base 7..13: mod_base = OTHER; note = 2'-methoxy nucleoside; note (original language) = 2'-甲氧基核苷
  modified_base 15: mod_base = OTHER; note = 2'-methoxy nucleoside; note (original language) = 2'-甲氧基核苷
  modified_base 17..21: mod_base = OTHER; note = 2'-methoxy nucleoside; note (original language) = 2'-甲氧基核苷
  modified_base 2: mod_base = OTHER; note = 2'-fluoro nucleoside; note (original language) = 2'-氟核苷
  modified_base 6: mod_base = OTHER; note = 2'-fluoro nucleoside; note (original language) = 2'-氟核苷
  modified_base 14: mod_base = OTHER; note = 2'-fluoro nucleoside; note (original language) = 2'-氟核苷
  modified_base 16: mod_base = OTHER; note = 2'-fluoro nucleoside; note (original language) = 2'-氟核苷
  modified_base 1..3: mod_base = OTHER; note = phosphorothioate bond; note (original language) = 硫代磷酸酯键
  modified_base 19..21: mod_base = OTHER; note = phosphorothioate bond; note (original language) = 硫代磷酸酯键
  source 1..21: mol_type = other RNA
ctgtgcatgccatatatacgg

SEQ ID NO: 701 - RNA, 21 nt, synthetic construct
  modified_base 1: mod_base = OTHER; note = 2'-methoxy nucleoside; note (original language) = 2'-甲氧基核苷
  modified_base 3..5: mod_base = OTHER; note = 2'-methoxy nucleoside; note (original language) = 2'-甲氧基核苷
  modified_base 7..13: mod_base = OTHER; note = 2'-methoxy nucleoside; note (original language) = 2'-甲氧基核苷
  modified_base 15: mod_base = OTHER; note = 2'-methoxy nucleoside; note (original language) = 2'-甲氧基核苷
  modified_base 17..21: mod_base = OTHER; note = 2'-methoxy nucleoside; note (original language) = 2'-甲氧基核苷
  modified_base 2: mod_base = OTHER; note = 2'-fluoro nucleoside; note (original language) = 2'-氟核苷
  modified_base 6: mod_base = OTHER; note = 2'-fluoro nucleoside; note (original language) = 2'-氟核苷
  modified_base 14: mod_base = OTHER; note = 2'-fluoro nucleoside; note (original language) = 2'-氟核苷
  modified_base 16: mod_base = OTHER; note = 2'-fluoro nucleoside; note (original language) = 2'-氟核苷
  modified_base 1..3: mod_base = OTHER; note = phosphorothioate bond; note (original language) = 硫代磷酸酯键
  modified_base 19..21: mod_base = OTHER; note = phosphorothioate bond; note (original language) = 硫代磷酸酯键
  source 1..21: mol_type = other RNA
gagaaataaccagctatggtt

SEQ ID NO: 702 - RNA, 21 nt, synthetic construct
  modified_base 1: mod_base = OTHER; note = 2'-methoxy nucleoside; note (original language) = 2'-甲氧基核苷
  modified_base 3..5: mod_base = OTHER; note = 2'-methoxy nucleoside; note (original language) = 2'-甲氧基核苷
  modified_base 7..13: mod_base = OTHER; note = 2'-methoxy nucleoside; note (original language) = 2'-甲氧基核苷
  modified_base 15: mod_base = OTHER; note = 2'-methoxy nucleoside; note (original language) = 2'-甲氧基核苷
  modified_base 17..21: mod_base = OTHER; note = 2'-methoxy nucleoside; note (original language) = 2'-甲氧基核苷
  modified_base 2: mod_base = OTHER; note = 2'-fluoro nucleoside; note (original language) = 2'-氟核苷
  modified_base 6: mod_base = OTHER; note = 2'-fluoro nucleoside; note (original language) = 2'-氟核苷
  modified_base 14: mod_base = OTHER; note = 2'-fluoro nucleoside; note (original language) = 2'-氟核苷
  modified_base 16: mod_base = OTHER; note = 2'-fluoro nucleoside; note (original language) = 2'-氟核苷
  modified_base 1..3: mod_base = OTHER; note = phosphorothioate bond; note (original language) = 硫代磷酸酯键
  modified_base 19..21: mod_base = OTHER; note = phosphorothioate bond; note (original language) = 硫代磷酸酯键
  source 1..21: mol_type = other RNA
ggaggtcatgttcttacattc

SEQ ID NO: 703 - RNA, 21 nt, synthetic construct
  modified_base 1: mod_base = OTHER; note = 2'-methoxy nucleoside; note (original language) = 2'-甲氧基核苷
  modified_base 3..5: mod_base = OTHER; note = 2'-methoxy nucleoside; note (original language) = 2'-甲氧基核苷
  modified_base 7..13: mod_base = OTHER; note = 2'-methoxy nucleoside; note (original language) = 2'-甲氧基核苷
  modified_base 15: mod_base = OTHER; note = 2'-methoxy nucleoside; note (original language) = 2'-甲氧基核苷
  modified_base 17..21: mod_base = OTHER; note = 2'-methoxy nucleoside; note (original language) = 2'-甲氧基核苷
  modified_base 2: mod_base = OTHER; note = 2'-fluoro nucleoside; note (original language) = 2'-氟核苷
  modified_base 6: mod_base = OTHER; note = 2'-fluoro nucleoside; note (original language) = 2'-氟核苷
  modified_base 14: mod_base = OTHER; note = 2'-fluoro nucleoside; note (original language) = 2'-氟核苷
  modified_base 16: mod_base = OTHER; note = 2'-fluoro nucleoside; note (original language) = 2'-氟核苷
  modified_base 1..3: mod_base = OTHER; note = phosphorothioate bond; note (original language) = 硫代磷酸酯键
  modified_base 19..21: mod_base = OTHER; note = phosphorothioate bond; note (original language) = 硫代磷酸酯键
  source 1..21: mol_type = other RNA
gtgcatgccatatatacggaa

SEQ ID NO: 704 - RNA, 21 nt, synthetic construct
  modified_base 1: mod_base = OTHER; note = 2'-methoxy nucleoside; note (original language) = 2'-甲氧基核苷
  modified_base 3..5: mod_base = OTHER; note = 2'-methoxy nucleoside; note (original language) = 2'-甲氧基核苷
  modified_base 7..13: mod_base = OTHER; note = 2'-methoxy nucleoside; note (original language) = 2'-甲氧基核苷
  modified_base 15: mod_base = OTHER; note = 2'-methoxy nucleoside; note (original language) = 2'-甲氧基核苷
  modified_base 17..21: mod_base = OTHER; note = 2'-methoxy nucleoside; note (original language) = 2'-甲氧基核苷
  modified_base 2: mod_base = OTHER; note = 2'-fluoro nucleoside; note (original language) = 2'-氟核苷
  modified_base 6: mod_base = OTHER; note = 2'-fluoro nucleoside; note (original language) = 2'-氟核苷
  modified_base 14: mod_base = OTHER; note = 2'-fluoro nucleoside; note (original language) = 2'-氟核苷
  modified_base 16: mod_base = OTHER; note = 2'-fluoro nucleoside; note (original language) = 2'-氟核苷
  modified_base 1..3: mod_base = OTHER; note = phosphorothioate bond; note (original language) = 硫代磷酸酯键
  modified_base 19..21: mod_base = OTHER; note = phosphorothioate bond; note (original language) = 硫代磷酸酯键
  source 1..21: mol_type = other RNA
gttcttacattcaagacacta

SEQ ID NO: 705 - RNA, 21 nt, synthetic construct
  modified_base 1: mod_base = OTHER; note = 2'-methoxy nucleoside; note (original language) = 2'-甲氧基核苷
  modified_base 3..5: mod_base = OTHER; note = 2'-methoxy nucleoside; note (original language) = 2'-甲氧基核苷
  modified_base 7..13: mod_base = OTHER; note = 2'-methoxy nucleoside; note (original language) = 2'-甲氧基核苷
  modified_base 15: mod_base = OTHER; note = 2'-methoxy nucleoside; note (original language) = 2'-甲氧基核苷
  modified_base 17..21: mod_base = OTHER; note = 2'-methoxy nucleoside; note (original language) = 2'-甲氧基核苷
  modified_base 2: mod_base = OTHER; note = 2'-fluoro nucleoside; note (original language) = 2'-氟核苷
  modified_base 6: mod_base = OTHER; note = 2'-fluoro nucleoside; note (original language) = 2'-氟核苷
  modified_base 14: mod_base = OTHER; note = 2'-fluoro nucleoside; note (original language) = 2'-氟核苷
  modified_base 16: mod_base = OTHER; note = 2'-fluoro nucleoside; note (original language) = 2'-氟核苷
  modified_base 1..3: mod_base = OTHER; note = phosphorothioate bond; note (original language) = 硫代磷酸酯键
  modified_base 19..21: mod_base = OTHER; note = phosphorothioate bond; note (original language) = 硫代磷酸酯键
  source 1..21: mol_type = other RNA
taaacactggttcttgcctcc

SEQ ID NO: 706 - RNA, 21 nt, synthetic construct
  modified_base 1: mod_base = OTHER; note = 2'-methoxy nucleoside; note (original language) = 2'-甲氧基核苷
  modified_base 3..5: mod_base = OTHER; note = 2'-methoxy nucleoside; note (original language) = 2'-甲氧基核苷
  modified_base 7..13: mod_base = OTHER; note = 2'-methoxy nucleoside; note (original language) = 2'-甲氧基核苷
  modified_base 15: mod_base = OTHER; note = 2'-methoxy nucleoside; note (original language) = 2'-甲氧基核苷
  modified_base 17..21: mod_base = OTHER; note = 2'-methoxy nucleoside; note (original language) = 2'-甲氧基核苷
  modified_base 2: mod_base = OTHER; note = 2'-fluoro nucleoside; note (original language) = 2'-氟核苷
  modified_base 6: mod_base = OTHER; note = 2'-fluoro nucleoside; note (original language) = 2'-氟核苷
  modified_base 14: mod_base = OTHER; note = 2'-fluoro nucleoside; note (original language) = 2'-氟核苷
  modified_base 16: mod_base = OTHER; note = 2'-fluoro nucleoside; note (original language) = 2'-氟核苷
  modified_base 1..3: mod_base = OTHER; note = phosphorothioate bond; note (original language) = 硫代磷酸酯键
  modified_base 19..21: mod_base = OTHER; note = phosphorothioate bond; note (original language) = 硫代磷酸酯键
  source 1..21: mol_type = other RNA
tacacagcaaacaggaatggg

SEQ ID NO: 707 - RNA, 21 nt, synthetic construct
  modified_base 1: mod_base = OTHER; note = 2'-methoxy nucleoside; note (original language) = 2'-甲氧基核苷
  modified_base 3..5: mod_base = OTHER; note = 2'-methoxy nucleoside; note (original language) = 2'-甲氧基核苷
  modified_base 7..13: mod_base = OTHER; note = 2'-methoxy nucleoside; note (original language) = 2'-甲氧基核苷
  modified_base 15: mod_base = OTHER; note = 2'-methoxy nucleoside; note (original language) = 2'-甲氧基核苷
  modified_base 17..21: mod_base = OTHER; note = 2'-methoxy nucleoside; note (original language) = 2'-甲氧基核苷
  modified_base 2: mod_base = OTHER; note = 2'-fluoro nucleoside; note (original language) = 2'-氟核苷
  modified_base 6: mod_base = OTHER; note = 2'-fluoro nucleoside; note (original language) = 2'-氟核苷
  modified_base 14: mod_base = OTHER; note = 2'-fluoro nucleoside; note (original language) = 2'-氟核苷
  modified_base 16: mod_base = OTHER; note = 2'-fluoro nucleoside; note (original language) = 2'-氟核苷
  modified_base 1..3: mod_base = OTHER; note = phosphorothioate bond; note (original language) = 硫代磷酸酯键
  modified_base 19..21: mod_base = OTHER; note = phosphorothioate bond; note (original language) = 硫代磷酸酯键
  source 1..21: mol_type = other RNA
tactttaattttaaaacccaa

SEQ ID NO: 708 - RNA, 21 nt, synthetic construct
  modified_base 1: mod_base = OTHER; note = 2'-methoxy nucleoside; note (original language) = 2'-甲氧基核苷
  modified_base 3..5: mod_base = OTHER; note = 2'-methoxy nucleoside; note (original language) = 2'-甲氧基核苷
  modified_base 7..13: mod_base = OTHER; note = 2'-methoxy nucleoside; note (original language) = 2'-甲氧基核苷
  modified_base 15: mod_base = OTHER; note = 2'-methoxy nucleoside; note (original language) = 2'-甲氧基核苷
  modified_base 17..21: mod_base = OTHER; note = 2'-methoxy nucleoside; note (original language) = 2'-甲氧基核苷
  modified_base 2: mod_base = OTHER; note = 2'-fluoro nucleoside; note (original language) = 2'-氟核苷
  modified_base 6: mod_base = OTHER; note = 2'-fluoro nucleoside; note (original language) = 2'-氟核苷
  modified_base 14: mod_base = OTHER; note = 2'-fluoro nucleoside; note (original language) = 2'-氟核苷
  modified_base 16: mod_base = OTHER; note = 2'-fluoro nucleoside; note (original language) = 2'-氟核苷
  modified_base 1..3: mod_base = OTHER; note = phosphorothioate bond; note (original language) = 硫代磷酸酯键
  modified_base 19..21: mod_base = OTHER; note = phosphorothioate bond; note (original language) = 硫代磷酸酯键
  source 1..21: mol_type = other RNA
tatacggaagcccaagaagtt

SEQ ID NO: 709 - RNA, 21 nt, synthetic construct
  modified_base 1: mod_base = OTHER; note = 2'-methoxy nucleoside; note (original language) = 2'-甲氧基核苷
  modified_base 3..5: mod_base = OTHER; note = 2'-methoxy nucleoside; note (original language) = 2'-甲氧基核苷
  modified_base 7..13: mod_base = OTHER; note = 2'-methoxy nucleoside; note (original language) = 2'-甲氧基核苷
  modified_base 15: mod_base = OTHER; note = 2'-methoxy nucleoside; note (original language) = 2'-甲氧基核苷
  modified_base 17..21: mod_base = OTHER; note = 2'-methoxy nucleoside; note (original language) = 2'-甲氧基核苷
  modified_base 2: mod_base = OTHER; note = 2'-fluoro nucleoside; note (original language) = 2'-氟核苷
  modified_base 6: mod_base = OTHER; note = 2'-fluoro nucleoside; note (original language) = 2'-氟核苷
  modified_base 14: mod_base = OTHER; note = 2'-fluoro nucleoside; note (original language) = 2'-氟核苷
  modified_base 16: mod_base = OTHER; note = 2'-fluoro nucleoside; note (original language) = 2'-氟核苷
  modified_base 1..3: mod_base = OTHER; note = phosphorothioate bond; note (original language) = 硫代磷酸酯键
  modified_base 19..21: mod_base = OTHER; note = phosphorothioate bond; note (original language) = 硫代磷酸酯键
  source 1..21: mol_type = other RNA
tatactttaattttaaaaccc

SEQ ID NO: 710 - RNA, 21 nt, synthetic construct
  modified_base 1: mod_base = OTHER; note = 2'-methoxy nucleoside; note (original language) = 2'-甲氧基核苷
  modified_base 3..5: mod_base = OTHER; note = 2'-methoxy nucleoside; note (original language) = 2'-甲氧基核苷
  modified_base 7..13: mod_base = OTHER; note = 2'-methoxy nucleoside; note (original language) = 2'-甲氧基核苷
  modified_base 15: mod_base = OTHER; note = 2'-methoxy nucleoside; note (original language) = 2'-甲氧基核苷
  modified_base 17..21: mod_base = OTHER; note = 2'-methoxy nucleoside; note (original language) = 2'-甲氧基核苷
  modified_base 2: mod_base = OTHER; note = 2'-fluoro nucleoside; note (original language) = 2'-氟核苷
  modified_base 6: mod_base = OTHER; note = 2'-fluoro nucleoside; note (original language) = 2'-氟核苷
  modified_base 14: mod_base = OTHER; note = 2'-fluoro nucleoside; note (original language) = 2'-氟核苷
  modified_base 16: mod_base = OTHER; note = 2'-fluoro nucleoside; note (original language) = 2'-氟核苷
  modified_base 1..3: mod_base = OTHER; note = phosphorothioate bond; note (original language) = 硫代磷酸酯键
  modified_base 19..21: mod_base = OTHER; note = phosphorothioate bond; note (original language) = 硫代磷酸酯键
  source 1..21: mol_type = other RNA
tcactgtgcatgccatatata

SEQ ID NO: 711 - RNA, 21 nt, synthetic construct
  modified_base 1: mod_base = OTHER; note = 2'-methoxy nucleoside; note (original language) = 2'-甲氧基核苷
  modified_base 3..5: mod_base = OTHER; note = 2'-methoxy nucleoside; note (original language) = 2'-甲氧基核苷
  modified_base 7..13: mod_base = OTHER; note = 2'-methoxy nucleoside; note (original language) = 2'-甲氧基核苷
  modified_base 15: mod_base = OTHER; note = 2'-methoxy nucleoside; note (original language) = 2'-甲氧基核苷
  modified_base 17..21: mod_base = OTHER; note = 2'-methoxy nucleoside; note (original language) = 2'-甲氧基核苷
  modified_base 2: mod_base = OTHER; note = 2'-fluoro nucleoside; note (original language) = 2'-氟核苷
  modified_base 6: mod_base = OTHER; note = 2'-fluoro nucleoside; note (original language) = 2'-氟核苷
  modified_base 14: mod_base = OTHER; note = 2'-fluoro nucleoside; note (original language) = 2'-氟核苷
  modified_base 16: mod_base = OTHER; note = 2'-fluoro nucleoside; note (original language) = 2'-氟核苷
  modified_base 1..3: mod_base = OTHER; note = phosphorothioate bond; note (original language) = 硫代磷酸酯键
  modified_base 19..21: mod_base = OTHER; note = phosphorothioate bond; note (original language) = 硫代磷酸酯键
  source 1..21: mol_type = other RNA
tcatgttcttacattcaagac

SEQ ID NO: 712 - RNA, 21 nt, synthetic construct
  modified_base 1: mod_base = OTHER; note = 2'-methoxy nucleoside; note (original language) = 2'-甲氧基核苷
  modified_base 3..5: mod_base = OTHER; note = 2'-methoxy nucleoside; note (original language) = 2'-甲氧基核苷
  modified_base 7..13: mod_base = OTHER; note = 2'-methoxy nucleoside; note (original language) = 2'-甲氧基核苷
  modified_base 15: mod_base = OTHER; note = 2'-methoxy nucleoside; note (original language) = 2'-甲氧基核苷
  modified_base 17..21: mod_base = OTHER; note = 2'-methoxy nucleoside; note (original language) = 2'-甲氧基核苷
  modified_base 2: mod_base = OTHER; note = 2'-fluoro nucleoside; note (original language) = 2'-氟核苷
  modified_base 6: mod_base = OTHER; note = 2'-fluoro nucleoside; note (original language) = 2'-氟核苷
  modified_base 14: mod_base = OTHER; note = 2'-fluoro nucleoside; note (original language) = 2'-氟核苷
  modified_base 16: mod_base = OTHER; note = 2'-fluoro nucleoside; note (original language) = 2'-氟核苷
  modified_base 1..3: mod_base = OTHER; note = phosphorothioate bond; note (original language) = 硫代磷酸酯键
  modified_base 19..21: mod_base = OTHER; note = phosphorothioate bond; note (original language) = 硫代磷酸酯键
  source 1..21: mol_type = other RNA
tcctgcaggtcataagatcct

SEQ ID NO: 713 - RNA, 21 nt, synthetic construct
  modified_base 1: mod_base = OTHER; note = 2'-methoxy nucleoside; note (original language) = 2'-甲氧基核苷
  modified_base 3..5: mod_base = OTHER; note = 2'-methoxy nucleoside; note (original language) = 2'-甲氧基核苷
  modified_base 7..13: mod_base = OTHER; note = 2'-methoxy nucleoside; note (original language) = 2'-甲氧基核苷
  modified_base 15: mod_base = OTHER; note = 2'-methoxy nucleoside; note (original language) = 2'-甲氧基核苷
  modified_base 17..21: mod_base = OTHER; note = 2'-methoxy nucleoside; note (original language) = 2'-甲氧基核苷
  modified_base 2: mod_base = OTHER; note = 2'-fluoro nucleoside; note (original language) = 2'-氟核苷
  modified_base 6: mod_base = OTHER; note = 2'-fluoro nucleoside; note (original language) = 2'-氟核苷
  modified_base 14: mod_base = OTHER; note = 2'-fluoro nucleoside; note (original language) = 2'-氟核苷
  modified_base 16: mod_base = OTHER; note = 2'-fluoro nucleoside; note (original language) = 2'-氟核苷
  modified_base 1..3: mod_base = OTHER; note = phosphorothioate bond; note (original language) = 硫代磷酸酯键
  modified_base 19..21: mod_base = OTHER; note = phosphorothioate bond; note (original language) = 硫代磷酸酯键
  source 1..21: mol_type = other RNA
tgaggtgctgttgtccaccca

SEQ ID NO: 714 - RNA, 21 nt, synthetic construct
  modified_base 1: mod_base = OTHER; note = 2'-methoxy nucleoside; note (original language) = 2'-甲氧基核苷
  modified_base 3..5: mod_base = OTHER; note = 2'-methoxy nucleoside; note (original language) = 2'-甲氧基核苷
  modified_base 7..13: mod_base = OTHER; note = 2'-methoxy nucleoside; note (original language) = 2'-甲氧基核苷
  modified_base 15: mod_base = OTHER; note = 2'-methoxy nucleoside; note (original language) = 2'-甲氧基核苷
  modified_base 17..21: mod_base = OTHER; note = 2'-methoxy nucleoside; note (original language) = 2'-甲氧基核苷
  modified_base 2: mod_base = OTHER; note = 2'-fluoro nucleoside; note (original language) = 2'-氟核苷
  modified_base 6: mod_base = OTHER; note = 2'-fluoro nucleoside; note (original language) = 2'-氟核苷
  modified_base 14: mod_base = OTHER; note = 2'-fluoro nucleoside; note (original language) = 2'-氟核苷
  modified_base 16: mod_base = OTHER; note = 2'-fluoro nucleoside; note (original language) = 2'-氟核苷
  modified_base 1..3: mod_base = OTHER; note = phosphorothioate bond; note (original language) = 硫代磷酸酯键
  modified_base 19..21: mod_base = OTHER; note = phosphorothioate bond; note (original language) = 硫代磷酸酯键
  source 1..21: mol_type = other RNA
tgcatgaacctgtcaatcttc

SEQ ID NO: 715 - RNA, 21 nt, synthetic construct
  modified_base 1: mod_base = OTHER; note = 2'-methoxy nucleoside; note (original language) = 2'-甲氧基核苷
  modified_base 3..5: mod_base = OTHER; note = 2'-methoxy nucleoside; note (original language) = 2'-甲氧基核苷
  modified_base 7..13: mod_base = OTHER; note = 2'-methoxy nucleoside; note (original language) = 2'-甲氧基核苷
  modified_base 15: mod_base = OTHER; note = 2'-methoxy nucleoside; note (original language) = 2'-甲氧基核苷
  modified_base 17..21: mod_base = OTHER; note = 2'-methoxy nucleoside; note (original language) = 2'-甲氧基核苷
  modified_base 2: mod_base = OTHER; note = 2'-fluoro nucleoside; note (original language) = 2'-氟核苷
  modified_base 6: mod_base = OTHER; note = 2'-fluoro nucleoside; note (original language) = 2'-氟核苷
  modified_base 14: mod_base = OTHER; note = 2'-fluoro nucleoside; note (original language) = 2'-氟核苷
  modified_base 16: mod_base = OTHER; note = 2'-fluoro nucleoside; note (original language) = 2'-氟核苷
  modified_base 1..3: mod_base = OTHER; note = phosphorothioate bond; note (original language) = 硫代磷酸酯键
  modified_base 19..21: mod_base = OTHER; note = phosphorothioate bond; note (original language) = 硫代磷酸酯键
  source 1..21: mol_type = other RNA
tgtcacagcctgcatgaacct

SEQ ID NO: 716 - RNA, 21 nt, synthetic construct
  modified_base 1: mod_base = OTHER; note = 2'-methoxy nucleoside; note (original language) = 2'-甲氧基核苷
  modified_base 3..5: mod_base = OTHER; note = 2'-methoxy nucleoside; note (original language) = 2'-甲氧基核苷
  modified_base 7..13: mod_base = OTHER; note = 2'-methoxy nucleoside; note (original language) = 2'-甲氧基核苷
  modified_base 15: mod_base = OTHER; note = 2'-methoxy nucleoside; note (original language) = 2'-甲氧基核苷
  modified_base 17..21: mod_base = OTHER; note = 2'-methoxy nucleoside; note (original language) = 2'-甲氧基核苷
  modified_base 2: mod_base = OTHER; note = 2'-fluoro nucleoside; note (original language) = 2'-氟核苷
  modified_base 6: mod_base = OTHER; note = 2'-fluoro nucleoside; note (original language) = 2'-氟核苷
  modified_base 14: mod_base = OTHER; note = 2'-fluoro nucleoside; note (original language) = 2'-氟核苷
  modified_base 16: mod_base = OTHER; note = 2'-fluoro nucleoside; note (original language) = 2'-氟核苷
  modified_base 1..3: mod_base = OTHER; note = phosphorothioate bond; note (original language) = 硫代磷酸酯键
  modified_base 19..21: mod_base = OTHER; note = phosphorothioate bond; note (original language) = 硫代磷酸酯键
  source 1..21: mol_type = other RNA
tgtccacccagaactcctggg

SEQ ID NO: 717 - RNA, 21 nt, synthetic construct
  modified_base 1: mod_base = OTHER; note = 2'-methoxy nucleoside; note (original language) = 2'-甲氧基核苷
  modified_base 3..5: mod_base = OTHER; note = 2'-methoxy nucleoside; note (original language) = 2'-甲氧基核苷
  modified_base 7..13: mod_base = OTHER; note = 2'-methoxy nucleoside; note (original language) = 2'-甲氧基核苷
  modified_base 15: mod_base = OTHER; note = 2'-methoxy nucleoside; note (original language) = 2'-甲氧基核苷
  modified_base 17..21: mod_base = OTHER; note = 2'-methoxy nucleoside; note (original language) = 2'-甲氧基核苷
  modified_base 2: mod_base = OTHER; note = 2'-fluoro nucleoside; note (original language) = 2'-氟核苷
  modified_base 6: mod_base = OTHER; note = 2'-fluoro nucleoside; note (original language) = 2'-氟核苷
  modified_base 14: mod_base = OTHER; note = 2'-fluoro nucleoside; note (original language) = 2'-氟核苷
  modified_base 16: mod_base = OTHER; note = 2'-fluoro nucleoside; note (original language) = 2'-氟核苷
  modified_base 1..3: mod_base = OTHER; note = phosphorothioate bond; note (original language) = 硫代磷酸酯键
  modified_base 19..21: mod_base = OTHER; note = phosphorothioate bond; note (original language) = 硫代磷酸酯键
  source 1..21: mol_type = other RNA
tgtgcatgccatatatacgga

SEQ ID NO: 718 - RNA, 21 nt, synthetic construct
  modified_base 1: mod_base = OTHER; note = 2'-methoxy nucleoside; note (original language) = 2'-甲氧基核苷
  modified_base 3..5: mod_base = OTHER; note = 2'-methoxy nucleoside; note (original language) = 2'-甲氧基核苷
  modified_base 7..13: mod_base = OTHER; note = 2'-methoxy nucleoside; note (original language) = 2'-甲氧基核苷
  modified_base 15: mod_base = OTHER; note = 2'-methoxy nucleoside; note (original language) = 2'-甲氧基核苷
  modified_base 17..21: mod_base = OTHER; note = 2'-methoxy nucleoside; note (original language) = 2'-甲氧基核苷
  modified_base 2: mod_base = OTHER; note = 2'-fluoro nucleoside; note (original language) = 2'-氟核苷
  modified_base 6: mod_base = OTHER; note = 2'-fluoro nucleoside; note (original language) = 2'-氟核苷
  modified_base 14: mod_base = OTHER; note = 2'-fluoro nucleoside; note (original language) = 2'-氟核苷
  modified_base 16: mod_base = OTHER; note = 2'-fluoro nucleoside; note (original language) = 2'-氟核苷
  modified_base 1..3: mod_base = OTHER; note = phosphorothioate bond; note (original language) = 硫代磷酸酯键
  modified_base 19..21: mod_base = OTHER; note = phosphorothioate bond; note (original language) = 硫代磷酸酯键
  source 1..21: mol_type = other RNA
ttcatccagttgagggagttt

SEQ ID NO: 719 - RNA, 21 nt, synthetic construct
  modified_base 1: mod_base = OTHER; note = 2'-methoxy nucleoside; note (original language) = 2'-甲氧基核苷
  modified_base 3..5: mod_base = OTHER; note = 2'-methoxy nucleoside; note (original language) = 2'-甲氧基核苷
  modified_base 7..13: mod_base = OTHER; note = 2'-methoxy nucleoside; note (original language) = 2'-甲氧基核苷
  modified_base 15: mod_base = OTHER; note = 2'-methoxy nucleoside; note (original language) = 2'-甲氧基核苷
  modified_base 17..21: mod_base = OTHER; note = 2'-methoxy nucleoside; note (original language) = 2'-甲氧基核苷
  modified_base 2: mod_base = OTHER; note = 2'-fluoro nucleoside; note (original language) = 2'-氟核苷
  modified_base 6: mod_base = OTHER; note = 2'-fluoro nucleoside; note (original language) = 2'-氟核苷
  modified_base 14: mod_base = OTHER; note = 2'-fluoro nucleoside; note (original language) = 2'-氟核苷
  modified_base 16: mod_base = OTHER; note = 2'-fluoro nucleoside; note (original language) = 2'-氟核苷
  modified_base 1..3: mod_base = OTHER; note = phosphorothioate bond; note (original language) = 硫代磷酸酯键
  modified_base 19..21: mod_base = OTHER; note = phosphorothioate bond; note (original language) = 硫代磷酸酯键
  source 1..21: mol_type = other RNA
ttgctggaaagtgagaccctc

SEQ ID NO: 720 - RNA, 21 nt, synthetic construct
  modified_base 1: mod_base = OTHER; note = 2'-methoxy nucleoside; note (original language) = 2'-甲氧基核苷
  modified_base 3..5: mod_base = OTHER; note = 2'-methoxy nucleoside; note (original language) = 2'-甲氧基核苷
  modified_base 7..13: mod_base = OTHER; note = 2'-methoxy nucleoside; note (original language) = 2'-甲氧基核苷
  modified_base 15: mod_base = OTHER; note = 2'-methoxy nucleoside; note (original language) = 2'-甲氧基核苷
  modified_base 17..21: mod_base = OTHER; note = 2'-methoxy nucleoside; note (original language) = 2'-甲氧基核苷
  modified_base 2: mod_base = OTHER; note = 2'-fluoro nucleoside; note (original language) = 2'-氟核苷
  modified_base 6: mod_base = OTHER; note = 2'-fluoro nucleoside; note (original language) = 2'-氟核苷
  modified_base 14: mod_base = OTHER; note = 2'-fluoro nucleoside; note (original language) = 2'-氟核苷
  modified_base 16: mod_base = OTHER; note = 2'-fluoro nucleoside; note (original language) = 2'-氟核苷
  modified_base 1..3: mod_base = OTHER; note = phosphorothioate bond; note (original language) = 硫代磷酸酯键
  modified_base 19..21: mod_base = OTHER; note = phosphorothioate bond; note (original language) = 硫代磷酸酯键
  source 1..21: mol_type = other RNA
ttgtccacccagaactcctgg

SEQ ID NO: 721 - RNA, 21 nt, synthetic construct
  modified_base 1: mod_base = OTHER; note = 2'-methoxy nucleoside; note (original language) = 2'-甲氧基核苷
  modified_base 3..5: mod_base = OTHER; note = 2'-methoxy nucleoside; note (original language) = 2'-甲氧基核苷
  modified_base 7..13: mod_base = OTHER; note = 2'-methoxy nucleoside; note (original language) = 2'-甲氧基核苷
  modified_base 15: mod_base = OTHER; note = 2'-methoxy nucleoside; note (original language) = 2'-甲氧基核苷
  modified_base 17..21: mod_base = OTHER; note = 2'-methoxy nucleoside; note (original language) = 2'-甲氧基核苷
  modified_base 2: mod_base = OTHER; note = 2'-fluoro nucleoside; note (original language) = 2'-氟核苷
  modified_base 6: mod_base = OTHER; note = 2'-fluoro nucleoside; note (original language) = 2'-氟核苷
  modified_base 14: mod_base = OTHER; note = 2'-fluoro nucleoside; note (original language) = 2'-氟核苷
  modified_base 16: mod_base = OTHER; note = 2'-fluoro nucleoside; note (original language) = 2'-氟核苷
  modified_base 1..3: mod_base = OTHER; note = phosphorothioate bond; note (original language) = 硫代磷酸酯键
  modified_base 19..21: mod_base = OTHER; note = phosphorothioate bond; note (original language) = 硫代磷酸酯键
  source 1..21: mol_type = other RNA
tttcacaaacaagctggtcgg

SEQ ID NO: 722 - RNA, 21 nt, synthetic construct
  modified_base 1: mod_base = OTHER; note = 2'-methoxy nucleoside; note (original language) = 2'-甲氧基核苷
  modified_base 3..5: mod_base = OTHER; note = 2'-methoxy nucleoside; note (original language) = 2'-甲氧基核苷
  modified_base 7..13: mod_base = OTHER; note = 2'-methoxy nucleoside; note (original language) = 2'-甲氧基核苷
  modified_base 15: mod_base = OTHER; note = 2'-methoxy nucleoside; note (original language) = 2'-甲氧基核苷
  modified_base 17..21: mod_base = OTHER; note = 2'-methoxy nucleoside; note (original language) = 2'-甲氧基核苷
  modified_base 2: mod_base = OTHER; note = 2'-fluoro nucleoside; note (original language) = 2'-氟核苷
  modified_base 6: mod_base = OTHER; note = 2'-fluoro nucleoside; note (original language) = 2'-氟核苷
  modified_base 14: mod_base = OTHER; note = 2'-fluoro nucleoside; note (original language) = 2'-氟核苷
  modified_base 16: mod_base = OTHER; note = 2'-fluoro nucleoside; note (original language) = 2'-氟核苷
  modified_base 1..3: mod_base = OTHER; note = phosphorothioate bond; note (original language) = 硫代磷酸酯键
  modified_base 19..21: mod_base = OTHER; note = phosphorothioate bond; note (original language) = 硫代磷酸酯键
  source 1..21: mol_type = other RNA
tttgccagctgctcacaggta

SEQ ID NO: 723 - RNA, 21 nt, synthetic construct
  modified_base 1: mod_base = OTHER; note = 2'-methoxy nucleoside; note (original language) = 2'-甲氧基核苷
  modified_base 3..5: mod_base = OTHER; note = 2'-methoxy nucleoside; note (original language) = 2'-甲氧基核苷
  modified_base 7..13: mod_base = OTHER; note = 2'-methoxy nucleoside; note (original language) = 2'-甲氧基核苷
  modified_base 15: mod_base = OTHER; note = 2'-methoxy nucleoside; note (original language) = 2'-甲氧基核苷
  modified_base 17..21: mod_base = OTHER; note = 2'-methoxy nucleoside; note (original language) = 2'-甲氧基核苷
  modified_base 2: mod_base = OTHER; note = 2'-fluoro nucleoside; note (original language) = 2'-氟核苷
  modified_base 6: mod_base = OTHER; note = 2'-fluoro nucleoside; note (original language) = 2'-氟核苷
  modified_base 14: mod_base = OTHER; note = 2'-fluoro nucleoside; note (original language) = 2'-氟核苷
  modified_base 16: mod_base = OTHER; note = 2'-fluoro nucleoside; note (original language) = 2'-氟核苷
  modified_base 1..3: mod_base = OTHER; note = phosphorothioate bond; note (original language) = 硫代磷酸酯键
  modified_base 19..21: mod_base = OTHER; note = phosphorothioate bond; note (original language) = 硫代磷酸酯键
  source 1..21: mol_type = other RNA
tttgctggaaagtgagaccct

SEQ ID NO: 724 - RNA, 21 nt, synthetic construct
  modified_base 1: mod_base = OTHER; note = 2'-methoxy nucleoside; note (original language) = 2'-甲氧基核苷
  modified_base 3..5: mod_base = OTHER; note = 2'-methoxy nucleoside; note (original language) = 2'-甲氧基核苷
  modified_base 7..13: mod_base = OTHER; note = 2'-methoxy nucleoside; note (original language) = 2'-甲氧基核苷
  modified_base 15: mod_base = OTHER; note = 2'-methoxy nucleoside; note (original language) = 2'-甲氧基核苷
  modified_base 17..21: mod_base = OTHER; note = 2'-methoxy nucleoside; note (original language) = 2'-甲氧基核苷
  modified_base 2: mod_base = OTHER; note = 2'-fluoro nucleoside; note (original language) = 2'-氟核苷
  modified_base 6: mod_base = OTHER; note = 2'-fluoro nucleoside; note (original language) = 2'-氟核苷
  modified_base 14: mod_base = OTHER; note = 2'-fluoro nucleoside; note (original language) = 2'-氟核苷
  modified_base 16: mod_base = OTHER; note = 2'-fluoro nucleoside; note (original language) = 2'-氟核苷
  modified_base 1..3: mod_base = OTHER; note = phosphorothioate bond; note (original language) = 硫代磷酸酯键
  modified_base 19..21: mod_base = OTHER; note = phosphorothioate bond; note (original language) = 硫代磷酸酯键
  source 1..21: mol_type = other RNA
ttttaaaacccaatttttgtt

SEQ ID NO: 725 - RNA, 21 nt, synthetic construct
  modified_base 1: mod_base = OTHER; note = 2'-methoxy nucleoside; note (original language) = 2'-甲氧基核苷
  modified_base 3..5: mod_base = OTHER; note = 2'-methoxy nucleoside; note (original language) = 2'-甲氧基核苷
  modified_base 7..13: mod_base = OTHER; note = 2'-methoxy nucleoside; note (original language) = 2'-甲氧基核苷
  modified_base 15: mod_base = OTHER; note = 2'-methoxy nucleoside; note (original language) = 2'-甲氧基核苷
  modified_base 17..21: mod_base = OTHER; note = 2'-methoxy nucleoside; note (original language) = 2'-甲氧基核苷
  modified_base 2: mod_base = OTHER; note = 2'-fluoro nucleoside; note (original language) = 2'-氟核苷
  modified_base 6: mod_base = OTHER; note = 2'-fluoro nucleoside; note (original language) = 2'-氟核苷
  modified_base 14: mod_base = OTHER; note = 2'-fluoro nucleoside; note (original language) = 2'-氟核苷
  modified_base 16: mod_base = OTHER; note = 2'-fluoro nucleoside; note (original language) = 2'-氟核苷
  modified_base 1..3: mod_base = OTHER; note = phosphorothioate bond; note (original language) = 硫代磷酸酯键
  modified_base 19..21: mod_base = OTHER; note = phosphorothioate bond; note (original language) = 硫代磷酸酯键
  source 1..21: mol_type = other RNA
ttttgtttcacaaacaagctg

SEQ ID NO: 726 - RNA, 21 nt, synthetic construct
  modified_base 1: mod_base = OTHER; note = 2'-methoxy nucleoside; note (original language) = 2'-甲氧基核苷
  modified_base 3..5: mod_base = OTHER; note = 2'-methoxy nucleoside; note (original language) = 2'-甲氧基核苷
  modified_base 7..13: mod_base = OTHER; note = 2'-methoxy nucleoside; note (original language) = 2'-甲氧基核苷
  modified_base 15: mod_base = OTHER; note = 2'-methoxy nucleoside; note (original language) = 2'-甲氧基核苷
  modified_base 17..21: mod_base = OTHER; note = 2'-methoxy nucleoside; note (original language) = 2'-甲氧基核苷
  modified_base 2: mod_base = OTHER; note = 2'-fluoro nucleoside; note (original language) = 2'-氟核苷
  modified_base 6: mod_base = OTHER; note = 2'-fluoro nucleoside; note (original language) = 2'-氟核苷
  modified_base 14: mod_base = OTHER; note = 2'-fluoro nucleoside; note (original language) = 2'-氟核苷
  modified_base 16: mod_base = OTHER; note = 2'-fluoro nucleoside; note (original language) = 2'-氟核苷
  modified_base 1..3: mod_base = OTHER; note = phosphorothioate bond; note (original language) = 硫代磷酸酯键
  modified_base 19..21: mod_base = OTHER; note = phosphorothioate bond; note (original language) = 硫代磷酸酯键
  source 1..21: mol_type = other RNA
tgttagtaataaacgtcttgc

SEQ ID NO: 727 - RNA, 21 nt, synthetic construct
  modified_base 1: mod_base = OTHER; note = 2'-methoxy nucleoside; note (original language) = 2'-甲氧基核苷
  modified_base 3..5: mod_base = OTHER; note = 2'-methoxy nucleoside; note (original language) = 2'-甲氧基核苷
  modified_base 7..13: mod_base = OTHER; note = 2'-methoxy nucleoside; note (original language) = 2'-甲氧基核苷
  modified_base 15: mod_base = OTHER; note = 2'-methoxy nucleoside; note (original language) = 2'-甲氧基核苷
  modified_base 17..21: mod_base = OTHER; note = 2'-methoxy nucleoside; note (original language) = 2'-甲氧基核苷
  modified_base 2: mod_base = OTHER; note = 2'-fluoro nucleoside; note (original language) = 2'-氟核苷
  modified_base 6: mod_base = OTHER; note = 2'-fluoro nucleoside; note (original language) = 2'-氟核苷
  modified_base 14: mod_base = OTHER; note = 2'-fluoro nucleoside; note (original language) = 2'-氟核苷
  modified_base 16: mod_base = OTHER; note = 2'-fluoro nucleoside; note (original language) = 2'-氟核苷
  modified_base 1..3: mod_base = OTHER; note = phosphorothioate bond; note (original language) = 硫代磷酸酯键
  modified_base 19..21: mod_base = OTHER; note = phosphorothioate bond; note (original language) = 硫代磷酸酯键
  source 1..21: mol_type = other RNA
ttcacaaacaagctggtcggt

SEQ ID NO: 728 - RNA, 21 nt, synthetic construct
  modified_base 1: mod_base = OTHER; note = 2'-methoxy nucleoside; note (original language) = 2'-甲氧基核苷
  modified_base 3..5: mod_base = OTHER; note = 2'-methoxy nucleoside; note (original language) = 2'-甲氧基核苷
  modified_base 7..13: mod_base = OTHER; note = 2'-methoxy nucleoside; note (original language) = 2'-甲氧基核苷
  modified_base 15: mod_base = OTHER; note = 2'-methoxy nucleoside; note (original language) = 2'-甲氧基核苷
  modified_base 17..21: mod_base = OTHER; note = 2'-methoxy nucleoside; note (original language) = 2'-甲氧基核苷
  modified_base 2: mod_base = OTHER; note = 2'-fluoro nucleoside; note (original language) = 2'-氟核苷
  modified_base 6: mod_base = OTHER; note = 2'-fluoro nucleoside; note (original language) = 2'-氟核苷
  modified_base 14: mod_base = OTHER; note = 2'-fluoro nucleoside; note (original language) = 2'-氟核苷
  modified_base 16: mod_base = OTHER; note = 2'-fluoro nucleoside; note (original language) = 2'-氟核苷
  modified_base 1..3: mod_base = OTHER; note = phosphorothioate bond; note (original language) = 硫代磷酸酯键
  modified_base 19..21: mod_base = OTHER; note = phosphorothioate bond; note (original language) = 硫代磷酸酯键
  source 1..21: mol_type = other RNA
tttttgtttcacaaacaagct

SEQ ID NO: 729 - RNA, 21 nt, synthetic construct
  modified_base 1: mod_base = OTHER; note = 2'-methoxy nucleoside; note (original language) = 2'-甲氧基核苷
  modified_base 3..5: mod_base = OTHER; note = 2'-methoxy nucleoside; note (original language) = 2'-甲氧基核苷
  modified_base 7..13: mod_base = OTHER; note = 2'-methoxy nucleoside; note (original language) = 2'-甲氧基核苷
  modified_base 15: mod_base = OTHER; note = 2'-methoxy nucleoside; note (original language) = 2'-甲氧基核苷
  modified_base 17..21: mod_base = OTHER; note = 2'-methoxy nucleoside; note (original language) = 2'-甲氧基核苷
  modified_base 2: mod_base = OTHER; note = 2'-fluoro nucleoside; note (original language) = 2'-氟核苷
  modified_base 6: mod_base = OTHER; note = 2'-fluoro nucleoside; note (original language) = 2'-氟核苷
  modified_base 14: mod_base = OTHER; note = 2'-fluoro nucleoside; note (original language) = 2'-氟核苷
  modified_base 16: mod_base = OTHER; note = 2'-fluoro nucleoside; note (original language) = 2'-氟核苷
  modified_base 1..3: mod_base = OTHER; note = phosphorothioate bond; note (original language) = 硫代磷酸酯键
  modified_base 19..21: mod_base = OTHER; note = phosphorothioate bond; note (original language) = 硫代磷酸酯键
  source 1..21: mol_type = other RNA
tgagtcaccgagaagttgtcc

SEQ ID NO: 730 - RNA, 21 nt, synthetic construct
  modified_base 1: mod_base = OTHER; note = 2'-methoxy nucleoside; note (original language) = 2'-甲氧基核苷
  modified_base 3..5: mod_base = OTHER; note = 2'-methoxy nucleoside; note (original language) = 2'-甲氧基核苷
  modified_base 7..13: mod_base = OTHER; note = 2'-methoxy nucleoside; note (original language) = 2'-甲氧基核苷
  modified_base 15: mod_base = OTHER; note = 2'-methoxy nucleoside; note (original language) = 2'-甲氧基核苷
  modified_base 17..21: mod_base = OTHER; note = 2'-methoxy nucleoside; note (original language) = 2'-甲氧基核苷
  modified_base 2: mod_base = OTHER; note = 2'-fluoro nucleoside; note (original language) = 2'-氟核苷
  modified_base 6: mod_base = OTHER; note = 2'-fluoro nucleoside; note (original language) = 2'-氟核苷
  modified_base 14: mod_base = OTHER; note = 2'-fluoro nucleoside; note (original language) = 2'-氟核苷
  modified_base 16: mod_base = OTHER; note = 2'-fluoro nucleoside; note (original language) = 2'-氟核苷
  modified_base 1..3: mod_base = OTHER; note = phosphorothioate bond; note (original language) = 硫代磷酸酯键
  modified_base 19..21: mod_base = OTHER; note = phosphorothioate bond; note (original language) = 硫代磷酸酯键
  source 1..21: mol_type = other RNA
ttggccagcatcccgaccatt

SEQ ID NO: 731 - RNA, 21 nt, synthetic construct
  modified_base 1: mod_base = OTHER; note = 2'-methoxy nucleoside; note (original language) = 2'-甲氧基核苷
  modified_base 3..5: mod_base = OTHER; note = 2'-methoxy nucleoside; note (original language) = 2'-甲氧基核苷
  modified_base 7..13: mod_base = OTHER; note = 2'-methoxy nucleoside; note (original language) = 2'-甲氧基核苷
  modified_base 15: mod_base = OTHER; note = 2'-methoxy nucleoside; note (original language) = 2'-甲氧基核苷
  modified_base 17..21: mod_base = OTHER; note = 2'-methoxy nucleoside; note (original language) = 2'-甲氧基核苷
  modified_base 2: mod_base = OTHER; note = 2'-fluoro nucleoside; note (original language) = 2'-氟核苷
  modified_base 6: mod_base = OTHER; note = 2'-fluoro nucleoside; note (original language) = 2'-氟核苷
  modified_base 14: mod_base = OTHER; note = 2'-fluoro nucleoside; note (original language) = 2'-氟核苷
  modified_base 16: mod_base = OTHER; note = 2'-fluoro nucleoside; note (original language) = 2'-氟核苷
  modified_base 1..3: mod_base = OTHER; note = phosphorothioate bond; note (original language) = 硫代磷酸酯键
  modified_base 19..21: mod_base = OTHER; note = phosphorothioate bond; note (original language) = 硫代磷酸酯键
  source 1..21: mol_type = other RNA
cattcaaacagaaattcaggt

SEQ ID NO: 732 - RNA, 21 nt, synthetic construct
  modified_base 1: mod_base = OTHER; note = 2'-methoxy nucleoside; note (original language) = 2'-甲氧基核苷
  modified_base 3..5: mod_base = OTHER; note = 2'-methoxy nucleoside; note (original language) = 2'-甲氧基核苷
  modified_base 7..13: mod_base = OTHER; note = 2'-methoxy nucleoside; note (original language) = 2'-甲氧基核苷
  modified_base 15: mod_base = OTHER; note = 2'-methoxy nucleoside; note (original language) = 2'-甲氧基核苷
  modified_base 17..21: mod_base = OTHER; note = 2'-methoxy nucleoside; note (original language) = 2'-甲氧基核苷
  modified_base 2: mod_base = OTHER; note = 2'-fluoro nucleoside; note (original language) = 2'-氟核苷
  modified_base 6: mod_base = OTHER; note = 2'-fluoro nucleoside; note (original language) = 2'-氟核苷
  modified_base 14: mod_base = OTHER; note = 2'-fluoro nucleoside; note (original language) = 2'-氟核苷
  modified_base 16: mod_base = OTHER; note = 2'-fluoro nucleoside; note (original language) = 2'-氟核苷
  modified_base 1..3: mod_base = OTHER; note = phosphorothioate bond; note (original language) = 硫代磷酸酯键
  modified_base 19..21: mod_base = OTHER; note = phosphorothioate bond; note (original language) = 硫代磷酸酯键
  source 1..21: mol_type = other RNA
ctgcaggtcataagatccttg

SEQ ID NO: 733 - RNA, 21 nt, synthetic construct
  modified_base 1: mod_base = OTHER; note = 2'-methoxy nucleoside; note (original language) = 2'-甲氧基核苷
  modified_base 3..5: mod_base = OTHER; note = 2'-methoxy nucleoside; note (original language) = 2'-甲氧基核苷
  modified_base 7..13: mod_base = OTHER; note = 2'-methoxy nucleoside; note (original language) = 2'-甲氧基核苷
  modified_base 15: mod_base = OTHER; note = 2'-methoxy nucleoside; note (original language) = 2'-甲氧基核苷
  modified_base 17..21: mod_base = OTHER; note = 2'-methoxy nucleoside; note (original language) = 2'-甲氧基核苷
  modified_base 2: mod_base = OTHER; note = 2'-fluoro nucleoside; note (original language) = 2'-氟核苷
  modified_base 6: mod_base = OTHER; note = 2'-fluoro nucleoside; note (original language) = 2'-氟核苷
  modified_base 14: mod_base = OTHER; note = 2'-fluoro nucleoside; note (original language) = 2'-氟核苷
  modified_base 16: mod_base = OTHER; note = 2'-fluoro nucleoside; note (original language) = 2'-氟核苷
  modified_base 1..3: mod_base = OTHER; note = phosphorothioate bond; note (original language) = 硫代磷酸酯键
  modified_base 19..21: mod_base = OTHER; note = phosphorothioate bond; note (original language) = 硫代磷酸酯键
  source 1..21: mol_type = other RNA
tgaacctgtcaatcttctcag

SEQ ID NO: 734 - RNA, 21 nt, synthetic construct
  modified_base 1: mod_base = OTHER; note = 2'-methoxy nucleoside; note (original language) = 2'-甲氧基核苷
  modified_base 3..5: mod_base = OTHER; note = 2'-methoxy nucleoside; note (original language) = 2'-甲氧基核苷
  modified_base 7..13: mod_base = OTHER; note = 2'-methoxy nucleoside; note (original language) = 2'-甲氧基核苷
  modified_base 15: mod_base = OTHER; note = 2'-methoxy nucleoside; note (original language) = 2'-甲氧基核苷
  modified_base 17..21: mod_base = OTHER; note = 2'-methoxy nucleoside; note (original language) = 2'-甲氧基核苷
  modified_base 2: mod_base = OTHER; note = 2'-fluoro nucleoside; note (original language) = 2'-氟核苷
  modified_base 6: mod_base = OTHER; note = 2'-fluoro nucleoside; note (original language) = 2'-氟核苷
  modified_base 14: mod_base = OTHER; note = 2'-fluoro nucleoside; note (original language) = 2'-氟核苷
  modified_base 16: mod_base = OTHER; note = 2'-fluoro nucleoside; note (original language) = 2'-氟核苷
  modified_base 1..3: mod_base = OTHER; note = phosphorothioate bond; note (original language) = 硫代磷酸酯键
  modified_base 19..21: mod_base = OTHER; note = phosphorothioate bond; note (original language) = 硫代磷酸酯键
  source 1..21: mol_type = other RNA
ttggaattctttttggaacag

SEQ ID NO: 735 - RNA, 21 nt, synthetic construct
  modified_base 1: mod_base = OTHER; note = 2'-methoxy nucleoside; note (original language) = 2'-甲氧基核苷
  modified_base 3..5: mod_base = OTHER; note = 2'-methoxy nucleoside; note (original language) = 2'-甲氧基核苷
  modified_base 7..13: mod_base = OTHER; note = 2'-methoxy nucleoside; note (original language) = 2'-甲氧基核苷
  modified_base 15: mod_base = OTHER; note = 2'-methoxy nucleoside; note (original language) = 2'-甲氧基核苷
  modified_base 17..21: mod_base = OTHER; note = 2'-methoxy nucleoside; note (original language) = 2'-甲氧基核苷
  modified_base 2: mod_base = OTHER; note = 2'-fluoro nucleoside; note (original language) = 2'-氟核苷
  modified_base 6: mod_base = OTHER; note = 2'-fluoro nucleoside; note (original language) = 2'-氟核苷
  modified_base 14: mod_base = OTHER; note = 2'-fluoro nucleoside; note (original language) = 2'-氟核苷
  modified_base 16: mod_base = OTHER; note = 2'-fluoro nucleoside; note (original language) = 2'-氟核苷
  modified_base 1..3: mod_base = OTHER; note = phosphorothioate bond; note (original language) = 硫代磷酸酯键
  modified_base 19..21: mod_base = OTHER; note = phosphorothioate bond; note (original language) = 硫代磷酸酯键
  source 1..21: mol_type = other RNA
cggaggtcatgttcttacatt

SEQ ID NO: 736 - RNA, 21 nt, synthetic construct
  modified_base 1: mod_base = OTHER; note = 2'-methoxy nucleoside; note (original language) = 2'-甲氧基核苷
  modified_base 3..5: mod_base = OTHER; note = 2'-methoxy nucleoside; note (original language) = 2'-甲氧基核苷
  modified_base 7..13: mod_base = OTHER; note = 2'-methoxy nucleoside; note (original language) = 2'-甲氧基核苷
  modified_base 15: mod_base = OTHER; note = 2'-methoxy nucleoside; note (original language) = 2'-甲氧基核苷
  modified_base 17..21: mod_base = OTHER; note = 2'-methoxy nucleoside; note (original language) = 2'-甲氧基核苷
  modified_base 2: mod_base = OTHER; note = 2'-fluoro nucleoside; note (original language) = 2'-氟核苷
  modified_base 6: mod_base = OTHER; note = 2'-fluoro nucleoside; note (original language) = 2'-氟核苷
  modified_base 14: mod_base = OTHER; note = 2'-fluoro nucleoside; note (original language) = 2'-氟核苷
  modified_base 16: mod_base = OTHER; note = 2'-fluoro nucleoside; note (original language) = 2'-氟核苷
  modified_base 1..3: mod_base = OTHER; note = phosphorothioate bond; note (original language) = 硫代磷酸酯键
  modified_base 19..21: mod_base = OTHER; note = phosphorothioate bond; note (original language) = 硫代磷酸酯键
  source 1..21: mol_type = other RNA
tagcaggccctgtacagcctg

SEQ ID NO: 737 - RNA, 21 nt, synthetic construct
  modified_base 1: mod_base = OTHER; note = 2'-methoxy nucleoside; note (original language) = 2'-甲氧基核苷
  modified_base 3..5: mod_base = OTHER; note = 2'-methoxy nucleoside; note (original language) = 2'-甲氧基核苷
  modified_base 7..13: mod_base = OTHER; note = 2'-methoxy nucleoside; note (original language) = 2'-甲氧基核苷
  modified_base 15: mod_base = OTHER; note = 2'-methoxy nucleoside; note (original language) = 2'-甲氧基核苷
  modified_base 17..21: mod_base = OTHER; note = 2'-methoxy nucleoside; note (original language) = 2'-甲氧基核苷
  modified_base 2: mod_base = OTHER; note = 2'-fluoro nucleoside; note (original language) = 2'-氟核苷
  modified_base 6: mod_base = OTHER; note = 2'-fluoro nucleoside; note (original language) = 2'-氟核苷
  modified_base 14: mod_base = OTHER; note = 2'-fluoro nucleoside; note (original language) = 2'-氟核苷
  modified_base 16: mod_base = OTHER; note = 2'-fluoro nucleoside; note (original language) = 2'-氟核苷
  modified_base 1..3: mod_base = OTHER; note = phosphorothioate bond; note (original language) = 硫代磷酸酯键
  modified_base 19..21: mod_base = OTHER; note = phosphorothioate bond; note (original language) = 硫代磷酸酯键
  source 1..21: mol_type = other RNA
tagtttcttcatccagttgag

SEQ ID NO: 738 - RNA, 21 nt, synthetic construct
  modified_base 1: mod_base = OTHER; note = 2'-methoxy nucleoside; note (original language) = 2'-甲氧基核苷
  modified_base 3..5: mod_base = OTHER; note = 2'-methoxy nucleoside; note (original language) = 2'-甲氧基核苷
  modified_base 7..13: mod_base = OTHER; note = 2'-methoxy nucleoside; note (original language) = 2'-甲氧基核苷
  modified_base 15: mod_base = OTHER; note = 2'-methoxy nucleoside; note (original language) = 2'-甲氧基核苷
  modified_base 17..21: mod_base = OTHER; note = 2'-methoxy nucleoside; note (original language) = 2'-甲氧基核苷
  modified_base 2: mod_base = OTHER; note = 2'-fluoro nucleoside; note (original language) = 2'-氟核苷
  modified_base 6: mod_base = OTHER; note = 2'-fluoro nucleoside; note (original language) = 2'-氟核苷
  modified_base 14: mod_base = OTHER; note = 2'-fluoro nucleoside; note (original language) = 2'-氟核苷
  modified_base 16: mod_base = OTHER; note = 2'-fluoro nucleoside; note (original language) = 2'-氟核苷
  modified_base 1..3: mod_base = OTHER; note = phosphorothioate bond; note (original language) = 硫代磷酸酯键
  modified_base 19..21: mod_base = OTHER; note = phosphorothioate bond; note (original language) = 硫代磷酸酯键
  source 1..21: mol_type = other RNA
ttcttcatccagttgagggag

SEQ ID NO: 739 - RNA, 21 nt, synthetic construct
  modified_base 1: mod_base = OTHER; note = 2'-methoxy nucleoside; note (original language) = 2'-甲氧基核苷
  modified_base 3..5: mod_base = OTHER; note = 2'-methoxy nucleoside; note (original language) = 2'-甲氧基核苷
  modified_base 7..13: mod_base = OTHER; note = 2'-methoxy nucleoside; note (original language) = 2'-甲氧基核苷
  modified_base 15: mod_base = OTHER; note = 2'-methoxy nucleoside; note (original language) = 2'-甲氧基核苷
  modified_base 17..21: mod_base = OTHER; note = 2'-methoxy nucleoside; note (original language) = 2'-甲氧基核苷
  modified_base 2: mod_base = OTHER; note = 2'-fluoro nucleoside; note (original language) = 2'-氟核苷
  modified_base 6: mod_base = OTHER; note = 2'-fluoro nucleoside; note (original language) = 2'-氟核苷
  modified_base 14: mod_base = OTHER; note = 2'-fluoro nucleoside; note (original language) = 2'-氟核苷
  modified_base 16: mod_base = OTHER; note = 2'-fluoro nucleoside; note (original language) = 2'-氟核苷
  modified_base 1..3: mod_base = OTHER; note = phosphorothioate bond; note (original language) = 硫代磷酸酯键
  modified_base 19..21: mod_base = OTHER; note = phosphorothioate bond; note (original language) = 硫代磷酸酯键
  source 1..21: mol_type = other RNA
tgcttgcatctttcacgtatt

SEQ ID NO: 740 - RNA, 21 nt, synthetic construct
  modified_base 1: mod_base = OTHER; note = 2'-methoxy nucleoside; note (original language) = 2'-甲氧基核苷
  modified_base 3..5: mod_base = OTHER; note = 2'-methoxy nucleoside; note (original language) = 2'-甲氧基核苷
  modified_base 7..13: mod_base = OTHER; note = 2'-methoxy nucleoside; note (original language) = 2'-甲氧基核苷
  modified_base 15: mod_base = OTHER; note = 2'-methoxy nucleoside; note (original language) = 2'-甲氧基核苷
  modified_base 17..21: mod_base = OTHER; note = 2'-methoxy nucleoside; note (original language) = 2'-甲氧基核苷
  modified_base 2: mod_base = OTHER; note = 2'-fluoro nucleoside; note (original language) = 2'-氟核苷
  modified_base 6: mod_base = OTHER; note = 2'-fluoro nucleoside; note (original language) = 2'-氟核苷
  modified_base 14: mod_base = OTHER; note = 2'-fluoro nucleoside; note (original language) = 2'-氟核苷
  modified_base 16: mod_base = OTHER; note = 2'-fluoro nucleoside; note (original language) = 2'-氟核苷
  modified_base 1..3: mod_base = OTHER; note = phosphorothioate bond; note (original language) = 硫代磷酸酯键
  modified_base 19..21: mod_base = OTHER; note = phosphorothioate bond; note (original language) = 硫代磷酸酯键
  source 1..21: mol_type = other RNA
atctgctgctggcctttgcct

SEQ ID NO: 741 - RNA, 21 nt, synthetic construct
  modified_base 1: mod_base = OTHER; note = 2'-methoxy nucleoside; note (original language) = 2'-甲氧基核苷
  modified_base 3..5: mod_base = OTHER; note = 2'-methoxy nucleoside; note (original language) = 2'-甲氧基核苷
  modified_base 7..13: mod_base = OTHER; note = 2'-methoxy nucleoside; note (original language) = 2'-甲氧基核苷
  modified_base 15: mod_base = OTHER; note = 2'-methoxy nucleoside; note (original language) = 2'-甲氧基核苷
  modified_base 17..21: mod_base = OTHER; note = 2'-methoxy nucleoside; note (original language) = 2'-甲氧基核苷
  modified_base 2: mod_base = OTHER; note = 2'-fluoro nucleoside; note (original language) = 2'-氟核苷
  modified_base 6: mod_base = OTHER; note = 2'-fluoro nucleoside; note (original language) = 2'-氟核苷
  modified_base 14: mod_base = OTHER; note = 2'-fluoro nucleoside; note (original language) = 2'-氟核苷
  modified_base 16: mod_base = OTHER; note = 2'-fluoro nucleoside; note (original language) = 2'-氟核苷
  modified_base 1..3: mod_base = OTHER; note = phosphorothioate bond; note (original language) = 硫代磷酸酯键
  modified_base 19..21: mod_base = OTHER; note = phosphorothioate bond; note (original language) = 硫代磷酸酯键
  source 1..21: mol_type = other RNA
caggtcataagatccttgcag

SEQ ID NO: 742 - RNA, 21 nt, synthetic construct
  modified_base 1: mod_base = OTHER; note = 2'-methoxy nucleoside; note (original language) = 2'-甲氧基核苷
  modified_base 3..5: mod_base = OTHER; note = 2'-methoxy nucleoside; note (original language) = 2'-甲氧基核苷
  modified_base 7..13: mod_base = OTHER; note = 2'-methoxy nucleoside; note (original language) = 2'-甲氧基核苷
  modified_base 15: mod_base = OTHER; note = 2'-methoxy nucleoside; note (original language) = 2'-甲氧基核苷
  modified_base 17..21: mod_base = OTHER; note = 2'-methoxy nucleoside; note (original language) = 2'-甲氧基核苷
  modified_base 2: mod_base = OTHER; note = 2'-fluoro nucleoside; note (original language) = 2'-氟核苷
  modified_base 6: mod_base = OTHER; note = 2'-fluoro nucleoside; note (original language) = 2'-氟核苷
  modified_base 14: mod_base = OTHER; note = 2'-fluoro nucleoside; note (original language) = 2'-氟核苷
  modified_base 16: mod_base = OTHER; note = 2'-fluoro nucleoside; note (original language) = 2'-氟核苷
  modified_base 1..3: mod_base = OTHER; note = phosphorothioate bond; note (original language) = 硫代磷酸酯键
  modified_base 19..21: mod_base = OTHER; note = phosphorothioate bond; note (original language) = 硫代磷酸酯键
  source 1..21: mol_type = other RNA
ttgcctgtagcctgtcagctg

SEQ ID NO: 743 - RNA, 21 nt, synthetic construct
  modified_base 1: mod_base = OTHER; note = 2'-methoxy nucleoside; note (original language) = 2'-甲氧基核苷
  modified_base 3..5: mod_base = OTHER; note = 2'-methoxy nucleoside; note (original language) = 2'-甲氧基核苷
  modified_base 7..13: mod_base = OTHER; note = 2'-methoxy nucleoside; note (original language) = 2'-甲氧基核苷
  modified_base 15: mod_base = OTHER; note = 2'-methoxy nucleoside; note (original language) = 2'-甲氧基核苷
  modified_base 17..21: mod_base = OTHER; note = 2'-methoxy nucleoside; note (original language) = 2'-甲氧基核苷
  modified_base 2: mod_base = OTHER; note = 2'-fluoro nucleoside; note (original language) = 2'-氟核苷
  modified_base 6: mod_base = OTHER; note = 2'-fluoro nucleoside; note (original language) = 2'-氟核苷
  modified_base 14: mod_base = OTHER; note = 2'-fluoro nucleoside; note (original language) = 2'-氟核苷
  modified_base 16: mod_base = OTHER; note = 2'-fluoro nucleoside; note (original language) = 2'-氟核苷
  modified_base 1..3: mod_base = OTHER; note = phosphorothioate bond; note (original language) = 硫代磷酸酯键
  modified_base 19..21: mod_base = OTHER; note = phosphorothioate bond; note (original language) = 硫代磷酸酯键
  source 1..21: mol_type = other RNA
tttattactaacacaagggag

SEQ ID NO: 744 - RNA, 21 nt, synthetic construct
  modified_base 1: mod_base = OTHER; note = 2'-methoxy nucleoside; note (original language) = 2'-甲氧基核苷
  modified_base 3..5: mod_base = OTHER; note = 2'-methoxy nucleoside; note (original language) = 2'-甲氧基核苷
  modified_base 7..13: mod_base = OTHER; note = 2'-methoxy nucleoside; note (original language) = 2'-甲氧基核苷
  modified_base 15: mod_base = OTHER; note = 2'-methoxy nucleoside; note (original language) = 2'-甲氧基核苷
  modified_base 17..21: mod_base = OTHER; note = 2'-methoxy nucleoside; note (original language) = 2'-甲氧基核苷
  modified_base 2: mod_base = OTHER; note = 2'-fluoro nucleoside; note (original language) = 2'-氟核苷
  modified_base 6: mod_base = OTHER; note = 2'-fluoro nucleoside; note (original language) = 2'-氟核苷
  modified_base 14: mod_base = OTHER; note = 2'-fluoro nucleoside; note (original language) = 2'-氟核苷
  modified_base 16: mod_base = OTHER; note = 2'-fluoro nucleoside; note (original language) = 2'-氟核苷
  modified_base 1..3: mod_base = OTHER; note = phosphorothioate bond; note (original language) = 硫代磷酸酯键
  modified_base 19..21: mod_base = OTHER; note = phosphorothioate bond; note (original language) = 硫代磷酸酯键
  source 1..21: mol_type = other RNA
caaacagaaattcaggtgctt

SEQ ID NO: 745 - RNA, 21 nt, synthetic construct
  modified_base 1: mod_base = OTHER; note = 2'-methoxy nucleoside; note (original language) = 2'-甲氧基核苷
  modified_base 3..5: mod_base = OTHER; note = 2'-methoxy nucleoside; note (original language) = 2'-甲氧基核苷
  modified_base 7..13: mod_base = OTHER; note = 2'-methoxy nucleoside; note (original language) = 2'-甲氧基核苷
  modified_base 15: mod_base = OTHER; note = 2'-methoxy nucleoside; note (original language) = 2'-甲氧基核苷
  modified_base 17..21: mod_base = OTHER; note = 2'-methoxy nucleoside; note (original language) = 2'-甲氧基核苷
  modified_base 2: mod_base = OTHER; note = 2'-fluoro nucleoside; note (original language) = 2'-氟核苷
  modified_base 6: mod_base = OTHER; note = 2'-fluoro nucleoside; note (original language) = 2'-氟核苷
  modified_base 14: mod_base = OTHER; note = 2'-fluoro nucleoside; note (original language) = 2'-氟核苷
  modified_base 16: mod_base = OTHER; note = 2'-fluoro nucleoside; note (original language) = 2'-氟核苷
  modified_base 1..3: mod_base = OTHER; note = phosphorothioate bond; note (original language) = 硫代磷酸酯键
  modified_base 19..21: mod_base = OTHER; note = phosphorothioate bond; note (original language) = 硫代磷酸酯键
  source 1..21: mol_type = other RNA
ctggcctcatgctgtgctcag

SEQ ID NO: 746 - RNA, 21 nt, synthetic construct
  modified_base 1: mod_base = OTHER; note = 2'-methoxy nucleoside; note (original language) = 2'-甲氧基核苷
  modified_base 3..5: mod_base = OTHER; note = 2'-methoxy nucleoside; note (original language) = 2'-甲氧基核苷
  modified_base 7..13: mod_base = OTHER; note = 2'-methoxy nucleoside; note (original language) = 2'-甲氧基核苷
  modified_base 15: mod_base = OTHER; note = 2'-methoxy nucleoside; note (original language) = 2'-甲氧基核苷
  modified_base 17..21: mod_base = OTHER; note = 2'-methoxy nucleoside; note (original language) = 2'-甲氧基核苷
  modified_base 2: mod_base = OTHER; note = 2'-fluoro nucleoside; note (original language) = 2'-氟核苷
  modified_base 6: mod_base = OTHER; note = 2'-fluoro nucleoside; note (original language) = 2'-氟核苷
  modified_base 14: mod_base = OTHER; note = 2'-fluoro nucleoside; note (original language) = 2'-氟核苷
  modified_base 16: mod_base = OTHER; note = 2'-fluoro nucleoside; note (original language) = 2'-氟核苷
  modified_base 1..3: mod_base = OTHER; note = phosphorothioate bond; note (original language) = 硫代磷酸酯键
  modified_base 19..21: mod_base = OTHER; note = phosphorothioate bond; note (original language) = 硫代磷酸酯键
  source 1..21: mol_type = other RNA
tattactaacacaagggagaa

SEQ ID NO: 747 - RNA, 21 nt, synthetic construct
  modified_base 1: mod_base = OTHER; note = 2'-methoxy nucleoside; note (original language) = 2'-甲氧基核苷
  modified_base 3..5: mod_base = OTHER; note = 2'-methoxy nucleoside; note (original language) = 2'-甲氧基核苷
  modified_base 7..13: mod_base = OTHER; note = 2'-methoxy nucleoside; note (original language) = 2'-甲氧基核苷
  modified_base 15: mod_base = OTHER; note = 2'-methoxy nucleoside; note (original language) = 2'-甲氧基核苷
  modified_base 17..21: mod_base = OTHER; note = 2'-methoxy nucleoside; note (original language) = 2'-甲氧基核苷
  modified_base 2: mod_base = OTHER; note = 2'-fluoro nucleoside; note (original language) = 2'-氟核苷
  modified_base 6: mod_base = OTHER; note = 2'-fluoro nucleoside; note (original language) = 2'-氟核苷
  modified_base 14: mod_base = OTHER; note = 2'-fluoro nucleoside; note (original language) = 2'-氟核苷
  modified_base 16: mod_base = OTHER; note = 2'-fluoro nucleoside; note (original language) = 2'-氟核苷
  modified_base 1..3: mod_base = OTHER; note = phosphorothioate bond; note (original language) = 硫代磷酸酯键
  modified_base 19..21: mod_base = OTHER; note = phosphorothioate bond; note (original language) = 硫代磷酸酯键
  source 1..21: mol_type = other RNA
tgcatctttcacgtattgttc

SEQ ID NO: 748 - RNA, 21 nt, synthetic construct
  modified_base 1: mod_base = OTHER; note = 2'-methoxy nucleoside; note (original language) = 2'-甲氧基核苷
  modified_base 3..5: mod_base = OTHER; note = 2'-methoxy nucleoside; note (original language) = 2'-甲氧基核苷
  modified_base 7..13: mod_base = OTHER; note = 2'-methoxy nucleoside; note (original language) = 2'-甲氧基核苷
  modified_base 15: mod_base = OTHER; note = 2'-methoxy nucleoside; note (original language) = 2'-甲氧基核苷
  modified_base 17..21: mod_base = OTHER; note = 2'-methoxy nucleoside; note (original language) = 2'-甲氧基核苷
  modified_base 2: mod_base = OTHER; note = 2'-fluoro nucleoside; note (original language) = 2'-氟核苷
  modified_base 6: mod_base = OTHER; note = 2'-fluoro nucleoside; note (original language) = 2'-氟核苷
  modified_base 14: mod_base = OTHER; note = 2'-fluoro nucleoside; note (original language) = 2'-氟核苷
  modified_base 16: mod_base = OTHER; note = 2'-fluoro nucleoside; note (original language) = 2'-氟核苷
  modified_base 1..3: mod_base = OTHER; note = phosphorothioate bond; note (original language) = 硫代磷酸酯键
  modified_base 19..21: mod_base = OTHER; note = phosphorothioate bond; note (original language) = 硫代磷酸酯键
  source 1..21: mol_type = other RNA
catctttcacgtattgttcaa

SEQ ID NO: 749 - RNA, 21 nt, synthetic construct
  modified_base 1: mod_base = OTHER; note = 2'-methoxy nucleoside; note (original language) = 2'-甲氧基核苷
  modified_base 3..5: mod_base = OTHER; note = 2'-methoxy nucleoside; note (original language) = 2'-甲氧基核苷
  modified_base 7..13: mod_base = OTHER; note = 2'-methoxy nucleoside; note (original language) = 2'-甲氧基核苷
  modified_base 15: mod_base = OTHER; note = 2'-methoxy nucleoside; note (original language) = 2'-甲氧基核苷
  modified_base 17..21: mod_base = OTHER; note = 2'-methoxy nucleoside; note (original language) = 2'-甲氧基核苷
  modified_base 2: mod_base = OTHER; note = 2'-fluoro nucleoside; note (original language) = 2'-氟核苷
  modified_base 6: mod_base = OTHER; note = 2'-fluoro nucleoside; note (original language) = 2'-氟核苷
  modified_base 14: mod_base = OTHER; note = 2'-fluoro nucleoside; note (original language) = 2'-氟核苷
  modified_base 16: mod_base = OTHER; note = 2'-fluoro nucleoside; note (original language) = 2'-氟核苷
  modified_base 1..3: mod_base = OTHER; note = phosphorothioate bond; note (original language) = 硫代磷酸酯键
  modified_base 19..21: mod_base = OTHER; note = phosphorothioate bond; note (original language) = 硫代磷酸酯键
  source 1..21: mol_type = other RNA
tactaacacaagggagaaata

SEQ ID NO: 750 - RNA, 21 nt, synthetic construct
  modified_base 1: mod_base = OTHER; note = 2'-methoxy nucleoside; note (original language) = 2'-甲氧基核苷
  modified_base 3..5: mod_base = OTHER; note = 2'-methoxy nucleoside; note (original language) = 2'-甲氧基核苷
  modified_base 7..13: mod_base = OTHER; note = 2'-methoxy nucleoside; note (original language) = 2'-甲氧基核苷
  modified_base 15: mod_base = OTHER; note = 2'-methoxy nucleoside; note (original language) = 2'-甲氧基核苷
  modified_base 17..21: mod_base = OTHER; note = 2'-methoxy nucleoside; note (original language) = 2'-甲氧基核苷
  modified_base 2: mod_base = OTHER; note = 2'-fluoro nucleoside; note (original language) = 2'-氟核苷
  modified_base 6: mod_base = OTHER; note = 2'-fluoro nucleoside; note (original language) = 2'-氟核苷
  modified_base 14: mod_base = OTHER; note = 2'-fluoro nucleoside; note (original language) = 2'-氟核苷
  modified_base 16: mod_base = OTHER; note = 2'-fluoro nucleoside; note (original language) = 2'-氟核苷
  modified_base 1..3: mod_base = OTHER; note = phosphorothioate bond; note (original language) = 硫代磷酸酯键
  modified_base 19..21: mod_base = OTHER; note = phosphorothioate bond; note (original language) = 硫代磷酸酯键
  source 1..21: mol_type = other RNA
ttgggcttcccggcattggcc

SEQ ID NO: 751 - RNA, 21 nt, synthetic construct
  modified_base 1: mod_base = OTHER; note = 2'-methoxy nucleoside; note (original language) = 2'-甲氧基核苷
  modified_base 3..5: mod_base = OTHER; note = 2'-methoxy nucleoside; note (original language) = 2'-甲氧基核苷
  modified_base 7..13: mod_base = OTHER; note = 2'-methoxy nucleoside; note (original language) = 2'-甲氧基核苷
  modified_base 15: mod_base = OTHER; note = 2'-methoxy nucleoside; note (original language) = 2'-甲氧基核苷
  modified_base 17..21: mod_base = OTHER; note = 2'-methoxy nucleoside; note (original language) = 2'-甲氧基核苷
  modified_base 2: mod_base = OTHER; note = 2'-fluoro nucleoside; note (original language) = 2'-氟核苷
  modified_base 6: mod_base = OTHER; note = 2'-fluoro nucleoside; note (original language) = 2'-氟核苷
  modified_base 14: mod_base = OTHER; note = 2'-fluoro nucleoside; note (original language) = 2'-氟核苷
  modified_base 16: mod_base = OTHER; note = 2'-fluoro nucleoside; note (original language) = 2'-氟核苷
  modified_base 1..3: mod_base = OTHER; note = phosphorothioate bond; note (original language) = 硫代磷酸酯键
  modified_base 19..21: mod_base = OTHER; note = phosphorothioate bond; note (original language) = 硫代磷酸酯键
  source 1..21: mol_type = other RNA
agaaattcaggtgcttgcatc

SEQ ID NO: 752 - RNA, 21 nt, synthetic construct
  modified_base 1: mod_base = OTHER; note = 2'-methoxy nucleoside; note (original language) = 2'-甲氧基核苷
  modified_base 3..5: mod_base = OTHER; note = 2'-methoxy nucleoside; note (original language) = 2'-甲氧基核苷
  modified_base 7..13: mod_base = OTHER; note = 2'-methoxy nucleoside; note (original language) = 2'-甲氧基核苷
  modified_base 15: mod_base = OTHER; note = 2'-methoxy nucleoside; note (original language) = 2'-甲氧基核苷
  modified_base 17..21: mod_base = OTHER; note = 2'-methoxy nucleoside; note (original language) = 2'-甲氧基核苷
  modified_base 2: mod_base = OTHER; note = 2'-fluoro nucleoside; note (original language) = 2'-氟核苷
  modified_base 6: mod_base = OTHER; note = 2'-fluoro nucleoside; note (original language) = 2'-氟核苷
  modified_base 14: mod_base = OTHER; note = 2'-fluoro nucleoside; note (original language) = 2'-氟核苷
  modified_base 16: mod_base = OTHER; note = 2'-fluoro nucleoside; note (original language) = 2'-氟核苷
  modified_base 1..3: mod_base = OTHER; note = phosphorothioate bond; note (original language) = 硫代磷酸酯键
  modified_base 19..21: mod_base = OTHER; note = phosphorothioate bond; note (original language) = 硫代磷酸酯键
  source 1..21: mol_type = other RNA
ataagatccttgcagcaccag

SEQ ID NO: 753 - RNA, 21 nt, synthetic construct
  modified_base 1: mod_base = OTHER; note = 2'-methoxy nucleoside; note (original language) = 2'-甲氧基核苷
  modified_base 3..5: mod_base = OTHER; note = 2'-methoxy nucleoside; note (original language) = 2'-甲氧基核苷
  modified_base 7..13: mod_base = OTHER; note = 2'-methoxy nucleoside; note (original language) = 2'-甲氧基核苷
  modified_base 15: mod_base = OTHER; note = 2'-methoxy nucleoside; note (original language) = 2'-甲氧基核苷
  modified_base 17..21: mod_base = OTHER; note = 2'-methoxy nucleoside; note (original language) = 2'-甲氧基核苷
  modified_base 2: mod_base = OTHER; note = 2'-fluoro nucleoside; note (original language) = 2'-氟核苷
  modified_base 6: mod_base = OTHER; note = 2'-fluoro nucleoside; note (original language) = 2'-氟核苷
  modified_base 14: mod_base = OTHER; note = 2'-fluoro nucleoside; note (original language) = 2'-氟核苷
  modified_base 16: mod_base = OTHER; note = 2'-fluoro nucleoside; note (original language) = 2'-氟核苷
  modified_base 1..3: mod_base = OTHER; note = phosphorothioate bond; note (original language) = 硫代磷酸酯键
  modified_base 19..21: mod_base = OTHER; note = phosphorothioate bond; note (original language) = 硫代磷酸酯键
  source 1..21: mol_type = other RNA
tagcctgtcagctgtgtggtc

SEQ ID NO: 754 - RNA, 21 nt, synthetic construct
  modified_base 1: mod_base = OTHER; note = 2'-methoxy nucleoside; note (original language) = 2'-甲氧基核苷
  modified_base 3..5: mod_base = OTHER; note = 2'-methoxy nucleoside; note (original language) = 2'-甲氧基核苷
  modified_base 7..13: mod_base = OTHER; note = 2'-methoxy nucleoside; note (original language) = 2'-甲氧基核苷
  modified_base 15: mod_base = OTHER; note = 2'-methoxy nucleoside; note (original language) = 2'-甲氧基核苷
  modified_base 17..21: mod_base = OTHER; note = 2'-methoxy nucleoside; note (original language) = 2'-甲氧基核苷
  modified_base 2: mod_base = OTHER; note = 2'-fluoro nucleoside; note (original language) = 2'-氟核苷
  modified_base 6: mod_base = OTHER; note = 2'-fluoro nucleoside; note (original language) = 2'-氟核苷
  modified_base 14: mod_base = OTHER; note = 2'-fluoro nucleoside; note (original language) = 2'-氟核苷
  modified_base 16: mod_base = OTHER; note = 2'-fluoro nucleoside; note (original language) = 2'-氟核苷
  modified_base 1..3: mod_base = OTHER; note = phosphorothioate bond; note (original language) = 硫代磷酸酯键
  modified_base 19..21: mod_base = OTHER; note = phosphorothioate bond; note (original language) = 硫代磷酸酯键
  source 1..21: mol_type = other RNA
tctttcacgtattgttcaaaa

SEQ ID NO: 755 - RNA, 21 nt, synthetic construct
  modified_base 1: mod_base = OTHER; note = 2'-methoxy nucleoside; note (original language) = 2'-甲氧基核苷
  modified_base 3..5: mod_base = OTHER; note = 2'-methoxy nucleoside; note (original language) = 2'-甲氧基核苷
  modified_base 7..13: mod_base = OTHER; note = 2'-methoxy nucleoside; note (original language) = 2'-甲氧基核苷
  modified_base 15: mod_base = OTHER; note = 2'-methoxy nucleoside; note (original language) = 2'-甲氧基核苷
  modified_base 17..21: mod_base = OTHER; note = 2'-methoxy nucleoside; note (original language) = 2'-甲氧基核苷
  modified_base 2: mod_base = OTHER; note = 2'-fluoro nucleoside; note (original language) = 2'-氟核苷
  modified_base 6: mod_base = OTHER; note = 2'-fluoro nucleoside; note (original language) = 2'-氟核苷
  modified_base 14: mod_base = OTHER; note = 2'-fluoro nucleoside; note (original language) = 2'-氟核苷
  modified_base 16: mod_base = OTHER; note = 2'-fluoro nucleoside; note (original language) = 2'-氟核苷
  modified_base 1..3: mod_base = OTHER; note = phosphorothioate bond; note (original language) = 硫代磷酸酯键
  modified_base 19..21: mod_base = OTHER; note = phosphorothioate bond; note (original language) = 硫代磷酸酯键
  source 1..21: mol_type = other RNA
tcaacttgtcttcggtgtcaa

SEQ ID NO: 756 - RNA, 21 nt, synthetic construct
  modified_base 1: mod_base = OTHER; note = 2'-methoxy nucleoside; note (original language) = 2'-甲氧基核苷
  modified_base 3..5: mod_base = OTHER; note = 2'-methoxy nucleoside; note (original language) = 2'-甲氧基核苷
  modified_base 7..13: mod_base = OTHER; note = 2'-methoxy nucleoside; note (original language) = 2'-甲氧基核苷
  modified_base 15: mod_base = OTHER; note = 2'-methoxy nucleoside; note (original language) = 2'-甲氧基核苷
  modified_base 17..21: mod_base = OTHER; note = 2'-methoxy nucleoside; note (original language) = 2'-甲氧基核苷
  modified_base 2: mod_base = OTHER; note = 2'-fluoro nucleoside; note (original language) = 2'-氟核苷
  modified_base 6: mod_base = OTHER; note = 2'-fluoro nucleoside; note (original language) = 2'-氟核苷
  modified_base 14: mod_base = OTHER; note = 2'-fluoro nucleoside; note (original language) = 2'-氟核苷
  modified_base 16: mod_base = OTHER; note = 2'-fluoro nucleoside; note (original language) = 2'-氟核苷
  modified_base 1..3: mod_base = OTHER; note = phosphorothioate bond; note (original language) = 硫代磷酸酯键
  modified_base 19..21: mod_base = OTHER; note = phosphorothioate bond; note (original language) = 硫代磷酸酯键
  source 1..21: mol_type = other RNA
gtgctgtccacactggctccc

SEQ ID NO: 757 - RNA, 21 nt, synthetic construct
  modified_base 1: mod_base = OTHER; note = 2'-methoxy nucleoside; note (original language) = 2'-甲氧基核苷
  modified_base 3..5: mod_base = OTHER; note = 2'-methoxy nucleoside; note (original language) = 2'-甲氧基核苷
  modified_base 7..13: mod_base = OTHER; note = 2'-methoxy nucleoside; note (original language) = 2'-甲氧基核苷
  modified_base 15: mod_base = OTHER; note = 2'-methoxy nucleoside; note (original language) = 2'-甲氧基核苷
  modified_base 17..21: mod_base = OTHER; note = 2'-methoxy nucleoside; note (original language) = 2'-甲氧基核苷
  modified_base 2: mod_base = OTHER; note = 2'-fluoro nucleoside; note (original language) = 2'-氟核苷
  modified_base 6: mod_base = OTHER; note = 2'-fluoro nucleoside; note (original language) = 2'-氟核苷
  modified_base 14: mod_base = OTHER; note = 2'-fluoro nucleoside; note (original language) = 2'-氟核苷
  modified_base 16: mod_base = OTHER; note = 2'-fluoro nucleoside; note (original language) = 2'-氟核苷
  modified_base 1..3: mod_base = OTHER; note = phosphorothioate bond; note (original language) = 硫代磷酸酯键
  modified_base 19..21: mod_base = OTHER; note = phosphorothioate bond; note (original language) = 硫代磷酸酯键
  source 1..21: mol_type = other RNA
tgcagttcttgtccttccaag

SEQ ID NO: 758 - RNA, 21 nt, synthetic construct
  modified_base 1: mod_base = OTHER; note = 2'-methoxy nucleoside; note (original language) = 2'-甲氧基核苷
  modified_base 3..5: mod_base = OTHER; note = 2'-methoxy nucleoside; note (original language) = 2'-甲氧基核苷
  modified_base 7..13: mod_base = OTHER; note = 2'-methoxy nucleoside; note (original language) = 2'-甲氧基核苷
  modified_base 15: mod_base = OTHER; note = 2'-methoxy nucleoside; note (original language) = 2'-甲氧基核苷
  modified_base 17..21: mod_base = OTHER; note = 2'-methoxy nucleoside; note (original language) = 2'-甲氧基核苷
  modified_base 2: mod_base = OTHER; note = 2'-fluoro nucleoside; note (original language) = 2'-氟核苷
  modified_base 6: mod_base = OTHER; note = 2'-fluoro nucleoside; note (original language) = 2'-氟核苷
  modified_base 14: mod_base = OTHER; note = 2'-fluoro nucleoside; note (original language) = 2'-氟核苷
  modified_base 16: mod_base = OTHER; note = 2'-fluoro nucleoside; note (original language) = 2'-氟核苷
  modified_base 1..3: mod_base = OTHER; note = phosphorothioate bond; note (original language) = 硫代磷酸酯键
  modified_base 19..21: mod_base = OTHER; note = phosphorothioate bond; note (original language) = 硫代磷酸酯键
  source 1..21: mol_type = other RNA
ttgagtcaccgagaagttgtc

SEQ ID NO: 759 - RNA, 21 nt, synthetic construct
  modified_base 1: mod_base = OTHER; note = 2'-methoxy nucleoside; note (original language) = 2'-甲氧基核苷
  modified_base 3..5: mod_base = OTHER; note = 2'-methoxy nucleoside; note (original language) = 2'-甲氧基核苷
  modified_base 7..13: mod_base = OTHER; note = 2'-methoxy nucleoside; note (original language) = 2'-甲氧基核苷
  modified_base 15: mod_base = OTHER; note = 2'-methoxy nucleoside; note (original language) = 2'-甲氧基核苷
  modified_base 17..21: mod_base = OTHER; note = 2'-methoxy nucleoside; note (original language) = 2'-甲氧基核苷
  modified_base 2: mod_base = OTHER; note = 2'-fluoro nucleoside; note (original language) = 2'-氟核苷
  modified_base 6: mod_base = OTHER; note = 2'-fluoro nucleoside; note (original language) = 2'-氟核苷
  modified_base 14: mod_base = OTHER; note = 2'-fluoro nucleoside; note (original language) = 2'-氟核苷
  modified_base 16: mod_base = OTHER; note = 2'-fluoro nucleoside; note (original language) = 2'-氟核苷
  modified_base 1..3: mod_base = OTHER; note = phosphorothioate bond; note (original language) = 硫代磷酸酯键
  modified_base 19..21: mod_base = OTHER; note = phosphorothioate bond; note (original language) = 硫代磷酸酯键
  source 1..21: mol_type = other RNA
cttattgtggcaagacgttta

SEQ ID NO: 760 - RNA, 21 nt, synthetic construct
  modified_base 1: mod_base = OTHER; note = 2'-methoxy nucleoside; note (original language) = 2'-甲氧基核苷
  modified_base 3..5: mod_base = OTHER; note = 2'-methoxy nucleoside; note (original language) = 2'-甲氧基核苷
  modified_base 7..13: mod_base = OTHER; note = 2'-methoxy nucleoside; note (original language) = 2'-甲氧基核苷
  modified_base 15: mod_base = OTHER; note = 2'-methoxy nucleoside; note (original language) = 2'-甲氧基核苷
  modified_base 17..21: mod_base = OTHER; note = 2'-methoxy nucleoside; note (original language) = 2'-甲氧基核苷
  modified_base 2: mod_base = OTHER; note = 2'-fluoro nucleoside; note (original language) = 2'-氟核苷
  modified_base 6: mod_base = OTHER; note = 2'-fluoro nucleoside; note (original language) = 2'-氟核苷
  modified_base 14: mod_base = OTHER; note = 2'-fluoro nucleoside; note (original language) = 2'-氟核苷
  modified_base 16: mod_base = OTHER; note = 2'-fluoro nucleoside; note (original language) = 2'-氟核苷
  modified_base 1..3: mod_base = OTHER; note = phosphorothioate bond; note (original language) = 硫代磷酸酯键
  modified_base 19..21: mod_base = OTHER; note = phosphorothioate bond; note (original language) = 硫代磷酸酯键
  source 1..21: mol_type = other RNA
aacctgtcaatcttctcagca

SEQ ID NO: 761 - RNA, 21 nt, synthetic construct
  modified_base 1: mod_base = OTHER; note = 2'-methoxy nucleoside; note (original language) = 2'-甲氧基核苷
  modified_base 3..5: mod_base = OTHER; note = 2'-methoxy nucleoside; note (original language) = 2'-甲氧基核苷
  modified_base 7..13: mod_base = OTHER; note = 2'-methoxy nucleoside; note (original language) = 2'-甲氧基核苷
  modified_base 15: mod_base = OTHER; note = 2'-methoxy nucleoside; note (original language) = 2'-甲氧基核苷
  modified_base 17..21: mod_base = OTHER; note = 2'-methoxy nucleoside; note (original language) = 2'-甲氧基核苷
  modified_base 2: mod_base = OTHER; note = 2'-fluoro nucleoside; note (original language) = 2'-氟核苷
  modified_base 6: mod_base = OTHER; note = 2'-fluoro nucleoside; note (original language) = 2'-氟核苷
  modified_base 14: mod_base = OTHER; note = 2'-fluoro nucleoside; note (original language) = 2'-氟核苷
  modified_base 16: mod_base = OTHER; note = 2'-fluoro nucleoside; note (original language) = 2'-氟核苷
  modified_base 1..3: mod_base = OTHER; note = phosphorothioate bond; note (original language) = 硫代磷酸酯键
  modified_base 19..21: mod_base = OTHER; note = phosphorothioate bond; note (original language) = 硫代磷酸酯键
  source 1..21: mol_type = other RNA
aataaacccagcaaactggga

SEQ ID NO: 762 - RNA, 21 nt, synthetic construct
  modified_base 1: mod_base = OTHER; note = 2'-methoxy nucleoside; note (original language) = 2'-甲氧基核苷
  modified_base 3..5: mod_base = OTHER; note = 2'-methoxy nucleoside; note (original language) = 2'-甲氧基核苷
  modified_base 7..13: mod_base = OTHER; note = 2'-methoxy nucleoside; note (original language) = 2'-甲氧基核苷
  modified_base 15: mod_base = OTHER; note = 2'-methoxy nucleoside; note (original language) = 2'-甲氧基核苷
  modified_base 17..21: mod_base = OTHER; note = 2'-methoxy nucleoside; note (original language) = 2'-甲氧基核苷
  modified_base 2: mod_base = OTHER; note = 2'-fluoro nucleoside; note (original language) = 2'-氟核苷
  modified_base 6: mod_base = OTHER; note = 2'-fluoro nucleoside; note (original language) = 2'-氟核苷
  modified_base 14: mod_base = OTHER; note = 2'-fluoro nucleoside; note (original language) = 2'-氟核苷
  modified_base 16: mod_base = OTHER; note = 2'-fluoro nucleoside; note (original language) = 2'-氟核苷
  modified_base 1..3: mod_base = OTHER; note = phosphorothioate bond; note (original language) = 硫代磷酸酯键
  modified_base 19..21: mod_base = OTHER; note = phosphorothioate bond; note (original language) = 硫代磷酸酯键
  source 1..21: mol_type = other RNA
acttgagtcaccgagaagttg

SEQ ID NO: 763 - RNA, 23 nt, synthetic construct
  modified_base 1: mod_base = OTHER; note = 2'-methoxy nucleoside; note (original language) = 2'-甲氧基核苷
  modified_base 3..5: mod_base = OTHER; note = 2'-methoxy nucleoside; note (original language) = 2'-甲氧基核苷
  modified_base 7: mod_base = OTHER; note = 2'-methoxy nucleoside; note (original language) = 2'-甲氧基核苷
  modified_base 9..13: mod_base = OTHER; note = 2'-methoxy nucleoside; note (original language) = 2'-甲氧基核苷
  modified_base 15: mod_base = OTHER; note = 2'-methoxy nucleoside; note (original language) = 2'-甲氧基核苷
  modified_base 17..23: mod_base = OTHER; note = 2'-methoxy nucleoside; note (original language) = 2'-甲氧基核苷
  modified_base 2: mod_base = OTHER; note = 2'-fluoro nucleoside; note (original language) = 2'-氟核苷
  modified_base 6: mod_base = OTHER; note = 2'-fluoro nucleoside; note (original language) = 2'-氟核苷
  modified_base 8: mod_base = OTHER; note = 2'-fluoro nucleoside; note (original language) = 2'-氟核苷
  modified_base 14: mod_base = OTHER; note = 2'-fluoro nucleoside; note (original language) = 2'-氟核苷
  modified_base 16: mod_base = OTHER; note = 2'-fluoro nucleoside; note (original language) = 2'-氟核苷
  modified_base 1..3: mod_base = OTHER; note = phosphorothioate bond; note (original language) = 硫代磷酸酯键
  modified_base 21..23: mod_base = OTHER; note = phosphorothioate bond; note (original language) = 硫代磷酸酯键
  source 1..23: mol_type = other RNA
acttagaccaaggagaaacgcct

SEQ ID NO: 764 - RNA, 23 nt, synthetic construct
  modified_base 1: mod_base = OTHER; note = 2'-methoxy nucleoside; note (original language) = 2'-甲氧基核苷
  modified_base 3..5: mod_base = OTHER; note = 2'-methoxy nucleoside; note (original language) = 2'-甲氧基核苷
  modified_base 7..8: mod_base = OTHER; note = 2'-methoxy nucleoside; note (original language) = 2'-甲氧基核苷
  modified_base 10..13: mod_base = OTHER; note = 2'-methoxy nucleoside; note (original language) = 2'-甲氧基核苷
  modified_base 15: mod_base = OTHER; note = 2'-methoxy nucleoside; note (original language) = 2'-甲氧基核苷
  modified_base 17..23: mod_base = OTHER; note = 2'-methoxy nucleoside; note (original language) = 2'-甲氧基核苷
  modified_base 2: mod_base = OTHER; note = 2'-fluoro nucleoside; note (original language) = 2'-氟核苷
  modified_base 6: mod_base = OTHER; note = 2'-fluoro nucleoside; note (original language) = 2'-氟核苷
  modified_base 9: mod_base = OTHER; note = 2'-fluoro nucleoside; note (original language) = 2'-氟核苷
  modified_base 14: mod_base = OTHER; note = 2'-fluoro nucleoside; note (original language) = 2'-氟核苷
  modified_base 16: mod_base = OTHER; note = 2'-fluoro nucleoside; note (original language) = 2'-氟核苷
  modified_base 1..3: mod_base = OTHER; note = phosphorothioate bond; note (original language) = 硫代磷酸酯键
  modified_base 21..23: mod_base = OTHER; note = phosphorothioate bond; note (original language) = 硫代磷酸酯键
  source 1..23: mol_type = other RNA
acttagaccaaggagaaacgcct

SEQ ID NO: 765 - RNA, 21 nt, synthetic construct
  modified_base 1: mod_base = OTHER; note = 2'-methoxy nucleoside; note (original language) = 2'-甲氧基核苷
  modified_base 3..5: mod_base = OTHER; note = 2'-methoxy nucleoside; note (original language) = 2'-甲氧基核苷
  modified_base 7..13: mod_base = OTHER; note = 2'-methoxy nucleoside; note (original language) = 2'-甲氧基核苷
  modified_base 15: mod_base = OTHER; note = 2'-methoxy nucleoside; note (original language) = 2'-甲氧基核苷
  modified_base 17..21: mod_base = OTHER; note = 2'-methoxy nucleoside; note (original language) = 2'-甲氧基核苷
  modified_base 2: mod_base = OTHER; note = 2'-fluoro nucleoside; note (original language) = 2'-氟核苷
  modified_base 6: mod_base = OTHER; note = 2'-fluoro nucleoside; note (original language) = 2'-氟核苷
  modified_base 14: mod_base = OTHER; note = 2'-fluoro nucleoside; note (original language) = 2'-氟核苷
  modified_base 16: mod_base = OTHER; note = 2'-fluoro nucleoside; note (original language) = 2'-氟核苷
  modified_base 1..3: mod_base = OTHER; note = phosphorothioate bond; note (original language) = 硫代磷酸酯键
  modified_base 19..21: mod_base = OTHER; note = phosphorothioate bond; note (original language) = 硫代磷酸酯键
  modified_base 1: mod_base = OTHER; note = 2'-methoxy-5'-vinyl phosphonate nucleoside; note (original language) = 2'-甲氧基-5'-乙烯基膦酸核苷
  source 1..21: mol_type = other RNA
ttagaagaaaaggtgggagac

SEQ ID NO: 766 - RNA, 21 nt, synthetic construct
  modified_base 1: mod_base = OTHER; note = 2'-methoxy nucleoside; note (original language) = 2'-甲氧基核苷
  modified_base 3..5: mod_base = OTHER; note = 2'-methoxy nucleoside; note (original language) = 2'-甲氧基核苷
  modified_base 7..13: mod_base = OTHER; note = 2'-methoxy nucleoside; note (original language) = 2'-甲氧基核苷
  modified_base 15: mod_base = OTHER; note = 2'-methoxy nucleoside; note (original language) = 2'-甲氧基核苷
  modified_base 17..21: mod_base = OTHER; note = 2'-methoxy nucleoside; note (original language) = 2'-甲氧基核苷
  modified_base 2: mod_base = OTHER; note = 2'-fluoro nucleoside; note (original language) = 2'-氟核苷
  modified_base 6: mod_base = OTHER; note = 2'-fluoro nucleoside; note (original language) = 2'-氟核苷
  modified_base 14: mod_base = OTHER; note = 2'-fluoro nucleoside; note (original language) = 2'-氟核苷
  modified_base 16: mod_base = OTHER; note = 2'-fluoro nucleoside; note (original language) = 2'-氟核苷
  modified_base 1..3: mod_base = OTHER; note = phosphorothioate bond; note (original language) = 硫代磷酸酯键
  modified_base 19..21: mod_base = OTHER; note = phosphorothioate bond; note (original language) = 硫代磷酸酯键
  modified_base 1: mod_base = OTHER; note = 2'-methoxy-5'-vinyl phosphonate nucleoside; note (original language) = 2'-甲氧基-5'-乙烯基膦酸核苷
  source 1..21: mol_type = other RNA
tattagaagaaaaggtgggag

SEQ ID NO: 767 - RNA, 21 nt, synthetic construct
  modified_base 1: mod_base = OTHER; note = 2'-methoxy nucleoside; note (original language) = 2'-甲氧基核苷
  modified_base 3..5: mod_base = OTHER; note = 2'-methoxy nucleoside; note (original language) = 2'-甲氧基核苷
  modified_base 7..13: mod_base = OTHER; note = 2'-methoxy nucleoside; note (original language) = 2'-甲氧基核苷
  modified_base 15: mod_base = OTHER; note = 2'-methoxy nucleoside; note (original language) = 2'-甲氧基核苷
  modified_base 17..21: mod_base = OTHER; note = 2'-methoxy nucleoside; note (original language) = 2'-甲氧基核苷
  modified_base 2: mod_base = OTHER; note = 2'-fluoro nucleoside; note (original language) = 2'-氟核苷
  modified_base 6: mod_base = OTHER; note = 2'-fluoro nucleoside; note (original language) = 2'-氟核苷
  modified_base 14: mod_base = OTHER; note = 2'-fluoro nucleoside; note (original language) = 2'-氟核苷
  modified_base 16: mod_base = OTHER; note = 2'-fluoro nucleoside; note (original language) = 2'-氟核苷
  modified_base 1..3: mod_base = OTHER; note = phosphorothioate bond; note (original language) = 硫代磷酸酯键
  modified_base 19..21: mod_base = OTHER; note = phosphorothioate bond; note (original language) = 硫代磷酸酯键
  modified_base 1: mod_base = OTHER; note = 2'-methoxy-5'-vinyl phosphonate nucleoside; note (original language) = 2'-甲氧基-5'-乙烯基膦酸核苷
  source 1..21: mol_type = other RNA
ttcattagaagaaaaggtggg

SEQ ID NO: 768 - RNA, 21 nt, synthetic construct
  modified_base 1: mod_base = OTHER; note = 2'-methoxy nucleoside; note (original language) = 2'-甲氧基核苷
  modified_base 3..5: mod_base = OTHER; note = 2'-methoxy nucleoside; note (original language) = 2'-甲氧基核苷
  modified_base 7..13: mod_base = OTHER; note = 2'-methoxy nucleoside; note (original language) = 2'-甲氧基核苷
  modified_base 15: mod_base = OTHER; note = 2'-methoxy nucleoside; note (original language) = 2'-甲氧基核苷
  modified_base 17..21: mod_base = OTHER; note = 2'-methoxy nucleoside; note (original language) = 2'-甲氧基核苷
  modified_base 2: mod_base = OTHER; note = 2'-fluoro nucleoside; note (original language) = 2'-氟核苷
  modified_base 6: mod_base = OTHER; note = 2'-fluoro nucleoside; note (original language) = 2'-氟核苷
  modified_base 14: mod_base = OTHER; note = 2'-fluoro nucleoside; note (original language) = 2'-氟核苷
  modified_base 16: mod_base = OTHER; note = 2'-fluoro nucleoside; note (original language) = 2'-氟核苷
  modified_base 1..3: mod_base = OTHER; note = phosphorothioate bond; note (original language) = 硫代磷酸酯键
  modified_base 19..21: mod_base = OTHER; note = phosphorothioate bond; note (original language) = 硫代磷酸酯键
  modified_base 1: mod_base = OTHER; note = 2'-methoxy-5'-vinyl phosphonate nucleoside; note (original language) = 2'-甲氧基-5'-乙烯基膦酸核苷
  source 1..21: mol_type = other RNA
tactcattagaagaaaaggtg

SEQ ID NO: 769 - RNA, 21 nt, synthetic construct
  modified_base 3..5: mod_base = OTHER; note = 2'-methoxy nucleoside; note (original language) = 2'-甲氧基核苷
  modified_base 7..13: mod_base = OTHER; note = 2'-methoxy nucleoside; note (original language) = 2'-甲氧基核苷
  modified_base 15: mod_base = OTHER; note = 2'-methoxy nucleoside; note (original language) = 2'-甲氧基核苷
  modified_base 17..21: mod_base = OTHER; note = 2'-methoxy nucleoside; note (original language) = 2'-甲氧基核苷
  modified_base 2: mod_base = OTHER; note = 2'-fluoro nucleoside; note (original language) = 2'-氟核苷
  modified_base 6: mod_base = OTHER; note = 2'-fluoro nucleoside; note (original language) = 2'-氟核苷
  modified_base 14: mod_base = OTHER; note = 2'-fluoro nucleoside; note (original language) = 2'-氟核苷
  modified_base 16: mod_base = OTHER; note = 2'-fluoro nucleoside; note (original language) = 2'-氟核苷
  modified_base 1..3: mod_base = OTHER; note = phosphorothioate bond; note (original language) = 硫代磷酸酯键
  modified_base 19..21: mod_base = OTHER; note = phosphorothioate bond; note (original language) = 硫代磷酸酯键
  modified_base 1: mod_base = OTHER; note = 2'-acetamido-5'-vinyl phosphonate nucleoside; note (original language) = 2'-乙酰氨基-5'-乙烯基膦酸核苷
  source 1..21: mol_type = other RNA
ttagaagaaaaggtgggagac

SEQ ID NO: 770 - RNA, 21 nt, synthetic construct
  modified_base 3..5: mod_base = OTHER; note = 2'-methoxy nucleoside; note (original language) = 2'-甲氧基核苷
  modified_base 7..13: mod_base = OTHER; note = 2'-methoxy nucleoside; note (original language) = 2'-甲氧基核苷
  modified_base 15: mod_base = OTHER; note = 2'-methoxy nucleoside; note (original language) = 2'-甲氧基核苷
  modified_base 17..21: mod_base = OTHER; note = 2'-methoxy nucleoside; note (original language) = 2'-甲氧基核苷
  modified_base 2: mod_base = OTHER; note = 2'-fluoro nucleoside; note (original language) = 2'-氟核苷
  modified_base 6: mod_base = OTHER; note = 2'-fluoro nucleoside; note (original language) = 2'-氟核苷
  modified_base 14: mod_base = OTHER; note = 2'-fluoro nucleoside; note (original language) = 2'-氟核苷
  modified_base 16: mod_base = OTHER; note = 2'-fluoro nucleoside; note (original language) = 2'-氟核苷
  modified_base 1..3: mod_base = OTHER; note = phosphorothioate bond; note (original language) = 硫代磷酸酯键
  modified_base 19..21: mod_base = OTHER; note = phosphorothioate bond; note (original language) = 硫代磷酸酯键
  modified_base 1: mod_base = OTHER; note = 2'-acetamido-5'-vinyl phosphonate nucleoside; note (original language) = 2'-乙酰氨基-5'-乙烯基膦酸核苷
  source 1..21: mol_type = other RNA
tattagaagaaaaggtgggag

SEQ ID NO: 771 - RNA, 21 nt, synthetic construct
  modified_base 3..5: mod_base = OTHER; note = 2'-methoxy nucleoside; note (original language) = 2'-甲氧基核苷
  modified_base 7..13: mod_base = OTHER; note = 2'-methoxy nucleoside; note (original language) = 2'-甲氧基核苷
  modified_base 15: mod_base = OTHER; note = 2'-methoxy nucleoside; note (original language) = 2'-甲氧基核苷
  modified_base 17..21: mod_base = OTHER; note = 2'-methoxy nucleoside; note (original language) = 2'-甲氧基核苷
  modified_base 2: mod_base = OTHER; note = 2'-fluoro nucleoside; note (original language) = 2'-氟核苷
  modified_base 6: mod_base = OTHER; note = 2'-fluoro nucleoside; note (original language) = 2'-氟核苷
  modified_base 14: mod_base = OTHER; note = 2'-fluoro nucleoside; note (original language) = 2'-氟核苷
  modified_base 16: mod_base = OTHER; note = 2'-fluoro nucleoside; note (original language) = 2'-氟核苷
  modified_base 1..3: mod_base = OTHER; note = phosphorothioate bond; note (original language) = 硫代磷酸酯键
  modified_base 19..21: mod_base = OTHER; note = phosphorothioate bond; note (original language) = 硫代磷酸酯键
  modified_base 1: mod_base = OTHER; note = 2'-acetamido-5'-vinyl phosphonate nucleoside; note (original language) = 2'-乙酰氨基-5'-乙烯基膦酸核苷
  source 1..21: mol_type = other RNA
ttcattagaagaaaaggtggg

SEQ ID NO: 772 - RNA, 21 nt, synthetic construct
  modified_base 3..5: mod_base = OTHER; note = 2'-methoxy nucleoside; note (original language) = 2'-甲氧基核苷
  modified_base 7..13: mod_base = OTHER; note = 2'-methoxy nucleoside; note (original language) = 2'-甲氧基核苷
  modified_base 15: mod_base = OTHER; note = 2'-methoxy nucleoside; note (original language) = 2'-甲氧基核苷
  modified_base 17..21: mod_base = OTHER; note = 2'-methoxy nucleoside; note (original language) = 2'-甲氧基核苷
  modified_base 2: mod_base = OTHER; note = 2'-fluoro nucleoside; note (original language) = 2'-氟核苷
  modified_base 6: mod_base = OTHER; note = 2'-fluoro nucleoside; note (original language) = 2'-氟核苷
  modified_base 14: mod_base = OTHER; note = 2'-fluoro nucleoside; note (original language) = 2'-氟核苷
  modified_base 16: mod_base = OTHER; note = 2'-fluoro nucleoside; note (original language) = 2'-氟核苷
  modified_base 1..3: mod_base = OTHER; note = phosphorothioate bond; note (original language) = 硫代磷酸酯键
  modified_base 19..21: mod_base = OTHER; note = phosphorothioate bond; note (original language) = 硫代磷酸酯键
  modified_base 1: mod_base = OTHER; note = 2'-acetamido-5'-vinyl phosphonate nucleoside; note (original language) = 2'-乙酰氨基-5'-乙烯基膦酸核苷
  source 1..21: mol_type = other RNA
tactcattagaagaaaaggtg

SEQ ID NO: 773 - RNA, 23 nt, synthetic construct
  modified_base 1: mod_base = OTHER; note = 2'-methoxy nucleoside; note (original language) = 2'-甲氧基核苷
  modified_base 3..5: mod_base = OTHER; note = 2'-methoxy nucleoside; note (original language) = 2'-甲氧基核苷
  modified_base 7..8: mod_base = OTHER; note = 2'-methoxy nucleoside; note (original language) = 2'-甲氧基核苷
  modified_base 10..13: mod_base = OTHER; note = 2'-methoxy nucleoside; note (original language) = 2'-甲氧基核苷
  modified_base 15: mod_base = OTHER; note = 2'-methoxy nucleoside; note (original language) = 2'-甲氧基核苷
  modified_base 17..23: mod_base = OTHER; note = 2'-methoxy nucleoside; note (original language) = 2'-甲氧基核苷
  modified_base 2: mod_base = OTHER; note = 2'-fluoro nucleoside; note (original language) = 2'-氟核苷
  modified_base 6: mod_base = OTHER; note = 2'-fluoro nucleoside; note (original language) = 2'-氟核苷
  modified_base 9: mod_base = OTHER; note = 2'-fluoro nucleoside; note (original language) = 2'-氟核苷
  modified_base 14: mod_base = OTHER; note = 2'-fluoro nucleoside; note (original language) = 2'-氟核苷
  modified_base 16: mod_base = OTHER; note = 2'-fluoro nucleoside; note (original language) = 2'-氟核苷
  modified_base 1..3: mod_base = OTHER; note = phosphorothioate bond; note (original language) = 硫代磷酸酯键
  modified_base 21..23: mod_base = OTHER; note = phosphorothioate bond; note (original language) = 硫代磷酸酯键
  source 1..23: mol_type = other RNA
tcttagaccaaggagaaacgcct

SEQ ID NO: 774 - RNA, 23 nt, synthetic construct
  modified_base 3..5: mod_base = OTHER; note = 2'-methoxy nucleoside; note (original language) = 2'-甲氧基核苷
  modified_base 7..8: mod_base = OTHER; note = 2'-methoxy nucleoside; note (original language) = 2'-甲氧基核苷
  modified_base 10..13: mod_base = OTHER; note = 2'-methoxy nucleoside; note (original language) = 2'-甲氧基核苷
  modified_base 15: mod_base = OTHER; note = 2'-methoxy nucleoside; note (original language) = 2'-甲氧基核苷
  modified_base 17..23: mod_base = OTHER; note = 2'-methoxy nucleoside; note (original language) = 2'-甲氧基核苷
  modified_base 2: mod_base = OTHER; note = 2'-fluoro nucleoside; note (original language) = 2'-氟核苷
  modified_base 6: mod_base = OTHER; note = 2'-fluoro nucleoside; note (original language) = 2'-氟核苷
  modified_base 9: mod_base = OTHER; note = 2'-fluoro nucleoside; note (original language) = 2'-氟核苷
  modified_base 14: mod_base = OTHER; note = 2'-fluoro nucleoside; note (original language) = 2'-氟核苷
  modified_base 16: mod_base = OTHER; note = 2'-fluoro nucleoside; note (original language) = 2'-氟核苷
  modified_base 1..3: mod_base = OTHER; note = phosphorothioate bond; note (original language) = 硫代磷酸酯键
  modified_base 21..23: mod_base = OTHER; note = phosphorothioate bond; note (original language) = 硫代磷酸酯键
  modified_base 1: mod_base = OTHER; note = 2'-acetamido-5'-vinyl phosphonate nucleoside; note (original language) = 2'-乙酰氨基-5'-乙烯基膦酸核苷
  source 1..23: mol_type = other RNA
tcttagaccaaggagaaacgcct

SEQ ID NO: 775 - RNA, 23 nt, synthetic construct
  modified_base 1: mod_base = OTHER; note = 2'-methoxy nucleoside; note (original language) = 2'-甲氧基核苷
  modified_base 3..5: mod_base = OTHER; note = 2'-methoxy nucleoside; note (original language) = 2'-甲氧基核苷
  modified_base 7..8: mod_base = OTHER; note = 2'-methoxy nucleoside; note (original language) = 2'-甲氧基核苷
  modified_base 10..13: mod_base = OTHER; note = 2'-methoxy nucleoside; note (original language) = 2'-甲氧基核苷
  modified_base 15: mod_base = OTHER; note = 2'-methoxy nucleoside; note (original language) = 2'-甲氧基核苷
  modified_base 17..23: mod_base = OTHER; note = 2'-methoxy nucleoside; note (original language) = 2'-甲氧基核苷
  modified_base 2: mod_base = OTHER; note = 2'-fluoro nucleoside; note (original language) = 2'-氟核苷
  modified_base 6: mod_base = OTHER; note = 2'-fluoro nucleoside; note (original language) = 2'-氟核苷
  modified_base 9: mod_base = OTHER; note = 2'-fluoro nucleoside; note (original language) = 2'-氟核苷
  modified_base 14: mod_base = OTHER; note = 2'-fluoro nucleoside; note (original language) = 2'-氟核苷
  modified_base 16: mod_base = OTHER; note = 2'-fluoro nucleoside; note (original language) = 2'-氟核苷
  modified_base 1..3: mod_base = OTHER; note = phosphorothioate bond; note (original language) = 硫代磷酸酯键
  modified_base 21..23: mod_base = OTHER; note = phosphorothioate bond; note (original language) = 硫代磷酸酯键
  modified_base 1: mod_base = OTHER; note = 2'-methoxy-5'-vinyl phosphonate nucleoside; note (original language) = 2'-甲氧基-5'-乙烯基膦酸核苷
  source 1..23: mol_type = other RNA
tcttagaccaaggagaaacgcct

SEQ ID NO: 776 - RNA, 21 nt, synthetic construct
  modified_base 3..5: mod_base = OTHER; note = 2'-methoxy nucleoside; note (original language) = 2'-甲氧基核苷
  modified_base 7..8: mod_base = OTHER; note = 2'-methoxy nucleoside; note (original language) = 2'-甲氧基核苷
  modified_base 10..13: mod_base = OTHER; note = 2'-methoxy nucleoside; note (original language) = 2'-甲氧基核苷
  modified_base 15: mod_base = OTHER; note = 2'-methoxy nucleoside; note (original language) = 2'-甲氧基核苷
  modified_base 17..21: mod_base = OTHER; note = 2'-methoxy nucleoside; note (original language) = 2'-甲氧基核苷
  modified_base 2: mod_base = OTHER; note = 2'-fluoro nucleoside; note (original language) = 2'-氟核苷
  modified_base 6: mod_base = OTHER; note = 2'-fluoro nucleoside; note (original language) = 2'-氟核苷
  modified_base 9: mod_base = OTHER; note = 2'-fluoro nucleoside; note (original language) = 2'-氟核苷
  modified_base 14: mod_base = OTHER; note = 2'-fluoro nucleoside; note (original language) = 2'-氟核苷
  modified_base 16: mod_base = OTHER; note = 2'-fluoro nucleoside; note (original language) = 2'-氟核苷
  modified_base 1..3: mod_base = OTHER; note = phosphorothioate bond; note (original language) = 硫代磷酸酯键
  modified_base 19..21: mod_base = OTHER; note = phosphorothioate bond; note (original language) = 硫代磷酸酯键
  modified_base 1: mod_base = OTHER; note = 2'-acetamido-5'-vinyl phosphonate nucleoside; note (original language) = 2'-乙酰氨基-5'-乙烯基膦酸核苷
  source 1..21: mol_type = other RNA
ttagaagaaaaggtgggagac

SEQ ID NO: 777 - RNA, 21 nt, synthetic construct
  modified_base 3..5: mod_base = OTHER; note = 2'-methoxy nucleoside; note (original language) = 2'-甲氧基核苷
  modified_base 7..8: mod_base = OTHER; note = 2'-methoxy nucleoside; note (original language) = 2'-甲氧基核苷
  modified_base 10..13: mod_base = OTHER; note = 2'-methoxy nucleoside; note (original language) = 2'-甲氧基核苷
  modified_base 15: mod_base = OTHER; note = 2'-methoxy nucleoside; note (original language) = 2'-甲氧基核苷
  modified_base 17..21: mod_base = OTHER; note = 2'-methoxy nucleoside; note (original language) = 2'-甲氧基核苷
  modified_base 2: mod_base = OTHER; note = 2'-fluoro nucleoside; note (original language) = 2'-氟核苷
  modified_base 6: mod_base = OTHER; note = 2'-fluoro nucleoside; note (original language) = 2'-氟核苷
  modified_base 9: mod_base = OTHER; note = 2'-fluoro nucleoside; note (original language) = 2'-氟核苷
  modified_base 14: mod_base = OTHER; note = 2'-fluoro nucleoside; note (original language) = 2'-氟核苷
  modified_base 16: mod_base = OTHER; note = 2'-fluoro nucleoside; note (original language) = 2'-氟核苷
  modified_base 1..3: mod_base = OTHER; note = phosphorothioate bond; note (original language) = 硫代磷酸酯键
  modified_base 19..21: mod_base = OTHER; note = phosphorothioate bond; note (original language) = 硫代磷酸酯键
  modified_base 1: mod_base = OTHER; note = 2'-acetamido-5'-vinyl phosphonate nucleoside; note (original language) = 2'-乙酰氨基-5'-乙烯基膦酸核苷
  source 1..21: mol_type = other RNA
tattagaagaaaaggtgggag

SEQ ID NO: 778 - RNA, 21 nt, synthetic construct
  modified_base 3..5: mod_base = OTHER; note = 2'-methoxy nucleoside; note (original language) = 2'-甲氧基核苷
  modified_base 7..8: mod_base = OTHER; note = 2'-methoxy nucleoside; note (original language) = 2'-甲氧基核苷
  modified_base 10..13: mod_base = OTHER; note = 2'-methoxy nucleoside; note (original language) = 2'-甲氧基核苷
  modified_base 15: mod_base = OTHER; note = 2'-methoxy nucleoside; note (original language) = 2'-甲氧基核苷
  modified_base 17..21: mod_base = OTHER; note = 2'-methoxy nucleoside; note (original language) = 2'-甲氧基核苷
  modified_base 2: mod_base = OTHER; note = 2'-fluoro nucleoside; note (original language) = 2'-氟核苷
  modified_base 6: mod_base = OTHER; note = 2'-fluoro nucleoside; note (original language) = 2'-氟核苷
  modified_base 9: mod_base = OTHER; note = 2'-fluoro nucleoside; note (original language) = 2'-氟核苷
  modified_base 14: mod_base = OTHER; note = 2'-fluoro nucleoside; note (original language) = 2'-氟核苷
  modified_base 16: mod_base = OTHER; note = 2'-fluoro nucleoside; note (original language) = 2'-氟核苷
  modified_base 1..3: mod_base = OTHER; note = phosphorothioate bond; note (original language) = 硫代磷酸酯键
  modified_base 19..21: mod_base = OTHER; note = phosphorothioate bond; note (original language) = 硫代磷酸酯键
  modified_base 1: mod_base = OTHER; note = 2'-acetamido-5'-vinyl phosphonate nucleoside; note (original language) = 2'-乙酰氨基-5'-乙烯基膦酸核苷
  source 1..21: mol_type = other RNA
ttcattagaagaaaaggtggg

SEQ ID NO: 779 - RNA, 21 nt, synthetic construct
  modified_base 3..5: mod_base = OTHER; note = 2'-methoxy nucleoside; note (original language) = 2'-甲氧基核苷
  modified_base 7..8: mod_base = OTHER; note = 2'-methoxy nucleoside; note (original language) = 2'-甲氧基核苷
  modified_base 10..13: mod_base = OTHER; note = 2'-methoxy nucleoside; note (original language) = 2'-甲氧基核苷
  modified_base 15: mod_base = OTHER; note = 2'-methoxy nucleoside; note (original language) = 2'-甲氧基核苷
  modified_base 17..21: mod_base = OTHER; note = 2'-methoxy nucleoside; note (original language) = 2'-甲氧基核苷
  modified_base 2: mod_base = OTHER; note = 2'-fluoro nucleoside; note (original language) = 2'-氟核苷
  modified_base 6: mod_base = OTHER; note = 2'-fluoro nucleoside; note (original language) = 2'-氟核苷
  modified_base 9: mod_base = OTHER; note = 2'-fluoro nucleoside; note (original language) = 2'-氟核苷
  modified_base 14: mod_base = OTHER; note = 2'-fluoro nucleoside; note (original language) = 2'-氟核苷
  modified_base 16: mod_base = OTHER; note = 2'-fluoro nucleoside; note (original language) = 2'-氟核苷
  modified_base 1..3: mod_base = OTHER; note = phosphorothioate bond; note (original language) = 硫代磷酸酯键
  modified_base 19..21: mod_base = OTHER; note = phosphorothioate bond; note (original language) = 硫代磷酸酯键
  modified_base 1: mod_base = OTHER; note = 2'-acetamido-5'-vinyl phosphonate nucleoside; note (original language) = 2'-乙酰氨基-5'-乙烯基膦酸核苷
  source 1..21: mol_type = other RNA
tactcattagaagaaaaggtg

SEQ ID NO: 780 - RNA, 21 nt, synthetic construct
  modified_base 1: mod_base = OTHER; note = 2'-methoxy nucleoside; note (original language) = 2'-甲氧基核苷
  modified_base 3..5: mod_base = OTHER; note = 2'-methoxy nucleoside; note (original language) = 2'-甲氧基核苷
  modified_base 7..8: mod_base = OTHER; note = 2'-methoxy nucleoside; note (original language) = 2'-甲氧基核苷
  modified_base 10..13: mod_base = OTHER; note = 2'-methoxy nucleoside; note (original language) = 2'-甲氧基核苷
  modified_base 15: mod_base = OTHER; note = 2'-methoxy nucleoside; note (original language) = 2'-甲氧基核苷
  modified_base 17..21: mod_base = OTHER; note = 2'-methoxy nucleoside; note (original language) = 2'-甲氧基核苷
  modified_base 2: mod_base = OTHER; note = 2'-fluoro nucleoside; note (original language) = 2'-氟核苷
  modified_base 6: mod_base = OTHER; note = 2'-fluoro nucleoside; note (original language) = 2'-氟核苷
  modified_base 9: mod_base = OTHER; note = 2'-fluoro nucleoside; note (original language) = 2'-氟核苷
  modified_base 14: mod_base = OTHER; note = 2'-fluoro nucleoside; note (original language) = 2'-氟核苷
  modified_base 16: mod_base = OTHER; note = 2'-fluoro nucleoside; note (original language) = 2'-氟核苷
  modified_base 1..3: mod_base = OTHER; note = phosphorothioate bond; note (original language) = 硫代磷酸酯键
  modified_base 19..21: mod_base = OTHER; note = phosphorothioate bond; note (original language) = 硫代磷酸酯键
  source 1..21: mol_type = other RNA
aatttttgttctcaacttgaa

SEQ ID NO: 781 - RNA, 21 nt, synthetic construct
  modified_base 3..5: mod_base = OTHER; note = 2'-methoxy nucleoside; note (original language) = 2'-甲氧基核苷
  modified_base 7..8: mod_base = OTHER; note = 2'-methoxy nucleoside; note (original language) = 2'-甲氧基核苷
  modified_base 10..13: mod_base = OTHER; note = 2'-methoxy nucleoside; note (original language) = 2'-甲氧基核苷
  modified_base 15: mod_base = OTHER; note = 2'-methoxy nucleoside; note (original language) = 2'-甲氧基核苷
  modified_base 17..21: mod_base = OTHER; note = 2'-methoxy nucleoside; note (original language) = 2'-甲氧基核苷
  modified_base 2: mod_base = OTHER; note = 2'-fluoro nucleoside; note (original language) = 2'-氟核苷
  modified_base 6: mod_base = OTHER; note = 2'-fluoro nucleoside; note (original language) = 2'-氟核苷
  modified_base 9: mod_base = OTHER; note = 2'-fluoro nucleoside; note (original language) = 2'-氟核苷
  modified_base 14: mod_base = OTHER; note = 2'-fluoro nucleoside; note (original language) = 2'-氟核苷
  modified_base 16: mod_base = OTHER; note = 2'-fluoro nucleoside; note (original language) = 2'-氟核苷
  modified_base 1..3: mod_base = OTHER; note = phosphorothioate bond; note (original language) = 硫代磷酸酯键
  modified_base 19..21: mod_base = OTHER; note = phosphorothioate bond; note (original language) = 硫代磷酸酯键
  modified_base 1: mod_base = OTHER; note = 2'-acetamido-5'-vinyl phosphonate nucleoside; note (original language) = 2'-乙酰氨基-5'-乙烯基膦酸核苷
  source 1..21: mol_type = other RNA
taaacactggttcttgcctcc

SEQ ID NO: 782 - RNA, 21 nt, synthetic construct
  modified_base 3..5: mod_base = OTHER; note = 2'-methoxy nucleoside; note (original language) = 2'-甲氧基核苷
  modified_base 7..8: mod_base = OTHER; note = 2'-methoxy nucleoside; note (original language) = 2'-甲氧基核苷
  modified_base 10..13: mod_base = OTHER; note = 2'-methoxy nucleoside; note (original language) = 2'-甲氧基核苷
  modified_base 15: mod_base = OTHER; note = 2'-methoxy nucleoside; note (original language) = 2'-甲氧基核苷
  modified_base 17..21: mod_base = OTHER; note = 2'-methoxy nucleoside; note (original language) = 2'-甲氧基核苷
  modified_base 2: mod_base = OTHER; note = 2'-fluoro nucleoside; note (original language) = 2'-氟核苷
  modified_base 6: mod_base = OTHER; note = 2'-fluoro nucleoside; note (original language) = 2'-氟核苷
  modified_base 9: mod_base = OTHER; note = 2'-fluoro nucleoside; note (original language) = 2'-氟核苷
  modified_base 14: mod_base = OTHER; note = 2'-fluoro nucleoside; note (original language) = 2'-氟核苷
  modified_base 16: mod_base = OTHER; note = 2'-fluoro nucleoside; note (original language) = 2'-氟核苷
  modified_base 1..3: mod_base = OTHER; note = phosphorothioate bond; note (original language) = 硫代磷酸酯键
  modified_base 19..21: mod_base = OTHER; note = phosphorothioate bond; note (original language) = 硫代磷酸酯键
  modified_base 1: mod_base = OTHER; note = 2'-acetamido-5'-vinyl phosphonate nucleoside; note (original language) = 2'-乙酰氨基-5'-乙烯基膦酸核苷
  source 1..21: mol_type = other RNA
tatactttaattttaaaaccc

SEQ ID NO: 783 - RNA, 21 nt, synthetic construct
  modified_base 3..5: mod_base = OTHER; note = 2'-methoxy nucleoside; note (original language) = 2'-甲氧基核苷
  modified_base 7..8: mod_base = OTHER; note = 2'-methoxy nucleoside; note (original language) = 2'-甲氧基核苷
  modified_base 10..13: mod_base = OTHER; note = 2'-methoxy nucleoside; note (original language) = 2'-甲氧基核苷
  modified_base 15: mod_base = OTHER; note = 2'-methoxy nucleoside; note (original language) = 2'-甲氧基核苷
  modified_base 17..21: mod_base = OTHER; note = 2'-methoxy nucleoside; note (original language) = 2'-甲氧基核苷
  modified_base 2: mod_base = OTHER; note = 2'-fluoro nucleoside; note (original language) = 2'-氟核苷
  modified_base 6: mod_base = OTHER; note = 2'-fluoro nucleoside; note (original language) = 2'-氟核苷
  modified_base 9: mod_base = OTHER; note = 2'-fluoro nucleoside; note (original language) = 2'-氟核苷
  modified_base 14: mod_base = OTHER; note = 2'-fluoro nucleoside; note (original language) = 2'-氟核苷
  modified_base 16: mod_base = OTHER; note = 2'-fluoro nucleoside; note (original language) = 2'-氟核苷
  modified_base 1..3: mod_base = OTHER; note = phosphorothioate bond; note (original language) = 硫代磷酸酯键
  modified_base 19..21: mod_base = OTHER; note = phosphorothioate bond; note (original language) = 硫代磷酸酯键
  modified_base 1: mod_base = OTHER; note = 2'-acetamido-5'-vinyl phosphonate nucleoside; note (original language) = 2'-乙酰氨基-5'-乙烯基膦酸核苷
  source 1..21: mol_type = other RNA
tttcacaaacaagctggtcgg

SEQ ID NO: 784 - RNA, 21 nt, synthetic construct
  modified_base 3..5: mod_base = OTHER; note = 2'-methoxy nucleoside; note (original language) = 2'-甲氧基核苷
  modified_base 7..8: mod_base = OTHER; note = 2'-methoxy nucleoside; note (original language) = 2'-甲氧基核苷
  modified_base 10..13: mod_base = OTHER; note = 2'-methoxy nucleoside; note (original language) = 2'-甲氧基核苷
  modified_base 15: mod_base = OTHER; note = 2'-methoxy nucleoside; note (original language) = 2'-甲氧基核苷
  modified_base 17..21: mod_base = OTHER; note = 2'-methoxy nucleoside; note (original language) = 2'-甲氧基核苷
  modified_base 2: mod_base = OTHER; note = 2'-fluoro nucleoside; note (original language) = 2'-氟核苷
  modified_base 6: mod_base = OTHER; note = 2'-fluoro nucleoside; note (original language) = 2'-氟核苷
  modified_base 9: mod_base = OTHER; note = 2'-fluoro nucleoside; note (original language) = 2'-氟核苷
  modified_base 14: mod_base = OTHER; note = 2'-fluoro nucleoside; note (original language) = 2'-氟核苷
  modified_base 16: mod_base = OTHER; note = 2'-fluoro nucleoside; note (original language) = 2'-氟核苷
  modified_base 1..3: mod_base = OTHER; note = phosphorothioate bond; note (original language) = 硫代磷酸酯键
  modified_base 19..21: mod_base = OTHER; note = phosphorothioate bond; note (original language) = 硫代磷酸酯键
  modified_base 1: mod_base = OTHER; note = 2'-acetamido-5'-vinyl phosphonate nucleoside; note (original language) = 2'-乙酰氨基-5'-乙烯基膦酸核苷
  source 1..21: mol_type = other RNA
tttgctggaaagtgagaccct

SEQ ID NO: 785 - RNA, 21 nt, synthetic construct
  modified_base 3..5: mod_base = OTHER; note = 2'-methoxy nucleoside; note (original language) = 2'-甲氧基核苷
  modified_base 7..8: mod_base = OTHER; note = 2'-methoxy nucleoside; note (original language) = 2'-甲氧基核苷
  modified_base 10..13: mod_base = OTHER; note = 2'-methoxy nucleoside; note (original language) = 2'-甲氧基核苷
  modified_base 15: mod_base = OTHER; note = 2'-methoxy nucleoside; note (original language) = 2'-甲氧基核苷
  modified_base 17..21: mod_base = OTHER; note = 2'-methoxy nucleoside; note (original language) = 2'-甲氧基核苷
  modified_base 2: mod_base = OTHER; note = 2'-fluoro nucleoside; note (original language) = 2'-氟核苷
  modified_base 6: mod_base = OTHER; note = 2'-fluoro nucleoside; note (original language) = 2'-氟核苷
  modified_base 9: mod_base = OTHER; note = 2'-fluoro nucleoside; note (original language) = 2'-氟核苷
  modified_base 14: mod_base = OTHER; note = 2'-fluoro nucleoside; note (original language) = 2'-氟核苷
  modified_base 16: mod_base = OTHER; note = 2'-fluoro nucleoside; note (original language) = 2'-氟核苷
  modified_base 1..3: mod_base = OTHER; note = phosphorothioate bond; note (original language) = 硫代磷酸酯键
  modified_base 19..21: mod_base = OTHER; note = phosphorothioate bond; note (original language) = 硫代磷酸酯键
  modified_base 1: mod_base = OTHER; note = 2'-acetamido-5'-vinyl phosphonate nucleoside; note (original language) = 2'-乙酰氨基-5'-乙烯基膦酸核苷
  source 1..21: mol_type = other RNA
ttcacaaacaagctggtcggt

SEQ ID NO: 786 - RNA, 21 nt, synthetic construct
  modified_base 1: mod_base = OTHER; note = 2'-methoxy nucleoside; note (original language) = 2'-甲氧基核苷
  modified_base 3..5: mod_base = OTHER; note = 2'-methoxy nucleoside; note (original language) = 2'-甲氧基核苷
  modified_base 7..13: mod_base = OTHER; note = 2'-methoxy nucleoside; note (original language) = 2'-甲氧基核苷
  modified_base 15: mod_base = OTHER; note = 2'-methoxy nucleoside; note (original language) = 2'-甲氧基核苷
  modified_base 17..21: mod_base = OTHER; note = 2'-methoxy nucleoside; note (original language) = 2'-甲氧基核苷
  modified_base 2: mod_base = OTHER; note = 2'-fluoro nucleoside; note (original language) = 2'-氟核苷
  modified_base 6: mod_base = OTHER; note = 2'-fluoro nucleoside; note (original language) = 2'-氟核苷
  modified_base 14: mod_base = OTHER; note = 2'-fluoro nucleoside; note (original language) = 2'-氟核苷
  modified_base 16: mod_base = OTHER; note = 2'-fluoro nucleoside; note (original language) = 2'-氟核苷
  modified_base 1..3: mod_base = OTHER; note = phosphorothioate bond; note (original language) = 硫代磷酸酯键
  modified_base 19..21: mod_base = OTHER; note = phosphorothioate bond; note (original language) = 硫代磷酸酯键
  source 1..21: mol_type = other RNA
tgactcattagaagaaaaggt

SEQ ID NO: 787 - RNA, 23 nt, synthetic construct
  modified_base 3..5: mod_base = OTHER; note = 2'-methoxy nucleoside; note (original language) = 2'-甲氧基核苷
  modified_base 7..8: mod_base = OTHER; note = 2'-methoxy nucleoside; note (original language) = 2'-甲氧基核苷
  modified_base 10..13: mod_base = OTHER; note = 2'-methoxy nucleoside; note (original language) = 2'-甲氧基核苷
  modified_base 15: mod_base = OTHER; note = 2'-methoxy nucleoside; note (original language) = 2'-甲氧基核苷
  modified_base 17..23: mod_base = OTHER; note = 2'-methoxy nucleoside; note (original language) = 2'-甲氧基核苷
  modified_base 2: mod_base = OTHER; note = 2'-fluoro nucleoside; note (original language) = 2'-氟核苷
  modified_base 6: mod_base = OTHER; note = 2'-fluoro nucleoside; note (original language) = 2'-氟核苷
  modified_base 9: mod_base = OTHER; note = 2'-fluoro nucleoside; note (original language) = 2'-氟核苷
  modified_base 14: mod_base = OTHER; note = 2'-fluoro nucleoside; note (original language) = 2'-氟核苷
  modified_base 16: mod_base = OTHER; note = 2'-fluoro nucleoside; note (original language) = 2'-氟核苷
  modified_base 1..3: mod_base = OTHER; note = phosphorothioate bond; note (original language) = 硫代磷酸酯键
  modified_base 21..23: mod_base = OTHER; note = phosphorothioate bond; note (original language) = 硫代磷酸酯键
  modified_base 1: mod_base = OTHER; note = 2'-acetamido-5'-vinyl phosphonate nucleoside; note (original language) = 2'-乙酰氨基-5'-乙烯基膦酸核苷
  source 1..23: mol_type = other RNA
tcttagaccaaggagaaacggct

SEQ ID NO: 788 - RNA, 23 nt, synthetic construct
  modified_base 3..5: mod_base = OTHER; note = 2'-methoxy nucleoside; note (original language) = 2'-甲氧基核苷
  modified_base 7..8: mod_base = OTHER; note = 2'-methoxy nucleoside; note (original language) = 2'-甲氧基核苷
  modified_base 10..13: mod_base = OTHER; note = 2'-methoxy nucleoside; note (original language) = 2'-甲氧基核苷
  modified_base 15: mod_base = OTHER; note = 2'-methoxy nucleoside; note (original language) = 2'-甲氧基核苷
  modified_base 17..23: mod_base = OTHER; note = 2'-methoxy nucleoside; note (original language) = 2'-甲氧基核苷
  modified_base 2: mod_base = OTHER; note = 2'-fluoro nucleoside; note (original language) = 2'-氟核苷
  modified_base 6: mod_base = OTHER; note = 2'-fluoro nucleoside; note (original language) = 2'-氟核苷
  modified_base 9: mod_base = OTHER; note = 2'-fluoro nucleoside; note (original language) = 2'-氟核苷
  modified_base 14: mod_base = OTHER; note = 2'-fluoro nucleoside; note (original language) = 2'-氟核苷
  modified_base 16: mod_base = OTHER; note = 2'-fluoro nucleoside; note (original language) = 2'-氟核苷
  modified_base 1..3: mod_base = OTHER; note = phosphorothioate bond; note (original language) = 硫代磷酸酯键
  modified_base 21..23: mod_base = OTHER; note = phosphorothioate bond; note (original language) = 硫代磷酸酯键
  modified_base 1: mod_base = OTHER; note = 2'-acetamido-5'-vinyl phosphonate nucleoside; note (original language) = 2'-乙酰氨基-5'-乙烯基膦酸核苷
  source 1..23: mol_type = other RNA
tttagaccaaggagaaacggctg

SEQ ID NO: 789 - RNA, 19 nt, synthetic construct
  source 1..19: mol_type = other RNA
gtcccaccttttcttctaa

SEQ ID NO: 790 - RNA, 19 nt, synthetic construct
  source 1..19: mol_type = other RNA
gtcccaccatttcttctaa

SEQ ID NO: 791 - RNA, 19 nt, synthetic construct
  source 1..19: mol_type = other RNA
gtcccaccctttcttctaa

SEQ ID NO: 792 - RNA, 19 nt, synthetic construct
  source 1..19: mol_type = other RNA
gtcccaccgtttcttctaa

SEQ ID NO: 793 - RNA, 19 nt, synthetic construct
  source 1..19: mol_type = other RNA
gtcccacctattcttctaa

SEQ ID NO: 794 - RNA, 19 nt, synthetic construct
  source 1..19: mol_type = other RNA
gtcccacctcttcttctaa

SEQ ID NO: 795 - RNA, 19 nt, synthetic construct
  source 1..19: mol_type = other RNA
gtcccacctgttcttctaa

SEQ ID NO: 796 - RNA, 19 nt, synthetic construct
  source 1..19: mol_type = other RNA
gtcccaccttatcttctaa

SEQ ID NO: 797 - RNA, 19 nt, synthetic construct
  source 1..19: mol_type = other RNA
gtcccaccttctcttctaa

SEQ ID NO: 798 - RNA, 19 nt, synthetic construct
  source 1..19: mol_type = other RNA
gtcccaccttgtcttctaa

SEQ ID NO: 799 - RNA, 19 nt, synthetic construct
  source 1..19: mol_type = other RNA
gccaccttttcttctaata

SEQ ID NO: 800 - RNA, 19 nt, synthetic construct
  source 1..19: mol_type = other RNA
gaccttttcttctaatgaa

SEQ ID NO: 801 - RNA, 19 nt, synthetic construct
  source 1..19: mol_type = other RNA
caagttgagaacaaaaata

SEQ ID NO: 802 - RNA, 19 nt, synthetic construct
  source 1..19: mol_type = other RNA
gggcaagaaccagtgttta

SEQ ID NO: 803 - RNA, 19 nt, synthetic construct
  source 1..19: mol_type = other RNA
ggaccagcttgtttgtgaa

SEQ ID NO: 804 - RNA, 19 nt, synthetic construct
  source 1..19: mol_type = other RNA
caccagcttgtttgtgaaa

SEQ ID NO: 805 - RNA, 21 nt, synthetic construct
  source 1..21: mol_type = other RNA
ttagaagaaaaggtgggacac

SEQ ID NO: 806 - RNA, 23 nt, synthetic construct
  modified_base 12: mod_base = i
  source 1..23: mol_type = other RNA
tcttagaccaangagaaacgcct

SEQ ID NO: 807 - RNA, 23 nt, synthetic construct
  modified_base 13: mod_base = i
  source 1..23: mol_type = other RNA
tcttagaccaagnagaaacgcct

SEQ ID NO: 808 - RNA, 23 nt, synthetic construct
  modified_base 15: mod_base = i
  source 1..23: mol_type = other RNA
tcttagaccaagganaaacgcct

SEQ ID NO: 809 - RNA, 23 nt, synthetic construct
  modified_base 17: mod_base = i
  source 1..23: mol_type = other RNA
tcttagaccaaggaganacgcct

SEQ ID NO: 810 - RNA, 23 nt, synthetic construct
  modified_base 18: mod_base = i
  source 1..23: mol_type = other RNA
tcttagaccaaggagaancgcct

SEQ ID NO: 811 - RNA, 23 nt, synthetic construct
  modified_base 20: mod_base = i
  source 1..23: mol_type = other RNA
tcttagaccaaggagaaacncct

SEQ ID NO: 812 - RNA, 21 nt, synthetic construct
  source 1..21: mol_type = other RNA
tattagaagaaaaggtggcag

SEQ ID NO: 813 - RNA, 21 nt, synthetic construct
  source 1..21: mol_type = other RNA
ttcattagaagaaaaggtcgg

SEQ ID NO: 814 - RNA, 21 nt, synthetic construct
  source 1..21: mol_type = other RNA
tatttttgttctcaacttgaa

SEQ ID NO: 815 - RNA, 21 nt, synthetic construct
  source 1..21: mol_type = other RNA
taaacactggttcttgccccc

SEQ ID NO: 816 - RNA, 21 nt, synthetic construct
  source 1..21: mol_type = other RNA
ttcacaaacaagctggtccgt

SEQ ID NO: 817 - RNA, 21 nt, synthetic construct
  source 1..21: mol_type = other RNA
tttcacaaacaagctggtggg

SEQ ID NO: 818 - RNA, 23 nt, synthetic construct
  modified_base 11: mod_base = i
  source 1..23: mol_type = other RNA
tcttagaccanggagaaacgcct

SEQ ID NO: 819 - RNA, 23 nt, synthetic construct
  modified_base 10: mod_base = i
  source 1..23: mol_type = other RNA
tcttagaccnaggagaaacgcct

SEQ ID NO: 820 - RNA, 23 nt, synthetic construct
  modified_base 7: mod_base = i
  source 1..23: mol_type = other RNA
tcttagnccaaggagaaacgcct

SEQ ID NO: 821 - RNA, 23 nt, synthetic construct
  modified_base 5: mod_base = i
  source 1..23: mol_type = other RNA
tcttngaccaaggagaaacgcct

SEQ ID NO: 822 - RNA, 19 nt, synthetic construct
  modified_base 1..6: mod_base = OTHER; note = 2'-methoxy nucleoside; note (original language) = 2'-甲氧基核苷
  modified_base 10..19: mod_base = OTHER; note = 2'-methoxy nucleoside; note (original language) = 2'-甲氧基核苷
  modified_base 7..9: mod_base = OTHER; note = 2'-fluoro nucleoside; note (original language) = 2'-氟核苷
  modified_base 1..3: mod_base = OTHER; note = phosphorothioate bond; note (original language) = 硫代磷酸酯键
  source 1..19: mol_type = other RNA
gtcccaccttttcttctaa

SEQ ID NO: 823 - RNA, 19 nt, synthetic construct
  modified_base 1..6: mod_base = OTHER; note = 2'-methoxy nucleoside; note (original language) = 2'-甲氧基核苷
  modified_base 10..19: mod_base = OTHER; note = 2'-methoxy nucleoside; note (original language) = 2'-甲氧基核苷
  modified_base 7..9: mod_base = OTHER; note = 2'-fluoro nucleoside; note (original language) = 2'-氟核苷
  modified_base 1..3: mod_base = OTHER; note = phosphorothioate bond; note (original language) = 硫代磷酸酯键
  source 1..19: mol_type = other RNA
gtcccaccatttcttctaa

SEQ ID NO: 824 - RNA, 19 nt, synthetic construct
  modified_base 1..6: mod_base = OTHER; note = 2'-methoxy nucleoside; note (original language) = 2'-甲氧基核苷
  modified_base 10..19: mod_base = OTHER; note = 2'-methoxy nucleoside; note (original language) = 2'-甲氧基核苷
  modified_base 7..9: mod_base = OTHER; note = 2'-fluoro nucleoside; note (original language) = 2'-氟核苷
  modified_base 1..3: mod_base = OTHER; note = phosphorothioate bond; note (original language) = 硫代磷酸酯键
  source 1..19: mol_type = other RNA
gtcccaccctttcttctaa

SEQ ID NO: 825 - RNA, 19 nt, synthetic construct
  modified_base 1..6: mod_base = OTHER; note = 2'-methoxy nucleoside; note (original language) = 2'-甲氧基核苷
  modified_base 10..19: mod_base = OTHER; note = 2'-methoxy nucleoside; note (original language) = 2'-甲氧基核苷
  modified_base 7..9: mod_base = OTHER; note = 2'-fluoro nucleoside; note (original language) = 2'-氟核苷
  modified_base 1..3: mod_base = OTHER; note = phosphorothioate bond; note (original language) = 硫代磷酸酯键
  source 1..19: mol_type = other RNA
gtcccaccgtttcttctaa

SEQ ID NO: 826 - RNA, 19 nt, synthetic construct
  modified_base 1..6: mod_base = OTHER; note = 2'-methoxy nucleoside; note (original language) = 2'-甲氧基核苷
  modified_base 10..19: mod_base = OTHER; note = 2'-methoxy nucleoside; note (original language) = 2'-甲氧基核苷
  modified_base 7..9: mod_base = OTHER; note = 2'-fluoro nucleoside; note (original language) = 2'-氟核苷
  modified_base 1..3: mod_base = OTHER; note = phosphorothioate bond; note (original language) = 硫代磷酸酯键
  source 1..19: mol_type = other RNA
gtcccacctattcttctaa

SEQ ID NO: 827 - RNA, 19 nt, synthetic construct
  modified_base 1..6: mod_base = OTHER; note = 2'-methoxy nucleoside; note (original language) = 2'-甲氧基核苷
  modified_base 10..19: mod_base = OTHER; note = 2'-methoxy nucleoside; note (original language) = 2'-甲氧基核苷
  modified_base 7..9: mod_base = OTHER; note = 2'-fluoro nucleoside; note (original language) = 2'-氟核苷
  modified_base 1..3: mod_base = OTHER; note = phosphorothioate bond; note (original language) = 硫代磷酸酯键
  source 1..19: mol_type = other RNA
gtcccacctcttcttctaa

SEQ ID NO: 828 - RNA, 19 nt, synthetic construct
  modified_base 1..6: mod_base = OTHER; note = 2'-methoxy nucleoside; note (original language) = 2'-甲氧基核苷
  modified_base 10..19: mod_base = OTHER; note = 2'-methoxy nucleoside; note (original language) = 2'-甲氧基核苷
  modified_base 7..9: mod_base = OTHER; note = 2'-fluoro nucleoside; note (original language) = 2'-氟核苷
  modified_base 1..3: mod_base = OTHER; note = phosphorothioate bond; note (original language) = 硫代磷酸酯键
  source 1..19: mol_type = other RNA
gtcccacctgttcttctaa

SEQ ID NO: 829 - RNA, 19 nt, synthetic construct
  modified_base 1..6: mod_base = OTHER; note = 2'-methoxy nucleoside; note (original language) = 2'-甲氧基核苷
  modified_base 10..19: mod_base = OTHER; note = 2'-methoxy nucleoside; note (original language) = 2'-甲氧基核苷
  modified_base 7..9: mod_base = OTHER; note = 2'-fluoro nucleoside; note (original language) = 2'-氟核苷
  modified_base 1..3: mod_base = OTHER; note = phosphorothioate bond; note (original language) = 硫代磷酸酯键
  source 1..19: mol_type = other RNA
gtcccaccttatcttctaa

SEQ ID NO: 830 - RNA, 19 nt, synthetic construct
  modified_base 1..6: mod_base = OTHER; note = 2'-methoxy nucleoside; note (original language) = 2'-甲氧基核苷
  modified_base 10..19: mod_base = OTHER; note = 2'-methoxy nucleoside; note (original language) = 2'-甲氧基核苷
  modified_base 7..9: mod_base = OTHER; note = 2'-fluoro nucleoside; note (original language) = 2'-氟核苷
  modified_base 1..3: mod_base = OTHER; note = phosphorothioate bond; note (original language) = 硫代磷酸酯键
  source 1..19: mol_type = other RNA
gtcccaccttctcttctaa

SEQ ID NO: 831 - RNA, 19 nt, synthetic construct
  modified_base 1..6: mod_base = OTHER; note = 2'-methoxy nucleoside; note (original language) = 2'-甲氧基核苷
  modified_base 10..19: mod_base = OTHER; note = 2'-methoxy nucleoside; note (original language) = 2'-甲氧基核苷
  modified_base 7..9: mod_base = OTHER; note = 2'-fluoro nucleoside; note (original language) = 2'-氟核苷
  modified_base 1..3: mod_base = OTHER; note = phosphorothioate bond; note (original language) = 硫代磷酸酯键
  source 1..19: mol_type = other RNA
gtcccaccttgtcttctaa

SEQ ID NO: 832 - RNA, 19 nt, synthetic construct
  modified_base 1..6: mod_base = OTHER; note = 2'-methoxy nucleoside; note (original language) = 2'-甲氧基核苷
  modified_base 8: mod_base = OTHER; note = 2'-methoxy nucleoside; note (original language) = 2'-甲氧基核苷
  modified_base 11..19: mod_base = OTHER; note = 2'-methoxy nucleoside; note (original language) = 2'-甲氧基核苷
  modified_base 7: mod_base = OTHER; note = 2'-fluoro nucleoside; note (original language) = 2'-氟核苷
  modified_base 9..10: mod_base = OTHER; note = 2'-fluoro nucleoside; note (original language) = 2'-氟核苷
  modified_base 1..3: mod_base = OTHER; note = phosphorothioate bond; note (original language) = 硫代磷酸酯键
  source 1..19: mol_type = other RNA
ccttttcttctaatgagta

SEQ ID NO: 833 - RNA, 19 nt, synthetic construct
  modified_base 1..6: mod_base = OTHER; note = 2'-methoxy nucleoside; note (original language) = 2'-甲氧基核苷
  modified_base 10..19: mod_base = OTHER; note = 2'-methoxy nucleoside; note (original language) = 2'-甲氧基核苷
  modified_base 7..9: mod_base = OTHER; note = 2'-fluoro nucleoside; note (original language) = 2'-氟核苷
  modified_base 1..3: mod_base = OTHER; note = phosphorothioate bond; note (original language) = 硫代磷酸酯键
  source 1..19: mol_type = other RNA
gccaccttttcttctaata

SEQ ID NO: 834 - RNA, 19 nt, synthetic construct
  modified_base 1..6: mod_base = OTHER; note = 2'-methoxy nucleoside; note (original language) = 2'-甲氧基核苷
  modified_base 10..19: mod_base = OTHER; note = 2'-methoxy nucleoside; note (original language) = 2'-甲氧基核苷
  modified_base 7..9: mod_base = OTHER; note = 2'-fluoro nucleoside; note (original language) = 2'-氟核苷
  modified_base 1..3: mod_base = OTHER; note = phosphorothioate bond; note (original language) = 硫代磷酸酯键
  source 1..19: mol_type = other RNA
gaccttttcttctaatgaa

SEQ ID NO: 835 - RNA, 19 nt, synthetic construct
  modified_base 1..6: mod_base = OTHER; note = 2'-methoxy nucleoside; note (original language) = 2'-甲氧基核苷
  modified_base 10..19: mod_base = OTHER; note = 2'-methoxy nucleoside; note (original language) = 2'-甲氧基核苷
  modified_base 7..9: mod_base = OTHER; note = 2'-fluoro nucleoside; note (original language) = 2'-氟核苷
  modified_base 1..3: mod_base = OTHER; note = phosphorothioate bond; note (original language) = 硫代磷酸酯键
  source 1..19: mol_type = other RNA
caagttgagaacaaaaata

SEQ ID NO: 836 - RNA, 19 nt, synthetic construct
  modified_base 1..6: mod_base = OTHER; note = 2'-methoxy nucleoside; note (original language) = 2'-甲氧基核苷
  modified_base 10..19: mod_base = OTHER; note = 2'-methoxy nucleoside; note (original language) = 2'-甲氧基核苷
  modified_base 7..9: mod_base = OTHER; note = 2'-fluoro nucleoside; note (original language) = 2'-氟核苷
  modified_base 1..3: mod_base = OTHER; note = phosphorothioate bond; note (original language) = 硫代磷酸酯键
  source 1..19: mol_type = other RNA
gggcaagaaccagtgttta

SEQ ID NO: 837 - RNA, 19 nt, synthetic construct
  modified_base 1..6: mod_base = OTHER; note = 2'-methoxy nucleoside; note (original language) = 2'-甲氧基核苷
  modified_base 10..19: mod_base = OTHER; note = 2'-methoxy nucleoside; note (original language) = 2'-甲氧基核苷
  modified_base 7..9: mod_base = OTHER; note = 2'-fluoro nucleoside; note (original language) = 2'-氟核苷
  modified_base 1..3: mod_base = OTHER; note = phosphorothioate bond; note (original language) = 硫代磷酸酯键
  source 1..19: mol_type = other RNA
ggaccagcttgtttgtgaa

SEQ ID NO: 838 - RNA, 19 nt, synthetic construct
  modified_base 1..6: mod_base = OTHER; note = 2'-methoxy nucleoside; note (original language) = 2'-甲氧基核苷
  modified_base 10..19: mod_base = OTHER; note = 2'-methoxy nucleoside; note (original language) = 2'-甲氧基核苷
  modified_base 7..9: mod_base = OTHER; note = 2'-fluoro nucleoside; note (original language) = 2'-氟核苷
  modified_base 1..3: mod_base = OTHER; note = phosphorothioate bond; note (original language) = 硫代磷酸酯键
  source 1..19: mol_type = other RNA
caccagcttgtttgtgaaa

SEQ ID NO: 839 - RNA, 21 nt, synthetic construct
  modified_base 1: mod_base = OTHER; note = 2'-methoxy nucleoside; note (original language) = 2'-甲氧基核苷
  modified_base 3..5: mod_base = OTHER; note = 2'-methoxy nucleoside; note (original language) = 2'-甲氧基核苷
  modified_base 7..8: mod_base = OTHER; note = 2'-methoxy nucleoside; note (original language) = 2'-甲氧基核苷
  modified_base 10..13: mod_base = OTHER; note = 2'-methoxy nucleoside; note (original language) = 2'-甲氧基核苷
  modified_base 15: mod_base = OTHER; note = 2'-methoxy nucleoside; note (original language) = 2'-甲氧基核苷
  modified_base 17..21: mod_base = OTHER; note = 2'-methoxy nucleoside; note (original language) = 2'-甲氧基核苷
  modified_base 2: mod_base = OTHER; note = 2'-fluoro nucleoside; note (original language) = 2'-氟核苷
  modified_base 6: mod_base = OTHER; note = 2'-fluoro nucleoside; note (original language) = 2'-氟核苷
  modified_base 9: mod_base = OTHER; note = 2'-fluoro nucleoside; note (original language) = 2'-氟核苷
  modified_base 14: mod_base = OTHER; note = 2'-fluoro nucleoside; note (original language) = 2'-氟核苷
  modified_base 16: mod_base = OTHER; note = 2'-fluoro nucleoside; note (original language) = 2'-氟核苷
  modified_base 1..3: mod_base = OTHER; note = phosphorothioate bond; note (original language) = 硫代磷酸酯键
  modified_base 19..21: mod_base = OTHER; note = phosphorothioate bond; note (original language) = 硫代磷酸酯键
  modified_base 1: mod_base = OTHER; note = 2'-methoxy-5'-vinyl phosphonate nucleoside; note (original language) = 2'-甲氧基-5'-乙烯基膦酸核苷
  source 1..21: mol_type = other RNA
ttagaagaaaaggtgggacac

SEQ ID NO: 840 - RNA, 21 nt, synthetic construct
  modified_base 1: mod_base = OTHER; note = 2'-methoxy nucleoside; note (original language) = 2'-甲氧基核苷
  modified_base 3..5: mod_base = OTHER; note = 2'-methoxy nucleoside; note (original language) = 2'-甲氧基核苷
  modified_base 7..8: mod_base = OTHER; note = 2'-methoxy nucleoside; note (original language) = 2'-甲氧基核苷
  modified_base 10..13: mod_base = OTHER; note = 2'-methoxy nucleoside; note (original language) = 2'-甲氧基核苷
  modified_base 15: mod_base = OTHER; note = 2'-methoxy nucleoside; note (original language) = 2'-甲氧基核苷
  modified_base 17..21: mod_base = OTHER; note = 2'-methoxy nucleoside; note (original language) = 2'-甲氧基核苷
  modified_base 2: mod_base = OTHER; note = 2'-fluoro nucleoside; note (original language) = 2'-氟核苷
  modified_base 6: mod_base = OTHER; note = 2'-fluoro nucleoside; note (original language) = 2'-氟核苷
  modified_base 9: mod_base = OTHER; note = 2'-fluoro nucleoside; note (original language) = 2'-氟核苷
  modified_base 14: mod_base = OTHER; note = 2'-fluoro nucleoside; note (original language) = 2'-氟核苷
  modified_base 16: mod_base = OTHER; note = 2'-fluoro nucleoside; note (original language) = 2'-氟核苷
  modified_base 1..3: mod_base = OTHER; note = phosphorothioate bond; note (original language) = 硫代磷酸酯键
  modified_base 19..21: mod_base = OTHER; note = phosphorothioate bond; note (original language) = 硫代磷酸酯键
  modified_base 1: mod_base = OTHER; note = 2'-methoxy-5'-vinyl phosphonate nucleoside; note (original language) = 2'-甲氧基-5'-乙烯基膦酸核苷
  source 1..21: mol_type = other RNA
tactcattagaagaaaaggtg

SEQ ID NO: 841 - RNA, 21 nt, synthetic construct
  modified_base 1: mod_base = OTHER; note = 2'-methoxy nucleoside; note (original language) = 2'-甲氧基核苷
  modified_base 3..5: mod_base = OTHER; note = 2'-methoxy nucleoside; note (original language) = 2'-甲氧基核苷
  modified_base 7: mod_base = OTHER; note = 2'-methoxy nucleoside; note (original language) = 2'-甲氧基核苷
  modified_base 9..11: mod_base = OTHER; note = 2'-methoxy nucleoside; note (original language) = 2'-甲氧基核苷
  modified_base 13: mod_base = OTHER; note = 2'-methoxy nucleoside; note (original language) = 2'-甲氧基核苷
  modified_base 15: mod_base = OTHER; note = 2'-methoxy nucleoside; note (original language) = 2'-甲氧基核苷
  modified_base 17: mod_base = OTHER; note = 2'-methoxy nucleoside; note (original language) = 2'-甲氧基核苷
  modified_base 19..21: mod_base = OTHER; note = 2'-methoxy nucleoside; note (original language) = 2'-甲氧基核苷
  modified_base 2: mod_base = OTHER; note = 2'-fluoro nucleoside; note (original language) = 2'-氟核苷
  modified_base 6: mod_base = OTHER; note = 2'-fluoro nucleoside; note (original language) = 2'-氟核苷
  modified_base 8: mod_base = OTHER; note = 2'-fluoro nucleoside; note (original language) = 2'-氟核苷
  modified_base 12: mod_base = OTHER; note = 2'-fluoro nucleoside; note (original language) = 2'-氟核苷
  modified_base 14: mod_base = OTHER; note = 2'-fluoro nucleoside; note (original language) = 2'-氟核苷
  modified_base 16: mod_base = OTHER; note = 2'-fluoro nucleoside; note (original language) = 2'-氟核苷
  modified_base 18: mod_base = OTHER; note = 2'-fluoro nucleoside; note (original language) = 2'-氟核苷
  modified_base 1..3: mod_base = OTHER; note = phosphorothioate bond; note (original language) = 硫代磷酸酯键
  modified_base 19..21: mod_base = OTHER; note = phosphorothioate bond; note (original language) = 硫代磷酸酯键
  modified_base 1: mod_base = OTHER; note = 2'-methoxy-5'-vinyl phosphonate nucleoside; note (original language) = 2'-甲氧基-5'-乙烯基膦酸核苷
  source 1..21: mol_type = other RNA
tactcattagaagaaaaggtg

SEQ ID NO: 842 - RNA, 21 nt, synthetic construct
  modified_base 1: mod_base = OTHER; note = 2'-methoxy nucleoside; note (original language) = 2'-甲氧基核苷
  modified_base 3: mod_base = OTHER; note = 2'-methoxy nucleoside; note (original language) = 2'-甲氧基核苷
  modified_base 5: mod_base = OTHER; note = 2'-methoxy nucleoside; note (original language) = 2'-甲氧基核苷
  modified_base 7: mod_base = OTHER; note = 2'-methoxy nucleoside; note (original language) = 2'-甲氧基核苷
  modified_base 9..11: mod_base = OTHER; note = 2'-methoxy nucleoside; note (original language) = 2'-甲氧基核苷
  modified_base 13: mod_base = OTHER; note = 2'-methoxy nucleoside; note (original language) = 2'-甲氧基核苷
  modified_base 15: mod_base = OTHER; note = 2'-methoxy nucleoside; note (original language) = 2'-甲氧基核苷
  modified_base 17: mod_base = OTHER; note = 2'-methoxy nucleoside; note (original language) = 2'-甲氧基核苷
  modified_base 19..21: mod_base = OTHER; note = 2'-methoxy nucleoside; note (original language) = 2'-甲氧基核苷
  modified_base 2: mod_base = OTHER; note = 2'-fluoro nucleoside; note (original language) = 2'-氟核苷
  modified_base 6: mod_base = OTHER; note = 2'-fluoro nucleoside; note (original language) = 2'-氟核苷
  modified_base 8: mod_base = OTHER; note = 2'-fluoro nucleoside; note (original language) = 2'-氟核苷
  modified_base 12: mod_base = OTHER; note = 2'-fluoro nucleoside; note (original language) = 2'-氟核苷
  modified_base 14: mod_base = OTHER; note = 2'-fluoro nucleoside; note (original language) = 2'-氟核苷
  modified_base 16: mod_base = OTHER; note = 2'-fluoro nucleoside; note (original language) = 2'-氟核苷
  modified_base 18: mod_base = OTHER; note = 2'-fluoro nucleoside; note (original language) = 2'-氟核苷
  modified_base 1..3: mod_base = OTHER; note = phosphorothioate bond; note (original language) = 硫代磷酸酯键
  modified_base 19..21: mod_base = OTHER; note = phosphorothioate bond; note (original language) = 硫代磷酸酯键
  modified_base 1: mod_base = OTHER; note = 2'-methoxy-5'-vinyl phosphonate nucleoside; note (original language) = 2'-甲氧基-5'-乙烯基膦酸核苷
  modified_base 4: mod_base = OTHER; note = 2,3-dihydroxypropyl nucleoside; note (original language) = 2,3-二羟丙基核苷
  modified_base 4: mod_base = OTHER; note = thymine; note (original language) = 胸腺嘧啶
  source 1..21: mol_type = other RNA
tactcattagaagaaaaggtg

SEQ ID NO: 843 - RNA, 21 nt, synthetic construct
  modified_base 1: mod_base = OTHER; note = 2'-methoxy nucleoside; note (original language) = 2'-甲氧基核苷
  modified_base 3..4: mod_base = OTHER; note = 2'-methoxy nucleoside; note (original language) = 2'-甲氧基核苷
  modified_base 7: mod_base = OTHER; note = 2'-methoxy nucleoside; note (original language) = 2'-甲氧基核苷
  modified_base 9..11: mod_base = OTHER; note = 2'-methoxy nucleoside; note (original language) = 2'-甲氧基核苷
  modified_base 13: mod_base = OTHER; note = 2'-methoxy nucleoside; note (original language) = 2'-甲氧基核苷
  modified_base 15: mod_base = OTHER; note = 2'-methoxy nucleoside; note (original language) = 2'-甲氧基核苷
  modified_base 17: mod_base = OTHER; note = 2'-methoxy nucleoside; note (original language) = 2'-甲氧基核苷
  modified_base 19..21: mod_base = OTHER; note = 2'-methoxy nucleoside; note (original language) = 2'-甲氧基核苷
  modified_base 2: mod_base = OTHER; note = 2'-fluoro nucleoside; note (original language) = 2'-氟核苷
  modified_base 6: mod_base = OTHER; note = 2'-fluoro nucleoside; note (original language) = 2'-氟核苷
  modified_base 8: mod_base = OTHER; note = 2'-fluoro nucleoside; note (original language) = 2'-氟核苷
  modified_base 12: mod_base = OTHER; note = 2'-fluoro nucleoside; note (original language) = 2'-氟核苷
  modified_base 14: mod_base = OTHER; note = 2'-fluoro nucleoside; note (original language) = 2'-氟核苷
  modified_base 16: mod_base = OTHER; note = 2'-fluoro nucleoside; note (original language) = 2'-氟核苷
  modified_base 18: mod_base = OTHER; note = 2'-fluoro nucleoside; note (original language) = 2'-氟核苷
  modified_base 1..3: mod_base = OTHER; note = phosphorothioate bond; note (original language) = 硫代磷酸酯键
  modified_base 19..21: mod_base = OTHER; note = phosphorothioate bond; note (original language) = 硫代磷酸酯键
  modified_base 1: mod_base = OTHER; note = 2'-methoxy-5'-vinyl phosphonate nucleoside; note (original language) = 2'-甲氧基-5'-乙烯基膦酸核苷
  modified_base 5: mod_base = OTHER; note = 2,3-dihydroxypropyl nucleoside; note (original language) = 2,3-二羟丙基核苷
  source 1..21: mol_type = other RNA
tactcattagaagaaaaggtg

SEQ ID NO: 844 - RNA, 21 nt, synthetic construct
  modified_base 1: mod_base = OTHER; note = 2'-methoxy nucleoside; note (original language) = 2'-甲氧基核苷
  modified_base 3..5: mod_base = OTHER; note = 2'-methoxy nucleoside; note (original language) = 2'-甲氧基核苷
  modified_base 7: mod_base = OTHER; note = 2'-methoxy nucleoside; note (original language) = 2'-甲氧基核苷
  modified_base 9..11: mod_base = OTHER; note = 2'-methoxy nucleoside; note (original language) = 2'-甲氧基核苷
  modified_base 13: mod_base = OTHER; note = 2'-methoxy nucleoside; note (original language) = 2'-甲氧基核苷
  modified_base 15: mod_base = OTHER; note = 2'-methoxy nucleoside; note (original language) = 2'-甲氧基核苷
  modified_base 17: mod_base = OTHER; note = 2'-methoxy nucleoside; note (original language) = 2'-甲氧基核苷
  modified_base 19..21: mod_base = OTHER; note = 2'-methoxy nucleoside; note (original language) = 2'-甲氧基核苷
  modified_base 2: mod_base = OTHER; note = 2'-fluoro nucleoside; note (original language) = 2'-氟核苷
  modified_base 8: mod_base = OTHER; note = 2'-fluoro nucleoside; note (original language) = 2'-氟核苷
  modified_base 12: mod_base = OTHER; note = 2'-fluoro nucleoside; note (original language) = 2'-氟核苷
  modified_base 14: mod_base = OTHER; note = 2'-fluoro nucleoside; note (original language) = 2'-氟核苷
  modified_base 16: mod_base = OTHER; note = 2'-fluoro nucleoside; note (original language) = 2'-氟核苷
  modified_base 18: mod_base = OTHER; note = 2'-fluoro nucleoside; note (original language) = 2'-氟核苷
  modified_base 1..3: mod_base = OTHER; note = phosphorothioate bond; note (original language) = 硫代磷酸酯键
  modified_base 19..21: mod_base = OTHER; note = phosphorothioate bond; note (original language) = 硫代磷酸酯键
  modified_base 1: mod_base = OTHER; note = 2'-methoxy-5'-vinyl phosphonate nucleoside; note (original language) = 2'-甲氧基-5'-乙烯基膦酸核苷
  modified_base 6: mod_base = OTHER; note = 2,3-dihydroxypropyl nucleoside; note (original language) = 2,3-二羟丙基核苷
  source 1..21: mol_type = other RNA
tactcattagaagaaaaggtg

SEQ ID NO: 845 - RNA, 21 nt, synthetic construct
  modified_base 1: mod_base = OTHER; note = 2'-methoxy nucleoside; note (original language) = 2'-甲氧基核苷
  modified_base 3..5: mod_base = OTHER; note = 2'-methoxy nucleoside; note (original language) = 2'-甲氧基核苷
  modified_base 9..11: mod_base = OTHER; note = 2'-methoxy nucleoside; note (original language) = 2'-甲氧基核苷
  modified_base 13: mod_base = OTHER; note = 2'-methoxy nucleoside; note (original language) = 2'-甲氧基核苷
  modified_base 15: mod_base = OTHER; note = 2'-methoxy nucleoside; note (original language) = 2'-甲氧基核苷
  modified_base 17: mod_base = OTHER; note = 2'-methoxy nucleoside; note (original language) = 2'-甲氧基核苷
  modified_base 19..21: mod_base = OTHER; note = 2'-methoxy nucleoside; note (original language) = 2'-甲氧基核苷
  modified_base 2: mod_base = OTHER; note = 2'-fluoro nucleoside; note (original language) = 2'-氟核苷
  modified_base 6: mod_base = OTHER; note = 2'-fluoro nucleoside; note (original language) = 2'-氟核苷
  modified_base 8: mod_base = OTHER; note = 2'-fluoro nucleoside; note (original language) = 2'-氟核苷
  modified_base 12: mod_base = OTHER; note = 2'-fluoro nucleoside; note (original language) = 2'-氟核苷
  modified_base 14: mod_base = OTHER; note = 2'-fluoro nucleoside; note (original language) = 2'-氟核苷
  modified_base 16: mod_base = OTHER; note = 2'-fluoro nucleoside; note (original language) = 2'-氟核苷
  modified_base 18: mod_base = OTHER; note = 2'-fluoro nucleoside; note (original language) = 2'-氟核苷
  modified_base 1..3: mod_base = OTHER; note = phosphorothioate bond; note (original language) = 硫代磷酸酯键
  modified_base 19..21: mod_base = OTHER; note = phosphorothioate bond; note (original language) = 硫代磷酸酯键
  modified_base 1: mod_base = OTHER; note = 2'-methoxy-5'-vinyl phosphonate nucleoside; note (original language) = 2'-甲氧基-5'-乙烯基膦酸核苷
  modified_base 7: mod_base = OTHER; note = 2,3-dihydroxypropyl nucleoside; note (original language) = 2,3-二羟丙基核苷
  modified_base 7: mod_base = OTHER; note = thymine; note (original language) = 胸腺嘧啶
  source 1..21: mol_type = other RNA
tactcattagaagaaaaggtg

SEQ ID NO: 846 - RNA, 21 nt, synthetic construct
  modified_base 1: mod_base = OTHER; note = 2'-methoxy nucleoside; note (original language) = 2'-甲氧基核苷
  modified_base 3..5: mod_base = OTHER; note = 2'-methoxy nucleoside; note (original language) = 2'-甲氧基核苷
  modified_base 7: mod_base = OTHER; note = 2'-methoxy nucleoside; note (original language) = 2'-甲氧基核苷
  modified_base 9..11: mod_base = OTHER; note = 2'-methoxy nucleoside; note (original language) = 2'-甲氧基核苷
  modified_base 13: mod_base = OTHER; note = 2'-methoxy nucleoside; note (original language) = 2'-甲氧基核苷
  modified_base 15: mod_base = OTHER; note = 2'-methoxy nucleoside; note (original language) = 2'-甲氧基核苷
  modified_base 17: mod_base = OTHER; note = 2'-methoxy nucleoside; note (original language) = 2'-甲氧基核苷
  modified_base 19..21: mod_base = OTHER; note = 2'-methoxy nucleoside; note (original language) = 2'-甲氧基核苷
  modified_base 2: mod_base = OTHER; note = 2'-fluoro nucleoside; note (original language) = 2'-氟核苷
  modified_base 6: mod_base = OTHER; note = 2'-fluoro nucleoside; note (original language) = 2'-氟核苷
  modified_base 12: mod_base = OTHER; note = 2'-fluoro nucleoside; note (original language) = 2'-氟核苷
  modified_base 14: mod_base = OTHER; note = 2'-fluoro nucleoside; note (original language) = 2'-氟核苷
  modified_base 16: mod_base = OTHER; note = 2'-fluoro nucleoside; note (original language) = 2'-氟核苷
  modified_base 18: mod_base = OTHER; note = 2'-fluoro nucleoside; note (original language) = 2'-氟核苷
  modified_base 1..3: mod_base = OTHER; note = phosphorothioate bond; note (original language) = 硫代磷酸酯键
  modified_base 19..21: mod_base = OTHER; note = phosphorothioate bond; note (original language) = 硫代磷酸酯键
  modified_base 1: mod_base = OTHER; note = 2'-methoxy-5'-vinyl phosphonate nucleoside; note (original language) = 2'-甲氧基-5'-乙烯基膦酸核苷
  modified_base 8: mod_base = OTHER; note = 2,3-dihydroxypropyl nucleoside; note (original language) = 2,3-二羟丙基核苷
  modified_base 8: mod_base = OTHER; note = thymine; note (original language) = 胸腺嘧啶
  source 1..21: mol_type = other RNA
tactcattagaagaaaaggtg

SEQ ID NO: 847 - RNA, 21 nt, synthetic construct
  modified_base 1: mod_base = OTHER; note = 2'-methoxy nucleoside; note (original language) = 2'-甲氧基核苷
  modified_base 3: mod_base = OTHER; note = 2'-methoxy nucleoside; note (original language) = 2'-甲氧基核苷
  modified_base 5: mod_base = OTHER; note = 2'-methoxy nucleoside; note (original language) = 2'-甲氧基核苷
  modified_base 7: mod_base = OTHER; note = 2'-methoxy nucleoside; note (original language) = 2'-甲氧基核苷
  modified_base 9..11: mod_base = OTHER; note = 2'-methoxy nucleoside; note (original language) = 2'-甲氧基核苷
  modified_base 13: mod_base = OTHER; note = 2'-methoxy nucleoside; note (original language) = 2'-甲氧基核苷
  modified_base 15: mod_base = OTHER; note = 2'-methoxy nucleoside; note (original language) = 2'-甲氧基核苷
  modified_base 17: mod_base = OTHER; note = 2'-methoxy nucleoside; note (original language) = 2'-甲氧基核苷
  modified_base 19..21: mod_base = OTHER; note = 2'-methoxy nucleoside; note (original language) = 2'-甲氧基核苷
  modified_base 2: mod_base = OTHER; note = 2'-fluoro nucleoside; note (original language) = 2'-氟核苷
  modified_base 6: mod_base = OTHER; note = 2'-fluoro nucleoside; note (original language) = 2'-氟核苷
  modified_base 8: mod_base = OTHER; note = 2'-fluoro nucleoside; note (original language) = 2'-氟核苷
  modified_base 12: mod_base = OTHER; note = 2'-fluoro nucleoside; note (original language) = 2'-氟核苷
  modified_base 14: mod_base = OTHER; note = 2'-fluoro nucleoside; note (original language) = 2'-氟核苷
  modified_base 16: mod_base = OTHER; note = 2'-fluoro nucleoside; note (original language) = 2'-氟核苷
  modified_base 18: mod_base = OTHER; note = 2'-fluoro nucleoside; note (original language) = 2'-氟核苷
  modified_base 1..3: mod_base = OTHER; note = phosphorothioate bond; note (original language) = 硫代磷酸酯键
  modified_base 19..21: mod_base = OTHER; note = phosphorothioate bond; note (original language) = 硫代磷酸酯键
  modified_base 1: mod_base = OTHER; note = 2'-methoxy-5'-vinyl phosphonate nucleoside; note (original language) = 2'-甲氧基-5'-乙烯基膦酸核苷
  modified_base 4..5: mod_base = OTHER; note = The nucleotide monomers are mutually linked by 2'-5'-phosphodiester bond.; note (original language) = 核苷酸单体通过2'-5'-磷酸二酯键相互连接
  source 1..21: mol_type = other RNA
tactcattagaagaaaaggtg

SEQ ID NO: 848 - RNA, 21 nt, synthetic construct
  modified_base 1: mod_base = OTHER; note = 2'-methoxy nucleoside; note (original language) = 2'-甲氧基核苷
  modified_base 3..4: mod_base = OTHER; note = 2'-methoxy nucleoside; note (original language) = 2'-甲氧基核苷
  modified_base 7: mod_base = OTHER; note = 2'-methoxy nucleoside; note (original language) = 2'-甲氧基核苷
  modified_base 9..11: mod_base = OTHER; note = 2'-methoxy nucleoside; note (original language) = 2'-甲氧基核苷
  modified_base 13: mod_base = OTHER; note = 2'-methoxy nucleoside; note (original language) = 2'-甲氧基核苷
  modified_base 15: mod_base = OTHER; note = 2'-methoxy nucleoside; note (original language) = 2'-甲氧基核苷
  modified_base 17: mod_base = OTHER; note = 2'-methoxy nucleoside; note (original language) = 2'-甲氧基核苷
  modified_base 19..21: mod_base = OTHER; note = 2'-methoxy nucleoside; note (original language) = 2'-甲氧基核苷
  modified_base 2: mod_base = OTHER; note = 2'-fluoro nucleoside; note (original language) = 2'-氟核苷
  modified_base 6: mod_base = OTHER; note = 2'-fluoro nucleoside; note (original language) = 2'-氟核苷
  modified_base 8: mod_base = OTHER; note = 2'-fluoro nucleoside; note (original language) = 2'-氟核苷
  modified_base 12: mod_base = OTHER; note = 2'-fluoro nucleoside; note (original language) = 2'-氟核苷
  modified_base 14: mod_base = OTHER; note = 2'-fluoro nucleoside; note (original language) = 2'-氟核苷
  modified_base 16: mod_base = OTHER; note = 2'-fluoro nucleoside; note (original language) = 2'-氟核苷
  modified_base 18: mod_base = OTHER; note = 2'-fluoro nucleoside; note (original language) = 2'-氟核苷
  modified_base 1..3: mod_base = OTHER; note = phosphorothioate bond; note (original language) = 硫代磷酸酯键
  modified_base 19..21: mod_base = OTHER; note = phosphorothioate bond; note (original language) = 硫代磷酸酯键
  modified_base 1: mod_base = OTHER; note = 2'-methoxy-5'-vinyl phosphonate nucleoside; note (original language) = 2'-甲氧基-5'-乙烯基膦酸核苷
  modified_base 5..6: mod_base = OTHER; note = The nucleotide monomers are mutually linked by 2'-5'-phosphodiester bond.; note (original language) = 核苷酸单体通过2'-5'-磷酸二酯键相互连接
  source 1..21: mol_type = other RNA
tactcattagaagaaaaggtg

SEQ ID NO: 849 - RNA, 21 nt, synthetic construct
  modified_base 1: mod_base = OTHER; note = 2'-methoxy nucleoside; note (original language) = 2'-甲氧基核苷
  modified_base 3..5: mod_base = OTHER; note = 2'-methoxy nucleoside; note (original language) = 2'-甲氧基核苷
  modified_base 7: mod_base = OTHER; note = 2'-methoxy nucleoside; note (original language) = 2'-甲氧基核苷
  modified_base 9..11: mod_base = OTHER; note = 2'-methoxy nucleoside; note (original language) = 2'-甲氧基核苷
  modified_base 13: mod_base = OTHER; note = 2'-methoxy nucleoside; note (original language) = 2'-甲氧基核苷
  modified_base 15: mod_base = OTHER; note = 2'-methoxy nucleoside; note (original language) = 2'-甲氧基核苷
  modified_base 17: mod_base = OTHER; note = 2'-methoxy nucleoside; note (original language) = 2'-甲氧基核苷
  modified_base 19..21: mod_base = OTHER; note = 2'-methoxy nucleoside; note (original language) = 2'-甲氧基核苷
  modified_base 2: mod_base = OTHER; note = 2'-fluoro nucleoside; note (original language) = 2'-氟核苷
  modified_base 8: mod_base = OTHER; note = 2'-fluoro nucleoside; note (original language) = 2'-氟核苷
  modified_base 12: mod_base = OTHER; note = 2'-fluoro nucleoside; note (original language) = 2'-氟核苷
  modified_base 14: mod_base = OTHER; note = 2'-fluoro nucleoside; note (original language) = 2'-氟核苷
  modified_base 16: mod_base = OTHER; note = 2'-fluoro nucleoside; note (original language) = 2'-氟核苷
  modified_base 18: mod_base = OTHER; note = 2'-fluoro nucleoside; note (original language) = 2'-氟核苷
  modified_base 1..3: mod_base = OTHER; note = phosphorothioate bond; note (original language) = 硫代磷酸酯键
  modified_base 19..21: mod_base = OTHER; note = phosphorothioate bond; note (original language) = 硫代磷酸酯键
  modified_base 1: mod_base = OTHER; note = 2'-methoxy-5'-vinyl phosphonate nucleoside; note (original language) = 2'-甲氧基-5'-乙烯基膦酸核苷
  modified_base 6..7: mod_base = OTHER; note = The nucleotide monomers are mutually linked by 2'-5'-phosphodiester bond.; note (original language) = 核苷酸单体通过2'-5'-磷酸二酯键相互连接
  source 1..21: mol_type = other RNA
tactcattagaagaaaaggtg

SEQ ID NO: 850 - RNA, 21 nt, synthetic construct
  modified_base 1: mod_base = OTHER; note = 2'-methoxy nucleoside; note (original language) = 2'-甲氧基核苷
  modified_base 3..5: mod_base = OTHER; note = 2'-methoxy nucleoside; note (original language) = 2'-甲氧基核苷
  modified_base 9..11: mod_base = OTHER; note = 2'-methoxy nucleoside; note (original language) = 2'-甲氧基核苷
  modified_base 13: mod_base = OTHER; note = 2'-methoxy nucleoside; note (original language) = 2'-甲氧基核苷
  modified_base 15: mod_base = OTHER; note = 2'-methoxy nucleoside; note (original language) = 2'-甲氧基核苷
  modified_base 17: mod_base = OTHER; note = 2'-methoxy nucleoside; note (original language) = 2'-甲氧基核苷
  modified_base 19..21: mod_base = OTHER; note = 2'-methoxy nucleoside; note (original language) = 2'-甲氧基核苷
  modified_base 2: mod_base = OTHER; note = 2'-fluoro nucleoside; note (original language) = 2'-氟核苷
  modified_base 6: mod_base = OTHER; note = 2'-fluoro nucleoside; note (original language) = 2'-氟核苷
  modified_base 8: mod_base = OTHER; note = 2'-fluoro nucleoside; note (original language) = 2'-氟核苷
  modified_base 12: mod_base = OTHER; note = 2'-fluoro nucleoside; note (original language) = 2'-氟核苷
  modified_base 14: mod_base = OTHER; note = 2'-fluoro nucleoside; note (original language) = 2'-氟核苷
  modified_base 16: mod_base = OTHER; note = 2'-fluoro nucleoside; note (original language) = 2'-氟核苷
  modified_base 18: mod_base = OTHER; note = 2'-fluoro nucleoside; note (original language) = 2'-氟核苷
  modified_base 1..3: mod_base = OTHER; note = phosphorothioate bond; note (original language) = 硫代磷酸酯键
  modified_base 19..21: mod_base = OTHER; note = phosphorothioate bond; note (original language) = 硫代磷酸酯键
  modified_base 1: mod_base = OTHER; note = 2'-methoxy-5'-vinyl phosphonate nucleoside; note (original language) = 2'-甲氧基-5'-乙烯基膦酸核苷
  modified_base 7..8: mod_base = OTHER; note = The nucleotide monomers are mutually linked by 2'-5'-phosphodiester bond.; note (original language) = 核苷酸单体通过2'-5'-磷酸二酯键相互连接
  source 1..21: mol_type = other RNA
tactcattagaagaaaaggtg

SEQ ID NO: 851 - RNA, 21 nt, synthetic construct
  modified_base 1: mod_base = OTHER; note = 2'-methoxy nucleoside; note (original language) = 2'-甲氧基核苷
  modified_base 3..5: mod_base = OTHER; note = 2'-methoxy nucleoside; note (original language) = 2'-甲氧基核苷
  modified_base 7: mod_base = OTHER; note = 2'-methoxy nucleoside; note (original language) = 2'-甲氧基核苷
  modified_base 9..11: mod_base = OTHER; note = 2'-methoxy nucleoside; note (original language) = 2'-甲氧基核苷
  modified_base 13: mod_base = OTHER; note = 2'-methoxy nucleoside; note (original language) = 2'-甲氧基核苷
  modified_base 15: mod_base = OTHER; note = 2'-methoxy nucleoside; note (original language) = 2'-甲氧基核苷
  modified_base 17: mod_base = OTHER; note = 2'-methoxy nucleoside; note (original language) = 2'-甲氧基核苷
  modified_base 19..21: mod_base = OTHER; note = 2'-methoxy nucleoside; note (original language) = 2'-甲氧基核苷
  modified_base 2: mod_base = OTHER; note = 2'-fluoro nucleoside; note (original language) = 2'-氟核苷
  modified_base 6: mod_base = OTHER; note = 2'-fluoro nucleoside; note (original language) = 2'-氟核苷
  modified_base 12: mod_base = OTHER; note = 2'-fluoro nucleoside; note (original language) = 2'-氟核苷
  modified_base 14: mod_base = OTHER; note = 2'-fluoro nucleoside; note (original language) = 2'-氟核苷
  modified_base 16: mod_base = OTHER; note = 2'-fluoro nucleoside; note (original language) = 2'-氟核苷
  modified_base 18: mod_base = OTHER; note = 2'-fluoro nucleoside; note (original language) = 2'-氟核苷
  modified_base 1..3: mod_base = OTHER; note = phosphorothioate bond; note (original language) = 硫代磷酸酯键
  modified_base 19..21: mod_base = OTHER; note = phosphorothioate bond; note (original language) = 硫代磷酸酯键
  modified_base 1: mod_base = OTHER; note = 2'-methoxy-5'-vinyl phosphonate nucleoside; note (original language) = 2'-甲氧基-5'-乙烯基膦酸核苷
  modified_base 8..9: mod_base = OTHER; note = The nucleotide monomers are mutually linked by 2'-5'-phosphodiester bond.; note (original language) = 核苷酸单体通过2'-5'-磷酸二酯键相互连接
  source 1..21: mol_type = other RNA
tactcattagaagaaaaggtg

SEQ ID NO: 852 - RNA, 23 nt, synthetic construct
  modified_base 1: mod_base = OTHER; note = 2'-methoxy nucleoside; note (original language) = 2'-甲氧基核苷
  modified_base 3..5: mod_base = OTHER; note = 2'-methoxy nucleoside; note (original language) = 2'-甲氧基核苷
  modified_base 7..8: mod_base = OTHER; note = 2'-methoxy nucleoside; note (original language) = 2'-甲氧基核苷
  modified_base 10..13: mod_base = OTHER; note = 2'-methoxy nucleoside; note (original language) = 2'-甲氧基核苷
  modified_base 15: mod_base = OTHER; note = 2'-methoxy nucleoside; note (original language) = 2'-甲氧基核苷
  modified_base 17..23: mod_base = OTHER; note = 2'-methoxy nucleoside; note (original language) = 2'-甲氧基核苷
  modified_base 2: mod_base = OTHER; note = 2'-fluoro nucleoside; note (original language) = 2'-氟核苷
  modified_base 6: mod_base = OTHER; note = 2'-fluoro nucleoside; note (original language) = 2'-氟核苷
  modified_base 9: mod_base = OTHER; note = 2'-fluoro nucleoside; note (original language) = 2'-氟核苷
  modified_base 14: mod_base = OTHER; note = 2'-fluoro nucleoside; note (original language) = 2'-氟核苷
  modified_base 16: mod_base = OTHER; note = 2'-fluoro nucleoside; note (original language) = 2'-氟核苷
  modified_base 1..3: mod_base = OTHER; note = phosphorothioate bond; note (original language) = 硫代磷酸酯键
  modified_base 21..23: mod_base = OTHER; note = phosphorothioate bond; note (original language) = 硫代磷酸酯键
  modified_base 1: mod_base = OTHER; note = 2'-methoxy-5'-vinyl phosphonate nucleoside; note (original language) = 2'-甲氧基-5'-乙烯基膦酸核苷
  modified_base 12: mod_base = i
  source 1..23: mol_type = other RNA
tcttagaccaangagaaacgcct

SEQ ID NO: 853 - RNA, 23 nt, synthetic construct
  modified_base 1: mod_base = OTHER; note = 2'-methoxy nucleoside; note (original language) = 2'-甲氧基核苷
  modified_base 3..5: mod_base = OTHER; note = 2'-methoxy nucleoside; note (original language) = 2'-甲氧基核苷
  modified_base 7..8: mod_base = OTHER; note = 2'-methoxy nucleoside; note (original language) = 2'-甲氧基核苷
  modified_base 10..13: mod_base = OTHER; note = 2'-methoxy nucleoside; note (original language) = 2'-甲氧基核苷
  modified_base 15: mod_base = OTHER; note = 2'-methoxy nucleoside; note (original language) = 2'-甲氧基核苷
  modified_base 17..23: mod_base = OTHER; note = 2'-methoxy nucleoside; note (original language) = 2'-甲氧基核苷
  modified_base 2: mod_base = OTHER; note = 2'-fluoro nucleoside; note (original language) = 2'-氟核苷
  modified_base 6: mod_base = OTHER; note = 2'-fluoro nucleoside; note (original language) = 2'-氟核苷
  modified_base 9: mod_base = OTHER; note = 2'-fluoro nucleoside; note (original language) = 2'-氟核苷
  modified_base 14: mod_base = OTHER; note = 2'-fluoro nucleoside; note (original language) = 2'-氟核苷
  modified_base 16: mod_base = OTHER; note = 2'-fluoro nucleoside; note (original language) = 2'-氟核苷
  modified_base 1..3: mod_base = OTHER; note = phosphorothioate bond; note (original language) = 硫代磷酸酯键
  modified_base 21..23: mod_base = OTHER; note = phosphorothioate bond; note (original language) = 硫代磷酸酯键
  modified_base 1: mod_base = OTHER; note = 2'-methoxy-5'-vinyl phosphonate nucleoside; note (original language) = 2'-甲氧基-5'-乙烯基膦酸核苷
  modified_base 13: mod_base = i
  source 1..23: mol_type = other RNA
tcttagaccaagnagaaacgcct

SEQ ID NO: 854 - RNA, 23 nt, synthetic construct
  modified_base 1: mod_base = OTHER; note = 2'-methoxy nucleoside; note (original language) = 2'-甲氧基核苷
  modified_base 3..5: mod_base = OTHER; note = 2'-methoxy nucleoside; note (original language) = 2'-甲氧基核苷
  modified_base 7..8: mod_base = OTHER; note = 2'-methoxy nucleoside; note (original language) = 2'-甲氧基核苷
  modified_base 10..13: mod_base = OTHER; note = 2'-methoxy nucleoside; note (original language) = 2'-甲氧基核苷
  modified_base 15: mod_base = OTHER; note = 2'-methoxy nucleoside; note (original language) = 2'-甲氧基核苷
  modified_base 17..23: mod_base = OTHER; note = 2'-methoxy nucleoside; note (original language) = 2'-甲氧基核苷
  modified_base 2: mod_base = OTHER; note = 2'-fluoro nucleoside; note (original language) = 2'-氟核苷
  modified_base 6: mod_base = OTHER; note = 2'-fluoro nucleoside; note (original language) = 2'-氟核苷
  modified_base 9: mod_base = OTHER; note = 2'-fluoro nucleoside; note (original language) = 2'-氟核苷
  modified_base 14: mod_base = OTHER; note = 2'-fluoro nucleoside; note (original language) = 2'-氟核苷
  modified_base 16: mod_base = OTHER; note = 2'-fluoro nucleoside; note (original language) = 2'-氟核苷
  modified_base 1..3: mod_base = OTHER; note = phosphorothioate bond; note (original language) = 硫代磷酸酯键
  modified_base 21..23: mod_base = OTHER; note = phosphorothioate bond; note (original language) = 硫代磷酸酯键
  modified_base 1: mod_base = OTHER; note = 2'-methoxy-5'-vinyl phosphonate nucleoside; note (original language) = 2'-甲氧基-5'-乙烯基膦酸核苷
  modified_base 15: mod_base = i
  source 1..23: mol_type = other RNA
tcttagaccaagganaaacgcct

SEQ ID NO: 855 - RNA, 23 nt, synthetic construct
  modified_base 1: mod_base = OTHER; note = 2'-methoxy nucleoside; note (original language) = 2'-甲氧基核苷
  modified_base 3..5: mod_base = OTHER; note = 2'-methoxy nucleoside; note (original language) = 2'-甲氧基核苷
  modified_base 7..8: mod_base = OTHER; note = 2'-methoxy nucleoside; note (original language) = 2'-甲氧基核苷
  modified_base 10..13: mod_base = OTHER; note = 2'-methoxy nucleoside; note (original language) = 2'-甲氧基核苷
  modified_base 15: mod_base = OTHER; note = 2'-methoxy nucleoside; note (original language) = 2'-甲氧基核苷
  modified_base 17..23: mod_base = OTHER; note = 2'-methoxy nucleoside; note (original language) = 2'-甲氧基核苷
  modified_base 2: mod_base = OTHER; note = 2'-fluoro nucleoside; note (original language) = 2'-氟核苷
  modified_base 6: mod_base = OTHER; note = 2'-fluoro nucleoside; note (original language) = 2'-氟核苷
  modified_base 9: mod_base = OTHER; note = 2'-fluoro nucleoside; note (original language) = 2'-氟核苷
  modified_base 14: mod_base = OTHER; note = 2'-fluoro nucleoside; note (original language) = 2'-氟核苷
  modified_base 16: mod_base = OTHER; note = 2'-fluoro nucleoside; note (original language) = 2'-氟核苷
  modified_base 1..3: mod_base = OTHER; note = phosphorothioate bond; note (original language) = 硫代磷酸酯键
  modified_base 21..23: mod_base = OTHER; note = phosphorothioate bond; note (original language) = 硫代磷酸酯键
  modified_base 1: mod_base = OTHER; note = 2'-methoxy-5'-vinyl phosphonate nucleoside; note (original language) = 2'-甲氧基-5'-乙烯基膦酸核苷
  modified_base 17: mod_base = i
  source 1..23: mol_type = other RNA
tcttagaccaaggaganacgcct

SEQ ID NO: 856 - RNA, 23 nt, synthetic construct
  modified_base 1: mod_base = OTHER; note = 2'-methoxy nucleoside; note (original language) = 2'-甲氧基核苷
  modified_base 3..5: mod_base = OTHER; note = 2'-methoxy nucleoside; note (original language) = 2'-甲氧基核苷
  modified_base 7..8: mod_base = OTHER; note = 2'-methoxy nucleoside; note (original language) = 2'-甲氧基核苷
  modified_base 10..13: mod_base = OTHER; note = 2'-methoxy nucleoside; note (original language) = 2'-甲氧基核苷
  modified_base 15: mod_base = OTHER; note = 2'-methoxy nucleoside; note (original language) = 2'-甲氧基核苷
  modified_base 17..23: mod_base = OTHER; note = 2'-methoxy nucleoside; note (original language) = 2'-甲氧基核苷
  modified_base 2: mod_base = OTHER; note = 2'-fluoro nucleoside; note (original language) = 2'-氟核苷
  modified_base 6: mod_base = OTHER; note = 2'-fluoro nucleoside; note (original language) = 2'-氟核苷
  modified_base 9: mod_base = OTHER; note = 2'-fluoro nucleoside; note (original language) = 2'-氟核苷
  modified_base 14: mod_base = OTHER; note = 2'-fluoro nucleoside; note (original language) = 2'-氟核苷
  modified_base 16: mod_base = OTHER; note = 2'-fluoro nucleoside; note (original language) = 2'-氟核苷
  modified_base 1..3: mod_base = OTHER; note = phosphorothioate bond; note (original language) = 硫代磷酸酯键
  modified_base 21..23: mod_base = OTHER; note = phosphorothioate bond; note (original language) = 硫代磷酸酯键
  modified_base 1: mod_base = OTHER; note = 2'-methoxy-5'-vinyl phosphonate nucleoside; note (original language) = 2'-甲氧基-5'-乙烯基膦酸核苷
  modified_base 18: mod_base = i
  source 1..23: mol_type = other RNA
tcttagaccaaggagaancgcct

SEQ ID NO: 857 - RNA, 23 nt, synthetic construct
  modified_base 1: mod_base = OTHER; note = 2'-methoxy nucleoside; note (original language) = 2'-甲氧基核苷
  modified_base 3..5: mod_base = OTHER; note = 2'-methoxy nucleoside; note (original language) = 2'-甲氧基核苷
  modified_base 7..8: mod_base = OTHER; note = 2'-methoxy nucleoside; note (original language) = 2'-甲氧基核苷
  modified_base 10..13: mod_base = OTHER; note = 2'-methoxy nucleoside; note (original language) = 2'-甲氧基核苷
  modified_base 15: mod_base = OTHER; note = 2'-methoxy nucleoside; note (original language) = 2'-甲氧基核苷
  modified_base 17..23: mod_base = OTHER; note = 2'-methoxy nucleoside; note (original language) = 2'-甲氧基核苷
  modified_base 2: mod_base = OTHER; note = 2'-fluoro nucleoside; note (original language) = 2'-氟核苷
  modified_base 6: mod_base = OTHER; note = 2'-fluoro nucleoside; note (original language) = 2'-氟核苷
  modified_base 9: mod_base = OTHER; note = 2'-fluoro nucleoside; note (original language) = 2'-氟核苷
  modified_base 14: mod_base = OTHER; note = 2'-fluoro nucleoside; note (original language) = 2'-氟核苷
  modified_base 16: mod_base = OTHER; note = 2'-fluoro nucleoside; note (original language) = 2'-氟核苷
  modified_base 1..3: mod_base = OTHER; note = phosphorothioate bond; note (original language) = 硫代磷酸酯键
  modified_base 21..23: mod_base = OTHER; note = phosphorothioate bond; note (original language) = 硫代磷酸酯键
  modified_base 1: mod_base = OTHER; note = 2'-methoxy-5'-vinyl phosphonate nucleoside; note (original language) = 2'-甲氧基-5'-乙烯基膦酸核苷
  modified_base 20: mod_base = i
  source 1..23: mol_type = other RNA
tcttagaccaaggagaaacncct

SEQ ID NO: 858 - RNA, 21 nt, synthetic construct
  modified_base 1: mod_base = OTHER; note = 2'-methoxy nucleoside; note (original language) = 2'-甲氧基核苷
  modified_base 3..5: mod_base = OTHER; note = 2'-methoxy nucleoside; note (original language) = 2'-甲氧基核苷
  modified_base 7..8: mod_base = OTHER; note = 2'-methoxy nucleoside; note (original language) = 2'-甲氧基核苷
  modified_base 10..13: mod_base = OTHER; note = 2'-methoxy nucleoside; note (original language) = 2'-甲氧基核苷
  modified_base 15: mod_base = OTHER; note = 2'-methoxy nucleoside; note (original language) = 2'-甲氧基核苷
  modified_base 17..21: mod_base = OTHER; note = 2'-methoxy nucleoside; note (original language) = 2'-甲氧基核苷
  modified_base 2: mod_base = OTHER; note = 2'-fluoro nucleoside; note (original language) = 2'-氟核苷
  modified_base 6: mod_base = OTHER; note = 2'-fluoro nucleoside; note (original language) = 2'-氟核苷
  modified_base 9: mod_base = OTHER; note = 2'-fluoro nucleoside; note (original language) = 2'-氟核苷
  modified_base 14: mod_base = OTHER; note = 2'-fluoro nucleoside; note (original language) = 2'-氟核苷
  modified_base 16: mod_base = OTHER; note = 2'-fluoro nucleoside; note (original language) = 2'-氟核苷
  modified_base 1..3: mod_base = OTHER; note = phosphorothioate bond; note (original language) = 硫代磷酸酯键
  modified_base 19..21: mod_base = OTHER; note = phosphorothioate bond; note (original language) = 硫代磷酸酯键
  modified_base 1: mod_base = OTHER; note = 2'-methoxy-5'-vinyl phosphonate nucleoside; note (original language) = 2'-甲氧基-5'-乙烯基膦酸核苷
  source 1..21: mol_type = other RNA
tattagaagaaaaggtggcag

SEQ ID NO: 859 - RNA, 21 nt, synthetic construct
  modified_base 1: mod_base = OTHER; note = 2'-methoxy nucleoside; note (original language) = 2'-甲氧基核苷
  modified_base 3..5: mod_base = OTHER; note = 2'-methoxy nucleoside; note (original language) = 2'-甲氧基核苷
  modified_base 7..8: mod_base = OTHER; note = 2'-methoxy nucleoside; note (original language) = 2'-甲氧基核苷
  modified_base 10..13: mod_base = OTHER; note = 2'-methoxy nucleoside; note (original language) = 2'-甲氧基核苷
  modified_base 15: mod_base = OTHER; note = 2'-methoxy nucleoside; note (original language) = 2'-甲氧基核苷
  modified_base 17..21: mod_base = OTHER; note = 2'-methoxy nucleoside; note (original language) = 2'-甲氧基核苷
  modified_base 2: mod_base = OTHER; note = 2'-fluoro nucleoside; note (original language) = 2'-氟核苷
  modified_base 6: mod_base = OTHER; note = 2'-fluoro nucleoside; note (original language) = 2'-氟核苷
  modified_base 9: mod_base = OTHER; note = 2'-fluoro nucleoside; note (original language) = 2'-氟核苷
  modified_base 14: mod_base = OTHER; note = 2'-fluoro nucleoside; note (original language) = 2'-氟核苷
  modified_base 16: mod_base = OTHER; note = 2'-fluoro nucleoside; note (original language) = 2'-氟核苷
  modified_base 1..3: mod_base = OTHER; note = phosphorothioate bond; note (original language) = 硫代磷酸酯键
  modified_base 19..21: mod_base = OTHER; note = phosphorothioate bond; note (original language) = 硫代磷酸酯键
  modified_base 1: mod_base = OTHER; note = 2'-methoxy-5'-vinyl phosphonate nucleoside; note (original language) = 2'-甲氧基-5'-乙烯基膦酸核苷
  source 1..21: mol_type = other RNA
ttcattagaagaaaaggtcgg

SEQ ID NO: 860 - RNA, 21 nt, synthetic construct
  modified_base 1: mod_base = OTHER; note = 2'-methoxy nucleoside; note (original language) = 2'-甲氧基核苷
  modified_base 3..5: mod_base = OTHER; note = 2'-methoxy nucleoside; note (original language) = 2'-甲氧基核苷
  modified_base 7..8: mod_base = OTHER; note = 2'-methoxy nucleoside; note (original language) = 2'-甲氧基核苷
  modified_base 10..13: mod_base = OTHER; note = 2'-methoxy nucleoside; note (original language) = 2'-甲氧基核苷
  modified_base 15: mod_base = OTHER; note = 2'-methoxy nucleoside; note (original language) = 2'-甲氧基核苷
  modified_base 17..21: mod_base = OTHER; note = 2'-methoxy nucleoside; note (original language) = 2'-甲氧基核苷
  modified_base 2: mod_base = OTHER; note = 2'-fluoro nucleoside; note (original language) = 2'-氟核苷
  modified_base 6: mod_base = OTHER; note = 2'-fluoro nucleoside; note (original language) = 2'-氟核苷
  modified_base 9: mod_base = OTHER; note = 2'-fluoro nucleoside; note (original language) = 2'-氟核苷
  modified_base 14: mod_base = OTHER; note = 2'-fluoro nucleoside; note (original language) = 2'-氟核苷
  modified_base 16: mod_base = OTHER; note = 2'-fluoro nucleoside; note (original language) = 2'-氟核苷
  modified_base 1..3: mod_base = OTHER; note = phosphorothioate bond; note (original language) = 硫代磷酸酯键
  modified_base 19..21: mod_base = OTHER; note = phosphorothioate bond; note (original language) = 硫代磷酸酯键
  modified_base 1: mod_base = OTHER; note = 2'-methoxy-5'-vinyl phosphonate nucleoside; note (original language) = 2'-甲氧基-5'-乙烯基膦酸核苷
  source 1..21: mol_type = other RNA
tatttttgttctcaacttgaa

SEQ ID NO: 861 - RNA, 21 nt, synthetic construct
  modified_base 1: mod_base = OTHER; note = 2'-methoxy nucleoside; note (original language) = 2'-甲氧基核苷
  modified_base 3..5: mod_base = OTHER; note = 2'-methoxy nucleoside; note (original language) = 2'-甲氧基核苷
  modified_base 7..8: mod_base = OTHER; note = 2'-methoxy nucleoside; note (original language) = 2'-甲氧基核苷
  modified_base 10..13: mod_base = OTHER; note = 2'-methoxy nucleoside; note (original language) = 2'-甲氧基核苷
  modified_base 15: mod_base = OTHER; note = 2'-methoxy nucleoside; note (original language) = 2'-甲氧基核苷
  modified_base 17..21: mod_base = OTHER; note = 2'-methoxy nucleoside; note (original language) = 2'-甲氧基核苷
  modified_base 2: mod_base = OTHER; note = 2'-fluoro nucleoside; note (original language) = 2'-氟核苷
  modified_base 6: mod_base = OTHER; note = 2'-fluoro nucleoside; note (original language) = 2'-氟核苷
  modified_base 9: mod_base = OTHER; note = 2'-fluoro nucleoside; note (original language) = 2'-氟核苷
  modified_base 14: mod_base = OTHER; note = 2'-fluoro nucleoside; note (original language) = 2'-氟核苷
  modified_base 16: mod_base = OTHER; note = 2'-fluoro nucleoside; note (original language) = 2'-氟核苷
  modified_base 1..3: mod_base = OTHER; note = phosphorothioate bond; note (original language) = 硫代磷酸酯键
  modified_base 19..21: mod_base = OTHER; note = phosphorothioate bond; note (original language) = 硫代磷酸酯键
  modified_base 1: mod_base = OTHER; note = 2'-methoxy-5'-vinyl phosphonate nucleoside; note (original language) = 2'-甲氧基-5'-乙烯基膦酸核苷
  source 1..21: mol_type = other RNA
taaacactggttcttgccccc

SEQ ID NO: 862 - RNA, 21 nt, synthetic construct
  modified_base 1: mod_base = OTHER; note = 2'-methoxy nucleoside; note (original language) = 2'-甲氧基核苷
  modified_base 3..5: mod_base = OTHER; note = 2'-methoxy nucleoside; note (original language) = 2'-甲氧基核苷
  modified_base 7..8: mod_base = OTHER; note = 2'-methoxy nucleoside; note (original language) = 2'-甲氧基核苷
  modified_base 10..13: mod_base = OTHER; note = 2'-methoxy nucleoside; note (original language) = 2'-甲氧基核苷
  modified_base 15: mod_base = OTHER; note = 2'-methoxy nucleoside; note (original language) = 2'-甲氧基核苷
  modified_base 17..21: mod_base = OTHER; note = 2'-methoxy nucleoside; note (original language) = 2'-甲氧基核苷
  modified_base 2: mod_base = OTHER; note = 2'-fluoro nucleoside; note (original language) = 2'-氟核苷
  modified_base 6: mod_base = OTHER; note = 2'-fluoro nucleoside; note (original language) = 2'-氟核苷
  modified_base 9: mod_base = OTHER; note = 2'-fluoro nucleoside; note (original language) = 2'-氟核苷
  modified_base 14: mod_base = OTHER; note = 2'-fluoro nucleoside; note (original language) = 2'-氟核苷
  modified_base 16: mod_base = OTHER; note = 2'-fluoro nucleoside; note (original language) = 2'-氟核苷
  modified_base 1..3: mod_base = OTHER; note = phosphorothioate bond; note (original language) = 硫代磷酸酯键
  modified_base 19..21: mod_base = OTHER; note = phosphorothioate bond; note (original language) = 硫代磷酸酯键
  modified_base 1: mod_base = OTHER; note = 2'-methoxy-5'-vinyl phosphonate nucleoside; note (original language) = 2'-甲氧基-5'-乙烯基膦酸核苷
  source 1..21: mol_type = other RNA
ttcacaaacaagctggtccgt

SEQ ID NO: 863 - RNA, 21 nt, synthetic construct
  modified_base 1: mod_base = OTHER; note = 2'-methoxy nucleoside; note (original language) = 2'-甲氧基核苷
  modified_base 3..5: mod_base = OTHER; note = 2'-methoxy nucleoside; note (original language) = 2'-甲氧基核苷
  modified_base 7..8: mod_base = OTHER; note = 2'-methoxy nucleoside; note (original language) = 2'-甲氧基核苷
  modified_base 10..13: mod_base = OTHER; note = 2'-methoxy nucleoside; note (original language) = 2'-甲氧基核苷
  modified_base 15: mod_base = OTHER; note = 2'-methoxy nucleoside; note (original language) = 2'-甲氧基核苷
  modified_base 17..21: mod_base = OTHER; note = 2'-methoxy nucleoside; note (original language) = 2'-甲氧基核苷
  modified_base 2: mod_base = OTHER; note = 2'-fluoro nucleoside; note (original language) = 2'-氟核苷
  modified_base 6: mod_base = OTHER; note = 2'-fluoro nucleoside; note (original language) = 2'-氟核苷
  modified_base 9: mod_base = OTHER; note = 2'-fluoro nucleoside; note (original language) = 2'-氟核苷
  modified_base 14: mod_base = OTHER; note = 2'-fluoro nucleoside; note (original language) = 2'-氟核苷
  modified_base 16: mod_base = OTHER; note = 2'-fluoro nucleoside; note (original language) = 2'-氟核苷
  modified_base 1..3: mod_base = OTHER; note = phosphorothioate bond; note (original language) = 硫代磷酸酯键
  modified_base 19..21: mod_base = OTHER; note = phosphorothioate bond; note (original language) = 硫代磷酸酯键
  modified_base 1: mod_base = OTHER; note = 2'-methoxy-5'-vinyl phosphonate nucleoside; note (original language) = 2'-甲氧基-5'-乙烯基膦酸核苷
  source 1..21: mol_type = other RNA
tttcacaaacaagctggtggg

SEQ ID NO: 864 - RNA, 23 nt, synthetic construct
  modified_base 1: mod_base = OTHER; note = 2'-methoxy nucleoside; note (original language) = 2'-甲氧基核苷
  modified_base 3..5: mod_base = OTHER; note = 2'-methoxy nucleoside; note (original language) = 2'-甲氧基核苷
  modified_base 7..8: mod_base = OTHER; note = 2'-methoxy nucleoside; note (original language) = 2'-甲氧基核苷
  modified_base 10..13: mod_base = OTHER; note = 2'-methoxy nucleoside; note (original language) = 2'-甲氧基核苷
  modified_base 15: mod_base = OTHER; note = 2'-methoxy nucleoside; note (original language) = 2'-甲氧基核苷
  modified_base 17..23: mod_base = OTHER; note = 2'-methoxy nucleoside; note (original language) = 2'-甲氧基核苷
  modified_base 2: mod_base = OTHER; note = 2'-fluoro nucleoside; note (original language) = 2'-氟核苷
  modified_base 6: mod_base = OTHER; note = 2'-fluoro nucleoside; note (original language) = 2'-氟核苷
  modified_base 9: mod_base = OTHER; note = 2'-fluoro nucleoside; note (original language) = 2'-氟核苷
  modified_base 14: mod_base = OTHER; note = 2'-fluoro nucleoside; note (original language) = 2'-氟核苷
  modified_base 16: mod_base = OTHER; note = 2'-fluoro nucleoside; note (original language) = 2'-氟核苷
  modified_base 1..3: mod_base = OTHER; note = phosphorothioate bond; note (original language) = 硫代磷酸酯键
  modified_base 21..23: mod_base = OTHER; note = phosphorothioate bond; note (original language) = 硫代磷酸酯键
  modified_base 1: mod_base = OTHER; note = 2'-methoxy-5'-vinyl phosphonate nucleoside; note (original language) = 2'-甲氧基-5'-乙烯基膦酸核苷
  modified_base 11: mod_base = i
  source 1..23: mol_type = other RNA
tcttagaccanggagaaacgcct

SEQ ID NO: 865 - RNA, 23 nt, synthetic construct
  modified_base 1: mod_base = OTHER; note = 2'-methoxy nucleoside; note (original language) = 2'-甲氧基核苷
  modified_base 3..5: mod_base = OTHER; note = 2'-methoxy nucleoside; note (original language) = 2'-甲氧基核苷
  modified_base 7..8: mod_base = OTHER; note = 2'-methoxy nucleoside; note (original language) = 2'-甲氧基核苷
  modified_base 10..13: mod_base = OTHER; note = 2'-methoxy nucleoside; note (original language) = 2'-甲氧基核苷
  modified_base 15: mod_base = OTHER; note = 2'-methoxy nucleoside; note (original language) = 2'-甲氧基核苷
  modified_base 17..23: mod_base = OTHER; note = 2'-methoxy nucleoside; note (original language) = 2'-甲氧基核苷
  modified_base 2: mod_base = OTHER; note = 2'-fluoro nucleoside; note (original language) = 2'-氟核苷
  modified_base 6: mod_base = OTHER; note = 2'-fluoro nucleoside; note (original language) = 2'-氟核苷
  modified_base 9: mod_base = OTHER; note = 2'-fluoro nucleoside; note (original language) = 2'-氟核苷
  modified_base 14: mod_base = OTHER; note = 2'-fluoro nucleoside; note (original language) = 2'-氟核苷
  modified_base 16: mod_base = OTHER; note = 2'-fluoro nucleoside; note (original language) = 2'-氟核苷
  modified_base 1..3: mod_base = OTHER; note = phosphorothioate bond; note (original language) = 硫代磷酸酯键
  modified_base 21..23: mod_base = OTHER; note = phosphorothioate bond; note (original language) = 硫代磷酸酯键
  modified_base 1: mod_base = OTHER; note = 2'-methoxy-5'-vinyl phosphonate nucleoside; note (original language) = 2'-甲氧基-5'-乙烯基膦酸核苷
  modified_base 10: mod_base = i
  source 1..23: mol_type = other RNA
tcttagaccnaggagaaacgcct

SEQ ID NO: 866 - RNA, 23 nt, synthetic construct
  modified_base 1: mod_base = OTHER; note = 2'-methoxy nucleoside; note (original language) = 2'-甲氧基核苷
  modified_base 3..5: mod_base = OTHER; note = 2'-methoxy nucleoside; note (original language) = 2'-甲氧基核苷
  modified_base 7..8: mod_base = OTHER; note = 2'-methoxy nucleoside; note (original language) = 2'-甲氧基核苷
  modified_base 10..13: mod_base = OTHER; note = 2'-methoxy nucleoside; note (original language) = 2'-甲氧基核苷
  modified_base 15: mod_base = OTHER; note = 2'-methoxy nucleoside; note (original language) = 2'-甲氧基核苷
  modified_base 17..23: mod_base = OTHER; note = 2'-methoxy nucleoside; note (original language) = 2'-甲氧基核苷
  modified_base 2: mod_base = OTHER; note = 2'-fluoro nucleoside; note (original language) = 2'-氟核苷
  modified_base 6: mod_base = OTHER; note = 2'-fluoro nucleoside; note (original language) = 2'-氟核苷
  modified_base 9: mod_base = OTHER; note = 2'-fluoro nucleoside; note (original language) = 2'-氟核苷
  modified_base 14: mod_base = OTHER; note = 2'-fluoro nucleoside; note (original language) = 2'-氟核苷
  modified_base 16: mod_base = OTHER; note = 2'-fluoro nucleoside; note (original language) = 2'-氟核苷
  modified_base 1..3: mod_base = OTHER; note = phosphorothioate bond; note (original language) = 硫代磷酸酯键
  modified_base 21..23: mod_base = OTHER; note = phosphorothioate bond; note (original language) = 硫代磷酸酯键
  modified_base 1: mod_base = OTHER; note = 2'-methoxy-5'-vinyl phosphonate nucleoside; note (original language) = 2'-甲氧基-5'-乙烯基膦酸核苷
  modified_base 7: mod_base = i
  source 1..23: mol_type = other RNA
tcttagnccaaggagaaacgcct

SEQ ID NO: 867 - RNA, 23 nt, synthetic construct
  modified_base 1: mod_base = OTHER; note = 2'-methoxy nucleoside; note (original language) = 2'-甲氧基核苷
  modified_base 3..5: mod_base = OTHER; note = 2'-methoxy nucleoside; note (original language) = 2'-甲氧基核苷
  modified_base 7..8: mod_base = OTHER; note = 2'-methoxy nucleoside; note (original language) = 2'-甲氧基核苷
  modified_base 10..13: mod_base = OTHER; note = 2'-methoxy nucleoside; note (original language) = 2'-甲氧基核苷
  modified_base 15: mod_base = OTHER; note = 2'-methoxy nucleoside; note (original language) = 2'-甲氧基核苷
  modified_base 17..23: mod_base = OTHER; note = 2'-methoxy nucleoside; note (original language) = 2'-甲氧基核苷
  modified_base 2: mod_base = OTHER; note = 2'-fluoro nucleoside; note (original language) = 2'-氟核苷
  modified_base 6: mod_base = OTHER; note = 2'-fluoro nucleoside; note (original language) = 2'-氟核苷
  modified_base 9: mod_base = OTHER; note = 2'-fluoro nucleoside; note (original language) = 2'-氟核苷
  modified_base 14: mod_base = OTHER; note = 2'-fluoro nucleoside; note (original language) = 2'-氟核苷
  modified_base 16: mod_base = OTHER; note = 2'-fluoro nucleoside; note (original language) = 2'-氟核苷
  modified_base 1..3: mod_base = OTHER; note = phosphorothioate bond; note (original language) = 硫代磷酸酯键
  modified_base 21..23: mod_base = OTHER; note = phosphorothioate bond; note (original language) = 硫代磷酸酯键
  modified_base 1: mod_base = OTHER; note = 2'-methoxy-5'-vinyl phosphonate nucleoside; note (original language) = 2'-甲氧基-5'-乙烯基膦酸核苷
  modified_base 5: mod_base = i
  source 1..23: mol_type = other RNA
tcttngaccaaggagaaacgcct

SEQ ID NO: 868 - RNA, 21 nt, synthetic construct
  source 1..21: mol_type = other RNA
gcacctcgtcatccacaatga

SEQ ID NO: 869 - RNA, 21 nt, synthetic construct
  source 1..21: mol_type = other RNA
gtgctgctgagaagattgaca

SEQ ID NO: 870 - RNA, 21 nt, synthetic construct
  source 1..21: mol_type = other RNA
gagagagagcccacagagtca

SEQ ID NO: 871 - RNA, 21 nt, synthetic construct
  source 1..21: mol_type = other RNA
gcttttcttctaatgagtcga

SEQ ID NO: 872 - RNA, 23 nt, synthetic construct
  source 1..23: mol_type = other RNA
tcattgtggatgacgaggtgcaa

SEQ ID NO: 873 - RNA, 23 nt, synthetic construct
  source 1..23: mol_type = other RNA
tgtcaatcttctcagcagcacca

SEQ ID NO: 874 - RNA, 23 nt, synthetic construct
  source 1..23: mol_type = other RNA
tgactctgtgggctctctctcat

SEQ ID NO: 875 - RNA, 23 nt, synthetic construct
  source 1..23: mol_type = other RNA
tcgactcattagaagaaaagctg

SEQ ID NO: 876 - RNA, 21 nt, synthetic construct
  modified_base 1..8: mod_base = OTHER; note = 2'-methoxy nucleoside; note (original language) = 2'-甲氧基核苷
  modified_base 12..21: mod_base = OTHER; note = 2'-methoxy nucleoside; note (original language) = 2'-甲氧基核苷
  modified_base 9..11: mod_base = OTHER; note = 2'-fluoro nucleoside; note (original language) = 2'-氟核苷
  modified_base 1..3: mod_base = OTHER; note = phosphorothioate bond; note (original language) = 硫代磷酸酯键
  source 1..21: mol_type = other RNA
ccacctcgtcatccacaatga

SEQ ID NO: 877 - RNA, 21 nt, synthetic construct
  modified_base 1..8: mod_base = OTHER; note = 2'-methoxy nucleoside; note (original language) = 2'-甲氧基核苷
  modified_base 12..21: mod_base = OTHER; note = 2'-methoxy nucleoside; note (original language) = 2'-甲氧基核苷
  modified_base 9..11: mod_base = OTHER; note = 2'-fluoro nucleoside; note (original language) = 2'-氟核苷
  modified_base 1..3: mod_base = OTHER; note = phosphorothioate bond; note (original language) = 硫代磷酸酯键
  source 1..21: mol_type = other RNA
gcacctcgtcatccacaatga

SEQ ID NO: 878 - RNA, 21 nt, synthetic construct
  modified_base 1..8: mod_base = OTHER; note = 2'-methoxy nucleoside; note (original language) = 2'-甲氧基核苷
  modified_base 12..21: mod_base = OTHER; note = 2'-methoxy nucleoside; note (original language) = 2'-甲氧基核苷
  modified_base 9..11: mod_base = OTHER; note = 2'-fluoro nucleoside; note (original language) = 2'-氟核苷
  modified_base 1..3: mod_base = OTHER; note = phosphorothioate bond; note (original language) = 硫代磷酸酯键
  source 1..21: mol_type = other RNA
ggcatgcacagtgagctatga

SEQ ID NO: 879 - RNA, 21 nt, synthetic construct
  modified_base 1..8: mod_base = OTHER; note = 2'-methoxy nucleoside; note (original language) = 2'-甲氧基核苷
  modified_base 12..21: mod_base = OTHER; note = 2'-methoxy nucleoside; note (original language) = 2'-甲氧基核苷
  modified_base 9..11: mod_base = OTHER; note = 2'-fluoro nucleoside; note (original language) = 2'-氟核苷
  modified_base 1..3: mod_base = OTHER; note = phosphorothioate bond; note (original language) = 硫代磷酸酯键
  source 1..21: mol_type = other RNA
ttgctgctgagaagattgaca

SEQ ID NO: 880 - RNA, 21 nt, synthetic construct
  modified_base 1..8: mod_base = OTHER; note = 2'-methoxy nucleoside; note (original language) = 2'-甲氧基核苷
  modified_base 12..21: mod_base = OTHER; note = 2'-methoxy nucleoside; note (original language) = 2'-甲氧基核苷
  modified_base 9..11: mod_base = OTHER; note = 2'-fluoro nucleoside; note (original language) = 2'-氟核苷
  modified_base 1..3: mod_base = OTHER; note = phosphorothioate bond; note (original language) = 硫代磷酸酯键
  source 1..21: mol_type = other RNA
gtgctgctgagaagattgaca

SEQ ID NO: 881 - RNA, 21 nt, synthetic construct
  modified_base 1..8: mod_base = OTHER; note = 2'-methoxy nucleoside; note (original language) = 2'-甲氧基核苷
  modified_base 12..21: mod_base = OTHER; note = 2'-methoxy nucleoside; note (original language) = 2'-甲氧基核苷
  modified_base 9..11: mod_base = OTHER; note = 2'-fluoro nucleoside; note (original language) = 2'-氟核苷
  modified_base 1..3: mod_base = OTHER; note = phosphorothioate bond; note (original language) = 硫代磷酸酯键
  source 1..21: mol_type = other RNA
gagaagattgacaggttcata

SEQ ID NO: 882 - RNA, 21 nt, synthetic construct
  modified_base 1..8: mod_base = OTHER; note = 2'-methoxy nucleoside; note (original language) = 2'-甲氧基核苷
  modified_base 12..21: mod_base = OTHER; note = 2'-methoxy nucleoside; note (original language) = 2'-甲氧基核苷
  modified_base 9..11: mod_base = OTHER; note = 2'-fluoro nucleoside; note (original language) = 2'-氟核苷
  modified_base 1..3: mod_base = OTHER; note = phosphorothioate bond; note (original language) = 硫代磷酸酯键
  source 1..21: mol_type = other RNA
gctgaacagcgttttttttga

SEQ ID NO: 883 - RNA, 21 nt, synthetic construct
  modified_base 1..8: mod_base = OTHER; note = 2'-methoxy nucleoside; note (original language) = 2'-甲氧基核苷
  modified_base 12..21: mod_base = OTHER; note = 2'-methoxy nucleoside; note (original language) = 2'-甲氧基核苷
  modified_base 9..11: mod_base = OTHER; note = 2'-fluoro nucleoside; note (original language) = 2'-氟核苷
  modified_base 1..3: mod_base = OTHER; note = phosphorothioate bond; note (original language) = 硫代磷酸酯键
  source 1..21: mol_type = other RNA
gagagagagcccacagagtct

SEQ ID NO: 884 - RNA, 21 nt, synthetic construct
  modified_base 1..8: mod_base = OTHER; note = 2'-methoxy nucleoside; note (original language) = 2'-甲氧基核苷
  modified_base 12..21: mod_base = OTHER; note = 2'-methoxy nucleoside; note (original language) = 2'-甲氧基核苷
  modified_base 9..11: mod_base = OTHER; note = 2'-fluoro nucleoside; note (original language) = 2'-氟核苷
  modified_base 1..3: mod_base = OTHER; note = phosphorothioate bond; note (original language) = 硫代磷酸酯键
  source 1..21: mol_type = other RNA
gagagagagcccacagagtca

SEQ ID NO: 885 - RNA, 21 nt, synthetic construct
  modified_base 1..8: mod_base = OTHER; note = 2'-methoxy nucleoside; note (original language) = 2'-甲氧基核苷
  modified_base 12..21: mod_base = OTHER; note = 2'-methoxy nucleoside; note (original language) = 2'-甲氧基核苷
  modified_base 9..11: mod_base = OTHER; note = 2'-fluoro nucleoside; note (original language) = 2'-氟核苷
  modified_base 1..3: mod_base = OTHER; note = phosphorothioate bond; note (original language) = 硫代磷酸酯键
  source 1..21: mol_type = other RNA
ccttttcttctaatgagtcga

SEQ ID NO: 886 - RNA, 21 nt, synthetic construct
  modified_base 1..8: mod_base = OTHER; note = 2'-methoxy nucleoside; note (original language) = 2'-甲氧基核苷
  modified_base 12..21: mod_base = OTHER; note = 2'-methoxy nucleoside; note (original language) = 2'-甲氧基核苷
  modified_base 9..11: mod_base = OTHER; note = 2'-fluoro nucleoside; note (original language) = 2'-氟核苷
  modified_base 1..3: mod_base = OTHER; note = phosphorothioate bond; note (original language) = 硫代磷酸酯键
  source 1..21: mol_type = other RNA
gcttttcttctaatgagtcga

SEQ ID NO: 887 - RNA, 23 nt, synthetic construct
  modified_base 1: mod_base = OTHER; note = 2'-methoxy nucleoside; note (original language) = 2'-甲氧基核苷
  modified_base 3..5: mod_base = OTHER; note = 2'-methoxy nucleoside; note (original language) = 2'-甲氧基核苷
  modified_base 7..8: mod_base = OTHER; note = 2'-methoxy nucleoside; note (original language) = 2'-甲氧基核苷
  modified_base 10..13: mod_base = OTHER; note = 2'-methoxy nucleoside; note (original language) = 2'-甲氧基核苷
  modified_base 15: mod_base = OTHER; note = 2'-methoxy nucleoside; note (original language) = 2'-甲氧基核苷
  modified_base 17..23: mod_base = OTHER; note = 2'-methoxy nucleoside; note (original language) = 2'-甲氧基核苷
  modified_base 2: mod_base = OTHER; note = 2'-fluoro nucleoside; note (original language) = 2'-氟核苷
  modified_base 6: mod_base = OTHER; note = 2'-fluoro nucleoside; note (original language) = 2'-氟核苷
  modified_base 9: mod_base = OTHER; note = 2'-fluoro nucleoside; note (original language) = 2'-氟核苷
  modified_base 14: mod_base = OTHER; note = 2'-fluoro nucleoside; note (original language) = 2'-氟核苷
  modified_base 16: mod_base = OTHER; note = 2'-fluoro nucleoside; note (original language) = 2'-氟核苷
  modified_base 1..3: mod_base = OTHER; note = phosphorothioate bond; note (original language) = 硫代磷酸酯键
  modified_base 21..23: mod_base = OTHER; note = phosphorothioate bond; note (original language) = 硫代磷酸酯键
  source 1..23: mol_type = other RNA
tcattgtggatgacgaggtgcaa

SEQ ID NO: 888 - RNA, 23 nt, synthetic construct
  modified_base 1: mod_base = OTHER; note = 2'-methoxy nucleoside; note (original language) = 2'-甲氧基核苷
  modified_base 3..5: mod_base = OTHER; note = 2'-methoxy nucleoside; note (original language) = 2'-甲氧基核苷
  modified_base 7..8: mod_base = OTHER; note = 2'-methoxy nucleoside; note (original language) = 2'-甲氧基核苷
  modified_base 10..13: mod_base = OTHER; note = 2'-methoxy nucleoside; note (original language) = 2'-甲氧基核苷
  modified_base 15: mod_base = OTHER; note = 2'-methoxy nucleoside; note (original language) = 2'-甲氧基核苷
  modified_base 17..23: mod_base = OTHER; note = 2'-methoxy nucleoside; note (original language) = 2'-甲氧基核苷
  modified_base 2: mod_base = OTHER; note = 2'-fluoro nucleoside; note (original language) = 2'-氟核苷
  modified_base 6: mod_base = OTHER; note = 2'-fluoro nucleoside; note (original language) = 2'-氟核苷
  modified_base 9: mod_base = OTHER; note = 2'-fluoro nucleoside; note (original language) = 2'-氟核苷
  modified_base 14: mod_base = OTHER; note = 2'-fluoro nucleoside; note (original language) = 2'-氟核苷
  modified_base 16: mod_base = OTHER; note = 2'-fluoro nucleoside; note (original language) = 2'-氟核苷
  modified_base 1..3: mod_base = OTHER; note = phosphorothioate bond; note (original language) = 硫代磷酸酯键
  modified_base 21..23: mod_base = OTHER; note = phosphorothioate bond; note (original language) = 硫代磷酸酯键
  modified_base 1: mod_base = OTHER; note = 2'-methoxy-5'-vinyl phosphonate nucleoside; note (original language) = 2'-甲氧基-5'-乙烯基膦酸核苷
  source 1..23: mol_type = other RNA
tcattgtggatgacgaggtgcaa

SEQ ID NO: 889 - RNA, 23 nt, synthetic construct
  modified_base 1: mod_base = OTHER; note = 2'-methoxy nucleoside; note (original language) = 2'-甲氧基核苷
  modified_base 3..5: mod_base = OTHER; note = 2'-methoxy nucleoside; note (original language) = 2'-甲氧基核苷
  modified_base 7..8: mod_base = OTHER; note = 2'-methoxy nucleoside; note (original language) = 2'-甲氧基核苷
  modified_base 10..13: mod_base = OTHER; note = 2'-methoxy nucleoside; note (original language) = 2'-甲氧基核苷
  modified_base 15: mod_base = OTHER; note = 2'-methoxy nucleoside; note (original language) = 2'-甲氧基核苷
  modified_base 17..23: mod_base = OTHER; note = 2'-methoxy nucleoside; note (original language) = 2'-甲氧基核苷
  modified_base 2: mod_base = OTHER; note = 2'-fluoro nucleoside; note (original language) = 2'-氟核苷
  modified_base 6: mod_base = OTHER; note = 2'-fluoro nucleoside; note (original language) = 2'-氟核苷
  modified_base 9: mod_base = OTHER; note = 2'-fluoro nucleoside; note (original language) = 2'-氟核苷
  modified_base 14: mod_base = OTHER; note = 2'-fluoro nucleoside; note (original language) = 2'-氟核苷
  modified_base 16: mod_base = OTHER; note = 2'-fluoro nucleoside; note (original language) = 2'-氟核苷
  modified_base 1..3: mod_base = OTHER; note = phosphorothioate bond; note (original language) = 硫代磷酸酯键
  modified_base 21..23: mod_base = OTHER; note = phosphorothioate bond; note (original language) = 硫代磷酸酯键
  modified_base 1: mod_base = OTHER; note = 2'-methoxy-5'-vinyl phosphonate nucleoside; note (original language) = 2'-甲氧基-5'-乙烯基膦酸核苷
  source 1..23: mol_type = other RNA
tcatagctcactgtgcatgccat

SEQ ID NO: 890 - RNA, 23 nt, synthetic construct
  modified_base 1: mod_base = OTHER; note = 2'-methoxy nucleoside; note (original language) = 2'-甲氧基核苷
  modified_base 3..5: mod_base = OTHER; note = 2'-methoxy nucleoside; note (original language) = 2'-甲氧基核苷
  modified_base 7..8: mod_base = OTHER; note = 2'-methoxy nucleoside; note (original language) = 2'-甲氧基核苷
  modified_base 10..13: mod_base = OTHER; note = 2'-methoxy nucleoside; note (original language) = 2'-甲氧基核苷
  modified_base 15: mod_base = OTHER; note = 2'-methoxy nucleoside; note (original language) = 2'-甲氧基核苷
  modified_base 17..23: mod_base = OTHER; note = 2'-methoxy nucleoside; note (original language) = 2'-甲氧基核苷
  modified_base 2: mod_base = OTHER; note = 2'-fluoro nucleoside; note (original language) = 2'-氟核苷
  modified_base 6: mod_base = OTHER; note = 2'-fluoro nucleoside; note (original language) = 2'-氟核苷
  modified_base 9: mod_base = OTHER; note = 2'-fluoro nucleoside; note (original language) = 2'-氟核苷
  modified_base 14: mod_base = OTHER; note = 2'-fluoro nucleoside; note (original language) = 2'-氟核苷
  modified_base 16: mod_base = OTHER; note = 2'-fluoro nucleoside; note (original language) = 2'-氟核苷
  modified_base 1..3: mod_base = OTHER; note = phosphorothioate bond; note (original language) = 硫代磷酸酯键
  modified_base 21..23: mod_base = OTHER; note = phosphorothioate bond; note (original language) = 硫代磷酸酯键
  source 1..23: mol_type = other RNA
tgtcaatcttctcagcagcaaca

SEQ ID NO: 891 - RNA, 23 nt, synthetic construct
  modified_base 1: mod_base = OTHER; note = 2'-methoxy nucleoside; note (original language) = 2'-甲氧基核苷
  modified_base 3..5: mod_base = OTHER; note = 2'-methoxy nucleoside; note (original language) = 2'-甲氧基核苷
  modified_base 7..8: mod_base = OTHER; note = 2'-methoxy nucleoside; note (original language) = 2'-甲氧基核苷
  modified_base 10..13: mod_base = OTHER; note = 2'-methoxy nucleoside; note (original language) = 2'-甲氧基核苷
  modified_base 15: mod_base = OTHER; note = 2'-methoxy nucleoside; note (original language) = 2'-甲氧基核苷
  modified_base 17..23: mod_base = OTHER; note = 2'-methoxy nucleoside; note (original language) = 2'-甲氧基核苷
  modified_base 2: mod_base = OTHER; note = 2'-fluoro nucleoside; note (original language) = 2'-氟核苷
  modified_base 6: mod_base = OTHER; note = 2'-fluoro nucleoside; note (original language) = 2'-氟核苷
  modified_base 9: mod_base = OTHER; note = 2'-fluoro nucleoside; note (original language) = 2'-氟核苷
  modified_base 14: mod_base = OTHER; note = 2'-fluoro nucleoside; note (original language) = 2'-氟核苷
  modified_base 16: mod_base = OTHER; note = 2'-fluoro nucleoside; note (original language) = 2'-氟核苷
  modified_base 1..3: mod_base = OTHER; note = phosphorothioate bond; note (original language) = 硫代磷酸酯键
  modified_base 21..23: mod_base = OTHER; note = phosphorothioate bond; note (original language) = 硫代磷酸酯键
  source 1..23: mol_type = other RNA
tgtcaatcttctcagcagcacca

SEQ ID NO: 892 - RNA, 23 nt, synthetic construct
  modified_base 1: mod_base = OTHER; note = 2'-methoxy nucleoside; note (original language) = 2'-甲氧基核苷
  modified_base 3..5: mod_base = OTHER; note = 2'-methoxy nucleoside; note (original language) = 2'-甲氧基核苷
  modified_base 7..8: mod_base = OTHER; note = 2'-methoxy nucleoside; note (original language) = 2'-甲氧基核苷
  modified_base 10..13: mod_base = OTHER; note = 2'-methoxy nucleoside; note (original language) = 2'-甲氧基核苷
  modified_base 15: mod_base = OTHER; note = 2'-methoxy nucleoside; note (original language) = 2'-甲氧基核苷
  modified_base 17..23: mod_base = OTHER; note = 2'-methoxy nucleoside; note (original language) = 2'-甲氧基核苷
  modified_base 2: mod_base = OTHER; note = 2'-fluoro nucleoside; note (original language) = 2'-氟核苷
  modified_base 6: mod_base = OTHER; note = 2'-fluoro nucleoside; note (original language) = 2'-氟核苷
  modified_base 9: mod_base = OTHER; note = 2'-fluoro nucleoside; note (original language) = 2'-氟核苷
  modified_base 14: mod_base = OTHER; note = 2'-fluoro nucleoside; note (original language) = 2'-氟核苷
  modified_base 16: mod_base = OTHER; note = 2'-fluoro nucleoside; note (original language) = 2'-氟核苷
  modified_base 1..3: mod_base = OTHER; note = phosphorothioate bond; note (original language) = 硫代磷酸酯键
  modified_base 21..23: mod_base = OTHER; note = phosphorothioate bond; note (original language) = 硫代磷酸酯键
  modified_base 1: mod_base = OTHER; note = 2'-methoxy-5'-vinyl phosphonate nucleoside; note (original language) = 2'-甲氧基-5'-乙烯基膦酸核苷
  source 1..23: mol_type = other RNA
tgtcaatcttctcagcagcacca

SEQ ID NO: 893 - RNA, 23 nt, synthetic construct
  modified_base 1: mod_base = OTHER; note = 2'-methoxy nucleoside; note (original language) = 2'-甲氧基核苷
  modified_base 3..5: mod_base = OTHER; note = 2'-methoxy nucleoside; note (original language) = 2'-甲氧基核苷
  modified_base 7..8: mod_base = OTHER; note = 2'-methoxy nucleoside; note (original language) = 2'-甲氧基核苷
  modified_base 10..13: mod_base = OTHER; note = 2'-methoxy nucleoside; note (original language) = 2'-甲氧基核苷
  modified_base 15: mod_base = OTHER; note = 2'-methoxy nucleoside; note (original language) = 2'-甲氧基核苷
  modified_base 17..23: mod_base = OTHER; note = 2'-methoxy nucleoside; note (original language) = 2'-甲氧基核苷
  modified_base 2: mod_base = OTHER; note = 2'-fluoro nucleoside; note (original language) = 2'-氟核苷
  modified_base 6: mod_base = OTHER; note = 2'-fluoro nucleoside; note (original language) = 2'-氟核苷
  modified_base 9: mod_base = OTHER; note = 2'-fluoro nucleoside; note (original language) = 2'-氟核苷
  modified_base 14: mod_base = OTHER; note = 2'-fluoro nucleoside; note (original language) = 2'-氟核苷
  modified_base 16: mod_base = OTHER; note = 2'-fluoro nucleoside; note (original language) = 2'-氟核苷
  modified_base 1..3: mod_base = OTHER; note = phosphorothioate bond; note (original language) = 硫代磷酸酯键
  modified_base 21..23: mod_base = OTHER; note = phosphorothioate bond; note (original language) = 硫代磷酸酯键
  modified_base 1: mod_base = OTHER; note = 2'-methoxy-5'-vinyl phosphonate nucleoside; note (original language) = 2'-甲氧基-5'-乙烯基膦酸核苷
  source 1..23: mol_type = other RNA
tatgaacctgtcaatcttctcag

SEQ ID NO: 894 - RNA, 23 nt, synthetic construct
  modified_base 1: mod_base = OTHER; note = 2'-methoxy nucleoside; note (original language) = 2'-甲氧基核苷
  modified_base 3..5: mod_base = OTHER; note = 2'-methoxy nucleoside; note (original language) = 2'-甲氧基核苷
  modified_base 7..8: mod_base = OTHER; note = 2'-methoxy nucleoside; note (original language) = 2'-甲氧基核苷
  modified_base 10..13: mod_base = OTHER; note = 2'-methoxy nucleoside; note (original language) = 2'-甲氧基核苷
  modified_base 15: mod_base = OTHER; note = 2'-methoxy nucleoside; note (original language) = 2'-甲氧基核苷
  modified_base 17..23: mod_base = OTHER; note = 2'-methoxy nucleoside; note (original language) = 2'-甲氧基核苷
  modified_base 2: mod_base = OTHER; note = 2'-fluoro nucleoside; note (original language) = 2'-氟核苷
  modified_base 6: mod_base = OTHER; note = 2'-fluoro nucleoside; note (original language) = 2'-氟核苷
  modified_base 9: mod_base = OTHER; note = 2'-fluoro nucleoside; note (original language) = 2'-氟核苷
  modified_base 14: mod_base = OTHER; note = 2'-fluoro nucleoside; note (original language) = 2'-氟核苷
  modified_base 16: mod_base = OTHER; note = 2'-fluoro nucleoside; note (original language) = 2'-氟核苷
  modified_base 1..3: mod_base = OTHER; note = phosphorothioate bond; note (original language) = 硫代磷酸酯键
  modified_base 21..23: mod_base = OTHER; note = phosphorothioate bond; note (original language) = 硫代磷酸酯键
  modified_base 1: mod_base = OTHER; note = 2'-methoxy-5'-vinyl phosphonate nucleoside; note (original language) = 2'-甲氧基-5'-乙烯基膦酸核苷
  source 1..23: mol_type = other RNA
tcaaaaaaaatgctgttcagcac

SEQ ID NO: 895 - RNA, 23 nt, synthetic construct
  modified_base 1: mod_base = OTHER; note = 2'-methoxy nucleoside; note (original language) = 2'-甲氧基核苷
  modified_base 3..5: mod_base = OTHER; note = 2'-methoxy nucleoside; note (original language) = 2'-甲氧基核苷
  modified_base 7..8: mod_base = OTHER; note = 2'-methoxy nucleoside; note (original language) = 2'-甲氧基核苷
  modified_base 10..13: mod_base = OTHER; note = 2'-methoxy nucleoside; note (original language) = 2'-甲氧基核苷
  modified_base 15: mod_base = OTHER; note = 2'-methoxy nucleoside; note (original language) = 2'-甲氧基核苷
  modified_base 17..23: mod_base = OTHER; note = 2'-methoxy nucleoside; note (original language) = 2'-甲氧基核苷
  modified_base 2: mod_base = OTHER; note = 2'-fluoro nucleoside; note (original language) = 2'-氟核苷
  modified_base 6: mod_base = OTHER; note = 2'-fluoro nucleoside; note (original language) = 2'-氟核苷
  modified_base 9: mod_base = OTHER; note = 2'-fluoro nucleoside; note (original language) = 2'-氟核苷
  modified_base 14: mod_base = OTHER; note = 2'-fluoro nucleoside; note (original language) = 2'-氟核苷
  modified_base 16: mod_base = OTHER; note = 2'-fluoro nucleoside; note (original language) = 2'-氟核苷
  modified_base 1..3: mod_base = OTHER; note = phosphorothioate bond; note (original language) = 硫代磷酸酯键
  modified_base 21..23: mod_base = OTHER; note = phosphorothioate bond; note (original language) = 硫代磷酸酯键
  source 1..23: mol_type = other RNA
tgactctgtgggctctctctcat

SEQ ID NO: 896 - RNA, 23 nt, synthetic construct
  modified_base 1: mod_base = OTHER; note = 2'-methoxy nucleoside; note (original language) = 2'-甲氧基核苷
  modified_base 3..5: mod_base = OTHER; note = 2'-methoxy nucleoside; note (original language) = 2'-甲氧基核苷
  modified_base 7..8: mod_base = OTHER; note = 2'-methoxy nucleoside; note (original language) = 2'-甲氧基核苷
  modified_base 10..13: mod_base = OTHER; note = 2'-methoxy nucleoside; note (original language) = 2'-甲氧基核苷
  modified_base 15: mod_base = OTHER; note = 2'-methoxy nucleoside; note (original language) = 2'-甲氧基核苷
  modified_base 17..23: mod_base = OTHER; note = 2'-methoxy nucleoside; note (original language) = 2'-甲氧基核苷
  modified_base 2: mod_base = OTHER; note = 2'-fluoro nucleoside; note (original language) = 2'-氟核苷
  modified_base 6: mod_base = OTHER; note = 2'-fluoro nucleoside; note (original language) = 2'-氟核苷
  modified_base 9: mod_base = OTHER; note = 2'-fluoro nucleoside; note (original language) = 2'-氟核苷
  modified_base 14: mod_base = OTHER; note = 2'-fluoro nucleoside; note (original language) = 2'-氟核苷
  modified_base 16: mod_base = OTHER; note = 2'-fluoro nucleoside; note (original language) = 2'-氟核苷
  modified_base 1..3: mod_base = OTHER; note = phosphorothioate bond; note (original language) = 硫代磷酸酯键
  modified_base 21..23: mod_base = OTHER; note = phosphorothioate bond; note (original language) = 硫代磷酸酯键
  modified_base 1: mod_base = OTHER; note = 2'-methoxy-5'-vinyl phosphonate nucleoside; note (original language) = 2'-甲氧基-5'-乙烯基膦酸核苷
  source 1..23: mol_type = other RNA
tgactctgtgggctctctctcat

SEQ ID NO: 897 - RNA, 23 nt, synthetic construct
  modified_base 1: mod_base = OTHER; note = 2'-methoxy nucleoside; note (original language) = 2'-甲氧基核苷
  modified_base 3..5: mod_base = OTHER; note = 2'-methoxy nucleoside; note (original language) = 2'-甲氧基核苷
  modified_base 7..8: mod_base = OTHER; note = 2'-methoxy nucleoside; note (original language) = 2'-甲氧基核苷
  modified_base 10..13: mod_base = OTHER; note = 2'-methoxy nucleoside; note (original language) = 2'-甲氧基核苷
  modified_base 15: mod_base = OTHER; note = 2'-methoxy nucleoside; note (original language) = 2'-甲氧基核苷
  modified_base 17..23: mod_base = OTHER; note = 2'-methoxy nucleoside; note (original language) = 2'-甲氧基核苷
  modified_base 2: mod_base = OTHER; note = 2'-fluoro nucleoside; note (original language) = 2'-氟核苷
  modified_base 6: mod_base = OTHER; note = 2'-fluoro nucleoside; note (original language) = 2'-氟核苷
  modified_base 9: mod_base = OTHER; note = 2'-fluoro nucleoside; note (original language) = 2'-氟核苷
  modified_base 14: mod_base = OTHER; note = 2'-fluoro nucleoside; note (original language) = 2'-氟核苷
  modified_base 16: mod_base = OTHER; note = 2'-fluoro nucleoside; note (original language) = 2'-氟核苷
  modified_base 1..3: mod_base = OTHER; note = phosphorothioate bond; note (original language) = 硫代磷酸酯键
  modified_base 21..23: mod_base = OTHER; note = phosphorothioate bond; note (original language) = 硫代磷酸酯键
  source 1..23: mol_type = other RNA
tcgactcattagaagaaaagctg

SEQ ID NO: 898 - DNA, 23 bp, synthetic construct
  modified_base 1: mod_base = OTHER; note = 2'-methoxy nucleoside; note (original language) = 2'-甲氧基核苷
  modified_base 3..4: mod_base = OTHER; note = 2'-methoxy nucleoside; note (original language) = 2'-甲氧基核苷
  modified_base 6: mod_base = OTHER; note = 2'-methoxy nucleoside; note (original language) = 2'-甲氧基核苷
  modified_base 8..11: mod_base = OTHER; note = 2'-methoxy nucleoside; note (original language) = 2'-甲氧基核苷
  modified_base 13: mod_base = OTHER; note = 2'-methoxy nucleoside; note (original language) = 2'-甲氧基核苷
  modified_base 15..23: mod_base = OTHER; note = 2'-methoxy nucleoside; note (original language) = 2'-甲氧基核苷
  modified_base 14: mod_base = OTHER; note = 2'-fluoro nucleoside; note (original language) = 2'-氟核苷
  modified_base 1..3: mod_base = OTHER; note = phosphorothioate bond; note (original language) = 硫代磷酸酯键
  modified_base 21..23: mod_base = OTHER; note = phosphorothioate bond; note (original language) = 硫代磷酸酯键
  modified_base 1: mod_base = OTHER; note = 2'-methoxy-5'-vinyl phosphonate nucleoside; note (original language) = 2'-甲氧基-5'-乙烯基膦酸核苷
  misc_feature 1: note = RNA fragment
  misc_feature 2: note = DNA fragment
  misc_feature 3..4: note = RNA fragment
  misc_feature 5: note = DNA fragment
  misc_feature 6: note = RNA fragment
  misc_feature 7: note = DNA fragment
  misc_feature 8..11: note = RNA fragment
  misc_feature 12: note = DNA fragment
  misc_feature 13..23: note = RNA fragment
  source 1..23: mol_type = other DNA
tcgactcattagaagaaaagctg

SEQ ID NO: 899 - DNA, 23 bp, synthetic construct
  modified_base 1: mod_base = OTHER; note = 2'-methoxy nucleoside; note (original language) = 2'-甲氧基核苷
  modified_base 3..4: mod_base = OTHER; note = 2'-methoxy nucleoside; note (original language) = 2'-甲氧基核苷
  modified_base 6: mod_base = OTHER; note = 2'-methoxy nucleoside; note (original language) = 2'-甲氧基核苷
  modified_base 8..11: mod_base = OTHER; note = 2'-methoxy nucleoside; note (original language) = 2'-甲氧基核苷
  modified_base 13: mod_base = OTHER; note = 2'-methoxy nucleoside; note (original language) = 2'-甲氧基核苷
  modified_base 15..23: mod_base = OTHER; note = 2'-methoxy nucleoside; note (original language) = 2'-甲氧基核苷
  modified_base 14: mod_base = OTHER; note = 2'-fluoro nucleoside; note (original language) = 2'-氟核苷
  modified_base 1..3: mod_base = OTHER; note = phosphorothioate bond; note (original language) = 硫代磷酸酯键
  modified_base 21..23: mod_base = OTHER; note = phosphorothioate bond; note (original language) = 硫代磷酸酯键
  modified_base 1: mod_base = OTHER; note = 2'-methoxy-5'-vinyl phosphonate nucleoside; note (original language) = 2'-甲氧基-5'-乙烯基膦酸核苷
  misc_feature 1: note = RNA fragment
  misc_feature 2: note = DNA fragment
  misc_feature 3..4: note = RNA fragment
  misc_feature 5: note = DNA fragment
  misc_feature 6: note = RNA fragment
  misc_feature 7: note = DNA fragment
  misc_feature 8..11: note = RNA fragment
  misc_feature 12: note = DNA fragment
  misc_feature 13..23: note = RNA fragment
  source 1..23: mol_type = other DNA
tgtcaatcttctcagcagcacca

SEQ ID NO: 900 - DNA, 23 bp, synthetic construct
  modified_base 1: mod_base = OTHER; note = 2'-methoxy nucleoside; note (original language) = 2'-甲氧基核苷
  modified_base 3..4: mod_base = OTHER; note = 2'-methoxy nucleoside; note (original language) = 2'-甲氧基核苷
  modified_base 6: mod_base = OTHER; note = 2'-methoxy nucleoside; note (original language) = 2'-甲氧基核苷
  modified_base 8..11: mod_base = OTHER; note = 2'-methoxy nucleoside; note (original language) = 2'-甲氧基核苷
  modified_base 13: mod_base = OTHER; note = 2'-methoxy nucleoside; note (original language) = 2'-甲氧基核苷
  modified_base 15..23: mod_base = OTHER; note = 2'-methoxy nucleoside; note (original language) = 2'-甲氧基核苷
  modified_base 14: mod_base = OTHER; note = 2'-fluoro nucleoside; note (original language) = 2'-氟核苷
  modified_base 1..3: mod_base = OTHER; note = phosphorothioate bond; note (original language) = 硫代磷酸酯键
  modified_base 21..23: mod_base = OTHER; note = phosphorothioate bond; note (original language) = 硫代磷酸酯键
  modified_base 1: mod_base = OTHER; note = 2'-methoxy-5'-vinyl phosphonate nucleoside; note (original language) = 2'-甲氧基-5'-乙烯基膦酸核苷
  misc_feature 1: note = RNA fragment
  misc_feature 2: note = DNA fragment
  misc_feature 3..4: note = RNA fragment
  misc_feature 5: note = DNA fragment
  misc_feature 6: note = RNA fragment
  misc_feature 7: note = DNA fragment
  misc_feature 8..11: note = RNA fragment
  misc_feature 12: note = DNA fragment
  misc_feature 13..23: note = RNA fragment
  source 1..23: mol_type = other DNA
tatgaacctgtcaatcttctcag

SEQ ID NO: 901 - DNA, 23 bp, synthetic construct
  modified_base 1: mod_base = OTHER; note = 2'-methoxy nucleoside; note (original language) = 2'-甲氧基核苷
  modified_base 3..4: mod_base = OTHER; note = 2'-methoxy nucleoside; note (original language) = 2'-甲氧基核苷
  modified_base 6: mod_base = OTHER; note = 2'-methoxy nucleoside; note (original language) = 2'-甲氧基核苷
  modified_base 8..11: mod_base = OTHER; note = 2'-methoxy nucleoside; note (original language) = 2'-甲氧基核苷
  modified_base 13: mod_base = OTHER; note = 2'-methoxy nucleoside; note (original language) = 2'-甲氧基核苷
  modified_base 15..23: mod_base = OTHER; note = 2'-methoxy nucleoside; note (original language) = 2'-甲氧基核苷
  modified_base 14: mod_base = OTHER; note = 2'-fluoro nucleoside; note (original language) = 2'-氟核苷
  modified_base 1..3: mod_base = OTHER; note = phosphorothioate bond; note (original language) = 硫代磷酸酯键
  modified_base 21..23: mod_base = OTHER; note = phosphorothioate bond; note (original language) = 硫代磷酸酯键
  misc_feature 1: note = RNA fragment
  misc_feature 2: note = DNA fragment
  misc_feature 3..4: note = RNA fragment
  misc_feature 5: note = DNA fragment
  misc_feature 6: note = RNA fragment
  misc_feature 7: note = DNA fragment
  misc_feature 8..11: note = RNA fragment
  misc_feature 12: note = DNA fragment
  misc_feature 13..23: note = RNA fragment
  source 1..23: mol_type = other DNA
tcaaaaaaaatgctgttcagcac

SEQ ID NO: 902 - DNA, 23 bp, synthetic construct
  modified_base 1: mod_base = OTHER; note = 2'-methoxy nucleoside; note (original language) = 2'-甲氧基核苷
  modified_base 3..4: mod_base = OTHER; note = 2'-methoxy nucleoside; note (original language) = 2'-甲氧基核苷
  modified_base 6: mod_base = OTHER; note = 2'-methoxy nucleoside; note (original language) = 2'-甲氧基核苷
  modified_base 8..11: mod_base = OTHER; note = 2'-methoxy nucleoside; note (original language) = 2'-甲氧基核苷
  modified_base 13: mod_base = OTHER; note = 2'-methoxy nucleoside; note (original language) = 2'-甲氧基核苷
  modified_base 15..23: mod_base = OTHER; note = 2'-methoxy nucleoside; note (original language) = 2'-甲氧基核苷
  modified_base 14: mod_base = OTHER; note = 2'-fluoro nucleoside; note (original language) = 2'-氟核苷
  modified_base 1..3: mod_base = OTHER; note = phosphorothioate bond; note (original language) = 硫代磷酸酯键
  modified_base 21..23: mod_base = OTHER; note = phosphorothioate bond; note (original language) = 硫代磷酸酯键
  modified_base 1: mod_base = OTHER; note = 2'-methoxy-5'-vinyl phosphonate nucleoside; note (original language) = 2'-甲氧基-5'-乙烯基膦酸核苷
  misc_feature 1: note = RNA fragment
  misc_feature 2: note = DNA fragment
  misc_feature 3..4: note = RNA fragment
  misc_feature 5: note = DNA fragment
  misc_feature 6: note = RNA fragment
  misc_feature 7: note = DNA fragment
  misc_feature 8..11: note = RNA fragment
  misc_feature 12: note = DNA fragment
  misc_feature 13..23: note = RNA fragment
  source 1..23: mol_type = other DNA
tcaaaaaaaatgctgttcagcac

SEQ ID NO: 903 - DNA, 23 bp, synthetic construct
  modified_base 1: mod_base = OTHER; note = 2'-methoxy nucleoside; note (original language) = 2'-甲氧基核苷
  modified_base 3..4: mod_base = OTHER; note = 2'-methoxy nucleoside; note (original language) = 2'-甲氧基核苷
  modified_base 6: mod_base = OTHER; note = 2'-methoxy nucleoside; note (original language) = 2'-甲氧基核苷
  modified_base 8..11: mod_base = OTHER; note = 2'-methoxy nucleoside; note (original language) = 2'-甲氧基核苷
  modified_base 13: mod_base = OTHER; note = 2'-methoxy nucleoside; note (original language) = 2'-甲氧基核苷
  modified_base 15..23: mod_base = OTHER; note = 2'-methoxy nucleoside; note (original language) = 2'-甲氧基核苷
  modified_base 14: mod_base = OTHER; note = 2'-fluoro nucleoside; note (original language) = 2'-氟核苷
  modified_base 1..3: mod_base = OTHER; note = phosphorothioate bond; note (original language) = 硫代磷酸酯键
  modified_base 21..23: mod_base = OTHER; note = phosphorothioate bond; note (original language) = 硫代磷酸酯键
  modified_base 1: mod_base = OTHER; note = 2'-methoxy-5'-vinyl phosphonate nucleoside; note (original language) = 2'-甲氧基-5'-乙烯基膦酸核苷
  misc_feature 1: note = RNA fragment
  misc_feature 2: note = DNA fragment
  misc_feature 3..4: note = RNA fragment
  misc_feature 5: note = DNA fragment
  misc_feature 6: note = RNA fragment
  misc_feature 7: note = DNA fragment
  misc_feature 8..11: note = RNA fragment
  misc_feature 12: note = DNA fragment
  misc_feature 13..23: note = RNA fragment
  source 1..23: mol_type = other DNA
tgactctgtgggctctctctcat

SEQ ID NO: 904 - RNA, 23 nt, synthetic construct
  modified_base 1: mod_base = OTHER; note = 2'-methoxy nucleoside; note (original language) = 2'-甲氧基核苷
  modified_base 3..5: mod_base = OTHER; note = 2'-methoxy nucleoside; note (original language) = 2'-甲氧基核苷
  modified_base 7..8: mod_base = OTHER; note = 2'-methoxy nucleoside; note (original language) = 2'-甲氧基核苷
  modified_base 10..13: mod_base = OTHER; note = 2'-methoxy nucleoside; note (original language) = 2'-甲氧基核苷
  modified_base 15: mod_base = OTHER; note = 2'-methoxy nucleoside; note (original language) = 2'-甲氧基核苷
  modified_base 17..23: mod_base = OTHER; note = 2'-methoxy nucleoside; note (original language) = 2'-甲氧基核苷
  modified_base 2: mod_base = OTHER; note = 2'-fluoro nucleoside; note (original language) = 2'-氟核苷
  modified_base 9: mod_base = OTHER; note = 2'-fluoro nucleoside; note (original language) = 2'-氟核苷
  modified_base 14: mod_base = OTHER; note = 2'-fluoro nucleoside; note (original language) = 2'-氟核苷
  modified_base 16: mod_base = OTHER; note = 2'-fluoro nucleoside; note (original language) = 2'-氟核苷
  modified_base 1..3: mod_base = OTHER; note = phosphorothioate bond; note (original language) = 硫代磷酸酯键
  modified_base 21..23: mod_base = OTHER; note = phosphorothioate bond; note (original language) = 硫代磷酸酯键
  modified_base 1: mod_base = OTHER; note = 2'-methoxy-5'-vinyl phosphonate nucleoside; note (original language) = 2'-甲氧基-5'-乙烯基膦酸核苷
  modified_base 20: mod_base = i
  modified_base 6..7: mod_base = OTHER; note = The nucleotide monomers are mutually linked by 2'-5'-phosphodiester bond.; note (original language) = 核苷酸单体通过2'-5'-磷酸二酯键相互连接
  source 1..23: mol_type = other RNA
tcttagaccaaggagaaacncct

SEQ ID NO: 905 - RNA, 23 nt, synthetic construct
  modified_base 1: mod_base = OTHER; note = 2'-methoxy nucleoside; note (original language) = 2'-甲氧基核苷
  modified_base 3..5: mod_base = OTHER; note = 2'-methoxy nucleoside; note (original language) = 2'-甲氧基核苷
  modified_base 8: mod_base = OTHER; note = 2'-methoxy nucleoside; note (original language) = 2'-甲氧基核苷
  modified_base 10..13: mod_base = OTHER; note = 2'-methoxy nucleoside; note (original language) = 2'-甲氧基核苷
  modified_base 15: mod_base = OTHER; note = 2'-methoxy nucleoside; note (original language) = 2'-甲氧基核苷
  modified_base 17..23: mod_base = OTHER; note = 2'-methoxy nucleoside; note (original language) = 2'-甲氧基核苷
  modified_base 2: mod_base = OTHER; note = 2'-fluoro nucleoside; note (original language) = 2'-氟核苷
  modified_base 6: mod_base = OTHER; note = 2'-fluoro nucleoside; note (original language) = 2'-氟核苷
  modified_base 9: mod_base = OTHER; note = 2'-fluoro nucleoside; note (original language) = 2'-氟核苷
  modified_base 14: mod_base = OTHER; note = 2'-fluoro nucleoside; note (original language) = 2'-氟核苷
  modified_base 16: mod_base = OTHER; note = 2'-fluoro nucleoside; note (original language) = 2'-氟核苷
  modified_base 1..3: mod_base = OTHER; note = phosphorothioate bond; note (original language) = 硫代磷酸酯键
  modified_base 21..23: mod_base = OTHER; note = phosphorothioate bond; note (original language) = 硫代磷酸酯键
  modified_base 1: mod_base = OTHER; note = 2'-methoxy-5'-vinyl phosphonate nucleoside; note (original language) = 2'-甲氧基-5'-乙烯基膦酸核苷
  modified_base 20: mod_base = i
  modified_base 7..8: mod_base = OTHER; note = The nucleotide monomers are mutually linked by 2'-5'-phosphodiester bond.; note (original language) = 核苷酸单体通过2'-5'-磷酸二酯键相互连接
  source 1..23: mol_type = other RNA
tcttagaccaaggagaaacncct

SEQ ID NO: 906 - RNA, 23 nt, synthetic construct
  modified_base 1: mod_base = OTHER; note = 2'-methoxy nucleoside; note (original language) = 2'-甲氧基核苷
  modified_base 3..6: mod_base = OTHER; note = 2'-methoxy nucleoside; note (original language) = 2'-甲氧基核苷
  modified_base 8: mod_base = OTHER; note = 2'-methoxy nucleoside; note (original language) = 2'-甲氧基核苷
  modified_base 10..13: mod_base = OTHER; note = 2'-methoxy nucleoside; note (original language) = 2'-甲氧基核苷
  modified_base 15: mod_base = OTHER; note = 2'-methoxy nucleoside; note (original language) = 2'-甲氧基核苷
  modified_base 17..23: mod_base = OTHER; note = 2'-methoxy nucleoside; note (original language) = 2'-甲氧基核苷
  modified_base 2: mod_base = OTHER; note = 2'-fluoro nucleoside; note (original language) = 2'-氟核苷
  modified_base 9: mod_base = OTHER; note = 2'-fluoro nucleoside; note (original language) = 2'-氟核苷
  modified_base 14: mod_base = OTHER; note = 2'-fluoro nucleoside; note (original language) = 2'-氟核苷
  modified_base 16: mod_base = OTHER; note = 2'-fluoro nucleoside; note (original language) = 2'-氟核苷
  modified_base 1..3: mod_base = OTHER; note = phosphorothioate bond; note (original language) = 硫代磷酸酯键
  modified_base 21..23: mod_base = OTHER; note = phosphorothioate bond; note (original language) = 硫代磷酸酯键
  modified_base 1: mod_base = OTHER; note = 2'-methoxy-5'-vinyl phosphonate nucleoside; note (original language) = 2'-甲氧基-5'-乙烯基膦酸核苷
  modified_base 20: mod_base = i
  modified_base 7..8: mod_base = OTHER; note = The nucleotide monomers are mutually linked by 2'-5'-phosphodiester bond.; note (original language) = 核苷酸单体通过2'-5'-磷酸二酯键相互连接
  source 1..23: mol_type = other RNA
tcttagaccaaggagaaacncct

SEQ ID NO: 907 - DNA, 23 bp, synthetic construct
  modified_base 1: mod_base = OTHER; note = 2'-methoxy nucleoside; note (original language) = 2'-甲氧基核苷
  modified_base 3..4: mod_base = OTHER; note = 2'-methoxy nucleoside; note (original language) = 2'-甲氧基核苷
  modified_base 6: mod_base = OTHER; note = 2'-methoxy nucleoside; note (original language) = 2'-甲氧基核苷
  modified_base 8: mod_base = OTHER; note = 2'-methoxy nucleoside; note (original language) = 2'-甲氧基核苷
  modified_base 10..13: mod_base = OTHER; note = 2'-methoxy nucleoside; note (original language) = 2'-甲氧基核苷
  modified_base 15: mod_base = OTHER; note = 2'-methoxy nucleoside; note (original language) = 2'-甲氧基核苷
  modified_base 17..23: mod_base = OTHER; note = 2'-methoxy nucleoside; note (original language) = 2'-甲氧基核苷
  modified_base 2: mod_base = OTHER; note = 2'-fluoro nucleoside; note (original language) = 2'-氟核苷
  modified_base 9: mod_base = OTHER; note = 2'-fluoro nucleoside; note (original language) = 2'-氟核苷
  modified_base 14: mod_base = OTHER; note = 2'-fluoro nucleoside; note (original language) = 2'-氟核苷
  modified_base 16: mod_base = OTHER; note = 2'-fluoro nucleoside; note (original language) = 2'-氟核苷
  modified_base 1..3: mod_base = OTHER; note = phosphorothioate bond; note (original language) = 硫代磷酸酯键
  modified_base 21..23: mod_base = OTHER; note = phosphorothioate bond; note (original language) = 硫代磷酸酯键
  modified_base 1: mod_base = OTHER; note = 2'-methoxy-5'-vinyl phosphonate nucleoside; note (original language) = 2'-甲氧基-5'-乙烯基膦酸核苷
  modified_base 20: mod_base = i
  modified_base 7..8: mod_base = OTHER; note = The nucleotide monomers are mutually linked by 2'-5'-phosphodiester bond.; note (original language) = 核苷酸单体通过2'-5'-磷酸二酯键相互连接
  misc_feature 1..4: note = RNA fragment
  misc_feature 5: note = DNA fragment
  misc_feature 6..23: note = RNA fragment
  source 1..23: mol_type = other DNA
tcttagaccaaggagaaacncct

SEQ ID NO: 908 - RNA, 23 nt, synthetic construct
  modified_base 1: mod_base = OTHER; note = 2'-methoxy nucleoside; note (original language) = 2'-甲氧基核苷
  modified_base 3..5: mod_base = OTHER; note = 2'-methoxy nucleoside; note (original language) = 2'-甲氧基核苷
  modified_base 7..8: mod_base = OTHER; note = 2'-methoxy nucleoside; note (original language) = 2'-甲氧基核苷
  modified_base 10..13: mod_base = OTHER; note = 2'-methoxy nucleoside; note (original language) = 2'-甲氧基核苷
  modified_base 15: mod_base = OTHER; note = 2'-methoxy nucleoside; note (original language) = 2'-甲氧基核苷
  modified_base 17..23: mod_base = OTHER; note = 2'-methoxy nucleoside; note (original language) = 2'-甲氧基核苷
  modified_base 2: mod_base = OTHER; note = 2'-fluoro nucleoside; note (original language) = 2'-氟核苷
  modified_base 9: mod_base = OTHER; note = 2'-fluoro nucleoside; note (original language) = 2'-氟核苷
  modified_base 14: mod_base = OTHER; note = 2'-fluoro nucleoside; note (original language) = 2'-氟核苷
  modified_base 16: mod_base = OTHER; note = 2'-fluoro nucleoside; note (original language) = 2'-氟核苷
  modified_base 1..3: mod_base = OTHER; note = phosphorothioate bond; note (original language) = 硫代磷酸酯键
  modified_base 21..23: mod_base = OTHER; note = phosphorothioate bond; note (original language) = 硫代磷酸酯键
  modified_base 1: mod_base = OTHER; note = 2'-methoxy-5'-vinyl phosphonate nucleoside; note (original language) = 2'-甲氧基-5'-乙烯基膦酸核苷
  modified_base 6..7: mod_base = OTHER; note = The nucleotide monomers are mutually linked by 2'-5'-phosphodiester bond.; note (original language) = 核苷酸单体通过2'-5'-磷酸二酯键相互连接
  source 1..23: mol_type = other RNA
tcaaaaaaaatgctgttcagcac

SEQ ID NO: 909 - RNA, 23 nt, synthetic construct
  modified_base 1: mod_base = OTHER; note = 2'-methoxy nucleoside; note (original language) = 2'-甲氧基核苷
  modified_base 3..5: mod_base = OTHER; note = 2'-methoxy nucleoside; note (original language) = 2'-甲氧基核苷
  modified_base 8: mod_base = OTHER; note = 2'-methoxy nucleoside; note (original language) = 2'-甲氧基核苷
  modified_base 10..13: mod_base = OTHER; note = 2'-methoxy nucleoside; note (original language) = 2'-甲氧基核苷
  modified_base 15: mod_base = OTHER; note = 2'-methoxy nucleoside; note (original language) = 2'-甲氧基核苷
  modified_base 17..23: mod_base = OTHER; note = 2'-methoxy nucleoside; note (original language) = 2'-甲氧基核苷
  modified_base 2: mod_base = OTHER; note = 2'-fluoro nucleoside; note (original language) = 2'-氟核苷
  modified_base 6: mod_base = OTHER; note = 2'-fluoro nucleoside; note (original language) = 2'-氟核苷
  modified_base 9: mod_base = OTHER; note = 2'-fluoro nucleoside; note (original language) = 2'-氟核苷
  modified_base 14: mod_base = OTHER; note = 2'-fluoro nucleoside; note (original language) = 2'-氟核苷
  modified_base 16: mod_base = OTHER; note = 2'-fluoro nucleoside; note (original language) = 2'-氟核苷
  modified_base 1..3: mod_base = OTHER; note = phosphorothioate bond; note (original language) = 硫代磷酸酯键
  modified_base 21..23: mod_base = OTHER; note = phosphorothioate bond; note (original language) = 硫代磷酸酯键
  modified_base 1: mod_base = OTHER; note = 2'-methoxy-5'-vinyl phosphonate nucleoside; note (original language) = 2'-甲氧基-5'-乙烯基膦酸核苷
  modified_base 7..8: mod_base = OTHER; note = The nucleotide monomers are mutually linked by 2'-5'-phosphodiester bond.; note (original language) = 核苷酸单体通过2'-5'-磷酸二酯键相互连接
  source 1..23: mol_type = other RNA
tcaaaaaaaatgctgttcagcac

SEQ ID NO: 910 - RNA, 23 nt, synthetic construct
  modified_base 1: mod_base = OTHER; note = 2'-methoxy nucleoside; note (original language) = 2'-甲氧基核苷
  modified_base 3..6: mod_base = OTHER; note = 2'-methoxy nucleoside; note (original language) = 2'-甲氧基核苷
  modified_base 8: mod_base = OTHER; note = 2'-methoxy nucleoside; note (original language) = 2'-甲氧基核苷
  modified_base 10..13: mod_base = OTHER; note = 2'-methoxy nucleoside; note (original language) = 2'-甲氧基核苷
  modified_base 15: mod_base = OTHER; note = 2'-methoxy nucleoside; note (original language) = 2'-甲氧基核苷
  modified_base 17..23: mod_base = OTHER; note = 2'-methoxy nucleoside; note (original language) = 2'-甲氧基核苷
  modified_base 2: mod_base = OTHER; note = 2'-fluoro nucleoside; note (original language) = 2'-氟核苷
  modified_base 9: mod_base = OTHER; note = 2'-fluoro nucleoside; note (original language) = 2'-氟核苷
  modified_base 14: mod_base = OTHER; note = 2'-fluoro nucleoside; note (original language) = 2'-氟核苷
  modified_base 16: mod_base = OTHER; note = 2'-fluoro nucleoside; note (original language) = 2'-氟核苷
  modified_base 1..3: mod_base = OTHER; note = phosphorothioate bond; note (original language) = 硫代磷酸酯键
  modified_base 21..23: mod_base = OTHER; note = phosphorothioate bond; note (original language) = 硫代磷酸酯键
  modified_base 1: mod_base = OTHER; note = 2'-methoxy-5'-vinyl phosphonate nucleoside; note (original language) = 2'-甲氧基-5'-乙烯基膦酸核苷
  modified_base 7..8: mod_base = OTHER; note = The nucleotide monomers are mutually linked by 2'-5'-phosphodiester bond.; note (original language) = 核苷酸单体通过2'-5'-磷酸二酯键相互连接
  source 1..23: mol_type = other RNA
tcaaaaaaaatgctgttcagcac

SEQ ID NO: 911 - DNA, 23 bp, synthetic construct
  modified_base 1: mod_base = OTHER; note = 2'-methoxy nucleoside; note (original language) = 2'-甲氧基核苷
  modified_base 3..4: mod_base = OTHER; note = 2'-methoxy nucleoside; note (original language) = 2'-甲氧基核苷
  modified_base 6: mod_base = OTHER; note = 2'-methoxy nucleoside; note (original language) = 2'-甲氧基核苷
  modified_base 8: mod_base = OTHER; note = 2'-methoxy nucleoside; note (original language) = 2'-甲氧基核苷
  modified_base 10..13: mod_base = OTHER; note = 2'-methoxy nucleoside; note (original language) = 2'-甲氧基核苷
  modified_base 15: mod_base = OTHER; note = 2'-methoxy nucleoside; note (original language) = 2'-甲氧基核苷
  modified_base 17..23: mod_base = OTHER; note = 2'-methoxy nucleoside; note (original language) = 2'-甲氧基核苷
  modified_base 2: mod_base = OTHER; note = 2'-fluoro nucleoside; note (original language) = 2'-氟核苷
  modified_base 9: mod_base = OTHER; note = 2'-fluoro nucleoside; note (original language) = 2'-氟核苷
  modified_base 14: mod_base = OTHER; note = 2'-fluoro nucleoside; note (original language) = 2'-氟核苷
  modified_base 16: mod_base = OTHER; note = 2'-fluoro nucleoside; note (original language) = 2'-氟核苷
  modified_base 1..3: mod_base = OTHER; note = phosphorothioate bond; note (original language) = 硫代磷酸酯键
  modified_base 21..23: mod_base = OTHER; note = phosphorothioate bond; note (original language) = 硫代磷酸酯键
  modified_base 1: mod_base = OTHER; note = 2'-methoxy-5'-vinyl phosphonate nucleoside; note (original language) = 2'-甲氧基-5'-乙烯基膦酸核苷
  modified_base 7..8: mod_base = OTHER; note = The nucleotide monomers are mutually linked by 2'-5'-phosphodiester bond.; note (original language) = 核苷酸单体通过2'-5'-磷酸二酯键相互连接
  misc_feature 1..4: note = RNA fragment
  misc_feature 5: note = DNA fragment
  misc_feature 6..23: note = RNA fragment
  source 1..23: mol_type = other DNA
tcaaaaaaaatgctgttcagcac